European Patent Application EP 4 538 286 A1, published April 16, 2025. Title: CD80 mutant polypeptide and use thereof. Applicant: 杭州阿诺生物医药科技有限公司. Application CN. The sequence listing filed with the application follows.

SEQUENCE LISTING (296 sequences)

SEQ ID NO: 1 - skipped

SEQ ID NO: 2 - protein, 208 aa, synthetic construct
  REGION 1..208: note = Artificial
VIHVTKEVKEVATLSCGHNVSVEELAQTRIYWQKNKKMVLTMMSGDMNIWPEYKNRTIFDITNNLSIVILELRPSDEGTYECVVLKYEKDAFKREHLAEVTLSVKADFPTPSISDFEIPTSNIRRIICSTSGGFPEPHLSWLENGEELNAINTTVSQDPETELYAVSSKLDFNMTTNHSFMCLIKYGHLRVNQTFNWNTTKQEHFPDN

SEQ ID NO: 3 - protein, 208 aa, synthetic construct
  REGION 1..208: note = Artificial
VIHVTKEVKEVATLSCGHNVSVEELAQTRIYWQKNKKMVLTMMSGDMNIWPEYKNRTIFDITNNLSIVILNLRPSDEGTYECVVLKYEKDAFKREHLAEVTLSVKADFPTPSISDFEIPTSNIRRIICSTSGGFPEPHLSWLENGEELNAINTTVSQDPETELYAVSSKLDFNMTTNHSFMCLIKYGHLRVNQTFNWNTTKQEHFPDN

SEQ ID NO: 4 - protein, 208 aa, synthetic construct
  REGION 1..208: note = Artificial
VIHVTKEVKEVATLSCGHNVSVEELAQTRIYWQKNKKMVLTMMSGDMNIWPEYKNRTIFDITNNLSIVILQLRPSDEGTYECVVLKYEKDAFKREHLAEVTLSVKADFPTPSISDFEIPTSNIRRIICSTSGGFPEPHLSWLENGEELNAINTTVSQDPETELYAVSSKLDFNMTTNHSFMCLIKYGHLRVNQTFNWNTTKQEHFPDN

SEQ ID NO: 5 - protein, 208 aa, synthetic construct
  REGION 1..208: note = Artificial
VIHVTKEVKEVATLSCGHNVSVEELAQTRIYWQKNKKMVLTMMSGDMNIWPEYKNRTIFDITNNLSIVILTLRPSDEGTYECVVLKYEKDAFKREHLAEVTLSVKADFPTPSISDFEIPTSNIRRIICSTSGGFPEPHLSWLENGEELNAINTTVSQDPETELYAVSSKLDFNMTTNHSFMCLIKYGHLRVNQTFNWNTTKQEHFPDN

SEQ ID NO: 6 - protein, 208 aa, synthetic construct
  REGION 1..208: note = Artificial
VIHVTKEVKEVATLSCGHNVSVEELAQTRIYWQKSKKMVLTMMSGDMNIWPEYKNRTIFDITNNLSIVILELRPSDEGTYECVVLKYEKDAFKREHLAEVTLSVKADFPTPSISDFEIPTSNIRRIICSTSGGFPEPHLSWLENGEELNAINTTVSQDPETELYAVSSKLDFNMTTNHSFMCLIKYGHLRVNQTFNWNTTKQEHFPDN

SEQ ID NO: 7 - protein, 208 aa, synthetic construct
  REGION 1..208: note = Artificial
VIHVTKEVKEVATLSCGHNVSVEELAQTRIYWQKSKKMVLTMMSGDMNIWPEYKNRTIFDITNNLSIVILNLRPSDEGTYECVVLKYEKDAFKREHLAEVTLSVKADFPTPSISDFEIPTSNIRRIICSTSGGFPEPHLSWLENGEELNAINTTVSQDPETELYAVSSKLDFNMTTNHSFMCLIKYGHLRVNQTFNWNTTKQEHFPDN

SEQ ID NO: 8 - protein, 208 aa, synthetic construct
  REGION 1..208: note = Artificial
VIHVTKEVKEVATLSCGHNVSVEELAQTRIYWQKSKKMVLTMMSGDMNIWPEYKNRTIFDITNNLSIVILQLRPSDEGTYECVVLKYEKDAFKREHLAEVTLSVKADFPTPSISDFEIPTSNIRRIICSTSGGFPEPHLSWLENGEELNAINTTVSQDPETELYAVSSKLDFNMTTNHSFMCLIKYGHLRVNQTFNWNTTKQEHFPDN

SEQ ID NO: 9 - protein, 208 aa, synthetic construct
  REGION 1..208: note = Artificial
VIHVTKEVKEVATLSCGHNVSVEELAQTRIYWQKSKKMVLTMMSGDMNIWPEYKNRTIFDITNNLSIVILTLRPSDEGTYECVVLKYEKDAFKREHLAEVTLSVKADFPTPSISDFEIPTSNIRRIICSTSGGFPEPHLSWLENGEELNAINTTVSQDPETELYAVSSKLDFNMTTNHSFMCLIKYGHLRVNQTFNWNTTKQEHFPDN

SEQ ID NO: 10 - protein, 208 aa, synthetic construct
  REGION 1..208: note = Artificial
VIHVTKEVKEVATLSCGHNVSVEELAQTRIYWQKQKKMVLTMMSGDMNIWPEYKNRTIFDITNNLSIVILELRPSDEGTYECVVLKYEKDAFKREHLAEVTLSVKADFPTPSISDFEIPTSNIRRIICSTSGGFPEPHLSWLENGEELNAINTTVSQDPETELYAVSSKLDFNMTTNHSFMCLIKYGHLRVNQTFNWNTTKQEHFPDN

SEQ ID NO: 11 - protein, 208 aa, synthetic construct
  REGION 1..208: note = Artificial
VIHVTKEVKEVATLSCGHNVSVEELAQTRIYWQKQKKMVLTMMSGDMNIWPEYKNRTIFDITNNLSIVILNLRPSDEGTYECVVLKYEKDAFKREHLAEVTLSVKADFPTPSISDFEIPTSNIRRIICSTSGGFPEPHLSWLENGEELNAINTTVSQDPETELYAVSSKLDFNMTTNHSFMCLIKYGHLRVNQTFNWNTTKQEHFPDN

SEQ ID NO: 12 - protein, 208 aa, synthetic construct
  REGION 1..208: note = Artificial
VIHVTKEVKEVATLSCGHNVSVEELAQTRIYWQKQKKMVLTMMSGDMNIWPEYKNRTIFDITNNLSIVILQLRPSDEGTYECVVLKYEKDAFKREHLAEVTLSVKADFPTPSISDFEIPTSNIRRIICSTSGGFPEPHLSWLENGEELNAINTTVSQDPETELYAVSSKLDFNMTTNHSFMCLIKYGHLRVNQTFNWNTTKQEHFPDN

SEQ ID NO: 13 - protein, 208 aa, synthetic construct
  REGION 1..208: note = Artificial
VIHVTKEVKEVATLSCGHNVSVEELAQTRIYWQKQKKMVLTMMSGDMNIWPEYKNRTIFDITNNLSIVILTLRPSDEGTYECVVLKYEKDAFKREHLAEVTLSVKADFPTPSISDFEIPTSNIRRIICSTSGGFPEPHLSWLENGEELNAINTTVSQDPETELYAVSSKLDFNMTTNHSFMCLIKYGHLRVNQTFNWNTTKQEHFPDN

SEQ ID NO: 14 - protein, 208 aa, synthetic construct
  REGION 1..208: note = Artificial
VIHVTKEVKEVATLSCGHNVSVEELAQTRIYWQKTKKMVLTMMSGDMNIWPEYKNRTIFDITNNLSIVILELRPSDEGTYECVVLKYEKDAFKREHLAEVTLSVKADFPTPSISDFEIPTSNIRRIICSTSGGFPEPHLSWLENGEELNAINTTVSQDPETELYAVSSKLDFNMTTNHSFMCLIKYGHLRVNQTFNWNTTKQEHFPDN

SEQ ID NO: 15 - protein, 208 aa, synthetic construct
  REGION 1..208: note = Artificial
VIHVTKEVKEVATLSCGHNVSVEELAQTRIYWQKTKKMVLTMMSGDMNIWPEYKNRTIFDITNNLSIVILNLRPSDEGTYECVVLKYEKDAFKREHLAEVTLSVKADFPTPSISDFEIPTSNIRRIICSTSGGFPEPHLSWLENGEELNAINTTVSQDPETELYAVSSKLDFNMTTNHSFMCLIKYGHLRVNQTFNWNTTKQEHFPDN

SEQ ID NO: 16 - protein, 208 aa, synthetic construct
  REGION 1..208: note = Artificial
VIHVTKEVKEVATLSCGHNVSVEELAQTRIYWQKTKKMVLTMMSGDMNIWPEYKNRTIFDITNNLSIVILQLRPSDEGTYECVVLKYEKDAFKREHLAEVTLSVKADFPTPSISDFEIPTSNIRRIICSTSGGFPEPHLSWLENGEELNAINTTVSQDPETELYAVSSKLDFNMTTNHSFMCLIKYGHLRVNQTFNWNTTKQEHFPDN

SEQ ID NO: 17 - protein, 208 aa, synthetic construct
  REGION 1..208: note = Artificial
VIHVTKEVKEVATLSCGHNVSVEELAQTRIYWQKTKKMVLTMMSGDMNIWPEYKNRTIFDITNNLSIVILTLRPSDEGTYECVVLKYEKDAFKREHLAEVTLSVKADFPTPSISDFEIPTSNIRRIICSTSGGFPEPHLSWLENGEELNAINTTVSQDPETELYAVSSKLDFNMTTNHSFMCLIKYGHLRVNQTFNWNTTKQEHFPDN

SEQ ID NO: 18 - protein, 208 aa, synthetic construct
  REGION 1..208: note = Artificial
VIHVTKEVKEVATLSCGHNVSVEELAQTRIYWQKEKKMVLTMMSGDANIWPEYKNRTIFDITNNLSIVYLELRPSDEGTYECLVLKYEKDAFKREHLAEVTLSVKADFPTPSISDFEIPTSNIRRIICSTSGGFPEPHLSWLENGEELNAINTTVSQDPETELYAVSSKLDFNMTTNHSFMCLIKYGHLRVNQTFNWNTTKQEHFPDN

SEQ ID NO: 19 - protein, 208 aa, synthetic construct
  REGION 1..208: note = Artificial
VIHVTKEVKEVATLSCGHNVSVEELAQTRIYWQKEKKMVLTMMSGDANIWPEYKNRTIFDITNNLSIVWLELRPSDEGTYECLVLKYEKDAFKREHLAEVTLSVKADFPTPSISDFEIPTSNIRRIICSTSGGFPEPHLSWLENGEELNAINTTVSQDPETELYAVSSKLDFNMTTNHSFMCLIKYGHLRVNQTFNWNTTKQEHFPDN

SEQ ID NO: 20 - protein, 208 aa, synthetic construct
  REGION 1..208: note = Artificial
VIHVTKEVKEVATLSCGHNVSVEELAQTRIYWQKEKKMVLTMMSGDANIWPEYKNRTIFDITNNLSIVYLELRPSDEGTYECVVLKYEKDAFKREHLAEVTLSVKADFPTPSISDFEIPTSNIRRIICSTSGGFPEPHLSWLENGEELNAINTTVSQDPETELYAVSSKLDFNMTTNHSFMCLIKYGHLRVNQTFNWNTTKQEHFPDN

SEQ ID NO: 21 - protein, 208 aa, synthetic construct
  REGION 1..208: note = Artificial
VIHVTKEVKEVATLSCGHNVSVEELAQTRIYWQKEKKMVLTMMSGDANIWPEYKNRTIFDITNNLSIVWLELRPSDEGTYECVVLKYEKDAFKREHLAEVTLSVKADFPTPSISDFEIPTSNIRRIICSTSGGFPEPHLSWLENGEELNAINTTVSQDPETELYAVSSKLDFNMTTNHSFMCLIKYGHLRVNQTFNWNTTKQEHFPDN

SEQ ID NO: 22 - protein, 208 aa, synthetic construct
  REGION 1..208: note = Artificial
VIHVTKEVKEVATLSCGHNVSVEELAQTRIYWQKEKKMVLTMMSGDMNIWPEYKNRTIFDITNNLSIVYLELRPSDEGTYECLVLKYEKDAFKREHLAEVTLSVKADFPTPSISDFEIPTSNIRRIICSTSGGFPEPHLSWLENGEELNAINTTVSQDPETELYAVSSKLDFNMTTNHSFMCLIKYGHLRVNQTFNWNTTKQEHFPDN

SEQ ID NO: 23 - protein, 208 aa, synthetic construct
  REGION 1..208: note = Artificial
VIHVTKEVKEVATLSCGHNVSVEELAQTRIYWQKEKKMVLTMMSGDMNIWPEYKNRTIFDITNNLSIVWLELRPSDEGTYECLVLKYEKDAFKREHLAEVTLSVKADFPTPSISDFEIPTSNIRRIICSTSGGFPEPHLSWLENGEELNAINTTVSQDPETELYAVSSKLDFNMTTNHSFMCLIKYGHLRVNQTFNWNTTKQEHFPDN

SEQ ID NO: 24 - protein, 208 aa, synthetic construct
  REGION 1..208: note = Artificial
VIHVTKEVKEVATLSCGHNVSVEELAQTRIYWQKEKKMVLTMMSGDMNIWPEYKNRTIFDITNNLSIVYLELRPSDEGTYECVVLKYEKDAFKREHLAEVTLSVKADFPTPSISDFEIPTSNIRRIICSTSGGFPEPHLSWLENGEELNAINTTVSQDPETELYAVSSKLDFNMTTNHSFMCLIKYGHLRVNQTFNWNTTKQEHFPDN

SEQ ID NO: 25 - protein, 208 aa, synthetic construct
  REGION 1..208: note = Artificial
VIHVTKEVKEVATLSCGHNVSVEELAQTRIYWQKEKKMVLTMMSGDMNIWPEYKNRTIFDITNNLSIVWLELRPSDEGTYECVVLKYEKDAFKREHLAEVTLSVKADFPTPSISDFEIPTSNIRRIICSTSGGFPEPHLSWLENGEELNAINTTVSQDPETELYAVSSKLDFNMTTNHSFMCLIKYGHLRVNQTFNWNTTKQEHFPDN

SEQ ID NO: 26 - protein, 208 aa, synthetic construct
  REGION 1..208: note = Artificial
VIHVTKEVKEVATLSCGWNVSVEELMQTRIYWQKEKKMVLTMMSGDMNIWPEYKNRTIFDITNNLSIVILELRPSDEGTYECVVNKYEKDAFKREHLAEVTLSVKADFPTPSISDFEIPTSNIRRIICSTSGGFPEPHLSWLENGEELNAINTTVSQDPETELYAVSSKLDFNMTTNHSFMCLIKYGHLRVNQTFNWNTTKQEHFPDN

SEQ ID NO: 27 - protein, 208 aa, synthetic construct
  REGION 1..208: note = Artificial
VIHVTKEVKEVATLSCGWNVSVEELMQTRIYWQKEKKMVLTMMSGDMNIWPEYKNRTIFDITNNLSIVILELRPSDEGTYECVVDKYEKDAFKREHLAEVTLSVKADFPTPSISDFEIPTSNIRRIICSTSGGFPEPHLSWLENGEELNAINTTVSQDPETELYAVSSKLDFNMTTNHSFMCLIKYGHLRVNQTFNWNTTKQEHFPDN

SEQ ID NO: 28 - protein, 208 aa, synthetic construct
  REGION 1..208: note = Artificial
VIHVTKEVKEVATLSCGWNVSVEELCQTRIYWQKEKKMVLTMMSGDMNIWPEYKNRTIFDITNNLSIVILELRPSDEGTYECVVNKYEKDAFKREHLAEVTLSVKADFPTPSISDFEIPTSNIRRIICSTSGGFPEPHLSWLENGEELNAINTTVSQDPETELYAVSSKLDFNMTTNHSFMCLIKYGHLRVNQTFNWNTTKQEHFPDN

SEQ ID NO: 29 - protein, 208 aa, synthetic construct
  REGION 1..208: note = Artificial
VIHVTKEVKEVATLSCGWNVSVEELCQTRIYWQKEKKMVLTMMSGDMNIWPEYKNRTIFDITNNLSIVILELRPSDEGTYECVVDKYEKDAFKREHLAEVTLSVKADFPTPSISDFEIPTSNIRRIICSTSGGFPEPHLSWLENGEELNAINTTVSQDPETELYAVSSKLDFNMTTNHSFMCLIKYGHLRVNQTFNWNTTKQEHFPDN

SEQ ID NO: 30 - protein, 208 aa, synthetic construct
  REGION 1..208: note = Artificial
VIHVTKEVKEVATLSCGHNVSVEELMQTRIYWQKEKKMVLTMMSGDMNIWPEYKNRTIFDITNNLSIVILELRPSDEGTYECVVNKYEKDAFKREHLAEVTLSVKADFPTPSISDFEIPTSNIRRIICSTSGGFPEPHLSWLENGEELNAINTTVSQDPETELYAVSSKLDFNMTTNHSFMCLIKYGHLRVNQTFNWNTTKQEHFPDN

SEQ ID NO: 31 - protein, 208 aa, synthetic construct
  REGION 1..208: note = Artificial
VIHVTKEVKEVATLSCGHNVSVEELMQTRIYWQKEKKMVLTMMSGDMNIWPEYKNRTIFDITNNLSIVILELRPSDEGTYECVVDKYEKDAFKREHLAEVTLSVKADFPTPSISDFEIPTSNIRRIICSTSGGFPEPHLSWLENGEELNAINTTVSQDPETELYAVSSKLDFNMTTNHSFMCLIKYGHLRVNQTFNWNTTKQEHFPDN

SEQ ID NO: 32 - protein, 208 aa, synthetic construct
  REGION 1..208: note = Artificial
VIHVTKEVKEVATLSCGHNVSVEELCQTRIYWQKEKKMVLTMMSGDMNIWPEYKNRTIFDITNNLSIVILELRPSDEGTYECVVDKYEKDAFKREHLAEVTLSVKADFPTPSISDFEIPTSNIRRIICSTSGGFPEPHLSWLENGEELNAINTTVSQDPETELYAVSSKLDFNMTTNHSFMCLIKYGHLRVNQTFNWNTTKQEHFPDN

SEQ ID NO: 33 - protein, 208 aa, synthetic construct
  REGION 1..208: note = Artificial
VIHVTKEVKEVATLSCGHNVSVEELCQTRIYWQKEKKMVLTMMSGDMNIWPEYKNRTIFDITNNLSIVILELRPSDEGTYECVVNKYEKDAFKREHLAEVTLSVKADFPTPSISDFEIPTSNIRRIICSTSGGFPEPHLSWLENGEELNAINTTVSQDPETELYAVSSKLDFNMTTNHSFMCLIKYGHLRVNQTFNWNTTKQEHFPDN

SEQ ID NO: 34 - protein, 208 aa, synthetic construct
  REGION 1..208: note = Artificial
VIHVTKEVKEVATLSCGHNVSVEELAQTRIYWQKEKKMVLTMMSGDMNIWPEYKNRTIFDITNNLSIVLLELRPSDEGTYECLVLKYEKDAFKREHLAEVTLSVKADFPTPSISDFEIPTSNIRRIICSTSGGFPEPHLSWLENGEELNAINTTVSQDPETELYAVSSKLDFNMTTNHSFMCLIKYGHLRVNQTFNWNTTKQEHFPDN

SEQ ID NO: 35 - protein, 208 aa, synthetic construct
  REGION 1..208: note = Artificial
VIHVTKEVKEVATLSCGWNVSVEELVQTRIYWQKNKKMVLTMMSGDMNIWPEYKNRTIFDITNNLSIVILELRPSDEGTYECVVNKYEKDAFKREHLAEVTLSVKADFPTPSISDFEIPTSNIRRIICSTSGGFPEPHLSWLENGEELNAINTTVSQDPETELYAVSSKLDFNMTTNHSFMCLIKYGHLRVNQTFNWNTTKQEHFPDN

SEQ ID NO: 36 - protein, 208 aa, synthetic construct
  REGION 1..208: note = Artificial
VIHVTKEVKEVAKLSCGHNVSVEELAQTRIYWQKEKKMVLTLMSGDHNIWPEYKNRTIFDITNNLSIVILELRPSDEGTYECVVLKYEKDAFKREHLAEVTLSVKADFPTPSISDFEIPTSNIRRIICSTSGGFPEPHLSWLENGEELNAINTTVSQDPETELYAVSSKLDFNMTTNHSFMCLIKYGHLRVNQTFNWNTTKQEHFPDN

SEQ ID NO: 37 - protein, 208 aa, synthetic construct
  REGION 1..208: note = Artificial
VIHVTKEVKEVAKLSCGHNVSVEELAQTRIYWQKEKKMVLTLMSGDQNIWPEYKNRTIFDITNNLSIVILELRPSDEGTYECVVLKYEKDAFKREHLAEVTLSVKADFPTPSISDFEIPTSNIRRIICSTSGGFPEPHLSWLENGEELNAINTTVSQDPETELYAVSSKLDFNMTTNHSFMCLIKYGHLRVNQTFNWNTTKQEHFPDN

SEQ ID NO: 38 - protein, 208 aa, synthetic construct
  REGION 1..208: note = Artificial
VIHVTKEVKEVAKLSCGHNVSVEELAQTRIYWQKEKKMVLTLMSGDMNIWPEYKNRTIFDITNNLSIVILELRPSDEGTYECVVLKYEKDAFKREHLAEVTLSVKADFPTPSISDFEIPTSNIRRIICSTSGGFPEPHLSWLENGEELNAINTTVSQDPETELYAVSSKLDFNMTTNHSFMCLIKYGHLRVNQTFNWNTTKQEHFPDN

SEQ ID NO: 39 - protein, 208 aa, synthetic construct
  REGION 1..208: note = Artificial
VIHVTKEVKEVAKLSCGHNVSVEELAQTRIYWQKEKKMVLTTMSGDHNIWPEYKNRTIFDITNNLSIVILELRPSDEGTYECVVLKYEKDAFKREHLAEVTLSVKADFPTPSISDFEIPTSNIRRIICSTSGGFPEPHLSWLENGEELNAINTTVSQDPETELYAVSSKLDFNMTTNHSFMCLIKYGHLRVNQTFNWNTTKQEHFPDN

SEQ ID NO: 40 - protein, 208 aa, synthetic construct
  REGION 1..208: note = Artificial
VIHVTKEVKEVAKLSCGHNVSVEELAQTRIYWQKEKKMVLTTMSGDQNIWPEYKNRTIFDITNNLSIVILELRPSDEGTYECVVLKYEKDAFKREHLAEVTLSVKADFPTPSISDFEIPTSNIRRIICSTSGGFPEPHLSWLENGEELNAINTTVSQDPETELYAVSSKLDFNMTTNHSFMCLIKYGHLRVNQTFNWNTTKQEHFPDN

SEQ ID NO: 41 - protein, 208 aa, synthetic construct
  REGION 1..208: note = Artificial
VIHVTKEVKEVAKLSCGHNVSVEELAQTRIYWQKEKKMVLTTMSGDMNIWPEYKNRTIFDITNNLSIVILELRPSDEGTYECVVLKYEKDAFKREHLAEVTLSVKADFPTPSISDFEIPTSNIRRIICSTSGGFPEPHLSWLENGEELNAINTTVSQDPETELYAVSSKLDFNMTTNHSFMCLIKYGHLRVNQTFNWNTTKQEHFPDN

SEQ ID NO: 42 - protein, 208 aa, synthetic construct
  REGION 1..208: note = Artificial
VIHVTKEVKEVATLSCGHNVSVEELAQTRIYWQKEKKMVLTMMSGDHNIWPEYKNRTIFDITNNLSIVYLELRPSDEGTYECLVLKYEKDAFKREHLAEVTLSVKADFPTPSISDFEIPTSNIRRIICSTSGGFPEPHLSWLENGEELNAINTTVSQDPETELYAVSSKLDFNMTTNHSFMCLIKYGHLRVNQTFNWNTTKQEHFPDN

SEQ ID NO: 43 - protein, 208 aa, synthetic construct
  REGION 1..208: note = Artificial
VIHVTKEVKEVATLSCGHNVSVEELAQTRIYWQKEKKMVLTMMSGDQNIWPEYKNRTIFDITNNLSIVYLELRPSDEGTYECLVLKYEKDAFKREHLAEVTLSVKADFPTPSISDFEIPTSNIRRIICSTSGGFPEPHLSWLENGEELNAINTTVSQDPETELYAVSSKLDFNMTTNHSFMCLIKYGHLRVNQTFNWNTTKQEHFPDN

SEQ ID NO: 44 - protein, 208 aa, synthetic construct
  REGION 1..208: note = Artificial
VIHVTKEVKEVATLSCGHNVSVEELAQTRIYWQKEKKMVLTMMSGDKNIWPEYKNRTIFDITNNLSIVYLELRPSDEGTYECLVLKYEKDAFKREHLAEVTLSVKADFPTPSISDFEIPTSNIRRIICSTSGGFPEPHLSWLENGEELNAINTTVSQDPETELYAVSSKLDFNMTTNHSFMCLIKYGHLRVNQTFNWNTTKQEHFPDN

SEQ ID NO: 45 - protein, 107 aa, Homo sapiens
VIHVTKEVKEVATLSCGHNVSVEELAQTRIYWQKEKKMVLTMMSGDMNIWPEYKNRTIFDITNNLSIVILALRPSDEGTYECVVLKYEKDAFKREHLAEVTLSVKAD

SEQ ID NO: 46 - protein, 107 aa, synthetic construct
  REGION 1..107: note = Artificial
VIHVTKEVKEVATLSCGHNVSVEELAQTRIYWQKNKKMVLTMMSGDMNIWPEYKNRTIFDITNNLSIVILELRPSDEGTYECVVLKYEKDAFKREHLAEVTLSVKAD

SEQ ID NO: 47 - protein, 107 aa, synthetic construct
  REGION 1..107: note = Artificial
VIHVTKEVKEVATLSCGHNVSVEELAQTRIYWQKNKKMVLTMMSGDMNIWPEYKNRTIFDITNNLSIVILNLRPSDEGTYECVVLKYEKDAFKREHLAEVTLSVKAD

SEQ ID NO: 48 - protein, 107 aa, synthetic construct
  REGION 1..107: note = Artificial
VIHVTKEVKEVATLSCGHNVSVEELAQTRIYWQKNKKMVLTMMSGDMNIWPEYKNRTIFDITNNLSIVILQLRPSDEGTYECVVLKYEKDAFKREHLAEVTLSVKAD

SEQ ID NO: 49 - protein, 107 aa, synthetic construct
  REGION 1..107: note = Artificial
VIHVTKEVKEVATLSCGHNVSVEELAQTRIYWQKNKKMVLTMMSGDMNIWPEYKNRTIFDITNNLSIVILTLRPSDEGTYECVVLKYEKDAFKREHLAEVTLSVKAD

SEQ ID NO: 50 - protein, 107 aa, synthetic construct
  REGION 1..107: note = Artificial
VIHVTKEVKEVATLSCGHNVSVEELAQTRIYWQKSKKMVLTMMSGDMNIWPEYKNRTIFDITNNLSIVILELRPSDEGTYECVVLKYEKDAFKREHLAEVTLSVKAD

SEQ ID NO: 51 - protein, 107 aa, synthetic construct
  REGION 1..107: note = Artificial
VIHVTKEVKEVATLSCGHNVSVEELAQTRIYWQKSKKMVLTMMSGDMNIWPEYKNRTIFDITNNLSIVILNLRPSDEGTYECVVLKYEKDAFKREHLAEVTLSVKAD

SEQ ID NO: 52 - protein, 107 aa, synthetic construct
  REGION 1..107: note = Artificial
VIHVTKEVKEVATLSCGHNVSVEELAQTRIYWQKSKKMVLTMMSGDMNIWPEYKNRTIFDITNNLSIVILQLRPSDEGTYECVVLKYEKDAFKREHLAEVTLSVKAD

SEQ ID NO: 53 - protein, 107 aa, synthetic construct
  REGION 1..107: note = Artificial
VIHVTKEVKEVATLSCGHNVSVEELAQTRIYWQKSKKMVLTMMSGDMNIWPEYKNRTIFDITNNLSIVILTLRPSDEGTYECVVLKYEKDAFKREHLAEVTLSVKAD

SEQ ID NO: 54 - protein, 107 aa, synthetic construct
  REGION 1..107: note = Artificial
VIHVTKEVKEVATLSCGHNVSVEELAQTRIYWQKQKKMVLTMMSGDMNIWPEYKNRTIFDITNNLSIVILELRPSDEGTYECVVLKYEKDAFKREHLAEVTLSVKAD

SEQ ID NO: 55 - protein, 107 aa, synthetic construct
  REGION 1..107: note = Artificial
VIHVTKEVKEVATLSCGHNVSVEELAQTRIYWQKQKKMVLTMMSGDMNIWPEYKNRTIFDITNNLSIVILNLRPSDEGTYECVVLKYEKDAFKREHLAEVTLSVKAD

SEQ ID NO: 56 - protein, 107 aa, synthetic construct
  REGION 1..107: note = Artificial
VIHVTKEVKEVATLSCGHNVSVEELAQTRIYWQKQKKMVLTMMSGDMNIWPEYKNRTIFDITNNLSIVILQLRPSDEGTYECVVLKYEKDAFKREHLAEVTLSVKAD

SEQ ID NO: 57 - protein, 107 aa, synthetic construct
  REGION 1..107: note = Artificial
VIHVTKEVKEVATLSCGHNVSVEELAQTRIYWQKQKKMVLTMMSGDMNIWPEYKNRTIFDITNNLSIVILTLRPSDEGTYECVVLKYEKDAFKREHLAEVTLSVKAD

SEQ ID NO: 58 - protein, 107 aa, synthetic construct
  REGION 1..107: note = Artificial
VIHVTKEVKEVATLSCGHNVSVEELAQTRIYWQKTKKMVLTMMSGDMNIWPEYKNRTIFDITNNLSIVILELRPSDEGTYECVVLKYEKDAFKREHLAEVTLSVKAD

SEQ ID NO: 59 - protein, 107 aa, synthetic construct
  REGION 1..107: note = Artificial
VIHVTKEVKEVATLSCGHNVSVEELAQTRIYWQKTKKMVLTMMSGDMNIWPEYKNRTIFDITNNLSIVILNLRPSDEGTYECVVLKYEKDAFKREHLAEVTLSVKAD

SEQ ID NO: 60 - protein, 107 aa, synthetic construct
  REGION 1..107: note = Artificial
VIHVTKEVKEVATLSCGHNVSVEELAQTRIYWQKTKKMVLTMMSGDMNIWPEYKNRTIFDITNNLSIVILQLRPSDEGTYECVVLKYEKDAFKREHLAEVTLSVKAD

SEQ ID NO: 61 - protein, 107 aa, synthetic construct
  REGION 1..107: note = Artificial
VIHVTKEVKEVATLSCGHNVSVEELAQTRIYWQKTKKMVLTMMSGDMNIWPEYKNRTIFDITNNLSIVILTLRPSDEGTYECVVLKYEKDAFKREHLAEVTLSVKAD

SEQ ID NO: 62 - protein, 107 aa, synthetic construct
  REGION 1..107: note = Artificial
VIHVTKEVKEVATLSCGHNVSVEELAQTRIYWQKEKKMVLTMMSGDANIWPEYKNRTIFDITNNLSIVYLELRPSDEGTYECLVLKYEKDAFKREHLAEVTLSVKAD

SEQ ID NO: 63 - protein, 107 aa, synthetic construct
  REGION 1..107: note = Artificial
VIHVTKEVKEVATLSCGHNVSVEELAQTRIYWQKEKKMVLTMMSGDANIWPEYKNRTIFDITNNLSIVWLELRPSDEGTYECLVLKYEKDAFKREHLAEVTLSVKAD

SEQ ID NO: 64 - protein, 107 aa, synthetic construct
  REGION 1..107: note = Artificial
VIHVTKEVKEVATLSCGHNVSVEELAQTRIYWQKEKKMVLTMMSGDANIWPEYKNRTIFDITNNLSIVYLELRPSDEGTYECVVLKYEKDAFKREHLAEVTLSVKAD

SEQ ID NO: 65 - protein, 107 aa, synthetic construct
  REGION 1..107: note = Artificial
VIHVTKEVKEVATLSCGHNVSVEELAQTRIYWQKEKKMVLTMMSGDANIWPEYKNRTIFDITNNLSIVWLELRPSDEGTYECVVLKYEKDAFKREHLAEVTLSVKAD

SEQ ID NO: 66 - protein, 107 aa, synthetic construct
  REGION 1..107: note = Artificial
VIHVTKEVKEVATLSCGHNVSVEELAQTRIYWQKEKKMVLTMMSGDMNIWPEYKNRTIFDITNNLSIVYLELRPSDEGTYECLVLKYEKDAFKREHLAEVTLSVKAD

SEQ ID NO: 67 - protein, 107 aa, synthetic construct
  REGION 1..107: note = Artificial
VIHVTKEVKEVATLSCGHNVSVEELAQTRIYWQKEKKMVLTMMSGDMNIWPEYKNRTIFDITNNLSIVWLELRPSDEGTYECLVLKYEKDAFKREHLAEVTLSVKAD

SEQ ID NO: 68 - protein, 107 aa, synthetic construct
  REGION 1..107: note = Artificial
VIHVTKEVKEVATLSCGHNVSVEELAQTRIYWQKEKKMVLTMMSGDMNIWPEYKNRTIFDITNNLSIVYLELRPSDEGTYECVVLKYEKDAFKREHLAEVTLSVKAD

SEQ ID NO: 69 - protein, 107 aa, synthetic construct
  REGION 1..107: note = Artificial
VIHVTKEVKEVATLSCGHNVSVEELAQTRIYWQKEKKMVLTMMSGDMNIWPEYKNRTIFDITNNLSIVWLELRPSDEGTYECVVLKYEKDAFKREHLAEVTLSVKAD

SEQ ID NO: 70 - protein, 107 aa, synthetic construct
  REGION 1..107: note = Artificial
VIHVTKEVKEVATLSCGWNVSVEELMQTRIYWQKEKKMVLTMMSGDMNIWPEYKNRTIFDITNNLSIVILELRPSDEGTYECVVNKYEKDAFKREHLAEVTLSVKAD

SEQ ID NO: 71 - protein, 107 aa, synthetic construct
  REGION 1..107: note = Artificial
VIHVTKEVKEVATLSCGWNVSVEELMQTRIYWQKEKKMVLTMMSGDMNIWPEYKNRTIFDITNNLSIVILELRPSDEGTYECVVDKYEKDAFKREHLAEVTLSVKAD

SEQ ID NO: 72 - protein, 107 aa, synthetic construct
  REGION 1..107: note = Artificial
VIHVTKEVKEVATLSCGWNVSVEELCQTRIYWQKEKKMVLTMMSGDMNIWPEYKNRTIFDITNNLSIVILELRPSDEGTYECVVNKYEKDAFKREHLAEVTLSVKAD

SEQ ID NO: 73 - protein, 107 aa, synthetic construct
  REGION 1..107: note = Artificial
VIHVTKEVKEVATLSCGWNVSVEELCQTRIYWQKEKKMVLTMMSGDMNIWPEYKNRTIFDITNNLSIVILELRPSDEGTYECVVDKYEKDAFKREHLAEVTLSVKAD

SEQ ID NO: 74 - protein, 107 aa, synthetic construct
  REGION 1..107: note = Artificial
VIHVTKEVKEVATLSCGHNVSVEELMQTRIYWQKEKKMVLTMMSGDMNIWPEYKNRTIFDITNNLSIVILELRPSDEGTYECVVNKYEKDAFKREHLAEVTLSVKAD

SEQ ID NO: 75 - protein, 107 aa, synthetic construct
  REGION 1..107: note = Artificial
VIHVTKEVKEVATLSCGHNVSVEELMQTRIYWQKEKKMVLTMMSGDMNIWPEYKNRTIFDITNNLSIVILELRPSDEGTYECVVDKYEKDAFKREHLAEVTLSVKAD

SEQ ID NO: 76 - protein, 107 aa, synthetic construct
  REGION 1..107: note = Artificial
VIHVTKEVKEVATLSCGHNVSVEELCQTRIYWQKEKKMVLTMMSGDMNIWPEYKNRTIFDITNNLSIVILELRPSDEGTYECVVDKYEKDAFKREHLAEVTLSVKAD

SEQ ID NO: 77 - protein, 107 aa, synthetic construct
  REGION 1..107: note = Artificial
VIHVTKEVKEVATLSCGHNVSVEELCQTRIYWQKEKKMVLTMMSGDMNIWPEYKNRTIFDITNNLSIVILELRPSDEGTYECVVNKYEKDAFKREHLAEVTLSVKAD

SEQ ID NO: 78 - protein, 107 aa, synthetic construct
  REGION 1..107: note = Artificial
VIHVTKEVKEVATLSCGHNVSVEELAQTRIYWQKEKKMVLTMMSGDMNIWPEYKNRTIFDITNNLSIVLLELRPSDEGTYECLVLKYEKDAFKREHLAEVTLSVKAD

SEQ ID NO: 79 - protein, 107 aa, synthetic construct
  REGION 1..107: note = Artificial
VIHVTKEVKEVATLSCGWNVSVEELVQTRIYWQKNKKMVLTMMSGDMNIWPEYKNRTIFDITNNLSIVILELRPSDEGTYECVVNKYEKDAFKREHLAEVTLSVKAD

SEQ ID NO: 80 - protein, 107 aa, synthetic construct
  REGION 1..107: note = Artificial
VIHVTKEVKEVAKLSCGHNVSVEELAQTRIYWQKEKKMVLTLMSGDHNIWPEYKNRTIFDITNNLSIVILELRPSDEGTYECVVLKYEKDAFKREHLAEVTLSVKAD

SEQ ID NO: 81 - protein, 107 aa, synthetic construct
  REGION 1..107: note = Artificial
VIHVTKEVKEVAKLSCGHNVSVEELAQTRIYWQKEKKMVLTLMSGDQNIWPEYKNRTIFDITNNLSIVILELRPSDEGTYECVVLKYEKDAFKREHLAEVTLSVKAD

SEQ ID NO: 82 - protein, 107 aa, synthetic construct
  REGION 1..107: note = Artificial
VIHVTKEVKEVAKLSCGHNVSVEELAQTRIYWQKEKKMVLTLMSGDMNIWPEYKNRTIFDITNNLSIVILELRPSDEGTYECVVLKYEKDAFKREHLAEVTLSVKAD

SEQ ID NO: 83 - protein, 107 aa, synthetic construct
  REGION 1..107: note = Artificial
VIHVTKEVKEVAKLSCGHNVSVEELAQTRIYWQKEKKMVLTTMSGDHNIWPEYKNRTIFDITNNLSIVILELRPSDEGTYECVVLKYEKDAFKREHLAEVTLSVKAD

SEQ ID NO: 84 - protein, 107 aa, synthetic construct
  REGION 1..107: note = Artificial
VIHVTKEVKEVAKLSCGHNVSVEELAQTRIYWQKEKKMVLTTMSGDQNIWPEYKNRTIFDITNNLSIVILELRPSDEGTYECVVLKYEKDAFKREHLAEVTLSVKAD

SEQ ID NO: 85 - protein, 107 aa, synthetic construct
  REGION 1..107: note = Artificial
VIHVTKEVKEVAKLSCGHNVSVEELAQTRIYWQKEKKMVLTTMSGDMNIWPEYKNRTIFDITNNLSIVILELRPSDEGTYECVVLKYEKDAFKREHLAEVTLSVKAD

SEQ ID NO: 86 - protein, 107 aa, synthetic construct
  REGION 1..107: note = Artificial
VIHVTKEVKEVATLSCGHNVSVEELAQTRIYWQKEKKMVLTMMSGDHNIWPEYKNRTIFDITNNLSIVYLELRPSDEGTYECLVLKYEKDAFKREHLAEVTLSVKAD

SEQ ID NO: 87 - protein, 107 aa, synthetic construct
  REGION 1..107: note = Artificial
VIHVTKEVKEVATLSCGHNVSVEELAQTRIYWQKEKKMVLTMMSGDQNIWPEYKNRTIFDITNNLSIVYLELRPSDEGTYECLVLKYEKDAFKREHLAEVTLSVKAD

SEQ ID NO: 88 - protein, 107 aa, synthetic construct
  REGION 1..107: note = Artificial
VIHVTKEVKEVATLSCGHNVSVEELAQTRIYWQKEKKMVLTMMSGDKNIWPEYKNRTIFDITNNLSIVYLELRPSDEGTYECLVLKYEKDAFKREHLAEVTLSVKAD

SEQ ID NO: 89 - protein, 254 aa, Homo sapiens
VIHVTKEVKEVATLSCGHNVSVEELAQTRIYWQKEKKMVLTMMSGDMNIWPEYKNRTIFDITNNLSIVILALRPSDEGTYECVVLKYEKDAFKREHLAEVTLSVKADFPTPSISDFEIPTSNIRRIICSTSGGFPEPHLSWLENGEELNAINTTVSQDPETELYAVSSKLDFNMTTNHSFMCLIKYGHLRVNQTFNWNTTKQEHFPDNLLPSWAITLISVNGIFVICCLTYCFAPRCRERRRNERLRRESVRPV

SEQ ID NO: 90 - protein, 232 aa, Homo sapiens
EPKSCDKTHTCPPCPAPELLGGPSVFLFPPKPKDTLMISRTPEVTCVVVDVSHEDPEVKFNWYVDGVEVHNAKTKPREEQYNSTYRVVSVLTVLHQDWLNGKEYKCKVSNKALPAPIEKTISKAKGQPREPQVYTLPPSRDELTKNQVSLTCLVKGFYPSDIAVEWESNGQPENNYKTTPPVLDSDGSFFLYSKLTVDKSRWQQGNVFSCSVMHEALHNHYTQKSLSLSPGK

SEQ ID NO: 91 - protein, 229 aa, Homo sapiens
ESKYGPPCPSCPAPEFLGGPSVFLFPPKPKDTLMISRTPEVTCVVVDVSQEDPEVQFNWYVDGVEVHNAKTKPREEQFNSTYRVVSVLTVLHQDWLNGKEYKCKVSNKGLPSSIEKTISKAKGQPREPQVYTLPPSQEEMTKNQVSLTCLVKGFYPSDIAVEWESNGQPENNYKTTPPVLDSDGSFFLYSRLTVDKSRWQEGNVFSCSVMHEALHNHYTQKSLSLSLGK

SEQ ID NO: 92 - protein, 5 aa, synthetic construct
  REGION 1..5: note = Artificial
GGGGS

SEQ ID NO: 93 - protein, 10 aa, synthetic construct
  REGION 1..10: note = Artificial
GGGGSGGGGS

SEQ ID NO: 94 - protein, 15 aa, synthetic construct
  REGION 1..15: note = Artificial
GGGGSGGGGSGGGGS

SEQ ID NO: 95 - protein, 20 aa, synthetic construct
  REGION 1..20: note = Artificial
GGGGSGGGGSGGGGSGGGGS

SEQ ID NO: 96 - protein, 9 aa, synthetic construct
  REGION 1..9: note = Artificial
GGGGSGGGS

SEQ ID NO: 97 - protein, 576 aa, synthetic construct
  REGION 1..576: note = Artificial
VIHVTKEVKEVATLSCGHNVSVEELAQTRIYWQKNKKMVLTMMSGDMNIWPEYKNRTIFDITNNLSIVILELRPSDEGTYECVVLKYEKDAFKREHLAEVTLSVKADGGGGSGGGGSGGGGSGGGGSGEVQLLESGGGLVQPGGSLRLSCAASGFTFSSYAMSWVRQAPGKGLEWVSGISGSGGFTYYADSVKGRFTISRDNSKNTLYLQMNSLRAEDTAVYYCAKPPRGYNYGPFDYWGQGTLVTVSSASTKGPSVFPLAPCSRSTSESTAALGCLVKDYFPEPVTVSWNSGALTSGVHTFPAVLQSSGLYSLSSVVTVPSSSLGTKTYTCNVDHKPSNTKVDKRVESKYGPPCPPCPAPEFLGGPSVFLFPPKPKDTLMISRTPEVTCVVVDVSQEDPEVQFNWYVDGVEVHNAKTKPREEQFNSTYRVVSVLAVLHQDWLNGKEYKCKVSNKGLPSSIEKTISKAKGQPREPQVYTLPPSQEEMTKNQVSLTCLVKGFYPSDIAVAWESNGQPENNYKTTPPVLDSDGSFFLYSRLTVDKSRWQEGNVFSCSVMHEALHAHYTQKSLSLSLGK

SEQ ID NO: 98 - protein, 576 aa, synthetic construct
  REGION 1..576: note = Artificial
VIHVTKEVKEVATLSCGHNVSVEELAQTRIYWQKNKKMVLTMMSGDMNIWPEYKNRTIFDITNNLSIVILNLRPSDEGTYECVVLKYEKDAFKREHLAEVTLSVKADGGGGSGGGGSGGGGSGGGGSGEVQLLESGGGLVQPGGSLRLSCAASGFTFSSYAMSWVRQAPGKGLEWVSGISGSGGFTYYADSVKGRFTISRDNSKNTLYLQMNSLRAEDTAVYYCAKPPRGYNYGPFDYWGQGTLVTVSSASTKGPSVFPLAPCSRSTSESTAALGCLVKDYFPEPVTVSWNSGALTSGVHTFPAVLQSSGLYSLSSVVTVPSSSLGTKTYTCNVDHKPSNTKVDKRVESKYGPPCPPCPAPEFLGGPSVFLFPPKPKDTLMISRTPEVTCVVVDVSQEDPEVQFNWYVDGVEVHNAKTKPREEQFNSTYRVVSVLAVLHQDWLNGKEYKCKVSNKGLPSSIEKTISKAKGQPREPQVYTLPPSQEEMTKNQVSLTCLVKGFYPSDIAVAWESNGQPENNYKTTPPVLDSDGSFFLYSRLTVDKSRWQEGNVFSCSVMHEALHAHYTQKSLSLSLGK

SEQ ID NO: 99 - protein, 576 aa, synthetic construct
  REGION 1..576: note = Artificial
VIHVTKEVKEVATLSCGHNVSVEELAQTRIYWQKNKKMVLTMMSGDMNIWPEYKNRTIFDITNNLSIVILQLRPSDEGTYECVVLKYEKDAFKREHLAEVTLSVKADGGGGSGGGGSGGGGSGGGGSGEVQLLESGGGLVQPGGSLRLSCAASGFTFSSYAMSWVRQAPGKGLEWVSGISGSGGFTYYADSVKGRFTISRDNSKNTLYLQMNSLRAEDTAVYYCAKPPRGYNYGPFDYWGQGTLVTVSSASTKGPSVFPLAPCSRSTSESTAALGCLVKDYFPEPVTVSWNSGALTSGVHTFPAVLQSSGLYSLSSVVTVPSSSLGTKTYTCNVDHKPSNTKVDKRVESKYGPPCPPCPAPEFLGGPSVFLFPPKPKDTLMISRTPEVTCVVVDVSQEDPEVQFNWYVDGVEVHNAKTKPREEQFNSTYRVVSVLAVLHQDWLNGKEYKCKVSNKGLPSSIEKTISKAKGQPREPQVYTLPPSQEEMTKNQVSLTCLVKGFYPSDIAVAWESNGQPENNYKTTPPVLDSDGSFFLYSRLTVDKSRWQEGNVFSCSVMHEALHAHYTQKSLSLSLGK

SEQ ID NO: 100 - protein, 576 aa, synthetic construct
  REGION 1..576: note = Artificial
VIHVTKEVKEVATLSCGHNVSVEELAQTRIYWQKNKKMVLTMMSGDMNIWPEYKNRTIFDITNNLSIVILTLRPSDEGTYECVVLKYEKDAFKREHLAEVTLSVKADGGGGSGGGGSGGGGSGGGGSGEVQLLESGGGLVQPGGSLRLSCAASGFTFSSYAMSWVRQAPGKGLEWVSGISGSGGFTYYADSVKGRFTISRDNSKNTLYLQMNSLRAEDTAVYYCAKPPRGYNYGPFDYWGQGTLVTVSSASTKGPSVFPLAPCSRSTSESTAALGCLVKDYFPEPVTVSWNSGALTSGVHTFPAVLQSSGLYSLSSVVTVPSSSLGTKTYTCNVDHKPSNTKVDKRVESKYGPPCPPCPAPEFLGGPSVFLFPPKPKDTLMISRTPEVTCVVVDVSQEDPEVQFNWYVDGVEVHNAKTKPREEQFNSTYRVVSVLAVLHQDWLNGKEYKCKVSNKGLPSSIEKTISKAKGQPREPQVYTLPPSQEEMTKNQVSLTCLVKGFYPSDIAVAWESNGQPENNYKTTPPVLDSDGSFFLYSRLTVDKSRWQEGNVFSCSVMHEALHAHYTQKSLSLSLGK

SEQ ID NO: 101 - protein, 576 aa, synthetic construct
  REGION 1..576: note = Artificial
VIHVTKEVKEVATLSCGHNVSVEELAQTRIYWQKSKKMVLTMMSGDMNIWPEYKNRTIFDITNNLSIVILELRPSDEGTYECVVLKYEKDAFKREHLAEVTLSVKADGGGGSGGGGSGGGGSGGGGSGEVQLLESGGGLVQPGGSLRLSCAASGFTFSSYAMSWVRQAPGKGLEWVSGISGSGGFTYYADSVKGRFTISRDNSKNTLYLQMNSLRAEDTAVYYCAKPPRGYNYGPFDYWGQGTLVTVSSASTKGPSVFPLAPCSRSTSESTAALGCLVKDYFPEPVTVSWNSGALTSGVHTFPAVLQSSGLYSLSSVVTVPSSSLGTKTYTCNVDHKPSNTKVDKRVESKYGPPCPPCPAPEFLGGPSVFLFPPKPKDTLMISRTPEVTCVVVDVSQEDPEVQFNWYVDGVEVHNAKTKPREEQFNSTYRVVSVLAVLHQDWLNGKEYKCKVSNKGLPSSIEKTISKAKGQPREPQVYTLPPSQEEMTKNQVSLTCLVKGFYPSDIAVAWESNGQPENNYKTTPPVLDSDGSFFLYSRLTVDKSRWQEGNVFSCSVMHEALHAHYTQKSLSLSLGK

SEQ ID NO: 102 - protein, 576 aa, synthetic construct
  REGION 1..576: note = Artificial
VIHVTKEVKEVATLSCGHNVSVEELAQTRIYWQKSKKMVLTMMSGDMNIWPEYKNRTIFDITNNLSIVILNLRPSDEGTYECVVLKYEKDAFKREHLAEVTLSVKADGGGGSGGGGSGGGGSGGGGSGEVQLLESGGGLVQPGGSLRLSCAASGFTFSSYAMSWVRQAPGKGLEWVSGISGSGGFTYYADSVKGRFTISRDNSKNTLYLQMNSLRAEDTAVYYCAKPPRGYNYGPFDYWGQGTLVTVSSASTKGPSVFPLAPCSRSTSESTAALGCLVKDYFPEPVTVSWNSGALTSGVHTFPAVLQSSGLYSLSSVVTVPSSSLGTKTYTCNVDHKPSNTKVDKRVESKYGPPCPPCPAPEFLGGPSVFLFPPKPKDTLMISRTPEVTCVVVDVSQEDPEVQFNWYVDGVEVHNAKTKPREEQFNSTYRVVSVLAVLHQDWLNGKEYKCKVSNKGLPSSIEKTISKAKGQPREPQVYTLPPSQEEMTKNQVSLTCLVKGFYPSDIAVAWESNGQPENNYKTTPPVLDSDGSFFLYSRLTVDKSRWQEGNVFSCSVMHEALHAHYTQKSLSLSLGK

SEQ ID NO: 103 - protein, 576 aa, synthetic construct
  REGION 1..576: note = Artificial
VIHVTKEVKEVATLSCGHNVSVEELAQTRIYWQKSKKMVLTMMSGDMNIWPEYKNRTIFDITNNLSIVILQLRPSDEGTYECVVLKYEKDAFKREHLAEVTLSVKADGGGGSGGGGSGGGGSGGGGSGEVQLLESGGGLVQPGGSLRLSCAASGFTFSSYAMSWVRQAPGKGLEWVSGISGSGGFTYYADSVKGRFTISRDNSKNTLYLQMNSLRAEDTAVYYCAKPPRGYNYGPFDYWGQGTLVTVSSASTKGPSVFPLAPCSRSTSESTAALGCLVKDYFPEPVTVSWNSGALTSGVHTFPAVLQSSGLYSLSSVVTVPSSSLGTKTYTCNVDHKPSNTKVDKRVESKYGPPCPPCPAPEFLGGPSVFLFPPKPKDTLMISRTPEVTCVVVDVSQEDPEVQFNWYVDGVEVHNAKTKPREEQFNSTYRVVSVLAVLHQDWLNGKEYKCKVSNKGLPSSIEKTISKAKGQPREPQVYTLPPSQEEMTKNQVSLTCLVKGFYPSDIAVAWESNGQPENNYKTTPPVLDSDGSFFLYSRLTVDKSRWQEGNVFSCSVMHEALHAHYTQKSLSLSLGK

SEQ ID NO: 104 - protein, 576 aa, synthetic construct
  REGION 1..576: note = Artificial
VIHVTKEVKEVATLSCGHNVSVEELAQTRIYWQKSKKMVLTMMSGDMNIWPEYKNRTIFDITNNLSIVILTLRPSDEGTYECVVLKYEKDAFKREHLAEVTLSVKADGGGGSGGGGSGGGGSGGGGSGEVQLLESGGGLVQPGGSLRLSCAASGFTFSSYAMSWVRQAPGKGLEWVSGISGSGGFTYYADSVKGRFTISRDNSKNTLYLQMNSLRAEDTAVYYCAKPPRGYNYGPFDYWGQGTLVTVSSASTKGPSVFPLAPCSRSTSESTAALGCLVKDYFPEPVTVSWNSGALTSGVHTFPAVLQSSGLYSLSSVVTVPSSSLGTKTYTCNVDHKPSNTKVDKRVESKYGPPCPPCPAPEFLGGPSVFLFPPKPKDTLMISRTPEVTCVVVDVSQEDPEVQFNWYVDGVEVHNAKTKPREEQFNSTYRVVSVLAVLHQDWLNGKEYKCKVSNKGLPSSIEKTISKAKGQPREPQVYTLPPSQEEMTKNQVSLTCLVKGFYPSDIAVAWESNGQPENNYKTTPPVLDSDGSFFLYSRLTVDKSRWQEGNVFSCSVMHEALHAHYTQKSLSLSLGK

SEQ ID NO: 105 - protein, 576 aa, synthetic construct
  REGION 1..576: note = Artificial
VIHVTKEVKEVATLSCGHNVSVEELAQTRIYWQKQKKMVLTMMSGDMNIWPEYKNRTIFDITNNLSIVILELRPSDEGTYECVVLKYEKDAFKREHLAEVTLSVKADGGGGSGGGGSGGGGSGGGGSGEVQLLESGGGLVQPGGSLRLSCAASGFTFSSYAMSWVRQAPGKGLEWVSGISGSGGFTYYADSVKGRFTISRDNSKNTLYLQMNSLRAEDTAVYYCAKPPRGYNYGPFDYWGQGTLVTVSSASTKGPSVFPLAPCSRSTSESTAALGCLVKDYFPEPVTVSWNSGALTSGVHTFPAVLQSSGLYSLSSVVTVPSSSLGTKTYTCNVDHKPSNTKVDKRVESKYGPPCPPCPAPEFLGGPSVFLFPPKPKDTLMISRTPEVTCVVVDVSQEDPEVQFNWYVDGVEVHNAKTKPREEQFNSTYRVVSVLAVLHQDWLNGKEYKCKVSNKGLPSSIEKTISKAKGQPREPQVYTLPPSQEEMTKNQVSLTCLVKGFYPSDIAVAWESNGQPENNYKTTPPVLDSDGSFFLYSRLTVDKSRWQEGNVFSCSVMHEALHAHYTQKSLSLSLGK

SEQ ID NO: 106 - protein, 576 aa, synthetic construct
  REGION 1..576: note = Artificial
VIHVTKEVKEVATLSCGHNVSVEELAQTRIYWQKQKKMVLTMMSGDMNIWPEYKNRTIFDITNNLSIVILNLRPSDEGTYECVVLKYEKDAFKREHLAEVTLSVKADGGGGSGGGGSGGGGSGGGGSGEVQLLESGGGLVQPGGSLRLSCAASGFTFSSYAMSWVRQAPGKGLEWVSGISGSGGFTYYADSVKGRFTISRDNSKNTLYLQMNSLRAEDTAVYYCAKPPRGYNYGPFDYWGQGTLVTVSSASTKGPSVFPLAPCSRSTSESTAALGCLVKDYFPEPVTVSWNSGALTSGVHTFPAVLQSSGLYSLSSVVTVPSSSLGTKTYTCNVDHKPSNTKVDKRVESKYGPPCPPCPAPEFLGGPSVFLFPPKPKDTLMISRTPEVTCVVVDVSQEDPEVQFNWYVDGVEVHNAKTKPREEQFNSTYRVVSVLAVLHQDWLNGKEYKCKVSNKGLPSSIEKTISKAKGQPREPQVYTLPPSQEEMTKNQVSLTCLVKGFYPSDIAVAWESNGQPENNYKTTPPVLDSDGSFFLYSRLTVDKSRWQEGNVFSCSVMHEALHAHYTQKSLSLSLGK

SEQ ID NO: 107 - protein, 576 aa, synthetic construct
  REGION 1..576: note = Artificial
VIHVTKEVKEVATLSCGHNVSVEELAQTRIYWQKQKKMVLTMMSGDMNIWPEYKNRTIFDITNNLSIVILQLRPSDEGTYECVVLKYEKDAFKREHLAEVTLSVKADGGGGSGGGGSGGGGSGGGGSGEVQLLESGGGLVQPGGSLRLSCAASGFTFSSYAMSWVRQAPGKGLEWVSGISGSGGFTYYADSVKGRFTISRDNSKNTLYLQMNSLRAEDTAVYYCAKPPRGYNYGPFDYWGQGTLVTVSSASTKGPSVFPLAPCSRSTSESTAALGCLVKDYFPEPVTVSWNSGALTSGVHTFPAVLQSSGLYSLSSVVTVPSSSLGTKTYTCNVDHKPSNTKVDKRVESKYGPPCPPCPAPEFLGGPSVFLFPPKPKDTLMISRTPEVTCVVVDVSQEDPEVQFNWYVDGVEVHNAKTKPREEQFNSTYRVVSVLAVLHQDWLNGKEYKCKVSNKGLPSSIEKTISKAKGQPREPQVYTLPPSQEEMTKNQVSLTCLVKGFYPSDIAVAWESNGQPENNYKTTPPVLDSDGSFFLYSRLTVDKSRWQEGNVFSCSVMHEALHAHYTQKSLSLSLGK

SEQ ID NO: 108 - protein, 576 aa, synthetic construct
  REGION 1..576: note = Artificial
VIHVTKEVKEVATLSCGHNVSVEELAQTRIYWQKQKKMVLTMMSGDMNIWPEYKNRTIFDITNNLSIVILTLRPSDEGTYECVVLKYEKDAFKREHLAEVTLSVKADGGGGSGGGGSGGGGSGGGGSGEVQLLESGGGLVQPGGSLRLSCAASGFTFSSYAMSWVRQAPGKGLEWVSGISGSGGFTYYADSVKGRFTISRDNSKNTLYLQMNSLRAEDTAVYYCAKPPRGYNYGPFDYWGQGTLVTVSSASTKGPSVFPLAPCSRSTSESTAALGCLVKDYFPEPVTVSWNSGALTSGVHTFPAVLQSSGLYSLSSVVTVPSSSLGTKTYTCNVDHKPSNTKVDKRVESKYGPPCPPCPAPEFLGGPSVFLFPPKPKDTLMISRTPEVTCVVVDVSQEDPEVQFNWYVDGVEVHNAKTKPREEQFNSTYRVVSVLAVLHQDWLNGKEYKCKVSNKGLPSSIEKTISKAKGQPREPQVYTLPPSQEEMTKNQVSLTCLVKGFYPSDIAVAWESNGQPENNYKTTPPVLDSDGSFFLYSRLTVDKSRWQEGNVFSCSVMHEALHAHYTQKSLSLSLGK

SEQ ID NO: 109 - protein, 576 aa, synthetic construct
  REGION 1..576: note = Artificial
VIHVTKEVKEVATLSCGHNVSVEELAQTRIYWQKTKKMVLTMMSGDMNIWPEYKNRTIFDITNNLSIVILELRPSDEGTYECVVLKYEKDAFKREHLAEVTLSVKADGGGGSGGGGSGGGGSGGGGSGEVQLLESGGGLVQPGGSLRLSCAASGFTFSSYAMSWVRQAPGKGLEWVSGISGSGGFTYYADSVKGRFTISRDNSKNTLYLQMNSLRAEDTAVYYCAKPPRGYNYGPFDYWGQGTLVTVSSASTKGPSVFPLAPCSRSTSESTAALGCLVKDYFPEPVTVSWNSGALTSGVHTFPAVLQSSGLYSLSSVVTVPSSSLGTKTYTCNVDHKPSNTKVDKRVESKYGPPCPPCPAPEFLGGPSVFLFPPKPKDTLMISRTPEVTCVVVDVSQEDPEVQFNWYVDGVEVHNAKTKPREEQFNSTYRVVSVLAVLHQDWLNGKEYKCKVSNKGLPSSIEKTISKAKGQPREPQVYTLPPSQEEMTKNQVSLTCLVKGFYPSDIAVAWESNGQPENNYKTTPPVLDSDGSFFLYSRLTVDKSRWQEGNVFSCSVMHEALHAHYTQKSLSLSLGK

SEQ ID NO: 110 - protein, 576 aa, synthetic construct
  REGION 1..576: note = Artificial
VIHVTKEVKEVATLSCGHNVSVEELAQTRIYWQKTKKMVLTMMSGDMNIWPEYKNRTIFDITNNLSIVILNLRPSDEGTYECVVLKYEKDAFKREHLAEVTLSVKADGGGGSGGGGSGGGGSGGGGSGEVQLLESGGGLVQPGGSLRLSCAASGFTFSSYAMSWVRQAPGKGLEWVSGISGSGGFTYYADSVKGRFTISRDNSKNTLYLQMNSLRAEDTAVYYCAKPPRGYNYGPFDYWGQGTLVTVSSASTKGPSVFPLAPCSRSTSESTAALGCLVKDYFPEPVTVSWNSGALTSGVHTFPAVLQSSGLYSLSSVVTVPSSSLGTKTYTCNVDHKPSNTKVDKRVESKYGPPCPPCPAPEFLGGPSVFLFPPKPKDTLMISRTPEVTCVVVDVSQEDPEVQFNWYVDGVEVHNAKTKPREEQFNSTYRVVSVLAVLHQDWLNGKEYKCKVSNKGLPSSIEKTISKAKGQPREPQVYTLPPSQEEMTKNQVSLTCLVKGFYPSDIAVAWESNGQPENNYKTTPPVLDSDGSFFLYSRLTVDKSRWQEGNVFSCSVMHEALHAHYTQKSLSLSLGK

SEQ ID NO: 111 - protein, 576 aa, synthetic construct
  REGION 1..576: note = Artificial
VIHVTKEVKEVATLSCGHNVSVEELAQTRIYWQKTKKMVLTMMSGDMNIWPEYKNRTIFDITNNLSIVILQLRPSDEGTYECVVLKYEKDAFKREHLAEVTLSVKADGGGGSGGGGSGGGGSGGGGSGEVQLLESGGGLVQPGGSLRLSCAASGFTFSSYAMSWVRQAPGKGLEWVSGISGSGGFTYYADSVKGRFTISRDNSKNTLYLQMNSLRAEDTAVYYCAKPPRGYNYGPFDYWGQGTLVTVSSASTKGPSVFPLAPCSRSTSESTAALGCLVKDYFPEPVTVSWNSGALTSGVHTFPAVLQSSGLYSLSSVVTVPSSSLGTKTYTCNVDHKPSNTKVDKRVESKYGPPCPPCPAPEFLGGPSVFLFPPKPKDTLMISRTPEVTCVVVDVSQEDPEVQFNWYVDGVEVHNAKTKPREEQFNSTYRVVSVLAVLHQDWLNGKEYKCKVSNKGLPSSIEKTISKAKGQPREPQVYTLPPSQEEMTKNQVSLTCLVKGFYPSDIAVAWESNGQPENNYKTTPPVLDSDGSFFLYSRLTVDKSRWQEGNVFSCSVMHEALHAHYTQKSLSLSLGK

SEQ ID NO: 112 - protein, 576 aa, synthetic construct
  REGION 1..576: note = Artificial
VIHVTKEVKEVATLSCGHNVSVEELAQTRIYWQKTKKMVLTMMSGDMNIWPEYKNRTIFDITNNLSIVILTLRPSDEGTYECVVLKYEKDAFKREHLAEVTLSVKADGGGGSGGGGSGGGGSGGGGSGEVQLLESGGGLVQPGGSLRLSCAASGFTFSSYAMSWVRQAPGKGLEWVSGISGSGGFTYYADSVKGRFTISRDNSKNTLYLQMNSLRAEDTAVYYCAKPPRGYNYGPFDYWGQGTLVTVSSASTKGPSVFPLAPCSRSTSESTAALGCLVKDYFPEPVTVSWNSGALTSGVHTFPAVLQSSGLYSLSSVVTVPSSSLGTKTYTCNVDHKPSNTKVDKRVESKYGPPCPPCPAPEFLGGPSVFLFPPKPKDTLMISRTPEVTCVVVDVSQEDPEVQFNWYVDGVEVHNAKTKPREEQFNSTYRVVSVLAVLHQDWLNGKEYKCKVSNKGLPSSIEKTISKAKGQPREPQVYTLPPSQEEMTKNQVSLTCLVKGFYPSDIAVAWESNGQPENNYKTTPPVLDSDGSFFLYSRLTVDKSRWQEGNVFSCSVMHEALHAHYTQKSLSLSLGK

SEQ ID NO: 113 - protein, 576 aa, synthetic construct
  REGION 1..576: note = Artificial
VIHVTKEVKEVATLSCGHNVSVEELAQTRIYWQKEKKMVLTMMSGDANIWPEYKNRTIFDITNNLSIVYLELRPSDEGTYECLVLKYEKDAFKREHLAEVTLSVKADGGGGSGGGGSGGGGSGGGGSGEVQLLESGGGLVQPGGSLRLSCAASGFTFSSYAMSWVRQAPGKGLEWVSGISGSGGFTYYADSVKGRFTISRDNSKNTLYLQMNSLRAEDTAVYYCAKPPRGYNYGPFDYWGQGTLVTVSSASTKGPSVFPLAPCSRSTSESTAALGCLVKDYFPEPVTVSWNSGALTSGVHTFPAVLQSSGLYSLSSVVTVPSSSLGTKTYTCNVDHKPSNTKVDKRVESKYGPPCPPCPAPEFLGGPSVFLFPPKPKDTLMISRTPEVTCVVVDVSQEDPEVQFNWYVDGVEVHNAKTKPREEQFNSTYRVVSVLAVLHQDWLNGKEYKCKVSNKGLPSSIEKTISKAKGQPREPQVYTLPPSQEEMTKNQVSLTCLVKGFYPSDIAVAWESNGQPENNYKTTPPVLDSDGSFFLYSRLTVDKSRWQEGNVFSCSVMHEALHAHYTQKSLSLSLGK

SEQ ID NO: 114 - protein, 576 aa, synthetic construct
  REGION 1..576: note = Artificial
VIHVTKEVKEVATLSCGHNVSVEELAQTRIYWQKEKKMVLTMMSGDANIWPEYKNRTIFDITNNLSIVWLELRPSDEGTYECLVLKYEKDAFKREHLAEVTLSVKADGGGGSGGGGSGGGGSGGGGSGEVQLLESGGGLVQPGGSLRLSCAASGFTFSSYAMSWVRQAPGKGLEWVSGISGSGGFTYYADSVKGRFTISRDNSKNTLYLQMNSLRAEDTAVYYCAKPPRGYNYGPFDYWGQGTLVTVSSASTKGPSVFPLAPCSRSTSESTAALGCLVKDYFPEPVTVSWNSGALTSGVHTFPAVLQSSGLYSLSSVVTVPSSSLGTKTYTCNVDHKPSNTKVDKRVESKYGPPCPPCPAPEFLGGPSVFLFPPKPKDTLMISRTPEVTCVVVDVSQEDPEVQFNWYVDGVEVHNAKTKPREEQFNSTYRVVSVLAVLHQDWLNGKEYKCKVSNKGLPSSIEKTISKAKGQPREPQVYTLPPSQEEMTKNQVSLTCLVKGFYPSDIAVAWESNGQPENNYKTTPPVLDSDGSFFLYSRLTVDKSRWQEGNVFSCSVMHEALHAHYTQKSLSLSLGK

SEQ ID NO: 115 - protein, 576 aa, synthetic construct
  REGION 1..576: note = Artificial
VIHVTKEVKEVATLSCGHNVSVEELAQTRIYWQKEKKMVLTMMSGDANIWPEYKNRTIFDITNNLSIVYLELRPSDEGTYECVVLKYEKDAFKREHLAEVTLSVKADGGGGSGGGGSGGGGSGGGGSGEVQLLESGGGLVQPGGSLRLSCAASGFTFSSYAMSWVRQAPGKGLEWVSGISGSGGFTYYADSVKGRFTISRDNSKNTLYLQMNSLRAEDTAVYYCAKPPRGYNYGPFDYWGQGTLVTVSSASTKGPSVFPLAPCSRSTSESTAALGCLVKDYFPEPVTVSWNSGALTSGVHTFPAVLQSSGLYSLSSVVTVPSSSLGTKTYTCNVDHKPSNTKVDKRVESKYGPPCPPCPAPEFLGGPSVFLFPPKPKDTLMISRTPEVTCVVVDVSQEDPEVQFNWYVDGVEVHNAKTKPREEQFNSTYRVVSVLAVLHQDWLNGKEYKCKVSNKGLPSSIEKTISKAKGQPREPQVYTLPPSQEEMTKNQVSLTCLVKGFYPSDIAVAWESNGQPENNYKTTPPVLDSDGSFFLYSRLTVDKSRWQEGNVFSCSVMHEALHAHYTQKSLSLSLGK

SEQ ID NO: 116 - protein, 576 aa, synthetic construct
  REGION 1..576: note = Artificial
VIHVTKEVKEVATLSCGHNVSVEELAQTRIYWQKEKKMVLTMMSGDANIWPEYKNRTIFDITNNLSIVWLELRPSDEGTYECVVLKYEKDAFKREHLAEVTLSVKADGGGGSGGGGSGGGGSGGGGSGEVQLLESGGGLVQPGGSLRLSCAASGFTFSSYAMSWVRQAPGKGLEWVSGISGSGGFTYYADSVKGRFTISRDNSKNTLYLQMNSLRAEDTAVYYCAKPPRGYNYGPFDYWGQGTLVTVSSASTKGPSVFPLAPCSRSTSESTAALGCLVKDYFPEPVTVSWNSGALTSGVHTFPAVLQSSGLYSLSSVVTVPSSSLGTKTYTCNVDHKPSNTKVDKRVESKYGPPCPPCPAPEFLGGPSVFLFPPKPKDTLMISRTPEVTCVVVDVSQEDPEVQFNWYVDGVEVHNAKTKPREEQFNSTYRVVSVLAVLHQDWLNGKEYKCKVSNKGLPSSIEKTISKAKGQPREPQVYTLPPSQEEMTKNQVSLTCLVKGFYPSDIAVAWESNGQPENNYKTTPPVLDSDGSFFLYSRLTVDKSRWQEGNVFSCSVMHEALHAHYTQKSLSLSLGK

SEQ ID NO: 117 - protein, 576 aa, synthetic construct
  REGION 1..576: note = Artificial
VIHVTKEVKEVATLSCGHNVSVEELAQTRIYWQKEKKMVLTMMSGDMNIWPEYKNRTIFDITNNLSIVYLELRPSDEGTYECLVLKYEKDAFKREHLAEVTLSVKADGGGGSGGGGSGGGGSGGGGSGEVQLLESGGGLVQPGGSLRLSCAASGFTFSSYAMSWVRQAPGKGLEWVSGISGSGGFTYYADSVKGRFTISRDNSKNTLYLQMNSLRAEDTAVYYCAKPPRGYNYGPFDYWGQGTLVTVSSASTKGPSVFPLAPCSRSTSESTAALGCLVKDYFPEPVTVSWNSGALTSGVHTFPAVLQSSGLYSLSSVVTVPSSSLGTKTYTCNVDHKPSNTKVDKRVESKYGPPCPPCPAPEFLGGPSVFLFPPKPKDTLMISRTPEVTCVVVDVSQEDPEVQFNWYVDGVEVHNAKTKPREEQFNSTYRVVSVLAVLHQDWLNGKEYKCKVSNKGLPSSIEKTISKAKGQPREPQVYTLPPSQEEMTKNQVSLTCLVKGFYPSDIAVAWESNGQPENNYKTTPPVLDSDGSFFLYSRLTVDKSRWQEGNVFSCSVMHEALHAHYTQKSLSLSLGK

SEQ ID NO: 118 - protein, 576 aa, synthetic construct
  REGION 1..576: note = Artificial
VIHVTKEVKEVATLSCGHNVSVEELAQTRIYWQKEKKMVLTMMSGDMNIWPEYKNRTIFDITNNLSIVWLELRPSDEGTYECLVLKYEKDAFKREHLAEVTLSVKADGGGGSGGGGSGGGGSGGGGSGEVQLLESGGGLVQPGGSLRLSCAASGFTFSSYAMSWVRQAPGKGLEWVSGISGSGGFTYYADSVKGRFTISRDNSKNTLYLQMNSLRAEDTAVYYCAKPPRGYNYGPFDYWGQGTLVTVSSASTKGPSVFPLAPCSRSTSESTAALGCLVKDYFPEPVTVSWNSGALTSGVHTFPAVLQSSGLYSLSSVVTVPSSSLGTKTYTCNVDHKPSNTKVDKRVESKYGPPCPPCPAPEFLGGPSVFLFPPKPKDTLMISRTPEVTCVVVDVSQEDPEVQFNWYVDGVEVHNAKTKPREEQFNSTYRVVSVLAVLHQDWLNGKEYKCKVSNKGLPSSIEKTISKAKGQPREPQVYTLPPSQEEMTKNQVSLTCLVKGFYPSDIAVAWESNGQPENNYKTTPPVLDSDGSFFLYSRLTVDKSRWQEGNVFSCSVMHEALHAHYTQKSLSLSLGK

SEQ ID NO: 119 - protein, 576 aa, synthetic construct
  REGION 1..576: note = Artificial
VIHVTKEVKEVATLSCGHNVSVEELAQTRIYWQKEKKMVLTMMSGDMNIWPEYKNRTIFDITNNLSIVYLELRPSDEGTYECVVLKYEKDAFKREHLAEVTLSVKADGGGGSGGGGSGGGGSGGGGSGEVQLLESGGGLVQPGGSLRLSCAASGFTFSSYAMSWVRQAPGKGLEWVSGISGSGGFTYYADSVKGRFTISRDNSKNTLYLQMNSLRAEDTAVYYCAKPPRGYNYGPFDYWGQGTLVTVSSASTKGPSVFPLAPCSRSTSESTAALGCLVKDYFPEPVTVSWNSGALTSGVHTFPAVLQSSGLYSLSSVVTVPSSSLGTKTYTCNVDHKPSNTKVDKRVESKYGPPCPPCPAPEFLGGPSVFLFPPKPKDTLMISRTPEVTCVVVDVSQEDPEVQFNWYVDGVEVHNAKTKPREEQFNSTYRVVSVLAVLHQDWLNGKEYKCKVSNKGLPSSIEKTISKAKGQPREPQVYTLPPSQEEMTKNQVSLTCLVKGFYPSDIAVAWESNGQPENNYKTTPPVLDSDGSFFLYSRLTVDKSRWQEGNVFSCSVMHEALHAHYTQKSLSLSLGK

SEQ ID NO: 120 - protein, 576 aa, synthetic construct
  REGION 1..576: note = Artificial
VIHVTKEVKEVATLSCGHNVSVEELAQTRIYWQKEKKMVLTMMSGDMNIWPEYKNRTIFDITNNLSIVWLELRPSDEGTYECVVLKYEKDAFKREHLAEVTLSVKADGGGGSGGGGSGGGGSGGGGSGEVQLLESGGGLVQPGGSLRLSCAASGFTFSSYAMSWVRQAPGKGLEWVSGISGSGGFTYYADSVKGRFTISRDNSKNTLYLQMNSLRAEDTAVYYCAKPPRGYNYGPFDYWGQGTLVTVSSASTKGPSVFPLAPCSRSTSESTAALGCLVKDYFPEPVTVSWNSGALTSGVHTFPAVLQSSGLYSLSSVVTVPSSSLGTKTYTCNVDHKPSNTKVDKRVESKYGPPCPPCPAPEFLGGPSVFLFPPKPKDTLMISRTPEVTCVVVDVSQEDPEVQFNWYVDGVEVHNAKTKPREEQFNSTYRVVSVLAVLHQDWLNGKEYKCKVSNKGLPSSIEKTISKAKGQPREPQVYTLPPSQEEMTKNQVSLTCLVKGFYPSDIAVAWESNGQPENNYKTTPPVLDSDGSFFLYSRLTVDKSRWQEGNVFSCSVMHEALHAHYTQKSLSLSLGK

SEQ ID NO: 121 - protein, 576 aa, synthetic construct
  REGION 1..576: note = Artificial
VIHVTKEVKEVATLSCGWNVSVEELMQTRIYWQKEKKMVLTMMSGDMNIWPEYKNRTIFDITNNLSIVILELRPSDEGTYECVVNKYEKDAFKREHLAEVTLSVKADGGGGSGGGGSGGGGSGGGGSGEVQLLESGGGLVQPGGSLRLSCAASGFTFSSYAMSWVRQAPGKGLEWVSGISGSGGFTYYADSVKGRFTISRDNSKNTLYLQMNSLRAEDTAVYYCAKPPRGYNYGPFDYWGQGTLVTVSSASTKGPSVFPLAPCSRSTSESTAALGCLVKDYFPEPVTVSWNSGALTSGVHTFPAVLQSSGLYSLSSVVTVPSSSLGTKTYTCNVDHKPSNTKVDKRVESKYGPPCPPCPAPEFLGGPSVFLFPPKPKDTLMISRTPEVTCVVVDVSQEDPEVQFNWYVDGVEVHNAKTKPREEQFNSTYRVVSVLAVLHQDWLNGKEYKCKVSNKGLPSSIEKTISKAKGQPREPQVYTLPPSQEEMTKNQVSLTCLVKGFYPSDIAVAWESNGQPENNYKTTPPVLDSDGSFFLYSRLTVDKSRWQEGNVFSCSVMHEALHAHYTQKSLSLSLGK

SEQ ID NO: 122 - protein, 576 aa, synthetic construct
  REGION 1..576: note = Artificial
VIHVTKEVKEVATLSCGWNVSVEELMQTRIYWQKEKKMVLTMMSGDMNIWPEYKNRTIFDITNNLSIVILELRPSDEGTYECVVDKYEKDAFKREHLAEVTLSVKADGGGGSGGGGSGGGGSGGGGSGEVQLLESGGGLVQPGGSLRLSCAASGFTFSSYAMSWVRQAPGKGLEWVSGISGSGGFTYYADSVKGRFTISRDNSKNTLYLQMNSLRAEDTAVYYCAKPPRGYNYGPFDYWGQGTLVTVSSASTKGPSVFPLAPCSRSTSESTAALGCLVKDYFPEPVTVSWNSGALTSGVHTFPAVLQSSGLYSLSSVVTVPSSSLGTKTYTCNVDHKPSNTKVDKRVESKYGPPCPPCPAPEFLGGPSVFLFPPKPKDTLMISRTPEVTCVVVDVSQEDPEVQFNWYVDGVEVHNAKTKPREEQFNSTYRVVSVLAVLHQDWLNGKEYKCKVSNKGLPSSIEKTISKAKGQPREPQVYTLPPSQEEMTKNQVSLTCLVKGFYPSDIAVAWESNGQPENNYKTTPPVLDSDGSFFLYSRLTVDKSRWQEGNVFSCSVMHEALHAHYTQKSLSLSLGK

SEQ ID NO: 123 - protein, 576 aa, synthetic construct
  REGION 1..576: note = Artificial
VIHVTKEVKEVATLSCGWNVSVEELCQTRIYWQKEKKMVLTMMSGDMNIWPEYKNRTIFDITNNLSIVILELRPSDEGTYECVVNKYEKDAFKREHLAEVTLSVKADGGGGSGGGGSGGGGSGGGGSGEVQLLESGGGLVQPGGSLRLSCAASGFTFSSYAMSWVRQAPGKGLEWVSGISGSGGFTYYADSVKGRFTISRDNSKNTLYLQMNSLRAEDTAVYYCAKPPRGYNYGPFDYWGQGTLVTVSSASTKGPSVFPLAPCSRSTSESTAALGCLVKDYFPEPVTVSWNSGALTSGVHTFPAVLQSSGLYSLSSVVTVPSSSLGTKTYTCNVDHKPSNTKVDKRVESKYGPPCPPCPAPEFLGGPSVFLFPPKPKDTLMISRTPEVTCVVVDVSQEDPEVQFNWYVDGVEVHNAKTKPREEQFNSTYRVVSVLAVLHQDWLNGKEYKCKVSNKGLPSSIEKTISKAKGQPREPQVYTLPPSQEEMTKNQVSLTCLVKGFYPSDIAVAWESNGQPENNYKTTPPVLDSDGSFFLYSRLTVDKSRWQEGNVFSCSVMHEALHAHYTQKSLSLSLGK

SEQ ID NO: 124 - protein, 576 aa, synthetic construct
  REGION 1..576: note = Artificial
VIHVTKEVKEVATLSCGWNVSVEELCQTRIYWQKEKKMVLTMMSGDMNIWPEYKNRTIFDITNNLSIVILELRPSDEGTYECVVDKYEKDAFKREHLAEVTLSVKADGGGGSGGGGSGGGGSGGGGSGEVQLLESGGGLVQPGGSLRLSCAASGFTFSSYAMSWVRQAPGKGLEWVSGISGSGGFTYYADSVKGRFTISRDNSKNTLYLQMNSLRAEDTAVYYCAKPPRGYNYGPFDYWGQGTLVTVSSASTKGPSVFPLAPCSRSTSESTAALGCLVKDYFPEPVTVSWNSGALTSGVHTFPAVLQSSGLYSLSSVVTVPSSSLGTKTYTCNVDHKPSNTKVDKRVESKYGPPCPPCPAPEFLGGPSVFLFPPKPKDTLMISRTPEVTCVVVDVSQEDPEVQFNWYVDGVEVHNAKTKPREEQFNSTYRVVSVLAVLHQDWLNGKEYKCKVSNKGLPSSIEKTISKAKGQPREPQVYTLPPSQEEMTKNQVSLTCLVKGFYPSDIAVAWESNGQPENNYKTTPPVLDSDGSFFLYSRLTVDKSRWQEGNVFSCSVMHEALHAHYTQKSLSLSLGK

SEQ ID NO: 125 - protein, 576 aa, synthetic construct
  REGION 1..576: note = Artificial
VIHVTKEVKEVATLSCGHNVSVEELMQTRIYWQKEKKMVLTMMSGDMNIWPEYKNRTIFDITNNLSIVILELRPSDEGTYECVVNKYEKDAFKREHLAEVTLSVKADGGGGSGGGGSGGGGSGGGGSGEVQLLESGGGLVQPGGSLRLSCAASGFTFSSYAMSWVRQAPGKGLEWVSGISGSGGFTYYADSVKGRFTISRDNSKNTLYLQMNSLRAEDTAVYYCAKPPRGYNYGPFDYWGQGTLVTVSSASTKGPSVFPLAPCSRSTSESTAALGCLVKDYFPEPVTVSWNSGALTSGVHTFPAVLQSSGLYSLSSVVTVPSSSLGTKTYTCNVDHKPSNTKVDKRVESKYGPPCPPCPAPEFLGGPSVFLFPPKPKDTLMISRTPEVTCVVVDVSQEDPEVQFNWYVDGVEVHNAKTKPREEQFNSTYRVVSVLAVLHQDWLNGKEYKCKVSNKGLPSSIEKTISKAKGQPREPQVYTLPPSQEEMTKNQVSLTCLVKGFYPSDIAVAWESNGQPENNYKTTPPVLDSDGSFFLYSRLTVDKSRWQEGNVFSCSVMHEALHAHYTQKSLSLSLGK

SEQ ID NO: 126 - protein, 576 aa, synthetic construct
  REGION 1..576: note = Artificial
VIHVTKEVKEVATLSCGHNVSVEELMQTRIYWQKEKKMVLTMMSGDMNIWPEYKNRTIFDITNNLSIVILELRPSDEGTYECVVDKYEKDAFKREHLAEVTLSVKADGGGGSGGGGSGGGGSGGGGSGEVQLLESGGGLVQPGGSLRLSCAASGFTFSSYAMSWVRQAPGKGLEWVSGISGSGGFTYYADSVKGRFTISRDNSKNTLYLQMNSLRAEDTAVYYCAKPPRGYNYGPFDYWGQGTLVTVSSASTKGPSVFPLAPCSRSTSESTAALGCLVKDYFPEPVTVSWNSGALTSGVHTFPAVLQSSGLYSLSSVVTVPSSSLGTKTYTCNVDHKPSNTKVDKRVESKYGPPCPPCPAPEFLGGPSVFLFPPKPKDTLMISRTPEVTCVVVDVSQEDPEVQFNWYVDGVEVHNAKTKPREEQFNSTYRVVSVLAVLHQDWLNGKEYKCKVSNKGLPSSIEKTISKAKGQPREPQVYTLPPSQEEMTKNQVSLTCLVKGFYPSDIAVAWESNGQPENNYKTTPPVLDSDGSFFLYSRLTVDKSRWQEGNVFSCSVMHEALHAHYTQKSLSLSLGK

SEQ ID NO: 127 - protein, 576 aa, synthetic construct
  REGION 1..576: note = Artificial
VIHVTKEVKEVATLSCGHNVSVEELCQTRIYWQKEKKMVLTMMSGDMNIWPEYKNRTIFDITNNLSIVILELRPSDEGTYECVVDKYEKDAFKREHLAEVTLSVKADGGGGSGGGGSGGGGSGGGGSGEVQLLESGGGLVQPGGSLRLSCAASGFTFSSYAMSWVRQAPGKGLEWVSGISGSGGFTYYADSVKGRFTISRDNSKNTLYLQMNSLRAEDTAVYYCAKPPRGYNYGPFDYWGQGTLVTVSSASTKGPSVFPLAPCSRSTSESTAALGCLVKDYFPEPVTVSWNSGALTSGVHTFPAVLQSSGLYSLSSVVTVPSSSLGTKTYTCNVDHKPSNTKVDKRVESKYGPPCPPCPAPEFLGGPSVFLFPPKPKDTLMISRTPEVTCVVVDVSQEDPEVQFNWYVDGVEVHNAKTKPREEQFNSTYRVVSVLAVLHQDWLNGKEYKCKVSNKGLPSSIEKTISKAKGQPREPQVYTLPPSQEEMTKNQVSLTCLVKGFYPSDIAVAWESNGQPENNYKTTPPVLDSDGSFFLYSRLTVDKSRWQEGNVFSCSVMHEALHAHYTQKSLSLSLGK

SEQ ID NO: 128 - protein, 576 aa, synthetic construct
  REGION 1..576: note = Artificial
VIHVTKEVKEVATLSCGHNVSVEELCQTRIYWQKEKKMVLTMMSGDMNIWPEYKNRTIFDITNNLSIVILELRPSDEGTYECVVNKYEKDAFKREHLAEVTLSVKADGGGGSGGGGSGGGGSGGGGSGEVQLLESGGGLVQPGGSLRLSCAASGFTFSSYAMSWVRQAPGKGLEWVSGISGSGGFTYYADSVKGRFTISRDNSKNTLYLQMNSLRAEDTAVYYCAKPPRGYNYGPFDYWGQGTLVTVSSASTKGPSVFPLAPCSRSTSESTAALGCLVKDYFPEPVTVSWNSGALTSGVHTFPAVLQSSGLYSLSSVVTVPSSSLGTKTYTCNVDHKPSNTKVDKRVESKYGPPCPPCPAPEFLGGPSVFLFPPKPKDTLMISRTPEVTCVVVDVSQEDPEVQFNWYVDGVEVHNAKTKPREEQFNSTYRVVSVLAVLHQDWLNGKEYKCKVSNKGLPSSIEKTISKAKGQPREPQVYTLPPSQEEMTKNQVSLTCLVKGFYPSDIAVAWESNGQPENNYKTTPPVLDSDGSFFLYSRLTVDKSRWQEGNVFSCSVMHEALHAHYTQKSLSLSLGK

SEQ ID NO: 129 - protein, 576 aa, synthetic construct
  REGION 1..576: note = Artificial
VIHVTKEVKEVATLSCGHNVSVEELAQTRIYWQKEKKMVLTMMSGDMNIWPEYKNRTIFDITNNLSIVLLELRPSDEGTYECLVLKYEKDAFKREHLAEVTLSVKADGGGGSGGGGSGGGGSGGGGSGEVQLLESGGGLVQPGGSLRLSCAASGFTFSSYAMSWVRQAPGKGLEWVSGISGSGGFTYYADSVKGRFTISRDNSKNTLYLQMNSLRAEDTAVYYCAKPPRGYNYGPFDYWGQGTLVTVSSASTKGPSVFPLAPCSRSTSESTAALGCLVKDYFPEPVTVSWNSGALTSGVHTFPAVLQSSGLYSLSSVVTVPSSSLGTKTYTCNVDHKPSNTKVDKRVESKYGPPCPPCPAPEFLGGPSVFLFPPKPKDTLMISRTPEVTCVVVDVSQEDPEVQFNWYVDGVEVHNAKTKPREEQFNSTYRVVSVLAVLHQDWLNGKEYKCKVSNKGLPSSIEKTISKAKGQPREPQVYTLPPSQEEMTKNQVSLTCLVKGFYPSDIAVAWESNGQPENNYKTTPPVLDSDGSFFLYSRLTVDKSRWQEGNVFSCSVMHEALHAHYTQKSLSLSLGK

SEQ ID NO: 130 - protein, 576 aa, synthetic construct
  REGION 1..576: note = Artificial
VIHVTKEVKEVATLSCGWNVSVEELVQTRIYWQKNKKMVLTMMSGDMNIWPEYKNRTIFDITNNLSIVILELRPSDEGTYECVVNKYEKDAFKREHLAEVTLSVKADGGGGSGGGGSGGGGSGGGGSGEVQLLESGGGLVQPGGSLRLSCAASGFTFSSYAMSWVRQAPGKGLEWVSGISGSGGFTYYADSVKGRFTISRDNSKNTLYLQMNSLRAEDTAVYYCAKPPRGYNYGPFDYWGQGTLVTVSSASTKGPSVFPLAPCSRSTSESTAALGCLVKDYFPEPVTVSWNSGALTSGVHTFPAVLQSSGLYSLSSVVTVPSSSLGTKTYTCNVDHKPSNTKVDKRVESKYGPPCPPCPAPEFLGGPSVFLFPPKPKDTLMISRTPEVTCVVVDVSQEDPEVQFNWYVDGVEVHNAKTKPREEQFNSTYRVVSVLAVLHQDWLNGKEYKCKVSNKGLPSSIEKTISKAKGQPREPQVYTLPPSQEEMTKNQVSLTCLVKGFYPSDIAVAWESNGQPENNYKTTPPVLDSDGSFFLYSRLTVDKSRWQEGNVFSCSVMHEALHAHYTQKSLSLSLGK

SEQ ID NO: 131 - protein, 576 aa, synthetic construct
  REGION 1..576: note = Artificial
VIHVTKEVKEVAKLSCGHNVSVEELAQTRIYWQKEKKMVLTLMSGDHNIWPEYKNRTIFDITNNLSIVILELRPSDEGTYECVVLKYEKDAFKREHLAEVTLSVKADGGGGSGGGGSGGGGSGGGGSGEVQLLESGGGLVQPGGSLRLSCAASGFTFSSYAMSWVRQAPGKGLEWVSGISGSGGFTYYADSVKGRFTISRDNSKNTLYLQMNSLRAEDTAVYYCAKPPRGYNYGPFDYWGQGTLVTVSSASTKGPSVFPLAPCSRSTSESTAALGCLVKDYFPEPVTVSWNSGALTSGVHTFPAVLQSSGLYSLSSVVTVPSSSLGTKTYTCNVDHKPSNTKVDKRVESKYGPPCPPCPAPEFLGGPSVFLFPPKPKDTLMISRTPEVTCVVVDVSQEDPEVQFNWYVDGVEVHNAKTKPREEQFNSTYRVVSVLAVLHQDWLNGKEYKCKVSNKGLPSSIEKTISKAKGQPREPQVYTLPPSQEEMTKNQVSLTCLVKGFYPSDIAVAWESNGQPENNYKTTPPVLDSDGSFFLYSRLTVDKSRWQEGNVFSCSVMHEALHAHYTQKSLSLSLGK

SEQ ID NO: 132 - protein, 576 aa, synthetic construct
  REGION 1..576: note = Artificial
VIHVTKEVKEVAKLSCGHNVSVEELAQTRIYWQKEKKMVLTLMSGDQNIWPEYKNRTIFDITNNLSIVILELRPSDEGTYECVVLKYEKDAFKREHLAEVTLSVKADGGGGSGGGGSGGGGSGGGGSGEVQLLESGGGLVQPGGSLRLSCAASGFTFSSYAMSWVRQAPGKGLEWVSGISGSGGFTYYADSVKGRFTISRDNSKNTLYLQMNSLRAEDTAVYYCAKPPRGYNYGPFDYWGQGTLVTVSSASTKGPSVFPLAPCSRSTSESTAALGCLVKDYFPEPVTVSWNSGALTSGVHTFPAVLQSSGLYSLSSVVTVPSSSLGTKTYTCNVDHKPSNTKVDKRVESKYGPPCPPCPAPEFLGGPSVFLFPPKPKDTLMISRTPEVTCVVVDVSQEDPEVQFNWYVDGVEVHNAKTKPREEQFNSTYRVVSVLAVLHQDWLNGKEYKCKVSNKGLPSSIEKTISKAKGQPREPQVYTLPPSQEEMTKNQVSLTCLVKGFYPSDIAVAWESNGQPENNYKTTPPVLDSDGSFFLYSRLTVDKSRWQEGNVFSCSVMHEALHAHYTQKSLSLSLGK

SEQ ID NO: 133 - protein, 576 aa, synthetic construct
  REGION 1..576: note = Artificial
VIHVTKEVKEVAKLSCGHNVSVEELAQTRIYWQKEKKMVLTLMSGDMNIWPEYKNRTIFDITNNLSIVILELRPSDEGTYECVVLKYEKDAFKREHLAEVTLSVKADGGGGSGGGGSGGGGSGGGGSGEVQLLESGGGLVQPGGSLRLSCAASGFTFSSYAMSWVRQAPGKGLEWVSGISGSGGFTYYADSVKGRFTISRDNSKNTLYLQMNSLRAEDTAVYYCAKPPRGYNYGPFDYWGQGTLVTVSSASTKGPSVFPLAPCSRSTSESTAALGCLVKDYFPEPVTVSWNSGALTSGVHTFPAVLQSSGLYSLSSVVTVPSSSLGTKTYTCNVDHKPSNTKVDKRVESKYGPPCPPCPAPEFLGGPSVFLFPPKPKDTLMISRTPEVTCVVVDVSQEDPEVQFNWYVDGVEVHNAKTKPREEQFNSTYRVVSVLAVLHQDWLNGKEYKCKVSNKGLPSSIEKTISKAKGQPREPQVYTLPPSQEEMTKNQVSLTCLVKGFYPSDIAVAWESNGQPENNYKTTPPVLDSDGSFFLYSRLTVDKSRWQEGNVFSCSVMHEALHAHYTQKSLSLSLGK

SEQ ID NO: 134 - protein, 576 aa, synthetic construct
  REGION 1..576: note = Artificial
VIHVTKEVKEVAKLSCGHNVSVEELAQTRIYWQKEKKMVLTTMSGDHNIWPEYKNRTIFDITNNLSIVILELRPSDEGTYECVVLKYEKDAFKREHLAEVTLSVKADGGGGSGGGGSGGGGSGGGGSGEVQLLESGGGLVQPGGSLRLSCAASGFTFSSYAMSWVRQAPGKGLEWVSGISGSGGFTYYADSVKGRFTISRDNSKNTLYLQMNSLRAEDTAVYYCAKPPRGYNYGPFDYWGQGTLVTVSSASTKGPSVFPLAPCSRSTSESTAALGCLVKDYFPEPVTVSWNSGALTSGVHTFPAVLQSSGLYSLSSVVTVPSSSLGTKTYTCNVDHKPSNTKVDKRVESKYGPPCPPCPAPEFLGGPSVFLFPPKPKDTLMISRTPEVTCVVVDVSQEDPEVQFNWYVDGVEVHNAKTKPREEQFNSTYRVVSVLAVLHQDWLNGKEYKCKVSNKGLPSSIEKTISKAKGQPREPQVYTLPPSQEEMTKNQVSLTCLVKGFYPSDIAVAWESNGQPENNYKTTPPVLDSDGSFFLYSRLTVDKSRWQEGNVFSCSVMHEALHAHYTQKSLSLSLGK

SEQ ID NO: 135 - protein, 576 aa, synthetic construct
  REGION 1..576: note = Artificial
VIHVTKEVKEVAKLSCGHNVSVEELAQTRIYWQKEKKMVLTTMSGDQNIWPEYKNRTIFDITNNLSIVILELRPSDEGTYECVVLKYEKDAFKREHLAEVTLSVKADGGGGSGGGGSGGGGSGGGGSGEVQLLESGGGLVQPGGSLRLSCAASGFTFSSYAMSWVRQAPGKGLEWVSGISGSGGFTYYADSVKGRFTISRDNSKNTLYLQMNSLRAEDTAVYYCAKPPRGYNYGPFDYWGQGTLVTVSSASTKGPSVFPLAPCSRSTSESTAALGCLVKDYFPEPVTVSWNSGALTSGVHTFPAVLQSSGLYSLSSVVTVPSSSLGTKTYTCNVDHKPSNTKVDKRVESKYGPPCPPCPAPEFLGGPSVFLFPPKPKDTLMISRTPEVTCVVVDVSQEDPEVQFNWYVDGVEVHNAKTKPREEQFNSTYRVVSVLAVLHQDWLNGKEYKCKVSNKGLPSSIEKTISKAKGQPREPQVYTLPPSQEEMTKNQVSLTCLVKGFYPSDIAVAWESNGQPENNYKTTPPVLDSDGSFFLYSRLTVDKSRWQEGNVFSCSVMHEALHAHYTQKSLSLSLGK

SEQ ID NO: 136 - protein, 576 aa, synthetic construct
  REGION 1..576: note = Artificial
VIHVTKEVKEVAKLSCGHNVSVEELAQTRIYWQKEKKMVLTTMSGDMNIWPEYKNRTIFDITNNLSIVILELRPSDEGTYECVVLKYEKDAFKREHLAEVTLSVKADGGGGSGGGGSGGGGSGGGGSGEVQLLESGGGLVQPGGSLRLSCAASGFTFSSYAMSWVRQAPGKGLEWVSGISGSGGFTYYADSVKGRFTISRDNSKNTLYLQMNSLRAEDTAVYYCAKPPRGYNYGPFDYWGQGTLVTVSSASTKGPSVFPLAPCSRSTSESTAALGCLVKDYFPEPVTVSWNSGALTSGVHTFPAVLQSSGLYSLSSVVTVPSSSLGTKTYTCNVDHKPSNTKVDKRVESKYGPPCPPCPAPEFLGGPSVFLFPPKPKDTLMISRTPEVTCVVVDVSQEDPEVQFNWYVDGVEVHNAKTKPREEQFNSTYRVVSVLAVLHQDWLNGKEYKCKVSNKGLPSSIEKTISKAKGQPREPQVYTLPPSQEEMTKNQVSLTCLVKGFYPSDIAVAWESNGQPENNYKTTPPVLDSDGSFFLYSRLTVDKSRWQEGNVFSCSVMHEALHAHYTQKSLSLSLGK

SEQ ID NO: 137 - protein, 576 aa, synthetic construct
  REGION 1..576: note = Artificial
VIHVTKEVKEVATLSCGHNVSVEELAQTRIYWQKEKKMVLTMMSGDHNIWPEYKNRTIFDITNNLSIVYLELRPSDEGTYECLVLKYEKDAFKREHLAEVTLSVKADGGGGSGGGGSGGGGSGGGGSGEVQLLESGGGLVQPGGSLRLSCAASGFTFSSYAMSWVRQAPGKGLEWVSGISGSGGFTYYADSVKGRFTISRDNSKNTLYLQMNSLRAEDTAVYYCAKPPRGYNYGPFDYWGQGTLVTVSSASTKGPSVFPLAPCSRSTSESTAALGCLVKDYFPEPVTVSWNSGALTSGVHTFPAVLQSSGLYSLSSVVTVPSSSLGTKTYTCNVDHKPSNTKVDKRVESKYGPPCPPCPAPEFLGGPSVFLFPPKPKDTLMISRTPEVTCVVVDVSQEDPEVQFNWYVDGVEVHNAKTKPREEQFNSTYRVVSVLAVLHQDWLNGKEYKCKVSNKGLPSSIEKTISKAKGQPREPQVYTLPPSQEEMTKNQVSLTCLVKGFYPSDIAVAWESNGQPENNYKTTPPVLDSDGSFFLYSRLTVDKSRWQEGNVFSCSVMHEALHAHYTQKSLSLSLGK

SEQ ID NO: 138 - protein, 576 aa, synthetic construct
  REGION 1..576: note = Artificial
VIHVTKEVKEVATLSCGHNVSVEELAQTRIYWQKEKKMVLTMMSGDQNIWPEYKNRTIFDITNNLSIVYLELRPSDEGTYECLVLKYEKDAFKREHLAEVTLSVKADGGGGSGGGGSGGGGSGGGGSGEVQLLESGGGLVQPGGSLRLSCAASGFTFSSYAMSWVRQAPGKGLEWVSGISGSGGFTYYADSVKGRFTISRDNSKNTLYLQMNSLRAEDTAVYYCAKPPRGYNYGPFDYWGQGTLVTVSSASTKGPSVFPLAPCSRSTSESTAALGCLVKDYFPEPVTVSWNSGALTSGVHTFPAVLQSSGLYSLSSVVTVPSSSLGTKTYTCNVDHKPSNTKVDKRVESKYGPPCPPCPAPEFLGGPSVFLFPPKPKDTLMISRTPEVTCVVVDVSQEDPEVQFNWYVDGVEVHNAKTKPREEQFNSTYRVVSVLAVLHQDWLNGKEYKCKVSNKGLPSSIEKTISKAKGQPREPQVYTLPPSQEEMTKNQVSLTCLVKGFYPSDIAVAWESNGQPENNYKTTPPVLDSDGSFFLYSRLTVDKSRWQEGNVFSCSVMHEALHAHYTQKSLSLSLGK

SEQ ID NO: 139 - protein, 576 aa, synthetic construct
  REGION 1..576: note = Artificial
VIHVTKEVKEVATLSCGHNVSVEELAQTRIYWQKEKKMVLTMMSGDKNIWPEYKNRTIFDITNNLSIVYLELRPSDEGTYECLVLKYEKDAFKREHLAEVTLSVKADGGGGSGGGGSGGGGSGGGGSGEVQLLESGGGLVQPGGSLRLSCAASGFTFSSYAMSWVRQAPGKGLEWVSGISGSGGFTYYADSVKGRFTISRDNSKNTLYLQMNSLRAEDTAVYYCAKPPRGYNYGPFDYWGQGTLVTVSSASTKGPSVFPLAPCSRSTSESTAALGCLVKDYFPEPVTVSWNSGALTSGVHTFPAVLQSSGLYSLSSVVTVPSSSLGTKTYTCNVDHKPSNTKVDKRVESKYGPPCPPCPAPEFLGGPSVFLFPPKPKDTLMISRTPEVTCVVVDVSQEDPEVQFNWYVDGVEVHNAKTKPREEQFNSTYRVVSVLAVLHQDWLNGKEYKCKVSNKGLPSSIEKTISKAKGQPREPQVYTLPPSQEEMTKNQVSLTCLVKGFYPSDIAVAWESNGQPENNYKTTPPVLDSDGSFFLYSRLTVDKSRWQEGNVFSCSVMHEALHAHYTQKSLSLSLGK

SEQ ID NO: 140 - protein, 576 aa, synthetic construct
  REGION 1..576: note = Artificial
VIHVTKEVKEVATLSCGHNVSVEELAQTRIYWQKEKKMVLTMMSGDMNIWPEYKNRTIFDITNNLSIVILALRPSDEGTYECVVLKYEKDAFKREHLAEVTLSVKADGGGGSGGGGSGGGGSGGGGSGEVQLLESGGGLVQPGGSLRLSCAASGFTFSSYAMSWVRQAPGKGLEWVSGISGSGGFTYYADSVKGRFTISRDNSKNTLYLQMNSLRAEDTAVYYCAKPPRGYNYGPFDYWGQGTLVTVSSASTKGPSVFPLAPCSRSTSESTAALGCLVKDYFPEPVTVSWNSGALTSGVHTFPAVLQSSGLYSLSSVVTVPSSSLGTKTYTCNVDHKPSNTKVDKRVESKYGPPCPPCPAPEFLGGPSVFLFPPKPKDTLMISRTPEVTCVVVDVSQEDPEVQFNWYVDGVEVHNAKTKPREEQFNSTYRVVSVLAVLHQDWLNGKEYKCKVSNKGLPSSIEKTISKAKGQPREPQVYTLPPSQEEMTKNQVSLTCLVKGFYPSDIAVAWESNGQPENNYKTTPPVLDSDGSFFLYSRLTVDKSRWQEGNVFSCSVMHEALHAHYTQKSLSLSLGK

SEQ ID NO: 141 - protein, 214 aa, synthetic construct
  REGION 1..214: note = Artificial
SYVLTQPPSVSVAPGQTARITCGGNNIGSKSVHWYQQKPGQAPVLVVYDDSDRPSGIPERFSGSNSGNTATLTISRVEAGDEADYYCQVWDSSSDHVVFGGGTKLTVLGQPKAAPSVTLFPPSSEELQANKATLVCLISDFYPGAVTVAWKADSSPVKAGVETTTPSKQSNNKYAASSYLSLTPEQWKSHRSYSCQVTHEGSTVEKTVAPTECS

SEQ ID NO: 142 - protein, 677 aa, synthetic construct
  REGION 1..677: note = Artificial
VIHVTKEVKEVATLSCGHNVSVEELAQTRIYWQKNKKMVLTMMSGDMNIWPEYKNRTIFDITNNLSIVILELRPSDEGTYECVVLKYEKDAFKREHLAEVTLSVKADFPTPSISDFEIPTSNIRRIICSTSGGFPEPHLSWLENGEELNAINTTVSQDPETELYAVSSKLDFNMTTNHSFMCLIKYGHLRVNQTFNWNTTKQEHFPDNGGGGSGGGGSGGGGSGGGGSGEVQLLESGGGLVQPGGSLRLSCAASGFTFSSYAMSWVRQAPGKGLEWVSGISGSGGFTYYADSVKGRFTISRDNSKNTLYLQMNSLRAEDTAVYYCAKPPRGYNYGPFDYWGQGTLVTVSSASTKGPSVFPLAPCSRSTSESTAALGCLVKDYFPEPVTVSWNSGALTSGVHTFPAVLQSSGLYSLSSVVTVPSSSLGTKTYTCNVDHKPSNTKVDKRVESKYGPPCPPCPAPEFLGGPSVFLFPPKPKDTLMISRTPEVTCVVVDVSQEDPEVQFNWYVDGVEVHNAKTKPREEQFNSTYRVVSVLAVLHQDWLNGKEYKCKVSNKGLPSSIEKTISKAKGQPREPQVYTLPPSQEEMTKNQVSLTCLVKGFYPSDIAVAWESNGQPENNYKTTPPVLDSDGSFFLYSRLTVDKSRWQEGNVFSCSVMHEALHAHYTQKSLSLSLGK

SEQ ID NO: 143 - protein, 677 aa, synthetic construct
  REGION 1..677: note = Artificial
VIHVTKEVKEVATLSCGHNVSVEELAQTRIYWQKNKKMVLTMMSGDMNIWPEYKNRTIFDITNNLSIVILNLRPSDEGTYECVVLKYEKDAFKREHLAEVTLSVKADFPTPSISDFEIPTSNIRRIICSTSGGFPEPHLSWLENGEELNAINTTVSQDPETELYAVSSKLDFNMTTNHSFMCLIKYGHLRVNQTFNWNTTKQEHFPDNGGGGSGGGGSGGGGSGGGGSGEVQLLESGGGLVQPGGSLRLSCAASGFTFSSYAMSWVRQAPGKGLEWVSGISGSGGFTYYADSVKGRFTISRDNSKNTLYLQMNSLRAEDTAVYYCAKPPRGYNYGPFDYWGQGTLVTVSSASTKGPSVFPLAPCSRSTSESTAALGCLVKDYFPEPVTVSWNSGALTSGVHTFPAVLQSSGLYSLSSVVTVPSSSLGTKTYTCNVDHKPSNTKVDKRVESKYGPPCPPCPAPEFLGGPSVFLFPPKPKDTLMISRTPEVTCVVVDVSQEDPEVQFNWYVDGVEVHNAKTKPREEQFNSTYRVVSVLAVLHQDWLNGKEYKCKVSNKGLPSSIEKTISKAKGQPREPQVYTLPPSQEEMTKNQVSLTCLVKGFYPSDIAVAWESNGQPENNYKTTPPVLDSDGSFFLYSRLTVDKSRWQEGNVFSCSVMHEALHAHYTQKSLSLSLGK

SEQ ID NO: 144 - protein, 677 aa, synthetic construct
  REGION 1..677: note = Artificial
VIHVTKEVKEVATLSCGHNVSVEELAQTRIYWQKNKKMVLTMMSGDMNIWPEYKNRTIFDITNNLSIVILQLRPSDEGTYECVVLKYEKDAFKREHLAEVTLSVKADFPTPSISDFEIPTSNIRRIICSTSGGFPEPHLSWLENGEELNAINTTVSQDPETELYAVSSKLDFNMTTNHSFMCLIKYGHLRVNQTFNWNTTKQEHFPDNGGGGSGGGGSGGGGSGGGGSGEVQLLESGGGLVQPGGSLRLSCAASGFTFSSYAMSWVRQAPGKGLEWVSGISGSGGFTYYADSVKGRFTISRDNSKNTLYLQMNSLRAEDTAVYYCAKPPRGYNYGPFDYWGQGTLVTVSSASTKGPSVFPLAPCSRSTSESTAALGCLVKDYFPEPVTVSWNSGALTSGVHTFPAVLQSSGLYSLSSVVTVPSSSLGTKTYTCNVDHKPSNTKVDKRVESKYGPPCPPCPAPEFLGGPSVFLFPPKPKDTLMISRTPEVTCVVVDVSQEDPEVQFNWYVDGVEVHNAKTKPREEQFNSTYRVVSVLAVLHQDWLNGKEYKCKVSNKGLPSSIEKTISKAKGQPREPQVYTLPPSQEEMTKNQVSLTCLVKGFYPSDIAVAWESNGQPENNYKTTPPVLDSDGSFFLYSRLTVDKSRWQEGNVFSCSVMHEALHAHYTQKSLSLSLGK

SEQ ID NO: 145 - protein, 677 aa, synthetic construct
  REGION 1..677: note = Artificial
VIHVTKEVKEVATLSCGHNVSVEELAQTRIYWQKNKKMVLTMMSGDMNIWPEYKNRTIFDITNNLSIVILTLRPSDEGTYECVVLKYEKDAFKREHLAEVTLSVKADFPTPSISDFEIPTSNIRRIICSTSGGFPEPHLSWLENGEELNAINTTVSQDPETELYAVSSKLDFNMTTNHSFMCLIKYGHLRVNQTFNWNTTKQEHFPDNGGGGSGGGGSGGGGSGGGGSGEVQLLESGGGLVQPGGSLRLSCAASGFTFSSYAMSWVRQAPGKGLEWVSGISGSGGFTYYADSVKGRFTISRDNSKNTLYLQMNSLRAEDTAVYYCAKPPRGYNYGPFDYWGQGTLVTVSSASTKGPSVFPLAPCSRSTSESTAALGCLVKDYFPEPVTVSWNSGALTSGVHTFPAVLQSSGLYSLSSVVTVPSSSLGTKTYTCNVDHKPSNTKVDKRVESKYGPPCPPCPAPEFLGGPSVFLFPPKPKDTLMISRTPEVTCVVVDVSQEDPEVQFNWYVDGVEVHNAKTKPREEQFNSTYRVVSVLAVLHQDWLNGKEYKCKVSNKGLPSSIEKTISKAKGQPREPQVYTLPPSQEEMTKNQVSLTCLVKGFYPSDIAVAWESNGQPENNYKTTPPVLDSDGSFFLYSRLTVDKSRWQEGNVFSCSVMHEALHAHYTQKSLSLSLGK

SEQ ID NO: 146 - protein, 677 aa, synthetic construct
  REGION 1..677: note = Artificial
VIHVTKEVKEVATLSCGHNVSVEELAQTRIYWQKSKKMVLTMMSGDMNIWPEYKNRTIFDITNNLSIVILELRPSDEGTYECVVLKYEKDAFKREHLAEVTLSVKADFPTPSISDFEIPTSNIRRIICSTSGGFPEPHLSWLENGEELNAINTTVSQDPETELYAVSSKLDFNMTTNHSFMCLIKYGHLRVNQTFNWNTTKQEHFPDNGGGGSGGGGSGGGGSGGGGSGEVQLLESGGGLVQPGGSLRLSCAASGFTFSSYAMSWVRQAPGKGLEWVSGISGSGGFTYYADSVKGRFTISRDNSKNTLYLQMNSLRAEDTAVYYCAKPPRGYNYGPFDYWGQGTLVTVSSASTKGPSVFPLAPCSRSTSESTAALGCLVKDYFPEPVTVSWNSGALTSGVHTFPAVLQSSGLYSLSSVVTVPSSSLGTKTYTCNVDHKPSNTKVDKRVESKYGPPCPPCPAPEFLGGPSVFLFPPKPKDTLMISRTPEVTCVVVDVSQEDPEVQFNWYVDGVEVHNAKTKPREEQFNSTYRVVSVLAVLHQDWLNGKEYKCKVSNKGLPSSIEKTISKAKGQPREPQVYTLPPSQEEMTKNQVSLTCLVKGFYPSDIAVAWESNGQPENNYKTTPPVLDSDGSFFLYSRLTVDKSRWQEGNVFSCSVMHEALHAHYTQKSLSLSLGK

SEQ ID NO: 147 - protein, 677 aa, synthetic construct
  REGION 1..677: note = Artificial
VIHVTKEVKEVATLSCGHNVSVEELAQTRIYWQKSKKMVLTMMSGDMNIWPEYKNRTIFDITNNLSIVILNLRPSDEGTYECVVLKYEKDAFKREHLAEVTLSVKADFPTPSISDFEIPTSNIRRIICSTSGGFPEPHLSWLENGEELNAINTTVSQDPETELYAVSSKLDFNMTTNHSFMCLIKYGHLRVNQTFNWNTTKQEHFPDNGGGGSGGGGSGGGGSGGGGSGEVQLLESGGGLVQPGGSLRLSCAASGFTFSSYAMSWVRQAPGKGLEWVSGISGSGGFTYYADSVKGRFTISRDNSKNTLYLQMNSLRAEDTAVYYCAKPPRGYNYGPFDYWGQGTLVTVSSASTKGPSVFPLAPCSRSTSESTAALGCLVKDYFPEPVTVSWNSGALTSGVHTFPAVLQSSGLYSLSSVVTVPSSSLGTKTYTCNVDHKPSNTKVDKRVESKYGPPCPPCPAPEFLGGPSVFLFPPKPKDTLMISRTPEVTCVVVDVSQEDPEVQFNWYVDGVEVHNAKTKPREEQFNSTYRVVSVLAVLHQDWLNGKEYKCKVSNKGLPSSIEKTISKAKGQPREPQVYTLPPSQEEMTKNQVSLTCLVKGFYPSDIAVAWESNGQPENNYKTTPPVLDSDGSFFLYSRLTVDKSRWQEGNVFSCSVMHEALHAHYTQKSLSLSLGK

SEQ ID NO: 148 - protein, 677 aa, synthetic construct
  REGION 1..677: note = Artificial
VIHVTKEVKEVATLSCGHNVSVEELAQTRIYWQKSKKMVLTMMSGDMNIWPEYKNRTIFDITNNLSIVILQLRPSDEGTYECVVLKYEKDAFKREHLAEVTLSVKADFPTPSISDFEIPTSNIRRIICSTSGGFPEPHLSWLENGEELNAINTTVSQDPETELYAVSSKLDFNMTTNHSFMCLIKYGHLRVNQTFNWNTTKQEHFPDNGGGGSGGGGSGGGGSGGGGSGEVQLLESGGGLVQPGGSLRLSCAASGFTFSSYAMSWVRQAPGKGLEWVSGISGSGGFTYYADSVKGRFTISRDNSKNTLYLQMNSLRAEDTAVYYCAKPPRGYNYGPFDYWGQGTLVTVSSASTKGPSVFPLAPCSRSTSESTAALGCLVKDYFPEPVTVSWNSGALTSGVHTFPAVLQSSGLYSLSSVVTVPSSSLGTKTYTCNVDHKPSNTKVDKRVESKYGPPCPPCPAPEFLGGPSVFLFPPKPKDTLMISRTPEVTCVVVDVSQEDPEVQFNWYVDGVEVHNAKTKPREEQFNSTYRVVSVLAVLHQDWLNGKEYKCKVSNKGLPSSIEKTISKAKGQPREPQVYTLPPSQEEMTKNQVSLTCLVKGFYPSDIAVAWESNGQPENNYKTTPPVLDSDGSFFLYSRLTVDKSRWQEGNVFSCSVMHEALHAHYTQKSLSLSLGK

SEQ ID NO: 149 - protein, 677 aa, synthetic construct
  REGION 1..677: note = Artificial
VIHVTKEVKEVATLSCGHNVSVEELAQTRIYWQKSKKMVLTMMSGDMNIWPEYKNRTIFDITNNLSIVILTLRPSDEGTYECVVLKYEKDAFKREHLAEVTLSVKADFPTPSISDFEIPTSNIRRIICSTSGGFPEPHLSWLENGEELNAINTTVSQDPETELYAVSSKLDFNMTTNHSFMCLIKYGHLRVNQTFNWNTTKQEHFPDNGGGGSGGGGSGGGGSGGGGSGEVQLLESGGGLVQPGGSLRLSCAASGFTFSSYAMSWVRQAPGKGLEWVSGISGSGGFTYYADSVKGRFTISRDNSKNTLYLQMNSLRAEDTAVYYCAKPPRGYNYGPFDYWGQGTLVTVSSASTKGPSVFPLAPCSRSTSESTAALGCLVKDYFPEPVTVSWNSGALTSGVHTFPAVLQSSGLYSLSSVVTVPSSSLGTKTYTCNVDHKPSNTKVDKRVESKYGPPCPPCPAPEFLGGPSVFLFPPKPKDTLMISRTPEVTCVVVDVSQEDPEVQFNWYVDGVEVHNAKTKPREEQFNSTYRVVSVLAVLHQDWLNGKEYKCKVSNKGLPSSIEKTISKAKGQPREPQVYTLPPSQEEMTKNQVSLTCLVKGFYPSDIAVAWESNGQPENNYKTTPPVLDSDGSFFLYSRLTVDKSRWQEGNVFSCSVMHEALHAHYTQKSLSLSLGK

SEQ ID NO: 150 - protein, 677 aa, synthetic construct
  REGION 1..677: note = Artificial
VIHVTKEVKEVATLSCGHNVSVEELAQTRIYWQKQKKMVLTMMSGDMNIWPEYKNRTIFDITNNLSIVILELRPSDEGTYECVVLKYEKDAFKREHLAEVTLSVKADFPTPSISDFEIPTSNIRRIICSTSGGFPEPHLSWLENGEELNAINTTVSQDPETELYAVSSKLDFNMTTNHSFMCLIKYGHLRVNQTFNWNTTKQEHFPDNGGGGSGGGGSGGGGSGGGGSGEVQLLESGGGLVQPGGSLRLSCAASGFTFSSYAMSWVRQAPGKGLEWVSGISGSGGFTYYADSVKGRFTISRDNSKNTLYLQMNSLRAEDTAVYYCAKPPRGYNYGPFDYWGQGTLVTVSSASTKGPSVFPLAPCSRSTSESTAALGCLVKDYFPEPVTVSWNSGALTSGVHTFPAVLQSSGLYSLSSVVTVPSSSLGTKTYTCNVDHKPSNTKVDKRVESKYGPPCPPCPAPEFLGGPSVFLFPPKPKDTLMISRTPEVTCVVVDVSQEDPEVQFNWYVDGVEVHNAKTKPREEQFNSTYRVVSVLAVLHQDWLNGKEYKCKVSNKGLPSSIEKTISKAKGQPREPQVYTLPPSQEEMTKNQVSLTCLVKGFYPSDIAVAWESNGQPENNYKTTPPVLDSDGSFFLYSRLTVDKSRWQEGNVFSCSVMHEALHAHYTQKSLSLSLGK

SEQ ID NO: 151 - protein, 677 aa, synthetic construct
  REGION 1..677: note = Artificial
VIHVTKEVKEVATLSCGHNVSVEELAQTRIYWQKQKKMVLTMMSGDMNIWPEYKNRTIFDITNNLSIVILNLRPSDEGTYECVVLKYEKDAFKREHLAEVTLSVKADFPTPSISDFEIPTSNIRRIICSTSGGFPEPHLSWLENGEELNAINTTVSQDPETELYAVSSKLDFNMTTNHSFMCLIKYGHLRVNQTFNWNTTKQEHFPDNGGGGSGGGGSGGGGSGGGGSGEVQLLESGGGLVQPGGSLRLSCAASGFTFSSYAMSWVRQAPGKGLEWVSGISGSGGFTYYADSVKGRFTISRDNSKNTLYLQMNSLRAEDTAVYYCAKPPRGYNYGPFDYWGQGTLVTVSSASTKGPSVFPLAPCSRSTSESTAALGCLVKDYFPEPVTVSWNSGALTSGVHTFPAVLQSSGLYSLSSVVTVPSSSLGTKTYTCNVDHKPSNTKVDKRVESKYGPPCPPCPAPEFLGGPSVFLFPPKPKDTLMISRTPEVTCVVVDVSQEDPEVQFNWYVDGVEVHNAKTKPREEQFNSTYRVVSVLAVLHQDWLNGKEYKCKVSNKGLPSSIEKTISKAKGQPREPQVYTLPPSQEEMTKNQVSLTCLVKGFYPSDIAVAWESNGQPENNYKTTPPVLDSDGSFFLYSRLTVDKSRWQEGNVFSCSVMHEALHAHYTQKSLSLSLGK

SEQ ID NO: 152 - protein, 677 aa, synthetic construct
  REGION 1..677: note = Artificial
VIHVTKEVKEVATLSCGHNVSVEELAQTRIYWQKQKKMVLTMMSGDMNIWPEYKNRTIFDITNNLSIVILQLRPSDEGTYECVVLKYEKDAFKREHLAEVTLSVKADFPTPSISDFEIPTSNIRRIICSTSGGFPEPHLSWLENGEELNAINTTVSQDPETELYAVSSKLDFNMTTNHSFMCLIKYGHLRVNQTFNWNTTKQEHFPDNGGGGSGGGGSGGGGSGGGGSGEVQLLESGGGLVQPGGSLRLSCAASGFTFSSYAMSWVRQAPGKGLEWVSGISGSGGFTYYADSVKGRFTISRDNSKNTLYLQMNSLRAEDTAVYYCAKPPRGYNYGPFDYWGQGTLVTVSSASTKGPSVFPLAPCSRSTSESTAALGCLVKDYFPEPVTVSWNSGALTSGVHTFPAVLQSSGLYSLSSVVTVPSSSLGTKTYTCNVDHKPSNTKVDKRVESKYGPPCPPCPAPEFLGGPSVFLFPPKPKDTLMISRTPEVTCVVVDVSQEDPEVQFNWYVDGVEVHNAKTKPREEQFNSTYRVVSVLAVLHQDWLNGKEYKCKVSNKGLPSSIEKTISKAKGQPREPQVYTLPPSQEEMTKNQVSLTCLVKGFYPSDIAVAWESNGQPENNYKTTPPVLDSDGSFFLYSRLTVDKSRWQEGNVFSCSVMHEALHAHYTQKSLSLSLGK

SEQ ID NO: 153 - protein, 677 aa, synthetic construct
  REGION 1..677: note = Artificial
VIHVTKEVKEVATLSCGHNVSVEELAQTRIYWQKQKKMVLTMMSGDMNIWPEYKNRTIFDITNNLSIVILTLRPSDEGTYECVVLKYEKDAFKREHLAEVTLSVKADFPTPSISDFEIPTSNIRRIICSTSGGFPEPHLSWLENGEELNAINTTVSQDPETELYAVSSKLDFNMTTNHSFMCLIKYGHLRVNQTFNWNTTKQEHFPDNGGGGSGGGGSGGGGSGGGGSGEVQLLESGGGLVQPGGSLRLSCAASGFTFSSYAMSWVRQAPGKGLEWVSGISGSGGFTYYADSVKGRFTISRDNSKNTLYLQMNSLRAEDTAVYYCAKPPRGYNYGPFDYWGQGTLVTVSSASTKGPSVFPLAPCSRSTSESTAALGCLVKDYFPEPVTVSWNSGALTSGVHTFPAVLQSSGLYSLSSVVTVPSSSLGTKTYTCNVDHKPSNTKVDKRVESKYGPPCPPCPAPEFLGGPSVFLFPPKPKDTLMISRTPEVTCVVVDVSQEDPEVQFNWYVDGVEVHNAKTKPREEQFNSTYRVVSVLAVLHQDWLNGKEYKCKVSNKGLPSSIEKTISKAKGQPREPQVYTLPPSQEEMTKNQVSLTCLVKGFYPSDIAVAWESNGQPENNYKTTPPVLDSDGSFFLYSRLTVDKSRWQEGNVFSCSVMHEALHAHYTQKSLSLSLGK

SEQ ID NO: 154 - protein, 677 aa, synthetic construct
  REGION 1..677: note = Artificial
VIHVTKEVKEVATLSCGHNVSVEELAQTRIYWQKTKKMVLTMMSGDMNIWPEYKNRTIFDITNNLSIVILELRPSDEGTYECVVLKYEKDAFKREHLAEVTLSVKADFPTPSISDFEIPTSNIRRIICSTSGGFPEPHLSWLENGEELNAINTTVSQDPETELYAVSSKLDFNMTTNHSFMCLIKYGHLRVNQTFNWNTTKQEHFPDNGGGGSGGGGSGGGGSGGGGSGEVQLLESGGGLVQPGGSLRLSCAASGFTFSSYAMSWVRQAPGKGLEWVSGISGSGGFTYYADSVKGRFTISRDNSKNTLYLQMNSLRAEDTAVYYCAKPPRGYNYGPFDYWGQGTLVTVSSASTKGPSVFPLAPCSRSTSESTAALGCLVKDYFPEPVTVSWNSGALTSGVHTFPAVLQSSGLYSLSSVVTVPSSSLGTKTYTCNVDHKPSNTKVDKRVESKYGPPCPPCPAPEFLGGPSVFLFPPKPKDTLMISRTPEVTCVVVDVSQEDPEVQFNWYVDGVEVHNAKTKPREEQFNSTYRVVSVLAVLHQDWLNGKEYKCKVSNKGLPSSIEKTISKAKGQPREPQVYTLPPSQEEMTKNQVSLTCLVKGFYPSDIAVAWESNGQPENNYKTTPPVLDSDGSFFLYSRLTVDKSRWQEGNVFSCSVMHEALHAHYTQKSLSLSLGK

SEQ ID NO: 155 - protein, 677 aa, synthetic construct
  REGION 1..677: note = Artificial
VIHVTKEVKEVATLSCGHNVSVEELAQTRIYWQKTKKMVLTMMSGDMNIWPEYKNRTIFDITNNLSIVILNLRPSDEGTYECVVLKYEKDAFKREHLAEVTLSVKADFPTPSISDFEIPTSNIRRIICSTSGGFPEPHLSWLENGEELNAINTTVSQDPETELYAVSSKLDFNMTTNHSFMCLIKYGHLRVNQTFNWNTTKQEHFPDNGGGGSGGGGSGGGGSGGGGSGEVQLLESGGGLVQPGGSLRLSCAASGFTFSSYAMSWVRQAPGKGLEWVSGISGSGGFTYYADSVKGRFTISRDNSKNTLYLQMNSLRAEDTAVYYCAKPPRGYNYGPFDYWGQGTLVTVSSASTKGPSVFPLAPCSRSTSESTAALGCLVKDYFPEPVTVSWNSGALTSGVHTFPAVLQSSGLYSLSSVVTVPSSSLGTKTYTCNVDHKPSNTKVDKRVESKYGPPCPPCPAPEFLGGPSVFLFPPKPKDTLMISRTPEVTCVVVDVSQEDPEVQFNWYVDGVEVHNAKTKPREEQFNSTYRVVSVLAVLHQDWLNGKEYKCKVSNKGLPSSIEKTISKAKGQPREPQVYTLPPSQEEMTKNQVSLTCLVKGFYPSDIAVAWESNGQPENNYKTTPPVLDSDGSFFLYSRLTVDKSRWQEGNVFSCSVMHEALHAHYTQKSLSLSLGK

SEQ ID NO: 156 - protein, 677 aa, synthetic construct
  REGION 1..677: note = Artificial
VIHVTKEVKEVATLSCGHNVSVEELAQTRIYWQKTKKMVLTMMSGDMNIWPEYKNRTIFDITNNLSIVILQLRPSDEGTYECVVLKYEKDAFKREHLAEVTLSVKADFPTPSISDFEIPTSNIRRIICSTSGGFPEPHLSWLENGEELNAINTTVSQDPETELYAVSSKLDFNMTTNHSFMCLIKYGHLRVNQTFNWNTTKQEHFPDNGGGGSGGGGSGGGGSGGGGSGEVQLLESGGGLVQPGGSLRLSCAASGFTFSSYAMSWVRQAPGKGLEWVSGISGSGGFTYYADSVKGRFTISRDNSKNTLYLQMNSLRAEDTAVYYCAKPPRGYNYGPFDYWGQGTLVTVSSASTKGPSVFPLAPCSRSTSESTAALGCLVKDYFPEPVTVSWNSGALTSGVHTFPAVLQSSGLYSLSSVVTVPSSSLGTKTYTCNVDHKPSNTKVDKRVESKYGPPCPPCPAPEFLGGPSVFLFPPKPKDTLMISRTPEVTCVVVDVSQEDPEVQFNWYVDGVEVHNAKTKPREEQFNSTYRVVSVLAVLHQDWLNGKEYKCKVSNKGLPSSIEKTISKAKGQPREPQVYTLPPSQEEMTKNQVSLTCLVKGFYPSDIAVAWESNGQPENNYKTTPPVLDSDGSFFLYSRLTVDKSRWQEGNVFSCSVMHEALHAHYTQKSLSLSLGK

SEQ ID NO: 157 - protein, 677 aa, synthetic construct
  REGION 1..677: note = Artificial
VIHVTKEVKEVATLSCGHNVSVEELAQTRIYWQKTKKMVLTMMSGDMNIWPEYKNRTIFDITNNLSIVILTLRPSDEGTYECVVLKYEKDAFKREHLAEVTLSVKADFPTPSISDFEIPTSNIRRIICSTSGGFPEPHLSWLENGEELNAINTTVSQDPETELYAVSSKLDFNMTTNHSFMCLIKYGHLRVNQTFNWNTTKQEHFPDNGGGGSGGGGSGGGGSGGGGSGEVQLLESGGGLVQPGGSLRLSCAASGFTFSSYAMSWVRQAPGKGLEWVSGISGSGGFTYYADSVKGRFTISRDNSKNTLYLQMNSLRAEDTAVYYCAKPPRGYNYGPFDYWGQGTLVTVSSASTKGPSVFPLAPCSRSTSESTAALGCLVKDYFPEPVTVSWNSGALTSGVHTFPAVLQSSGLYSLSSVVTVPSSSLGTKTYTCNVDHKPSNTKVDKRVESKYGPPCPPCPAPEFLGGPSVFLFPPKPKDTLMISRTPEVTCVVVDVSQEDPEVQFNWYVDGVEVHNAKTKPREEQFNSTYRVVSVLAVLHQDWLNGKEYKCKVSNKGLPSSIEKTISKAKGQPREPQVYTLPPSQEEMTKNQVSLTCLVKGFYPSDIAVAWESNGQPENNYKTTPPVLDSDGSFFLYSRLTVDKSRWQEGNVFSCSVMHEALHAHYTQKSLSLSLGK

SEQ ID NO: 158 - protein, 208 aa, synthetic construct; identical to SEQ ID NO: 2
  REGION 1..208: note = Artificial

SEQ ID NO: 159 - protein, 208 aa, synthetic construct; identical to SEQ ID NO: 3
  REGION 1..208: note = Artificial

SEQ ID NO: 160 - protein, 437 aa, synthetic construct
  REGION 1..437: note = Artificial
VIHVTKEVKEVATLSCGHNVSVEELAQTRIYWQKNKKMVLTMMSGDMNIWPEYKNRTIFDITNNLSIVILQLRPSDEGTYECVVLKYEKDAFKREHLAEVTLSVKADFPTPSISDFEIPTSNIRRIICSTSGGFPEPHLSWLENGEELNAINTTVSQDPETELYAVSSKLDFNMTTNHSFMCLIKYGHLRVNQTFNWNTTKQEHFPDNESKYGPPCPSCPAPEFLGGPSVFLFPPKPKDTLMISRTPEVTCVVVDVSQEDPEVQFNWYVDGVEVHNAKTKPREEQFNSTYRVVSVLTVLHQDWLNGKEYKCKVSNKGLPSSIEKTISKAKGQPREPQVYTLPPSQEEMTKNQVSLTCLVKGFYPSDIAVEWESNGQPENNYKTTPPVLDSDGSFFLYSRLTVDKSRWQEGNVFSCSVMHEALHNHYTQKSLSLSLGK

SEQ ID NO: 161 - protein, 437 aa, synthetic construct
  REGION 1..437: note = Artificial
VIHVTKEVKEVATLSCGHNVSVEELAQTRIYWQKNKKMVLTMMSGDMNIWPEYKNRTIFDITNNLSIVILTLRPSDEGTYECVVLKYEKDAFKREHLAEVTLSVKADFPTPSISDFEIPTSNIRRIICSTSGGFPEPHLSWLENGEELNAINTTVSQDPETELYAVSSKLDFNMTTNHSFMCLIKYGHLRVNQTFNWNTTKQEHFPDNESKYGPPCPSCPAPEFLGGPSVFLFPPKPKDTLMISRTPEVTCVVVDVSQEDPEVQFNWYVDGVEVHNAKTKPREEQFNSTYRVVSVLTVLHQDWLNGKEYKCKVSNKGLPSSIEKTISKAKGQPREPQVYTLPPSQEEMTKNQVSLTCLVKGFYPSDIAVEWESNGQPENNYKTTPPVLDSDGSFFLYSRLTVDKSRWQEGNVFSCSVMHEALHNHYTQKSLSLSLGK

SEQ ID NO: 162 - protein, 437 aa, synthetic construct
  REGION 1..437: note = Artificial
VIHVTKEVKEVATLSCGHNVSVEELAQTRIYWQKSKKMVLTMMSGDMNIWPEYKNRTIFDITNNLSIVILELRPSDEGTYECVVLKYEKDAFKREHLAEVTLSVKADFPTPSISDFEIPTSNIRRIICSTSGGFPEPHLSWLENGEELNAINTTVSQDPETELYAVSSKLDFNMTTNHSFMCLIKYGHLRVNQTFNWNTTKQEHFPDNESKYGPPCPSCPAPEFLGGPSVFLFPPKPKDTLMISRTPEVTCVVVDVSQEDPEVQFNWYVDGVEVHNAKTKPREEQFNSTYRVVSVLTVLHQDWLNGKEYKCKVSNKGLPSSIEKTISKAKGQPREPQVYTLPPSQEEMTKNQVSLTCLVKGFYPSDIAVEWESNGQPENNYKTTPPVLDSDGSFFLYSRLTVDKSRWQEGNVFSCSVMHEALHNHYTQKSLSLSLGK

SEQ ID NO: 163 - protein, 437 aa, synthetic construct
  REGION 1..437: note = Artificial
VIHVTKEVKEVATLSCGHNVSVEELAQTRIYWQKSKKMVLTMMSGDMNIWPEYKNRTIFDITNNLSIVILNLRPSDEGTYECVVLKYEKDAFKREHLAEVTLSVKADFPTPSISDFEIPTSNIRRIICSTSGGFPEPHLSWLENGEELNAINTTVSQDPETELYAVSSKLDFNMTTNHSFMCLIKYGHLRVNQTFNWNTTKQEHFPDNESKYGPPCPSCPAPEFLGGPSVFLFPPKPKDTLMISRTPEVTCVVVDVSQEDPEVQFNWYVDGVEVHNAKTKPREEQFNSTYRVVSVLTVLHQDWLNGKEYKCKVSNKGLPSSIEKTISKAKGQPREPQVYTLPPSQEEMTKNQVSLTCLVKGFYPSDIAVEWESNGQPENNYKTTPPVLDSDGSFFLYSRLTVDKSRWQEGNVFSCSVMHEALHNHYTQKSLSLSLGK

SEQ ID NO: 164 - protein, 437 aa, synthetic construct
  REGION 1..437: note = Artificial
VIHVTKEVKEVATLSCGHNVSVEELAQTRIYWQKSKKMVLTMMSGDMNIWPEYKNRTIFDITNNLSIVILQLRPSDEGTYECVVLKYEKDAFKREHLAEVTLSVKADFPTPSISDFEIPTSNIRRIICSTSGGFPEPHLSWLENGEELNAINTTVSQDPETELYAVSSKLDFNMTTNHSFMCLIKYGHLRVNQTFNWNTTKQEHFPDNESKYGPPCPSCPAPEFLGGPSVFLFPPKPKDTLMISRTPEVTCVVVDVSQEDPEVQFNWYVDGVEVHNAKTKPREEQFNSTYRVVSVLTVLHQDWLNGKEYKCKVSNKGLPSSIEKTISKAKGQPREPQVYTLPPSQEEMTKNQVSLTCLVKGFYPSDIAVEWESNGQPENNYKTTPPVLDSDGSFFLYSRLTVDKSRWQEGNVFSCSVMHEALHNHYTQKSLSLSLGK

SEQ ID NO: 165 - protein, 437 aa, synthetic construct
  REGION 1..437: note = Artificial
VIHVTKEVKEVATLSCGHNVSVEELAQTRIYWQKSKKMVLTMMSGDMNIWPEYKNRTIFDITNNLSIVILTLRPSDEGTYECVVLKYEKDAFKREHLAEVTLSVKADFPTPSISDFEIPTSNIRRIICSTSGGFPEPHLSWLENGEELNAINTTVSQDPETELYAVSSKLDFNMTTNHSFMCLIKYGHLRVNQTFNWNTTKQEHFPDNESKYGPPCPSCPAPEFLGGPSVFLFPPKPKDTLMISRTPEVTCVVVDVSQEDPEVQFNWYVDGVEVHNAKTKPREEQFNSTYRVVSVLTVLHQDWLNGKEYKCKVSNKGLPSSIEKTISKAKGQPREPQVYTLPPSQEEMTKNQVSLTCLVKGFYPSDIAVEWESNGQPENNYKTTPPVLDSDGSFFLYSRLTVDKSRWQEGNVFSCSVMHEALHNHYTQKSLSLSLGK

SEQ ID NO: 166 - protein, 437 aa, synthetic construct
  REGION 1..437: note = Artificial
VIHVTKEVKEVATLSCGHNVSVEELAQTRIYWQKQKKMVLTMMSGDMNIWPEYKNRTIFDITNNLSIVILELRPSDEGTYECVVLKYEKDAFKREHLAEVTLSVKADFPTPSISDFEIPTSNIRRIICSTSGGFPEPHLSWLENGEELNAINTTVSQDPETELYAVSSKLDFNMTTNHSFMCLIKYGHLRVNQTFNWNTTKQEHFPDNESKYGPPCPSCPAPEFLGGPSVFLFPPKPKDTLMISRTPEVTCVVVDVSQEDPEVQFNWYVDGVEVHNAKTKPREEQFNSTYRVVSVLTVLHQDWLNGKEYKCKVSNKGLPSSIEKTISKAKGQPREPQVYTLPPSQEEMTKNQVSLTCLVKGFYPSDIAVEWESNGQPENNYKTTPPVLDSDGSFFLYSRLTVDKSRWQEGNVFSCSVMHEALHNHYTQKSLSLSLGK

SEQ ID NO: 167 - protein, 437 aa, synthetic construct
  REGION 1..437: note = Artificial
VIHVTKEVKEVATLSCGHNVSVEELAQTRIYWQKQKKMVLTMMSGDMNIWPEYKNRTIFDITNNLSIVILNLRPSDEGTYECVVLKYEKDAFKREHLAEVTLSVKADFPTPSISDFEIPTSNIRRIICSTSGGFPEPHLSWLENGEELNAINTTVSQDPETELYAVSSKLDFNMTTNHSFMCLIKYGHLRVNQTFNWNTTKQEHFPDNESKYGPPCPSCPAPEFLGGPSVFLFPPKPKDTLMISRTPEVTCVVVDVSQEDPEVQFNWYVDGVEVHNAKTKPREEQFNSTYRVVSVLTVLHQDWLNGKEYKCKVSNKGLPSSIEKTISKAKGQPREPQVYTLPPSQEEMTKNQVSLTCLVKGFYPSDIAVEWESNGQPENNYKTTPPVLDSDGSFFLYSRLTVDKSRWQEGNVFSCSVMHEALHNHYTQKSLSLSLGK

SEQ ID NO: 168 - protein, 437 aa, synthetic construct
  REGION 1..437: note = Artificial
VIHVTKEVKEVATLSCGHNVSVEELAQTRIYWQKQKKMVLTMMSGDMNIWPEYKNRTIFDITNNLSIVILQLRPSDEGTYECVVLKYEKDAFKREHLAEVTLSVKADFPTPSISDFEIPTSNIRRIICSTSGGFPEPHLSWLENGEELNAINTTVSQDPETELYAVSSKLDFNMTTNHSFMCLIKYGHLRVNQTFNWNTTKQEHFPDNESKYGPPCPSCPAPEFLGGPSVFLFPPKPKDTLMISRTPEVTCVVVDVSQEDPEVQFNWYVDGVEVHNAKTKPREEQFNSTYRVVSVLTVLHQDWLNGKEYKCKVSNKGLPSSIEKTISKAKGQPREPQVYTLPPSQEEMTKNQVSLTCLVKGFYPSDIAVEWESNGQPENNYKTTPPVLDSDGSFFLYSRLTVDKSRWQEGNVFSCSVMHEALHNHYTQKSLSLSLGK

SEQ ID NO: 169 - protein, 437 aa, synthetic construct
  REGION 1..437: note = Artificial
VIHVTKEVKEVATLSCGHNVSVEELAQTRIYWQKQKKMVLTMMSGDMNIWPEYKNRTIFDITNNLSIVILTLRPSDEGTYECVVLKYEKDAFKREHLAEVTLSVKADFPTPSISDFEIPTSNIRRIICSTSGGFPEPHLSWLENGEELNAINTTVSQDPETELYAVSSKLDFNMTTNHSFMCLIKYGHLRVNQTFNWNTTKQEHFPDNESKYGPPCPSCPAPEFLGGPSVFLFPPKPKDTLMISRTPEVTCVVVDVSQEDPEVQFNWYVDGVEVHNAKTKPREEQFNSTYRVVSVLTVLHQDWLNGKEYKCKVSNKGLPSSIEKTISKAKGQPREPQVYTLPPSQEEMTKNQVSLTCLVKGFYPSDIAVEWESNGQPENNYKTTPPVLDSDGSFFLYSRLTVDKSRWQEGNVFSCSVMHEALHNHYTQKSLSLSLGK

SEQ ID NO: 170 - protein, 437 aa, synthetic construct
  REGION 1..437: note = Artificial
VIHVTKEVKEVATLSCGHNVSVEELAQTRIYWQKTKKMVLTMMSGDMNIWPEYKNRTIFDITNNLSIVILELRPSDEGTYECVVLKYEKDAFKREHLAEVTLSVKADFPTPSISDFEIPTSNIRRIICSTSGGFPEPHLSWLENGEELNAINTTVSQDPETELYAVSSKLDFNMTTNHSFMCLIKYGHLRVNQTFNWNTTKQEHFPDNESKYGPPCPSCPAPEFLGGPSVFLFPPKPKDTLMISRTPEVTCVVVDVSQEDPEVQFNWYVDGVEVHNAKTKPREEQFNSTYRVVSVLTVLHQDWLNGKEYKCKVSNKGLPSSIEKTISKAKGQPREPQVYTLPPSQEEMTKNQVSLTCLVKGFYPSDIAVEWESNGQPENNYKTTPPVLDSDGSFFLYSRLTVDKSRWQEGNVFSCSVMHEALHNHYTQKSLSLSLGK

SEQ ID NO: 171 - protein, 437 aa, synthetic construct
  REGION 1..437: note = Artificial
VIHVTKEVKEVATLSCGHNVSVEELAQTRIYWQKTKKMVLTMMSGDMNIWPEYKNRTIFDITNNLSIVILNLRPSDEGTYECVVLKYEKDAFKREHLAEVTLSVKADFPTPSISDFEIPTSNIRRIICSTSGGFPEPHLSWLENGEELNAINTTVSQDPETELYAVSSKLDFNMTTNHSFMCLIKYGHLRVNQTFNWNTTKQEHFPDNESKYGPPCPSCPAPEFLGGPSVFLFPPKPKDTLMISRTPEVTCVVVDVSQEDPEVQFNWYVDGVEVHNAKTKPREEQFNSTYRVVSVLTVLHQDWLNGKEYKCKVSNKGLPSSIEKTISKAKGQPREPQVYTLPPSQEEMTKNQVSLTCLVKGFYPSDIAVEWESNGQPENNYKTTPPVLDSDGSFFLYSRLTVDKSRWQEGNVFSCSVMHEALHNHYTQKSLSLSLGK

SEQ ID NO: 172 - protein, 437 aa, synthetic construct
  REGION 1..437: note = Artificial
VIHVTKEVKEVATLSCGHNVSVEELAQTRIYWQKTKKMVLTMMSGDMNIWPEYKNRTIFDITNNLSIVILQLRPSDEGTYECVVLKYEKDAFKREHLAEVTLSVKADFPTPSISDFEIPTSNIRRIICSTSGGFPEPHLSWLENGEELNAINTTVSQDPETELYAVSSKLDFNMTTNHSFMCLIKYGHLRVNQTFNWNTTKQEHFPDNESKYGPPCPSCPAPEFLGGPSVFLFPPKPKDTLMISRTPEVTCVVVDVSQEDPEVQFNWYVDGVEVHNAKTKPREEQFNSTYRVVSVLTVLHQDWLNGKEYKCKVSNKGLPSSIEKTISKAKGQPREPQVYTLPPSQEEMTKNQVSLTCLVKGFYPSDIAVEWESNGQPENNYKTTPPVLDSDGSFFLYSRLTVDKSRWQEGNVFSCSVMHEALHNHYTQKSLSLSLGK

SEQ ID NO: 173 - protein, 437 aa, synthetic construct
  REGION 1..437: note = Artificial
VIHVTKEVKEVATLSCGHNVSVEELAQTRIYWQKTKKMVLTMMSGDMNIWPEYKNRTIFDITNNLSIVILTLRPSDEGTYECVVLKYEKDAFKREHLAEVTLSVKADFPTPSISDFEIPTSNIRRIICSTSGGFPEPHLSWLENGEELNAINTTVSQDPETELYAVSSKLDFNMTTNHSFMCLIKYGHLRVNQTFNWNTTKQEHFPDNESKYGPPCPSCPAPEFLGGPSVFLFPPKPKDTLMISRTPEVTCVVVDVSQEDPEVQFNWYVDGVEVHNAKTKPREEQFNSTYRVVSVLTVLHQDWLNGKEYKCKVSNKGLPSSIEKTISKAKGQPREPQVYTLPPSQEEMTKNQVSLTCLVKGFYPSDIAVEWESNGQPENNYKTTPPVLDSDGSFFLYSRLTVDKSRWQEGNVFSCSVMHEALHNHYTQKSLSLSLGK

SEQ ID NO: 174 - protein, 437 aa, synthetic construct
  REGION 1..437: note = Artificial
VIHVTKEVKEVATLSCGHNVSVEELAQTRIYWQKEKKMVLTMMSGDMNIWPEYKNRTIFDITNNLSIVILALRPSDEGTYECVVLKYEKDAFKREHLAEVTLSVKADFPTPSISDFEIPTSNIRRIICSTSGGFPEPHLSWLENGEELNAINTTVSQDPETELYAVSSKLDFNMTTNHSFMCLIKYGHLRVNQTFNWNTTKQEHFPDNESKYGPPCPSCPAPEFLGGPSVFLFPPKPKDTLMISRTPEVTCVVVDVSQEDPEVQFNWYVDGVEVHNAKTKPREEQFNSTYRVVSVLTVLHQDWLNGKEYKCKVSNKGLPSSIEKTISKAKGQPREPQVYTLPPSQEEMTKNQVSLTCLVKGFYPSDIAVEWESNGQPENNYKTTPPVLDSDGSFFLYSRLTVDKSRWQEGNVFSCSVMHEALHNHYTQKSLSLSLGK

SEQ ID NO: 175 - protein, 336 aa, synthetic construct
  REGION 1..336: note = Artificial
VIHVTKEVKEVATLSCGHNVSVEELAQTRIYWQKNKKMVLTMMSGDMNIWPEYKNRTIFDITNNLSIVILELRPSDEGTYECVVLKYEKDAFKREHLAEVTLSVKADESKYGPPCPSCPAPEFLGGPSVFLFPPKPKDTLMISRTPEVTCVVVDVSQEDPEVQFNWYVDGVEVHNAKTKPREEQFNSTYRVVSVLTVLHQDWLNGKEYKCKVSNKGLPSSIEKTISKAKGQPREPQVYTLPPSQEEMTKNQVSLTCLVKGFYPSDIAVEWESNGQPENNYKTTPPVLDSDGSFFLYSRLTVDKSRWQEGNVFSCSVMHEALHNHYTQKSLSLSLGK

SEQ ID NO: 176 - protein, 336 aa, synthetic construct
  REGION 1..336: note = Artificial
VIHVTKEVKEVATLSCGHNVSVEELAQTRIYWQKNKKMVLTMMSGDMNIWPEYKNRTIFDITNNLSIVILNLRPSDEGTYECVVLKYEKDAFKREHLAEVTLSVKADESKYGPPCPSCPAPEFLGGPSVFLFPPKPKDTLMISRTPEVTCVVVDVSQEDPEVQFNWYVDGVEVHNAKTKPREEQFNSTYRVVSVLTVLHQDWLNGKEYKCKVSNKGLPSSIEKTISKAKGQPREPQVYTLPPSQEEMTKNQVSLTCLVKGFYPSDIAVEWESNGQPENNYKTTPPVLDSDGSFFLYSRLTVDKSRWQEGNVFSCSVMHEALHNHYTQKSLSLSLGK

SEQ ID NO: 177 - protein, 336 aa, synthetic construct
  REGION 1..336: note = Artificial
VIHVTKEVKEVATLSCGHNVSVEELAQTRIYWQKNKKMVLTMMSGDMNIWPEYKNRTIFDITNNLSIVILQLRPSDEGTYECVVLKYEKDAFKREHLAEVTLSVKADESKYGPPCPSCPAPEFLGGPSVFLFPPKPKDTLMISRTPEVTCVVVDVSQEDPEVQFNWYVDGVEVHNAKTKPREEQFNSTYRVVSVLTVLHQDWLNGKEYKCKVSNKGLPSSIEKTISKAKGQPREPQVYTLPPSQEEMTKNQVSLTCLVKGFYPSDIAVEWESNGQPENNYKTTPPVLDSDGSFFLYSRLTVDKSRWQEGNVFSCSVMHEALHNHYTQKSLSLSLGK

SEQ ID NO: 178 - protein, 336 aa, synthetic construct
  REGION 1..336: note = Artificial
VIHVTKEVKEVATLSCGHNVSVEELAQTRIYWQKNKKMVLTMMSGDMNIWPEYKNRTIFDITNNLSIVILTLRPSDEGTYECVVLKYEKDAFKREHLAEVTLSVKADESKYGPPCPSCPAPEFLGGPSVFLFPPKPKDTLMISRTPEVTCVVVDVSQEDPEVQFNWYVDGVEVHNAKTKPREEQFNSTYRVVSVLTVLHQDWLNGKEYKCKVSNKGLPSSIEKTISKAKGQPREPQVYTLPPSQEEMTKNQVSLTCLVKGFYPSDIAVEWESNGQPENNYKTTPPVLDSDGSFFLYSRLTVDKSRWQEGNVFSCSVMHEALHNHYTQKSLSLSLGK

SEQ ID NO: 179 - protein, 336 aa, synthetic construct
  REGION 1..336: note = Artificial
VIHVTKEVKEVATLSCGHNVSVEELAQTRIYWQKSKKMVLTMMSGDMNIWPEYKNRTIFDITNNLSIVILELRPSDEGTYECVVLKYEKDAFKREHLAEVTLSVKADESKYGPPCPSCPAPEFLGGPSVFLFPPKPKDTLMISRTPEVTCVVVDVSQEDPEVQFNWYVDGVEVHNAKTKPREEQFNSTYRVVSVLTVLHQDWLNGKEYKCKVSNKGLPSSIEKTISKAKGQPREPQVYTLPPSQEEMTKNQVSLTCLVKGFYPSDIAVEWESNGQPENNYKTTPPVLDSDGSFFLYSRLTVDKSRWQEGNVFSCSVMHEALHNHYTQKSLSLSLGK

SEQ ID NO: 180 - protein, 336 aa, synthetic construct
  REGION 1..336: note = Artificial
VIHVTKEVKEVATLSCGHNVSVEELAQTRIYWQKSKKMVLTMMSGDMNIWPEYKNRTIFDITNNLSIVILNLRPSDEGTYECVVLKYEKDAFKREHLAEVTLSVKADESKYGPPCPSCPAPEFLGGPSVFLFPPKPKDTLMISRTPEVTCVVVDVSQEDPEVQFNWYVDGVEVHNAKTKPREEQFNSTYRVVSVLTVLHQDWLNGKEYKCKVSNKGLPSSIEKTISKAKGQPREPQVYTLPPSQEEMTKNQVSLTCLVKGFYPSDIAVEWESNGQPENNYKTTPPVLDSDGSFFLYSRLTVDKSRWQEGNVFSCSVMHEALHNHYTQKSLSLSLGK

SEQ ID NO: 181 - protein, 336 aa, synthetic construct
  REGION 1..336: note = Artificial
VIHVTKEVKEVATLSCGHNVSVEELAQTRIYWQKSKKMVLTMMSGDMNIWPEYKNRTIFDITNNLSIVILQLRPSDEGTYECVVLKYEKDAFKREHLAEVTLSVKADESKYGPPCPSCPAPEFLGGPSVFLFPPKPKDTLMISRTPEVTCVVVDVSQEDPEVQFNWYVDGVEVHNAKTKPREEQFNSTYRVVSVLTVLHQDWLNGKEYKCKVSNKGLPSSIEKTISKAKGQPREPQVYTLPPSQEEMTKNQVSLTCLVKGFYPSDIAVEWESNGQPENNYKTTPPVLDSDGSFFLYSRLTVDKSRWQEGNVFSCSVMHEALHNHYTQKSLSLSLGK

SEQ ID NO: 182 - protein, 336 aa, synthetic construct
  REGION 1..336: note = Artificial
VIHVTKEVKEVATLSCGHNVSVEELAQTRIYWQKSKKMVLTMMSGDMNIWPEYKNRTIFDITNNLSIVILTLRPSDEGTYECVVLKYEKDAFKREHLAEVTLSVKADESKYGPPCPSCPAPEFLGGPSVFLFPPKPKDTLMISRTPEVTCVVVDVSQEDPEVQFNWYVDGVEVHNAKTKPREEQFNSTYRVVSVLTVLHQDWLNGKEYKCKVSNKGLPSSIEKTISKAKGQPREPQVYTLPPSQEEMTKNQVSLTCLVKGFYPSDIAVEWESNGQPENNYKTTPPVLDSDGSFFLYSRLTVDKSRWQEGNVFSCSVMHEALHNHYTQKSLSLSLGK

SEQ ID NO: 183 - protein, 336 aa, synthetic construct
  REGION 1..336: note = Artificial
VIHVTKEVKEVATLSCGHNVSVEELAQTRIYWQKQKKMVLTMMSGDMNIWPEYKNRTIFDITNNLSIVILELRPSDEGTYECVVLKYEKDAFKREHLAEVTLSVKADESKYGPPCPSCPAPEFLGGPSVFLFPPKPKDTLMISRTPEVTCVVVDVSQEDPEVQFNWYVDGVEVHNAKTKPREEQFNSTYRVVSVLTVLHQDWLNGKEYKCKVSNKGLPSSIEKTISKAKGQPREPQVYTLPPSQEEMTKNQVSLTCLVKGFYPSDIAVEWESNGQPENNYKTTPPVLDSDGSFFLYSRLTVDKSRWQEGNVFSCSVMHEALHNHYTQKSLSLSLGK

SEQ ID NO: 184 - protein, 336 aa, synthetic construct
  REGION 1..336: note = Artificial
VIHVTKEVKEVATLSCGHNVSVEELAQTRIYWQKQKKMVLTMMSGDMNIWPEYKNRTIFDITNNLSIVILNLRPSDEGTYECVVLKYEKDAFKREHLAEVTLSVKADESKYGPPCPSCPAPEFLGGPSVFLFPPKPKDTLMISRTPEVTCVVVDVSQEDPEVQFNWYVDGVEVHNAKTKPREEQFNSTYRVVSVLTVLHQDWLNGKEYKCKVSNKGLPSSIEKTISKAKGQPREPQVYTLPPSQEEMTKNQVSLTCLVKGFYPSDIAVEWESNGQPENNYKTTPPVLDSDGSFFLYSRLTVDKSRWQEGNVFSCSVMHEALHNHYTQKSLSLSLGK

SEQ ID NO: 185 - protein, 336 aa, synthetic construct
  REGION 1..336: note = Artificial
VIHVTKEVKEVATLSCGHNVSVEELAQTRIYWQKQKKMVLTMMSGDMNIWPEYKNRTIFDITNNLSIVILQLRPSDEGTYECVVLKYEKDAFKREHLAEVTLSVKADESKYGPPCPSCPAPEFLGGPSVFLFPPKPKDTLMISRTPEVTCVVVDVSQEDPEVQFNWYVDGVEVHNAKTKPREEQFNSTYRVVSVLTVLHQDWLNGKEYKCKVSNKGLPSSIEKTISKAKGQPREPQVYTLPPSQEEMTKNQVSLTCLVKGFYPSDIAVEWESNGQPENNYKTTPPVLDSDGSFFLYSRLTVDKSRWQEGNVFSCSVMHEALHNHYTQKSLSLSLGK

SEQ ID NO: 186 - protein, 336 aa, synthetic construct
  REGION 1..336: note = Artificial
VIHVTKEVKEVATLSCGHNVSVEELAQTRIYWQKQKKMVLTMMSGDMNIWPEYKNRTIFDITNNLSIVILTLRPSDEGTYECVVLKYEKDAFKREHLAEVTLSVKADESKYGPPCPSCPAPEFLGGPSVFLFPPKPKDTLMISRTPEVTCVVVDVSQEDPEVQFNWYVDGVEVHNAKTKPREEQFNSTYRVVSVLTVLHQDWLNGKEYKCKVSNKGLPSSIEKTISKAKGQPREPQVYTLPPSQEEMTKNQVSLTCLVKGFYPSDIAVEWESNGQPENNYKTTPPVLDSDGSFFLYSRLTVDKSRWQEGNVFSCSVMHEALHNHYTQKSLSLSLGK

SEQ ID NO: 187 - protein, 336 aa, synthetic construct
  REGION 1..336: note = Artificial
VIHVTKEVKEVATLSCGHNVSVEELAQTRIYWQKTKKMVLTMMSGDMNIWPEYKNRTIFDITNNLSIVILELRPSDEGTYECVVLKYEKDAFKREHLAEVTLSVKADESKYGPPCPSCPAPEFLGGPSVFLFPPKPKDTLMISRTPEVTCVVVDVSQEDPEVQFNWYVDGVEVHNAKTKPREEQFNSTYRVVSVLTVLHQDWLNGKEYKCKVSNKGLPSSIEKTISKAKGQPREPQVYTLPPSQEEMTKNQVSLTCLVKGFYPSDIAVEWESNGQPENNYKTTPPVLDSDGSFFLYSRLTVDKSRWQEGNVFSCSVMHEALHNHYTQKSLSLSLGK

SEQ ID NO: 188 - protein, 336 aa, synthetic construct
  REGION 1..336: note = Artificial
VIHVTKEVKEVATLSCGHNVSVEELAQTRIYWQKTKKMVLTMMSGDMNIWPEYKNRTIFDITNNLSIVILNLRPSDEGTYECVVLKYEKDAFKREHLAEVTLSVKADESKYGPPCPSCPAPEFLGGPSVFLFPPKPKDTLMISRTPEVTCVVVDVSQEDPEVQFNWYVDGVEVHNAKTKPREEQFNSTYRVVSVLTVLHQDWLNGKEYKCKVSNKGLPSSIEKTISKAKGQPREPQVYTLPPSQEEMTKNQVSLTCLVKGFYPSDIAVEWESNGQPENNYKTTPPVLDSDGSFFLYSRLTVDKSRWQEGNVFSCSVMHEALHNHYTQKSLSLSLGK

SEQ ID NO: 189 - protein, 336 aa, synthetic construct
  REGION 1..336: note = Artificial
VIHVTKEVKEVATLSCGHNVSVEELAQTRIYWQKTKKMVLTMMSGDMNIWPEYKNRTIFDITNNLSIVILQLRPSDEGTYECVVLKYEKDAFKREHLAEVTLSVKADESKYGPPCPSCPAPEFLGGPSVFLFPPKPKDTLMISRTPEVTCVVVDVSQEDPEVQFNWYVDGVEVHNAKTKPREEQFNSTYRVVSVLTVLHQDWLNGKEYKCKVSNKGLPSSIEKTISKAKGQPREPQVYTLPPSQEEMTKNQVSLTCLVKGFYPSDIAVEWESNGQPENNYKTTPPVLDSDGSFFLYSRLTVDKSRWQEGNVFSCSVMHEALHNHYTQKSLSLSLGK

SEQ ID NO: 190 - protein, 336 aa, synthetic construct
  REGION 1..336: note = Artificial
VIHVTKEVKEVATLSCGHNVSVEELAQTRIYWQKTKKMVLTMMSGDMNIWPEYKNRTIFDITNNLSIVILTLRPSDEGTYECVVLKYEKDAFKREHLAEVTLSVKADESKYGPPCPSCPAPEFLGGPSVFLFPPKPKDTLMISRTPEVTCVVVDVSQEDPEVQFNWYVDGVEVHNAKTKPREEQFNSTYRVVSVLTVLHQDWLNGKEYKCKVSNKGLPSSIEKTISKAKGQPREPQVYTLPPSQEEMTKNQVSLTCLVKGFYPSDIAVEWESNGQPENNYKTTPPVLDSDGSFFLYSRLTVDKSRWQEGNVFSCSVMHEALHNHYTQKSLSLSLGK

SEQ ID NO: 191 - protein, 336 aa, Homo sapiens
VIHVTKEVKEVATLSCGHNVSVEELAQTRIYWQKEKKMVLTMMSGDMNIWPEYKNRTIFDITNNLSIVILALRPSDEGTYECVVLKYEKDAFKREHLAEVTLSVKADESKYGPPCPSCPAPEFLGGPSVFLFPPKPKDTLMISRTPEVTCVVVDVSQEDPEVQFNWYVDGVEVHNAKTKPREEQFNSTYRVVSVLTVLHQDWLNGKEYKCKVSNKGLPSSIEKTISKAKGQPREPQVYTLPPSQEEMTKNQVSLTCLVKGFYPSDIAVEWESNGQPENNYKTTPPVLDSDGSFFLYSRLTVDKSRWQEGNVFSCSVMHEALHNHYTQKSLSLSLGK

SEQ ID NO: 192 - protein, 676 aa, synthetic construct
  REGION 1..676: note = Artificial
VIHVTKEVKEVATLSCGHNVSVEELAQTRIYWQKNKKMVLTMMSGDMNIWPEYKNRTIFDITNNLSIVILELRPSDEGTYECVVLKYEKDAFKREHLAEVTLSVKADFPTPSISDFEIPTSNIRRIICSTSGGFPEPHLSWLENGEELNAINTTVSQDPETELYAVSSKLDFNMTTNHSFMCLIKYGHLRVNQTFNWNTTKQEHFPDNGGGGSGGGGSGGGGSGGGGSGQVQLQQWGAGLLKPSETLSLTCAVYGGSFSDYYWNWIRQPPGKGLEWIGEINHRGSTNSNPSLKSRVTLSLDTSKNQFSLKLRSVTAADTAVYYCAFGYSDYEYNWFDPWGQGTLVTVSSASTKGPSVFPLAPCSRSTSESTAALGCLVKDYFPEPVTVSWNSGALTSGVHTFPAVLQSSGLYSLSSVVTVPSSSLGTKTYTCNVDHKPSNTKVDKRVESKYGPPCPPCPAPEFLGGPSVFLFPPKPKDTLMISRTPEVTCVVVDVSQEDPEVQFNWYVDGVEVHNAKTKPREEQFNSTYRVVSVLTVLHQDWLNGKEYKCKVSNKGLPSSIEKTISKAKGQPREPQVYTLPPSQEEMTKNQVSLTCLVKGFYPSDIAVEWESNGQPENNYKTTPPVLDSDGSFFLYSRLTVDKSRWQEGNVFSCSVMHEALHNHYTQKSLSLSLGK

SEQ ID NO: 193 - protein, 676 aa, synthetic construct
  REGION 1..676: note = Artificial
VIHVTKEVKEVATLSCGHNVSVEELAQTRIYWQKNKKMVLTMMSGDMNIWPEYKNRTIFDITNNLSIVILNLRPSDEGTYECVVLKYEKDAFKREHLAEVTLSVKADFPTPSISDFEIPTSNIRRIICSTSGGFPEPHLSWLENGEELNAINTTVSQDPETELYAVSSKLDFNMTTNHSFMCLIKYGHLRVNQTFNWNTTKQEHFPDNGGGGSGGGGSGGGGSGGGGSGQVQLQQWGAGLLKPSETLSLTCAVYGGSFSDYYWNWIRQPPGKGLEWIGEINHRGSTNSNPSLKSRVTLSLDTSKNQFSLKLRSVTAADTAVYYCAFGYSDYEYNWFDPWGQGTLVTVSSASTKGPSVFPLAPCSRSTSESTAALGCLVKDYFPEPVTVSWNSGALTSGVHTFPAVLQSSGLYSLSSVVTVPSSSLGTKTYTCNVDHKPSNTKVDKRVESKYGPPCPPCPAPEFLGGPSVFLFPPKPKDTLMISRTPEVTCVVVDVSQEDPEVQFNWYVDGVEVHNAKTKPREEQFNSTYRVVSVLTVLHQDWLNGKEYKCKVSNKGLPSSIEKTISKAKGQPREPQVYTLPPSQEEMTKNQVSLTCLVKGFYPSDIAVEWESNGQPENNYKTTPPVLDSDGSFFLYSRLTVDKSRWQEGNVFSCSVMHEALHNHYTQKSLSLSLGK

SEQ ID NO: 194 - protein, 676 aa, synthetic construct
  REGION 1..676: note = Artificial
VIHVTKEVKEVATLSCGHNVSVEELAQTRIYWQKNKKMVLTMMSGDMNIWPEYKNRTIFDITNNLSIVILQLRPSDEGTYECVVLKYEKDAFKREHLAEVTLSVKADFPTPSISDFEIPTSNIRRIICSTSGGFPEPHLSWLENGEELNAINTTVSQDPETELYAVSSKLDFNMTTNHSFMCLIKYGHLRVNQTFNWNTTKQEHFPDNGGGGSGGGGSGGGGSGGGGSGQVQLQQWGAGLLKPSETLSLTCAVYGGSFSDYYWNWIRQPPGKGLEWIGEINHRGSTNSNPSLKSRVTLSLDTSKNQFSLKLRSVTAADTAVYYCAFGYSDYEYNWFDPWGQGTLVTVSSASTKGPSVFPLAPCSRSTSESTAALGCLVKDYFPEPVTVSWNSGALTSGVHTFPAVLQSSGLYSLSSVVTVPSSSLGTKTYTCNVDHKPSNTKVDKRVESKYGPPCPPCPAPEFLGGPSVFLFPPKPKDTLMISRTPEVTCVVVDVSQEDPEVQFNWYVDGVEVHNAKTKPREEQFNSTYRVVSVLTVLHQDWLNGKEYKCKVSNKGLPSSIEKTISKAKGQPREPQVYTLPPSQEEMTKNQVSLTCLVKGFYPSDIAVEWESNGQPENNYKTTPPVLDSDGSFFLYSRLTVDKSRWQEGNVFSCSVMHEALHNHYTQKSLSLSLGK

SEQ ID NO: 195 - protein, 676 aa, synthetic construct
  REGION 1..676: note = Artificial
VIHVTKEVKEVATLSCGHNVSVEELAQTRIYWQKNKKMVLTMMSGDMNIWPEYKNRTIFDITNNLSIVILTLRPSDEGTYECVVLKYEKDAFKREHLAEVTLSVKADFPTPSISDFEIPTSNIRRIICSTSGGFPEPHLSWLENGEELNAINTTVSQDPETELYAVSSKLDFNMTTNHSFMCLIKYGHLRVNQTFNWNTTKQEHFPDNGGGGSGGGGSGGGGSGGGGSGQVQLQQWGAGLLKPSETLSLTCAVYGGSFSDYYWNWIRQPPGKGLEWIGEINHRGSTNSNPSLKSRVTLSLDTSKNQFSLKLRSVTAADTAVYYCAFGYSDYEYNWFDPWGQGTLVTVSSASTKGPSVFPLAPCSRSTSESTAALGCLVKDYFPEPVTVSWNSGALTSGVHTFPAVLQSSGLYSLSSVVTVPSSSLGTKTYTCNVDHKPSNTKVDKRVESKYGPPCPPCPAPEFLGGPSVFLFPPKPKDTLMISRTPEVTCVVVDVSQEDPEVQFNWYVDGVEVHNAKTKPREEQFNSTYRVVSVLTVLHQDWLNGKEYKCKVSNKGLPSSIEKTISKAKGQPREPQVYTLPPSQEEMTKNQVSLTCLVKGFYPSDIAVEWESNGQPENNYKTTPPVLDSDGSFFLYSRLTVDKSRWQEGNVFSCSVMHEALHNHYTQKSLSLSLGK

SEQ ID NO: 196 - protein, 676 aa, synthetic construct
  REGION 1..676: note = Artificial
VIHVTKEVKEVATLSCGHNVSVEELAQTRIYWQKEKKMVLTMMSGDMNIWPEYKNRTIFDITNNLSIVILALRPSDEGTYECVVLKYEKDAFKREHLAEVTLSVKADFPTPSISDFEIPTSNIRRIICSTSGGFPEPHLSWLENGEELNAINTTVSQDPETELYAVSSKLDFNMTTNHSFMCLIKYGHLRVNQTFNWNTTKQEHFPDNGGGGSGGGGSGGGGSGGGGSGQVQLQQWGAGLLKPSETLSLTCAVYGGSFSDYYWNWIRQPPGKGLEWIGEINHRGSTNSNPSLKSRVTLSLDTSKNQFSLKLRSVTAADTAVYYCAFGYSDYEYNWFDPWGQGTLVTVSSASTKGPSVFPLAPCSRSTSESTAALGCLVKDYFPEPVTVSWNSGALTSGVHTFPAVLQSSGLYSLSSVVTVPSSSLGTKTYTCNVDHKPSNTKVDKRVESKYGPPCPPCPAPEFLGGPSVFLFPPKPKDTLMISRTPEVTCVVVDVSQEDPEVQFNWYVDGVEVHNAKTKPREEQFNSTYRVVSVLTVLHQDWLNGKEYKCKVSNKGLPSSIEKTISKAKGQPREPQVYTLPPSQEEMTKNQVSLTCLVKGFYPSDIAVEWESNGQPENNYKTTPPVLDSDGSFFLYSRLTVDKSRWQEGNVFSCSVMHEALHNHYTQKSLSLSLGK

SEQ ID NO: 197 - protein, 214 aa, synthetic construct
  REGION 1..214: note = Artificial
EIVLTQSPATLSLSPGERATLSCRASQSISSYLAWYQQKPGQAPRLLIYDASNRATGIPARFSGSGSGTDFTLTISSLEPEDFAVYYCQQRSNWPLTFGQGINLEIKRTVAAPSVFIFPPSDEQLKSGTASVVCLLNNFYPREAKVQWKVDNALQSGNSQESVTEQDSKDSTYSLSSTLTLSKADYEKHKVYACEVTHQGLSSPVTKSFNRGEC

SEQ ID NO: 198 - protein, 575 aa, synthetic construct
  REGION 1..575: note = Artificial
VIHVTKEVKEVATLSCGHNVSVEELAQTRIYWQKNKKMVLTMMSGDMNIWPEYKNRTIFDITNNLSIVILELRPSDEGTYECVVLKYEKDAFKREHLAEVTLSVKADGGGGSGGGGSGGGGSGGGGSGQVQLQQWGAGLLKPSETLSLTCAVYGGSFSDYYWNWIRQPPGKGLEWIGEINHRGSTNSNPSLKSRVTLSLDTSKNQFSLKLRSVTAADTAVYYCAFGYSDYEYNWFDPWGQGTLVTVSSASTKGPSVFPLAPCSRSTSESTAALGCLVKDYFPEPVTVSWNSGALTSGVHTFPAVLQSSGLYSLSSVVTVPSSSLGTKTYTCNVDHKPSNTKVDKRVESKYGPPCPPCPAPEFLGGPSVFLFPPKPKDTLMISRTPEVTCVVVDVSQEDPEVQFNWYVDGVEVHNAKTKPREEQFNSTYRVVSVLTVLHQDWLNGKEYKCKVSNKGLPSSIEKTISKAKGQPREPQVYTLPPSQEEMTKNQVSLTCLVKGFYPSDIAVEWESNGQPENNYKTTPPVLDSDGSFFLYSRLTVDKSRWQEGNVFSCSVMHEALHNHYTQKSLSLSLGK

SEQ ID NO: 199 - protein, 575 aa, synthetic construct
  REGION 1..575: note = Artificial
VIHVTKEVKEVATLSCGHNVSVEELAQTRIYWQKNKKMVLTMMSGDMNIWPEYKNRTIFDITNNLSIVILNLRPSDEGTYECVVLKYEKDAFKREHLAEVTLSVKADGGGGSGGGGSGGGGSGGGGSGQVQLQQWGAGLLKPSETLSLTCAVYGGSFSDYYWNWIRQPPGKGLEWIGEINHRGSTNSNPSLKSRVTLSLDTSKNQFSLKLRSVTAADTAVYYCAFGYSDYEYNWFDPWGQGTLVTVSSASTKGPSVFPLAPCSRSTSESTAALGCLVKDYFPEPVTVSWNSGALTSGVHTFPAVLQSSGLYSLSSVVTVPSSSLGTKTYTCNVDHKPSNTKVDKRVESKYGPPCPPCPAPEFLGGPSVFLFPPKPKDTLMISRTPEVTCVVVDVSQEDPEVQFNWYVDGVEVHNAKTKPREEQFNSTYRVVSVLTVLHQDWLNGKEYKCKVSNKGLPSSIEKTISKAKGQPREPQVYTLPPSQEEMTKNQVSLTCLVKGFYPSDIAVEWESNGQPENNYKTTPPVLDSDGSFFLYSRLTVDKSRWQEGNVFSCSVMHEALHNHYTQKSLSLSLGK

SEQ ID NO: 200 - protein, 575 aa, synthetic construct
  REGION 1..575: note = Artificial
VIHVTKEVKEVATLSCGHNVSVEELAQTRIYWQKNKKMVLTMMSGDMNIWPEYKNRTIFDITNNLSIVILQLRPSDEGTYECVVLKYEKDAFKREHLAEVTLSVKADGGGGSGGGGSGGGGSGGGGSGQVQLQQWGAGLLKPSETLSLTCAVYGGSFSDYYWNWIRQPPGKGLEWIGEINHRGSTNSNPSLKSRVTLSLDTSKNQFSLKLRSVTAADTAVYYCAFGYSDYEYNWFDPWGQGTLVTVSSASTKGPSVFPLAPCSRSTSESTAALGCLVKDYFPEPVTVSWNSGALTSGVHTFPAVLQSSGLYSLSSVVTVPSSSLGTKTYTCNVDHKPSNTKVDKRVESKYGPPCPPCPAPEFLGGPSVFLFPPKPKDTLMISRTPEVTCVVVDVSQEDPEVQFNWYVDGVEVHNAKTKPREEQFNSTYRVVSVLTVLHQDWLNGKEYKCKVSNKGLPSSIEKTISKAKGQPREPQVYTLPPSQEEMTKNQVSLTCLVKGFYPSDIAVEWESNGQPENNYKTTPPVLDSDGSFFLYSRLTVDKSRWQEGNVFSCSVMHEALHNHYTQKSLSLSLGK

SEQ ID NO: 201 - protein, 575 aa, synthetic construct
  REGION 1..575: note = Artificial
VIHVTKEVKEVATLSCGHNVSVEELAQTRIYWQKNKKMVLTMMSGDMNIWPEYKNRTIFDITNNLSIVILTLRPSDEGTYECVVLKYEKDAFKREHLAEVTLSVKADGGGGSGGGGSGGGGSGGGGSGQVQLQQWGAGLLKPSETLSLTCAVYGGSFSDYYWNWIRQPPGKGLEWIGEINHRGSTNSNPSLKSRVTLSLDTSKNQFSLKLRSVTAADTAVYYCAFGYSDYEYNWFDPWGQGTLVTVSSASTKGPSVFPLAPCSRSTSESTAALGCLVKDYFPEPVTVSWNSGALTSGVHTFPAVLQSSGLYSLSSVVTVPSSSLGTKTYTCNVDHKPSNTKVDKRVESKYGPPCPPCPAPEFLGGPSVFLFPPKPKDTLMISRTPEVTCVVVDVSQEDPEVQFNWYVDGVEVHNAKTKPREEQFNSTYRVVSVLTVLHQDWLNGKEYKCKVSNKGLPSSIEKTISKAKGQPREPQVYTLPPSQEEMTKNQVSLTCLVKGFYPSDIAVEWESNGQPENNYKTTPPVLDSDGSFFLYSRLTVDKSRWQEGNVFSCSVMHEALHNHYTQKSLSLSLGK

SEQ ID NO: 202 - protein, 575 aa, synthetic construct
  REGION 1..575: note = Artificial
VIHVTKEVKEVATLSCGHNVSVEELAQTRIYWQKEKKMVLTMMSGDMNIWPEYKNRTIFDITNNLSIVILALRPSDEGTYECVVLKYEKDAFKREHLAEVTLSVKADGGGGSGGGGSGGGGSGGGGSGQVQLQQWGAGLLKPSETLSLTCAVYGGSFSDYYWNWIRQPPGKGLEWIGEINHRGSTNSNPSLKSRVTLSLDTSKNQFSLKLRSVTAADTAVYYCAFGYSDYEYNWFDPWGQGTLVTVSSASTKGPSVFPLAPCSRSTSESTAALGCLVKDYFPEPVTVSWNSGALTSGVHTFPAVLQSSGLYSLSSVVTVPSSSLGTKTYTCNVDHKPSNTKVDKRVESKYGPPCPPCPAPEFLGGPSVFLFPPKPKDTLMISRTPEVTCVVVDVSQEDPEVQFNWYVDGVEVHNAKTKPREEQFNSTYRVVSVLTVLHQDWLNGKEYKCKVSNKGLPSSIEKTISKAKGQPREPQVYTLPPSQEEMTKNQVSLTCLVKGFYPSDIAVEWESNGQPENNYKTTPPVLDSDGSFFLYSRLTVDKSRWQEGNVFSCSVMHEALHNHYTQKSLSLSLGK

SEQ ID NO: 203 - protein, 684 aa, synthetic construct
  REGION 1..684: note = Artificial
VIHVTKEVKEVATLSCGHNVSVEELAQTRIYWQKNKKMVLTMMSGDMNIWPEYKNRTIFDITNNLSIVILELRPSDEGTYECVVLKYEKDAFKREHLAEVTLSVKADFPTPSISDFEIPTSNIRRIICSTSGGFPEPHLSWLENGEELNAINTTVSQDPETELYAVSSKLDFNMTTNHSFMCLIKYGHLRVNQTFNWNTTKQEHFPDNGGGGSGGGGSGGGGSGGGGSGEVQLVESGGGLVQPGGSLRLSCAASGFTFNTYAMNWVRQAPGKGLEWVARIRSKYNNYATYYAASVKGRFTISRDDSKNSLYLQMNSLKTEDTAVYYCARHGNFGNSYVSWFAYWGQGTLVTVSSASTKGPSVFPLAPSSKSTSGGTAALGCLVKDYFPEPVTVSWNSGALTSGVHTFPAVLQSSGLYSLSSVVTVPSSSLGTQTYICNVNHKPSNTKVDKKVEPKSCDKTHTCPPCPAPELLGGPSVFLFPPKPKDTLMISRTPEVTCVVVDVSHEDPEVKFNWYVDGVEVHNAKTKPREEQYNSTYRVVSVLTVLHQDWLNGKEYKCKVSNKALPAPIEKTISKAKGQPREPQVYTLPPSRDELTKNQVSLTCLVKGFYPSDIAVEWESNGQPENNYKTTPPVLDSDGSFFLYSKLTVDKSRWQQGNVFSCSVMHEALHNHYTQKSLSLSPGK

SEQ ID NO: 204 - protein, 684 aa, synthetic construct
  REGION 1..684: note = Artificial
VIHVTKEVKEVATLSCGHNVSVEELAQTRIYWQKNKKMVLTMMSGDMNIWPEYKNRTIFDITNNLSIVILNLRPSDEGTYECVVLKYEKDAFKREHLAEVTLSVKADFPTPSISDFEIPTSNIRRIICSTSGGFPEPHLSWLENGEELNAINTTVSQDPETELYAVSSKLDFNMTTNHSFMCLIKYGHLRVNQTFNWNTTKQEHFPDNGGGGSGGGGSGGGGSGGGGSGEVQLVESGGGLVQPGGSLRLSCAASGFTFNTYAMNWVRQAPGKGLEWVARIRSKYNNYATYYAASVKGRFTISRDDSKNSLYLQMNSLKTEDTAVYYCARHGNFGNSYVSWFAYWGQGTLVTVSSASTKGPSVFPLAPSSKSTSGGTAALGCLVKDYFPEPVTVSWNSGALTSGVHTFPAVLQSSGLYSLSSVVTVPSSSLGTQTYICNVNHKPSNTKVDKKVEPKSCDKTHTCPPCPAPELLGGPSVFLFPPKPKDTLMISRTPEVTCVVVDVSHEDPEVKFNWYVDGVEVHNAKTKPREEQYNSTYRVVSVLTVLHQDWLNGKEYKCKVSNKALPAPIEKTISKAKGQPREPQVYTLPPSRDELTKNQVSLTCLVKGFYPSDIAVEWESNGQPENNYKTTPPVLDSDGSFFLYSKLTVDKSRWQQGNVFSCSVMHEALHNHYTQKSLSLSPGK

SEQ ID NO: 205 - protein, 684 aa, synthetic construct
  REGION 1..684: note = Artificial
VIHVTKEVKEVATLSCGHNVSVEELAQTRIYWQKNKKMVLTMMSGDMNIWPEYKNRTIFDITNNLSIVILQLRPSDEGTYECVVLKYEKDAFKREHLAEVTLSVKADFPTPSISDFEIPTSNIRRIICSTSGGFPEPHLSWLENGEELNAINTTVSQDPETELYAVSSKLDFNMTTNHSFMCLIKYGHLRVNQTFNWNTTKQEHFPDNGGGGSGGGGSGGGGSGGGGSGEVQLVESGGGLVQPGGSLRLSCAASGFTFNTYAMNWVRQAPGKGLEWVARIRSKYNNYATYYAASVKGRFTISRDDSKNSLYLQMNSLKTEDTAVYYCARHGNFGNSYVSWFAYWGQGTLVTVSSASTKGPSVFPLAPSSKSTSGGTAALGCLVKDYFPEPVTVSWNSGALTSGVHTFPAVLQSSGLYSLSSVVTVPSSSLGTQTYICNVNHKPSNTKVDKKVEPKSCDKTHTCPPCPAPELLGGPSVFLFPPKPKDTLMISRTPEVTCVVVDVSHEDPEVKFNWYVDGVEVHNAKTKPREEQYNSTYRVVSVLTVLHQDWLNGKEYKCKVSNKALPAPIEKTISKAKGQPREPQVYTLPPSRDELTKNQVSLTCLVKGFYPSDIAVEWESNGQPENNYKTTPPVLDSDGSFFLYSKLTVDKSRWQQGNVFSCSVMHEALHNHYTQKSLSLSPGK

SEQ ID NO: 206 - protein, 684 aa, synthetic construct
  REGION 1..684: note = Artificial
VIHVTKEVKEVATLSCGHNVSVEELAQTRIYWQKNKKMVLTMMSGDMNIWPEYKNRTIFDITNNLSIVILTLRPSDEGTYECVVLKYEKDAFKREHLAEVTLSVKADFPTPSISDFEIPTSNIRRIICSTSGGFPEPHLSWLENGEELNAINTTVSQDPETELYAVSSKLDFNMTTNHSFMCLIKYGHLRVNQTFNWNTTKQEHFPDNGGGGSGGGGSGGGGSGGGGSGEVQLVESGGGLVQPGGSLRLSCAASGFTFNTYAMNWVRQAPGKGLEWVARIRSKYNNYATYYAASVKGRFTISRDDSKNSLYLQMNSLKTEDTAVYYCARHGNFGNSYVSWFAYWGQGTLVTVSSASTKGPSVFPLAPSSKSTSGGTAALGCLVKDYFPEPVTVSWNSGALTSGVHTFPAVLQSSGLYSLSSVVTVPSSSLGTQTYICNVNHKPSNTKVDKKVEPKSCDKTHTCPPCPAPELLGGPSVFLFPPKPKDTLMISRTPEVTCVVVDVSHEDPEVKFNWYVDGVEVHNAKTKPREEQYNSTYRVVSVLTVLHQDWLNGKEYKCKVSNKALPAPIEKTISKAKGQPREPQVYTLPPSRDELTKNQVSLTCLVKGFYPSDIAVEWESNGQPENNYKTTPPVLDSDGSFFLYSKLTVDKSRWQQGNVFSCSVMHEALHNHYTQKSLSLSPGK

SEQ ID NO: 207 - protein, 684 aa, synthetic construct
  REGION 1..684: note = Artificial
VIHVTKEVKEVATLSCGHNVSVEELAQTRIYWQKEKKMVLTMMSGDMNIWPEYKNRTIFDITNNLSIVILALRPSDEGTYECVVLKYEKDAFKREHLAEVTLSVKADFPTPSISDFEIPTSNIRRIICSTSGGFPEPHLSWLENGEELNAINTTVSQDPETELYAVSSKLDFNMTTNHSFMCLIKYGHLRVNQTFNWNTTKQEHFPDNGGGGSGGGGSGGGGSGGGGSGEVQLVESGGGLVQPGGSLRLSCAASGFTFNTYAMNWVRQAPGKGLEWVARIRSKYNNYATYYAASVKGRFTISRDDSKNSLYLQMNSLKTEDTAVYYCARHGNFGNSYVSWFAYWGQGTLVTVSSASTKGPSVFPLAPSSKSTSGGTAALGCLVKDYFPEPVTVSWNSGALTSGVHTFPAVLQSSGLYSLSSVVTVPSSSLGTQTYICNVNHKPSNTKVDKKVEPKSCDKTHTCPPCPAPELLGGPSVFLFPPKPKDTLMISRTPEVTCVVVDVSHEDPEVKFNWYVDGVEVHNAKTKPREEQYNSTYRVVSVLTVLHQDWLNGKEYKCKVSNKALPAPIEKTISKAKGQPREPQVYTLPPSRDELTKNQVSLTCLVKGFYPSDIAVEWESNGQPENNYKTTPPVLDSDGSFFLYSKLTVDKSRWQQGNVFSCSVMHEALHNHYTQKSLSLSPGK

SEQ ID NO: 208 - protein, 215 aa, synthetic construct
  REGION 1..215: note = Artificial
QTVVTQEPSLTVSPGGTVTLTCRSSTGAVTTSNYANWVQQKPGQAPRGLIGGTNKRAPGTPARFSGSLLGGKAALTLSGVQPEDEAEYYCALWYSNLWVFGGGTKLTVLGQPKAAPSVTLFPPSSEELQANKATLVCLISDFYPGAVTVAWKADSSPVKAGVETTTPSKQSNNKYAASSYLSLTPEQWKSHRSYSCQVTHEGSTVEKTVAPTECS

SEQ ID NO: 209 - protein, 583 aa, synthetic construct
  REGION 1..583: note = Artificial
VIHVTKEVKEVATLSCGHNVSVEELAQTRIYWQKNKKMVLTMMSGDMNIWPEYKNRTIFDITNNLSIVILELRPSDEGTYECVVLKYEKDAFKREHLAEVTLSVKADGGGGSGGGGSGGGGSGGGGSGEVQLVESGGGLVQPGGSLRLSCAASGFTFNTYAMNWVRQAPGKGLEWVARIRSKYNNYATYYAASVKGRFTISRDDSKNSLYLQMNSLKTEDTAVYYCARHGNFGNSYVSWFAYWGQGTLVTVSSASTKGPSVFPLAPSSKSTSGGTAALGCLVKDYFPEPVTVSWNSGALTSGVHTFPAVLQSSGLYSLSSVVTVPSSSLGTQTYICNVNHKPSNTKVDKKVEPKSCDKTHTCPPCPAPELLGGPSVFLFPPKPKDTLMISRTPEVTCVVVDVSHEDPEVKFNWYVDGVEVHNAKTKPREEQYNSTYRVVSVLTVLHQDWLNGKEYKCKVSNKALPAPIEKTISKAKGQPREPQVYTLPPSRDELTKNQVSLTCLVKGFYPSDIAVEWESNGQPENNYKTTPPVLDSDGSFFLYSKLTVDKSRWQQGNVFSCSVMHEALHNHYTQKSLSLSPGK

SEQ ID NO: 210 - protein, 583 aa, synthetic construct
  REGION 1..583: note = Artificial
VIHVTKEVKEVATLSCGHNVSVEELAQTRIYWQKNKKMVLTMMSGDMNIWPEYKNRTIFDITNNLSIVILNLRPSDEGTYECVVLKYEKDAFKREHLAEVTLSVKADGGGGSGGGGSGGGGSGGGGSGEVQLVESGGGLVQPGGSLRLSCAASGFTFNTYAMNWVRQAPGKGLEWVARIRSKYNNYATYYAASVKGRFTISRDDSKNSLYLQMNSLKTEDTAVYYCARHGNFGNSYVSWFAYWGQGTLVTVSSASTKGPSVFPLAPSSKSTSGGTAALGCLVKDYFPEPVTVSWNSGALTSGVHTFPAVLQSSGLYSLSSVVTVPSSSLGTQTYICNVNHKPSNTKVDKKVEPKSCDKTHTCPPCPAPELLGGPSVFLFPPKPKDTLMISRTPEVTCVVVDVSHEDPEVKFNWYVDGVEVHNAKTKPREEQYNSTYRVVSVLTVLHQDWLNGKEYKCKVSNKALPAPIEKTISKAKGQPREPQVYTLPPSRDELTKNQVSLTCLVKGFYPSDIAVEWESNGQPENNYKTTPPVLDSDGSFFLYSKLTVDKSRWQQGNVFSCSVMHEALHNHYTQKSLSLSPGK

SEQ ID NO: 211 - protein, 583 aa, synthetic construct
  REGION 1..583: note = Artificial
VIHVTKEVKEVATLSCGHNVSVEELAQTRIYWQKNKKMVLTMMSGDMNIWPEYKNRTIFDITNNLSIVILQLRPSDEGTYECVVLKYEKDAFKREHLAEVTLSVKADGGGGSGGGGSGGGGSGGGGSGEVQLVESGGGLVQPGGSLRLSCAASGFTFNTYAMNWVRQAPGKGLEWVARIRSKYNNYATYYAASVKGRFTISRDDSKNSLYLQMNSLKTEDTAVYYCARHGNFGNSYVSWFAYWGQGTLVTVSSASTKGPSVFPLAPSSKSTSGGTAALGCLVKDYFPEPVTVSWNSGALTSGVHTFPAVLQSSGLYSLSSVVTVPSSSLGTQTYICNVNHKPSNTKVDKKVEPKSCDKTHTCPPCPAPELLGGPSVFLFPPKPKDTLMISRTPEVTCVVVDVSHEDPEVKFNWYVDGVEVHNAKTKPREEQYNSTYRVVSVLTVLHQDWLNGKEYKCKVSNKALPAPIEKTISKAKGQPREPQVYTLPPSRDELTKNQVSLTCLVKGFYPSDIAVEWESNGQPENNYKTTPPVLDSDGSFFLYSKLTVDKSRWQQGNVFSCSVMHEALHNHYTQKSLSLSPGK

SEQ ID NO: 212 - protein, 583 aa, synthetic construct
  REGION 1..583: note = Artificial
VIHVTKEVKEVATLSCGHNVSVEELAQTRIYWQKNKKMVLTMMSGDMNIWPEYKNRTIFDITNNLSIVILTLRPSDEGTYECVVLKYEKDAFKREHLAEVTLSVKADGGGGSGGGGSGGGGSGGGGSGEVQLVESGGGLVQPGGSLRLSCAASGFTFNTYAMNWVRQAPGKGLEWVARIRSKYNNYATYYAASVKGRFTISRDDSKNSLYLQMNSLKTEDTAVYYCARHGNFGNSYVSWFAYWGQGTLVTVSSASTKGPSVFPLAPSSKSTSGGTAALGCLVKDYFPEPVTVSWNSGALTSGVHTFPAVLQSSGLYSLSSVVTVPSSSLGTQTYICNVNHKPSNTKVDKKVEPKSCDKTHTCPPCPAPELLGGPSVFLFPPKPKDTLMISRTPEVTCVVVDVSHEDPEVKFNWYVDGVEVHNAKTKPREEQYNSTYRVVSVLTVLHQDWLNGKEYKCKVSNKALPAPIEKTISKAKGQPREPQVYTLPPSRDELTKNQVSLTCLVKGFYPSDIAVEWESNGQPENNYKTTPPVLDSDGSFFLYSKLTVDKSRWQQGNVFSCSVMHEALHNHYTQKSLSLSPGK

SEQ ID NO: 213 - protein, 583 aa, synthetic construct
  REGION 1..583: note = Artificial
VIHVTKEVKEVATLSCGHNVSVEELAQTRIYWQKEKKMVLTMMSGDMNIWPEYKNRTIFDITNNLSIVILALRPSDEGTYECVVLKYEKDAFKREHLAEVTLSVKADGGGGSGGGGSGGGGSGGGGSGEVQLVESGGGLVQPGGSLRLSCAASGFTFNTYAMNWVRQAPGKGLEWVARIRSKYNNYATYYAASVKGRFTISRDDSKNSLYLQMNSLKTEDTAVYYCARHGNFGNSYVSWFAYWGQGTLVTVSSASTKGPSVFPLAPSSKSTSGGTAALGCLVKDYFPEPVTVSWNSGALTSGVHTFPAVLQSSGLYSLSSVVTVPSSSLGTQTYICNVNHKPSNTKVDKKVEPKSCDKTHTCPPCPAPELLGGPSVFLFPPKPKDTLMISRTPEVTCVVVDVSHEDPEVKFNWYVDGVEVHNAKTKPREEQYNSTYRVVSVLTVLHQDWLNGKEYKCKVSNKALPAPIEKTISKAKGQPREPQVYTLPPSRDELTKNQVSLTCLVKGFYPSDIAVEWESNGQPENNYKTTPPVLDSDGSFFLYSKLTVDKSRWQQGNVFSCSVMHEALHNHYTQKSLSLSPGK

SEQ ID NO: 214 - DNA, 1785 bp, synthetic construct
  misc_feature 1..1785: note = Artificial
  source 1..1785: mol_type = other DNA
atgggttggagttgcatcatcctatttctagtggccaccgctaccggcgtgcactccgtgatccacgtgaccaaagaagtcaaggaagtggctaccctgtcttgcggccacaacgtgagcgtagaagagctggctcagaccaggatctactggcagaaaaacaagaagatggtgctgaccatgatgagcggcgacatgaacatctggcctgagtacaagaatagaaccatcttcgacatcaccaacaacctgtctatcgtgatcctggaactgagaccttccgacgagggcacctacgagtgcgtggtgctgaagtacgagaaggatgccttcaagagagagcacctggctgaggtgacactgtccgtgaaggccgacggcggcggcggctctggcggcggcggatctggcggaggaggctccggtggaggcggctcaggcgaggtgcagctgctggaatccggtggcggcctggtccagcctggcggatccctgcggctgtcttgtgcggccagcggctttaccttctccagctacgccatgtcctgggtgcggcaggcccccggcaagggcctggagtgggtcagcggcatcagcggaagtggcggattcacctactacgccgactccgtcaagggcagattcacaatctcccgggacaactccaagaataccctgtacctgcagatgaacagcctgcgggccgaggataccgccgtgtactactgcgccaagccccctagaggctacaactacggccctttcgactactggggacagggcactctcgtgaccgtctcttccgcctctaccaagggccctagcgtgtttcctctggccccatgcagcagatccacctccgagtctacagctgctctgggctgcctggtgaaggattacttccccgagcctgtgaccgtttcttggaactccggcgctctgacctctggcgtgcacacctttccggctgtgctgcagtcctccggcctgtattctctgtcgtctgtggttacagtgcctagctcttctctcggcaccaagacctatacctgcaacgtggaccacaagcctagcaacaccaaagtggacaagcgggtggaatctaagtacggcccaccttgtcccccctgccctgctcctgagttcctgggaggcccatctgtgtttctgttccctcctaagcctaaggacaccctgatgatctctcgcacccctgaagtgacctgtgtggtggtggacgtgtctcaagaggaccccgaggtgcagttcaactggtacgtggatggcgtcgaggtgcataacgccaaaacaaagcctcgggaagagcagttcaattctacatacagagtggtttccgtgctggccgtgctgcaccaggactggctgaacggcaaagagtacaagtgcaaggtgtccaacaagggcctgccttcctcaatcgagaaaactatttccaaggctaagggccagcctagagaacctcaagtgtataccctgcctccatcccaggaagagatgaccaagaaccaggtgtctctgacctgtctggtcaaaggcttctacccctccgatatcgccgtggcctgggagtctaatggccagcctgagaacaactacaagaccaccccccctgtgctggactctgatggctccttcttcctgtactccagactgacagtggacaagtcccggtggcaagaaggcaacgtgttctcctgctccgtgatgcacgaggccctgcatgcacactacacccagaagtccctgtccctgtctttgggcaag

SEQ ID NO: 215 - DNA, 699 bp, synthetic construct
  misc_feature 1..699: note = Artificial
  source 1..699: mol_type = other DNA
atgcacagctcagcactgctctgttgcctggtcctcctgactggggtgagggccagctacgtgctgacccagcccccctccgtgagcgtggctcctggacagaccgccagaatcacctgcggcggaaacaacatcggatcaaaaagcgtgcactggtaccagcagaaacccggacaggcccccgtgctggtggtgtacgatgactctgatagacccagcggcattcccgagagattctctggaagcaacagcggcaacaccgccaccctgaccatcagcagagtggaagccggcgatgaagctgactattattgccaggtgtgggacagcagcagcgaccacgtggtgttcggcggcggaaccaagctgacagtgctgggtcagcccaaggccaaccccactgtcactctgttcccgccctcctctgaggagctccaagccaacaaggccacactagtgtgtctgatcagtgacttctacccgggagctgtgacagtggcctggaaggcagatggcagccccgtcaaggcgggagtggagaccaccaaaccctccaaacagagcaacaacaagtacgcggccagcagctacctgagcctgacgcccgagcagtggaagtcccacagaagctacagctgccaggtcacgcatgaagggagcaccgtggagaagacagtggcccctacagaatgttcatga

SEQ ID NO: 216 - DNA, 1785 bp, synthetic construct
  misc_feature 1..1785: note = Artificial
  source 1..1785: mol_type = other DNA
atgggttggagttgcatcatcctatttctagtggctaccgccaccggcgtgcattccgtgatccacgtgaccaaagaagtgaaagaggtggctaccctgtcctgcggacataatgtgagcgtcgaggaactggcccagacccggatctactggcagaaaaataagaagatggtgctgaccatgatgtctggcgacatgaacatctggcctgagtacaagaaccggaccatcttcgacatcaccaacaacctgtccatcgtgatcctgaacctgagaccttccgacgagggcacctacgagtgcgtggtgctgaagtacgagaaggacgccttcaagcgggagcacctggccgaagtgacccttagcgtgaaggctgacggaggaggcggctctggcggcggcggctcaggcggtggcgggtccggcggcggcggctccggcgaggtgcagctgctggaatctggcggaggactggtgcagcctggcggctccctgagactgagctgtgccgcttcagggttcacatttagttcgtacgccatgtcctgggtgcggcaggcccctggcaagggcctggagtgggtctccggcatctctggcagcgggggcttcacgtactacgctgatagcgtgaaaggcagattcaccattagccgggacaattcgaagaacacactgtacctgcagatgaacagtctgagagccgaggacacagctgtgtactactgcgccaagcccccacggggctacaactacggtcctttcgactattggggccagggcaccctcgtgacagtctcttctgcttctaccaagggaccttccgtgttccctctggctccttgctccagatccacatctgagtctaccgctgctctgggctgcctggtgaaggactacttcccagagcctgttacagtgtcttggaactccggcgctctcacctccggcgtgcacacctttcctgccgttctgcaatcttctggcctgtactccttatcctccgtggtgacagtgccttcatcctccctcggcactaaaacctacacatgcaacgtggaccacaagccttccaacaccaaagtggacaagagagtggaaagcaagtatggccccccctgccctccttgtcctgcacccgagttcctgggcggccccagcgtgtttctcttcccccctaagccaaaggacaccctgatgatctcccgcacccctgaggtgacctgtgtggtcgtggacgtgtctcaagaggatcctgaagtgcagttcaactggtacgtggatggagtggaagtgcacaacgccaagaccaagcctagagaggaacagttcaactccacctacagagtggtatccgtcctggccgtgctgcaccaggactggctgaacggcaaggagtacaagtgcaaggtgtccaacaagggcctgccttcttctatcgagaagaccatctccaaggccaagggccagcccagagaacctcaagtgtacaccctgcctccttctcaggaagagatgaccaagaaccaggtgagcctgacctgtctggtcaagggcttctacccatctgatatcgccgtggcctgggagtctaatggccagcctgagaacaactacaagaccacccccccagtgctggacagcgatggctccttcttcctgtacagccggctgaccgtggataagtccagatggcaggaaggcaacgtgttttcttgctctgtgatgcacgaggccctgcacgcccactatacccagaagtccctgtctctgtccctgggaaaa

SEQ ID NO: 217 - DNA, 1785 bp, synthetic construct
  misc_feature 1..1785: note = Artificial
  source 1..1785: mol_type = other DNA
atgggttggagttgcatcatcctatttctagtggccaccgctaccggcgtccactccgtcatccacgtgaccaaagaggtgaaagaggtggctacactgtcttgcggccacaatgtgtccgtggaagagctggctcagacccggatctactggcagaagaacaagaagatggtactgaccatgatgtccggcgacatgaacatctggcctgagtacaagaacagaaccatcttcgacatcaccaacaacctgtctatcgtgatcctgcagctgagaccctctgacgagggcacctacgagtgcgtggtgctgaagtacgagaaggatgcctttaagagagagcacctggccgaagtgacactgtccgtgaaggccgatggcggaggaggttctggcgggggcggatctggcggcggcggctccggcggcggcggctctggcgaggttcagctgctggaatccggcggaggactggtgcagcctggaggctccctgagactgagctgtgccgcctctggcttcaccttttcttcctacgccatgtcttgggtgcggcaggctcctggcaagggcctggaatgggtctccggcatctccggcagcggcggctttacatactacgccgactctgtgaagggcagattcaccatctcccgggacaactccaagaacaccctgtatctgcagatgaactctctgagagccgaggacacagcagtgtactactgcgccaagcccccaagaggctacaactacggccctttcgattactggggccagggcaccctggttacagtctcttccgccagcaccaagggaccttccgtgtttcctctggccccttgctccagatccacctccgagtccacagctgctctgggctgcctggtcaaggactacttccctgaacccgtgaccgtgtcctggaactctggcgccctgacctctggagtgcacaccttccccgccgtgctgcagtccagcggcctgtactccctgagctccgtggtcaccgtgccttcctcttctctgggaaccaagacctatacctgcaacgtggaccacaagccatctaataccaaggtggacaagcgggtggaatctaagtacggccctccatgtcctccatgccctgctcccgagttcctcggcggaccttctgtgttcctgttcccacctaagcccaaggacaccctgatgatctctcggacacctgaggtgacttgtgtggtggtggacgtgtcccaagaagaccctgaagtgcagttcaactggtacgtggatggcgtggaagtgcataacgccaagaccaagcctcgcgaggagcagttcaacagcacctacagagtggtgtctgtgctggctgtgctgcaccaggactggctgaacggcaaagaatacaagtgcaaggtgagcaataagggcctgcccagctctatcgagaaaaccatttccaaggctaaaggccaacctcgggagcctcaggtgtacaccctgcctcctagccaggaggagatgaccaaaaaccaggtgtctctgacctgtctggtgaagggcttctaccccagcgatatcgccgtggcctgggagagcaatggccagcccgagaacaactataagaccacccctcctgtgctggactccgacggctccttcttcctttactctcggctgacagtggataagtccagatggcaagaaggcaacgtgttctcctgctccgtgatgcacgaggctctgcatgctcactacacccagaagagcctctctctgtctctgggcaag

SEQ ID NO: 218 - DNA, 1785 bp, synthetic construct
  misc_feature 1..1785: note = Artificial
  source 1..1785: mol_type = other DNA
atgggttggagttgcatcatcctatttctagtggccaccgccacaggcgtgcattctgtcatccacgtgaccaaggaagtgaaagaagtggctaccctgtcctgcggccacaatgtgtccgtggaagaactggctcagaccagaatctactggcagaagaacaagaagatggtgctgaccatgatgtctggcgacatgaacatctggcctgagtacaagaaccggaccatcttcgatatcaccaacaacctgtccatcgtgatcctgacgctgcggcctagtgacgagggcacctatgagtgcgtggttctgaagtacgagaaggatgccttcaagagagaacacctggccgaggtcaccttatccgttaaggccgacggcggaggaggaagcggcggcggcggctccggcgggggcggctccggaggcggaggctccggcgaggtgcagctgctggaatccggcggcggactggtgcaacccggtggcagcctgagactgtcttgcgccgccagtggcttcaccttctcctcctacgccatgtcctgggtgcggcaggcccctggcaagggcctggaatgggtctctggcatctctgggtccggcggatttacctactacgctgactccgtgaagggcagattcacaatctctcgggacaactctaagaacaccctgtacctgcagatgaacagcctgagagccgaggataccgctgtgtactactgcgctaagccacctagaggctacaactacggacccttcgactactggggccagggcaccctggtgaccgtgtcctccgccagcacaaagggcccatccgtgttcccactggcaccctgttctagatctacctccgagtctaccgctgctctgggctgcctggtcaaggattacttccccgaacctgtgacagtgtcttggaactccggcgctctgacttctggcgtgcacacctttcctgctgtgttgcagtcttctggcctgtacagcctgagttctgtggtgaccgtgccctcttcctccctgggcacaaagacctacacctgcaacgtggaccacaagccttccaataccaaagtggacaagcgcgtcgaatccaagtacggccctccttgccctccttgccccgctcccgagttcctgggaggaccctccgtgtttctgttccctccaaagcctaaggacaccctgatgatcagccggacccctgaggtgacatgtgtggtggtcgacgtgtctcaggaggaccctgaggtgcagtttaactggtacgtggatggcgtcgaggtgcataacgccaagaccaaacctagagaggaacagttcaacagcacctacagagtggtgtctgtgctggccgtgctccaccaggactggctgaacggcaaagagtacaagtgcaaggtgtccaacaagggtctgccttctagcatcgagaaaaccatctccaaggccaagggccagcctcgggagcctcaggtgtacactctgcctcctagccaagaagagatgaccaagaaccaggtgtctctcacctgtctggtgaaaggcttctacccctcagatattgccgtggcttgggagtccaacggccagcctgagaacaattacaagaccacacctccagtgctggactccgacggctccttcttcctgtattcccggctgaccgtggacaagtccagatggcaagagggcaacgtgttctcttgttccgtgatgcacgaggccctgcacgcgcactacacccagaaatctctgtctctgagcctgggcaag

SEQ ID NO: 219 - DNA, 1785 bp, synthetic construct
  misc_feature 1..1785: note = Artificial
  source 1..1785: mol_type = other DNA
atgggttggagttgcatcatcctatttctagtggccaccgctaccggcgtgcactccgtaattcacgtgaccaaagaggttaaagaagtggctacactgagctgcggccacaatgtgagcgtcgaggagttggctcagacccggatctactggcagaagtccaagaagatggtgctgaccatgatgtctggcgacatgaacatctggcctgagtacaagaacagaaccatctttgatatcaccaacaacctgtctatcgtgatcctggaactgcggccttctgacgagggcacatatgaatgcgtggtgctgaagtacgagaaggacgccttcaagagggagcacctggccgaggtgaccctctccgtcaaggccgatggcggtggcggttcgggaggcggaggaagcggcggcggcggcagcggaggaggtggctctggcgaggtgcagctgctggaatctggcggcggcctggtgcagcctggcggctctctgagactgagctgtgctgcctccggcttcaccttctcctcctacgccatgtcctgggtcagacaggcccccggcaagggcctggaatgggtgtctggaatcagtggctccggaggctttacctactacgccgactctgtgaaaggccggttcaccatctctcgggacaactccaagaataccctgtacctgcagatgaactccctcagagccgaggatacagctgtgtactactgcgccaagccccctagaggctacaactacggccctttcgactactggggccagggcaccctggtcaccgtgtcctctgcctctaccaagggcccctctgtgttccctctggctccttgctctagatccacctccgagtccaccgccgctctgggctgcctggtgaaggattacttcccggaacccgtgacagtttcttggaactccggcgctctgacctctggcgtgcacacctttcctgctgtgctgcagtcctccggcctgtattccctgtcgtccgtggtgaccgtgcctagtagctctctgggaaccaagacttacacctgcaacgtggaccacaagccctctaacacaaaagtggacaagcgggtggagagtaagtatggcccaccctgccctccttgtcctgcccctgagttcctgggcggaccctccgtgtttctcttccctcccaagcctaaggacaccctgatgatctcccggaccccagaagtgacctgtgtggtggtcgacgtgtctcaagaggaccctgaagtgcagttcaactggtacgtggacggcgtggaagtccataacgccaagaccaagcctagagaggaacagttcaacagcacctacagagtggtgagcgtgctggccgtgctgcaccaggattggctgaacggcaaagagtacaagtgcaaggtgtccaacaagggactgccttcctccatcgagaagacaatctccaaggctaagggccagcctcgcgagcctcaggtgtacaccctgcctccatctcaggaagagatgaccaagaaccaggtgagcctgacctgtctggtgaagggcttctacccttccgacatcgccgtggcctgggagtccaatggccaacctgagaacaactacaagaccacccctcctgtgctggactccgacggctccttcttcctgtactcccggctgacagtggataagtccagatggcaagaaggcaacgtgttctcttgctcggtgatgcacgaggccctgcatgctcactacacccagaaaagcttatctctgtctctgggcaag

SEQ ID NO: 220 - DNA, 1785 bp, synthetic construct
  misc_feature 1..1785: note = Artificial
  source 1..1785: mol_type = other DNA
atgggttggagttgcatcatcctatttctagtcgcaaccgctaccggcgtgcactccgtgatccacgtgaccaaagaagtgaaagaggtcgccaccctgtcttgtggccacaacgtgtctgtggaggaactggctcagaccagaatctactggcagaaatctaagaagatggtcctgacaatgatgtctggcgacatgaacatctggcctgaatataagaaccggaccatcttcgacatcaccaacaacctgtctatcgtgatcctgaacctgcggccttccgacgaggggacgtacgagtgcgtggtgctgaagtacgagaaggacgccttcaagagagagcacctcgctgaagtcaccctgagcgtgaaggccgatggcggcggcggctccggcggcggcggttccggaggcggcggctccggaggcggcggatccggcgaggtgcagctgctggaatccggcggaggactggtgcagcctggcggatccctgagactgtcttgcgccgcttctggcttcaccttttcctcttacgctatgagctgggtgcggcaggcccccggaaaaggcctggaatgggtcagtggcatctctggctctggcggctttacctactacgccgactccgtgaagggaagattcactatctcccgggacaactccaagaataccctgtacctgcagatgaattctctgagagccgaggacaccgccgtgtactactgcgctaagcctcctagaggctacaactacggccctttcgactattggggccagggcaccctggtcaccgtgtcttccgcctctaccaagggcccatccgtgtttcctctggccccttgtagccggtccacctccgagtcaacagctgctttgggctgcctggtgaaggactacttccccgagcctgtgacagtgtcttggaactctggcgctctgaccagcggcgtgcacaccttccctgctgtgctgcagtccagcggcctgtatagcctgtcctccgtggtgaccgtgccttcctcctctctgggaacaaagacctacacctgcaacgtggaccacaagcccagcaacaccaaagtggacaagcgggtcgaatccaagtacggccctccatgtcctccttgccctgctccagagttcctgggcggcccctccgtgtttctgttccctcccaagcctaaggatacactgatgatcagcagaacccctgaagtgacctgtgtggtggtggacgtgtcccaagaggatcccgaggtgcagttcaactggtacgtggacggcgtggaagtgcataacgccaagaccaagcctagagaagagcagttcaactccacctacagagtggtttctgtgctggccgtgctgcaccaggactggctgaacggcaaagaatacaagtgcaaggtgtccaacaaaggcctcccctcatccatcgagaagacaatttctaaggctaagggccaaccccgcgaacctcaggtgtacactctgcctccatctcaggaggagatgaccaagaaccaggtctctctgacctgcttggtgaagggcttctacccttccgatatcgccgtggcctgggagtccaatggccagcctgagaacaactacaagaccacccctcccgtgctggactctgatgggtccttcttcctgtacagccggctgacagtggataagtccagatggcaagagggcaacgtgttcagctgctccgtgatgcacgaggccctgcatgcccactacacccagaagtctctttcgctgtcactgggcaag

SEQ ID NO: 221 - DNA, 1785 bp, synthetic construct
  misc_feature 1..1785: note = Artificial
  source 1..1785: mol_type = other DNA
atgggttggagttgcatcatcctatttctagtggctacagctaccggcgtgcattccgtgatccacgtgaccaaagaggtcaaggaagtggccacactgtcttgcggccacaatgtgtccgtggaagagctggcccagacacgcatctactggcagaagtccaagaagatggtgctgaccatgatgtccggcgacatgaacatctggcctgagtacaagaacagaaccatcttcgacatcaccaacaacctgtccatcgtgatcctgcagctgaggccatccgacgaaggcacatatgagtgcgtagtgctgaagtacgagaaggacgccttcaagcgggagcacctggctgaagtgactctctccgtgaaagccgatgggggcggcggctccggcggcggcggaagcggcggcggcggctctggcggcggcggctctggcgaggtgcagctgctggaatctggaggcggactggtgcaacccggcggcagcctccggctgtcctgcgctgcttctggctttaccttctccagctacgctatgtcttgggtgcggcaggcccctggcaagggcctggagtgggtctccggcatctctggttcgggaggcttcacttactacgccgatagcgtgaagggcagattcaccatttcccgggacaactccaagaatacactgtatctgcagatgaacagcctgagagccgaggacaccgctgtgtactactgcgccaagcctcctagaggctacaactacggtcctttcgattactggggccagggcaccctggtcaccgtgtcttccgcctccaccaagggaccttctgtgttccctctggctccttgctcccggtcaacctccgagtccaccgccgccctgggctgcctggtgaaggactacttccccgaacccgtgaccgtgagctggaactctggtgctctgacctctggcgtgcacacctttcctgctgtgttgcagtccagcggcctgtactccttgtcatccgtggtgaccgtgccctcctctagcctgggcaccaaaacctatacctgcaacgtggaccacaagccttccaacaccaaagtggacaagagagtggaatctaagtacggccccccttgccctccttgtcctgccccagagttcctgggcggacctagcgtgtttctgttccctcctaagcccaaggataccctgatgatctcccggacccccgaagtgacctgtgtggtggtggacgtctcccaggaagatcctgaagtgcagttcaactggtacgtggacggcgtcgaggtgcacaacgccaaaacaaagcccagagaggaacagttcaactctacctacagagtggtgtcagtgctggccgtgctgcaccaggactggctgaacggcaaagagtacaagtgcaaggtctccaacaagggcctgcctagctcaatcgagaagaccatctctaaggccaagggacagcctcgggagcctcaggtctacaccctgcctccatctcaagaggagatgaccaagaaccaggtgagtctgacatgtctggtgaagggattctacccttctgatatcgctgtggcctgggaaagcaatggccagcctgagaacaactacaagaccacccccccagtgctggactccgacggatccttcttcctgtactctagactgaccgttgacaagtccagatggcaagagggcaacgtgttttcttgttctgtgatgcacgaggccctgcatgctcactacacccagaaatctttgtccctgtccctgggcaag

SEQ ID NO: 222 - DNA, 1785 bp, synthetic construct
  misc_feature 1..1785: note = Artificial
  source 1..1785: mol_type = other DNA
atgggttggagttgcatcatcctatttctagtcgccaccgccaccggcgtgcattccgtgatccacgtgaccaaagaagtgaaagaggtggccactctgtcttgcggccataacgtgagcgtcgaggaactggcccagaccaggatctactggcagaagtccaagaagatggtgctgaccatgatgtccggcgacatgaacatctggcctgaatataagaaccggaccatcttcgacatcaccaacaacctgtccatcgtgatcctgaccctgcggccttccgacgagggcacctacgagtgcgtggtgctgaagtacgagaaggatgccttcaagcgggagcacctggctgaagtgacactgagcgtgaaggccgacggcggcggcggctctggcggcggaggctccggcggaggcggatccgggggcggcggctcgggcgaggtccagctgctggaaagcggaggaggcttagtgcaacctggaggctctctcagactgtcctgtgctgcctctggcttcaccttctcttcctacgccatgtcttgggtcagacaggcccctggcaagggcctggaatgggtgagcggcatttctggctctggaggctttacctactatgctgactccgttaaaggcagattcaccatctcccgggacaactccaagaatacactgtacctgcagatgaactctctgagagccgaggatacagctgtgtactactgcgccaaaccccccagaggctacaactacggccctttcgactactggggccagggcaccctcgtgaccgtgtcctccgcttccaccaagggcccatctgtgtttcctctggctccttgctctcggtctacctccgagtccaccgctgctctgggctgcctggtgaaggactacttccccgagcctgtgaccgtgtcctggaactccggcgctctgacctctggcgtgcacacctttcctgccgtgctgcagagttccggcctgtactccctgagctctgtggtgacagtgcctagttccagcctgggaaccaagacctatacctgcaacgtggaccacaagcccagcaataccaaagtggacaagcgggtggagtctaagtacggccccccatgtcctccatgtcctgctcctgagttcctgggcggaccatctgtatttttgttccctcccaagcctaaggacaccctgatgatctccagaacccctgaagtgacctgcgttgtggtggacgtgtctcaagaggaccccgaggtgcagttcaactggtacgtggatggagtggaagtgcacaacgccaaaaccaagcctagagaagagcagttcaacagcacctacagagtggtctccgtgctggccgtgctgcaccaggactggctgaacggcaaagagtacaagtgcaaggtgtccaacaagggcctgccttcctctatcgagaagacaatcagcaaggctaagggccagccccgcgaacctcaggtgtacaccctgcctccttctcaagaagagatgacaaagaaccaggtgtccctgacctgtctggtgaagggattctacccctccgatatcgccgtggcttgggagtccaatggccagcctgagaacaactataagaccacacctcctgttctggactctgatggctccttcttcctgtacagccggctgaccgtggataagtcaagatggcaggaaggcaacgtgttctcctgctccgtaatgcacgaggccctgcacgcccactacacccagaagagcctgtctctgtccctgggcaag

SEQ ID NO: 223 - DNA, 1785 bp, synthetic construct
  misc_feature 1..1785: note = Artificial
  source 1..1785: mol_type = other DNA
atgggttggagttgcatcatcctatttctagtggccaccgctaccggcgtgcactccgtgatccacgtcacaaaagaggtgaaagaggtggctacactgtcctgcggccacaacgtgtctgtggaggagctggcccagaccagaatctattggcagaagcagaagaagatggtgctgaccatgatgtccggcgacatgaacatctggcctgagtacaagaaccggaccatcttcgacatcaccaacaatctgtctatcgtgatcctggaactgcggccttccgacgagggcacctacgagtgcgtggtgctgaagtacgagaaggacgccttcaagcgcgagcacttggctgaggtgacactgtccgtgaaggccgacggcggcggcggctcaggcggcggcggatctggcggcggaggctccggtggcggaggcagcggggaagtgcagctgctggaatctggcggcggcctggtgcagcctggcggatctctgagactgagctgtgctgcctctggcttcactttctcctcctacgccatgtcctgggtgcggcaggctcctggaaagggactggagtgggtttcgggcatcagcggctctggcggcttcacctactacgccgattccgtgaaaggcagattcacaatctctcgggacaacagcaagaacaccctgtacctgcagatgaactccctgagagccgaggacaccgccgtgtactactgcgctaagcctccaagaggctacaactacggccccttcgattactggggccagggcaccctcgtgactgtgtcctctgcctccaccaagggcccttccgtgttccctctggccccttgcagccggtctacctctgagtccaccgccgctctgggctgcctggtgaaggactacttcccagaacctgtgaccgtgtcttggaactctggcgctctgacctccggcgtgcacacttttcctgccgtgctgcagtctagtggcctgtactccctgtcctccgtcgtcaccgtgcctagcagcagcctgggcacaaagacctacacctgcaacgttgaccacaagccctccaatacaaaagtggacaagagagtggaatctaagtacggccccccttgtcctccttgccctgctcctgagttcctgggaggcccctccgtgtttctgttccccccaaagcctaaggataccctgatgattagtagaacccccgaagtgacctgtgtcgtggtggacgtgtcccaagaggatcctgaagtgcagttcaactggtacgtggatggcgtcgaggttcataacgccaagaccaagcccagggaggaacagttcaatagcacctatagagtcgtgagcgtgctggctgtgctgcaccaggactggctgaacggcaaggaatacaagtgcaaggtgtccaacaagggcctgccttcctccatcgagaagaccatctccaaggctaagggccagcctagagaacctcaagtgtatacactgccaccttctcaggaagagatgaccaagaaccaggtgtccctgacctgtctggtcaaaggattctacccttctgatatcgccgtggcctgggagtccaacggccagcccgagaacaattacaaaaccacccctcccgtgctggactccgacggctccttcttcctgtactctcggctgaccgtggacaagtccagatggcaagaaggtaacgtgttttcttgctccgtgatgcacgaggccctgcatgctcactacacccagaaatctctgtctctgtcgctcggcaag

SEQ ID NO: 224 - DNA, 1785 bp, synthetic construct
  misc_feature 1..1785: note = Artificial
  source 1..1785: mol_type = other DNA
atgggttggagttgcatcatcctatttctagtggctaccgccaccggcgtgcattccgtgatccacgtgaccaaggaagtgaaagaggtggccaccctgtcctgcggccacaatgtgtctgtcgaggaactggcccagaccagaatctactggcagaagcagaagaagatggtgctgaccatgatgtccggcgacatgaacatctggcctgagtataagaatagaacaatcttcgatatcaccaacaacctgtccatcgtgatcctgaacctgcggccttctgacgagggcacctacgagtgcgtggtgctgaagtacgaaaaagacgccttcaagagggagcacctggctgaagttacactgtcggtgaaggccgatggcggcggcggatctggcgggggcggctctggcggaggcggctccggcggcggcggcagcggcgaggtgcagctgctggaatctggaggcggcctggtgcagcctggcggatcgctgagactgtcgtgcgcagcttccgggtttaccttctcctcctacgccatgtcttgggtcagacaggctcctggaaagggcctggaatgggtgtctggcatcagcggctctggaggctttacctactacgctgacagcgtcaaaggccggttcaccatttctagagacaactccaagaacaccctgtacctgcagatgaactccctgcgggccgaggacaccgctgtgtactactgcgccaagccccctagaggctacaactatggccctttcgactactggggtcagggcacactggtcacagtgtcctcagccagtaccaaaggcccctccgtgttccctctggccccttgttctcggtctacctccgagtccaccgccgccctgggctgcctggtgaaggactacttccctgagcccgtgaccgtgtcctggaactctggcgccctgacatctggcgtgcacacctttcctgctgtgctgcagtcctccggactgtactctctgtctagcgtggtgaccgtgccttcttcttccctgggcacgaagacctatacttgcaacgtggaccacaagccttctaataccaaggtggacaagcgggtcgaaagcaagtacggcccaccttgcccaccatgtcctgctcctgagttcctgggaggcccatctgtgtttctgttcccgcccaagcctaaggatacactgatgatctcccggacccccgaggtgacctgtgtggtcgtcgacgtgtctcaggaggatcctgaagtgcagttcaactggtacgtggacggcgtggaagtgcacaacgccaagaccaagccccgcgaagagcagttcaacagcacctacagagtggtgtccgtgctggctgtgctgcatcaggactggctgaacggcaaagagtacaagtgcaaggtgtccaacaagggcctgccttcttccatcgagaagaccatctccaaggctaagggacagcctcgggagcctcaggtgtacaccctacctcccagccaagaagagatgaccaagaaccaggtctccctcacctgtctggtaaagggcttctacccttccgacatcgccgtggcctgggaatccaacggccaacccgagaacaattacaaaaccacccctccagtgctggactccgatggctccttcttcctgtactccagactgaccgtggataagtccagatggcaagagggcaacgtgttcagctgctccgtgatgcacgaggctctgcacgcccactacacccagaaatctctgtccttatctctcggcaag

SEQ ID NO: 225 - DNA, 1785 bp, synthetic construct
  misc_feature 1..1785: note = Artificial
  source 1..1785: mol_type = other DNA
atgggttggagttgcatcatcctatttctagtggctaccgctacaggagtgcactccgtgatccacgtgaccaaagaagtgaaagaggtggccaccctgagctgcggccataatgtgagcgtcgaggaactggcccagacccggatctactggcagaagcagaagaagatggtgctgaccatgatgtccggcgacatgaacatctggcctgagtacaagaacagaaccatcttcgatatcaccaacaatctgtccatcgtgattctgcagctgagaccctctgacgagggcacatacgagtgcgtggtgctgaagtacgagaaggacgccttcaagcgcgagcacctggctgaggtcacactgtccgtgaaggccgatggcggaggcggcagcggaggcggcggctctggcggcggcggctctggcggaggcggttctggcgaggtacagctgctggaatctggcggcggactggtgcagcctggcggctctctccggctgtcctgcgccgcctccggcttcaccttttcctcctacgccatgtcttgggtcagacaggcccctggcaagggactggaatgggtgtccggcatctctggatctggaggctttacctactacgccgactccgtcaagggcagattcaccatctcccgggacaactccaagaacaccctgtacctgcagatgaactctctgagagccgaggacactgctgtgtactactgcgctaagccacctagaggctacaactacggccctttcgactactggggccagggcaccctggtgacagtaagctctgcttctaccaagggcccttctgtgttccctctggctccttgctcccgttccacctctgagtcaaccgccgctctgggctgcctggtgaaggattacttccccgaacccgtcaccgtttcctggaactccggcgctctgacctccggcgtgcacacctttcctgccgtgctgcagtcctctggcctgtacagtctgtcttccgtggtgacagtgccttcctccagtttgggcaccaagacttacacctgcaacgtggaccacaagccgtcaaataccaaagtggacaagagagtggaatccaagtacggacctccttgtcctccatgccctgctcccgagttcctcggaggcccctccgtgtttctgttccctcctaaacccaaggacaccctgatgatctctcggacccccgaggtcacctgtgtggtggtggacgtgtctcaggaagatcctgaagtgcagttcaactggtacgtggatggcgtggaagtgcacaacgccaagacaaagcctagagaagagcagttcaacagtacctaccgggtggttagcgtgttagctgtgctgcatcaggactggctgaacggcaaagagtacaagtgcaaggtgtccaacaagggcctgccttcctctatcgagaaaaccatcagcaaggctaagggccaaccccgggaacctcaggtgtataccctgcctccatcccaagaggagatgaccaagaaccaggtgtccctgacctgtctggtgaagggcttctacccttccgacatcgccgtggcctgggagtccaacggccagcctgagaacaactataagaccacccctcctgtgctggactctgacggctccttcttcctgtactccagactgaccgtggataagtctagatggcaagaaggcaacgtgttcagctgtagcgtgatgcacgaggccctgcacgcccactacacacagaagtctctcagcctgtctctgggaaaa

SEQ ID NO: 226 - DNA, 1785 bp, synthetic construct
  misc_feature 1..1785: note = Artificial
  source 1..1785: mol_type = other DNA
atgggttggagttgcatcatcctatttctagttgctaccgccaccggcgtgcactccgtcatccacgtgaccaaagaggtgaaagaggtggctacactgtcttgtggccacaacgtgtccgtggaggaactggcccagaccaggatctactggcagaagcagaagaagatggtgctgaccatgatgtctggcgacatgaacatttggcctgagtataagaaccggaccatcttcgatatcaccaacaacctgtccatcgtgatcctgacactgcggccttcggacgagggcacctacgagtgtgtggtgctgaagtacgagaaggacgccttcaagcgcgagcacctggctgaagtgacattgtccgtgaaggctgatggcggaggcggctccggaggaggaggctccggcggcggcggctctggcggaggcggatccggcgaggtgcagctgctggaaagcggcggcgggctcgtgcaacctggaggcagcctgagactgtcctgcgccgcttctggatttaccttctcctcctacgccatgtcctgggtgcggcaggccccaggcaagggcctggaatgggtctccggcatcagcggctctggtggcttcacctattatgccgactctgtgaaaggcagattcaccatctctcgggataactccaagaataccctgtacctgcagatgaactctctgagagccgaggatactgctgtgtactactgcgctaagccacccagaggctacaactacggccctttcgactactggggccagggcaccctggtcaccgtgtcttccgcctctaccaagggcccttctgtgttccccctggctccttgcagtagatccacctccgagtccaccgctgctctgggctgcctggtgaaggactacttccccgaacctgtgaccgtgtcctggaactccggcgccttaacctctggcgtccacacctttcctgctgtgctgcagtccagcggcctgtactccctgtcttctgtggtgaccgtgccttcttcctccctgggaaccaagacctacacttgcaacgtggaccacaagcctagcaacaccaaagtggacaagcgggtggaatccaagtacggccccccctgccctccttgtcctgccccggagttcctgggcggccctagcgtgtttctgttcccccctaagcccaaggacaccctgatgatctccagaacccctgaagttacctgcgttgtcgtggatgtgtcacaggaggaccccgaggtgcagttcaactggtacgtggacggcgtggaagtgcataatgccaaaaccaagcctcgggaagagcagttcaactctacatacagagtggtgtctgtgctggccgtcctgcatcaggactggctgaacggcaaggaatacaagtgcaaggtgtccaacaagggactgccctcttctatcgagaagacaatcagcaaggccaagggacagcctagagagcctcaggtgtacacactgcctccttcccaagaggagatgaccaagaaccaggtgagtctgacctgtctggtgaaaggcttctacccctccgacatcgccgtggcctgggagtctaatggccagcctgagaacaactacaagaccacccctccagtgctggactccgacggctccttcttcctgtactctcggctgacagttgataagtccagatggcaagaaggcaacgtgttctcttgctccgtgatgcacgaggccctgcacgcccactacacccagaagtctctgtctctcagcctgggcaaa

SEQ ID NO: 227 - DNA, 1785 bp, synthetic construct; identical to SEQ ID NO: 226
  misc_feature 1..1785: note = Artificial
  source 1..1785: mol_type = other DNA

SEQ ID NO: 228 - DNA, 1785 bp, synthetic construct
  misc_feature 1..1785: note = Artificial
  source 1..1785: mol_type = other DNA
atgggttggagttgcatcatcctatttctagtggccaccgcaacaggcgtgcactccgtgatccacgtgaccaaagaagtgaaagaggtggctacactgtcctgcggccataatgtgtctgtcgaagagctggctcagaccagaatctactggcagaaaaccaagaagatggtccttaccatgatgtccggcgacatgaacatctggcctgagtacaagaacagaaccatcttcgacatcaccaacaacctgtccatcgtgatcctgaacctgagaccttccgacgagggcacctatgagtgcgtggtgctcaagtacgagaaggacgccttcaagagagagcacctggctgaggtcacactgtccgtgaaggccgatggcggcggaggctctggcggcggaggctctggcgggggcggttctggaggcggcggctctggcgaggtgcagctgctggaaagcggcggcggcctggtgcagcctggaggctccctgcggctgtcttgtgctgccagcggatttaccttttccagctacgccatgtcttgggtccggcaggcccctggcaagggcctggaatgggtgagcggcatctctggatctggcggcttcacctactacgccgactccgtgaagggcagattcaccatctcccgggacaactccaagaacaccctgtacctgcagatgaactctctcagagccgaggacaccgccgtgtactactgcgccaagcctcctagaggctacaactatggccccttcgattactggggccagggcaccctcgtgaccgtgagttctgcctccaccaagggaccttctgtgtttcctctggctccttgcagccggagcacatccgagtccacagctgctctgggctgtctggtcaaggactacttcccagaacccgtgacagtatcctggaactccggagccctgacctctggcgtgcacaccttccctgccgtcctgcagtcctccggcctgtactccctgtcttctgtagtgaccgtgccttcttccagccttggcaccaagacatatacctgcaacgtggaccacaagccttctaataccaaagtggataagcgggtggaatccaagtacggccctccttgccctccttgtcctgctcccgagttcctgggcggcccatctgtctttctgttcccccccaagcctaaggataccctgatgatctcgcggacccctgaagtgacctgtgtggtagtcgacgtgtctcaagaggatccagaagtgcagttcaactggtacgtggacggcgtggaagtgcacaacgctaagaccaagccccgggaagaacagttcaattctacctacagagtggtgtccgtgctggctgtgctgcaccaggactggctgaatggaaaagagtacaagtgcaaggtgtccaacaagggcctgcctagctctatcgagaaaaccatttctaaggccaagggccagccccgcgagcctcaggtgtacaccctgcctccatctcaagaggagatgaccaagaaccaggttagtctgacctgcctggtgaaaggcttctacccctcagatatcgccgtggcctgggagtccaacggccagcctgagaacaactacaagaccacacctcctgtgctggactccgacggctccttcttcctgtactccagactgactgtggacaagtctagatggcaagagggcaacgtgttctcctgctccgtgatgcacgaggccctgcatgctcactacacccagaagtccctgtccctgtcactgggcaag

SEQ ID NO: 229 - DNA, 1785 bp, synthetic construct
  misc_feature 1..1785: note = Artificial
  source 1..1785: mol_type = other DNA
atgggttggagttgcatcatcctatttctagttgctaccgctaccggcgtgcactccgtgatccacgtgacaaaggaggtgaaagaagtggccacactgtcttgcggccataacgtgagcgtggaagagctggcccagaccagaatctactggcagaaaaccaagaagatggtgctgaccatgatgtctggcgacatgaacatctggcctgaatacaagaatcggaccatcttcgacatcaccaacaacctgtccatcgtgatcctgcagctgagaccttcggacgagggcacatacgagtgcgtcgtgctgaagtacgagaaggacgccttcaagagagagcacctggccgaagtgacactgtctgtgaaggctgacggcggcggaggatctggcggcggcggctctggaggcggcggatctggcggcggcggatcaggcgaagtgcagctgttggagagtggcggcggcctggtacagcccggaggttctctgagactgtcctgcgctgcctctggctttaccttctcctcctacgccatgtcctgggtgcggcaggcccctggcaaaggcctggaatgggtgtccggaatctctggctctggcggattcacttactacgccgactctgtgaagggccggttcacaatctcccgggacaactccaagaataccctctacctgcagatgaactccctgagagccgaggacaccgccgtctattactgcgccaagcctcctagaggctacaactacggccccttcgattactggggccagggcaccttggtgaccgtgtcttctgcctccaccaagggcccttccgtgttccctctcgctccttgctcccggtctacctctgagtctaccgctgctctgggctgcctggtgaaggactatttccctgaacctgtgaccgtgtcctggaactccggcgctctgacctccggtgtgcacacctttcctgccgtgctgcagtcctctggactgtactctctgtcctctgtggtcaccgtgccttcctcctctctgggcaccaagacctatacctgcaacgtcgatcacaagccctctaacacgaaagtggataagagagtggaaagcaagtacggccctccatgtcctccttgtcctgctcctgagttcctgggcggcccttccgtgtttctgttcccacctaagcccaaggataccctgatgatctccagaacacctgaagtcacctgcgtggtggtggatgtgagccaagaggaccccgaggtgcagtttaactggtacgtggatggcgtggaggtgcacaacgccaagaccaagcctagagaagagcagttcaatagcacctaccgggtggtgtctgttctggctgtgctgcaccaggactggctgaacggcaaagagtacaagtgcaaggtgtccaacaagggcctgcccagctccatcgagaaaacaatttccaaggccaaaggccagcctcgcgagcctcaggtgtacaccctgccaccgtcccaagaggagatgaccaagaaccaggtgtccctgacctgtctggtcaaaggcttctacccttctgacatcgccgtcgcttgggagtccaatggccagcccgagaacaactacaagaccaccccacccgtgctggactccgacggctccttcttcctgtactcccggctgacagtggacaagtccagatggcaagaaggcaacgtgttcagctgttccgtgatgcacgaggccctgcatgcccactacacccagaagagcctgtcactgagcctcggcaag

SEQ ID NO: 230 - DNA, 1785 bp, synthetic construct
  misc_feature 1..1785: note = Artificial
  source 1..1785: mol_type = other DNA
atgggttggagttgcatcatcctatttctagtggctaccgctacaggagtgcattccgtcatccacgtgaccaaagaggtgaaggaagtggccaccctgtcctgcggccacaatgtgtctgtggaagagctggctcagaccagaatctactggcagaagaccaagaagatggtgctgaccatgatgtccggcgacatgaacatctggcctgagtacaagaacagaaccatcttcgacatcaccaataatctgtccatcgtgatcctgacactgaggccttctgacgagggcacctacgagtgcgtggtgctgaagtacgaaaaggatgccttcaagcgggagcatctggctgaagtgaccctgtctgtgaaggctgacggcggcggaggctcaggcggcggcggctctggcggaggtggctctggaggcggcggctccggcgaggtccagctgctggaatccggcggcggactggtgcagcccggaggctccctgcggctgtcttgcgccgcctccggctttacttttagttcctatgccatgtcttgggtgcggcaggcccccggcaagggcctggaatgggtctctggcatctccggctctggcggcttcacctactacgccgactccgtcaaaggcagattcaccatttctcgggacaacagcaagaatacactgtacctgcagatgaactctctgcgggccgaggatacggctgtgtactactgcgctaagccccccagaggctacaactacggccctttcgactactggggccagggcacccttgtgaccgtgtcctccgcctccaccaagggcccttccgtgtttcctctggccccttgctcccggtccacctccgagtccaccgccgctctgggctgcctggtgaaggattacttccccgagcctgtgacagtgtcctggaacagcggcgctctgacctccggcgtgcacaccttccctgccgttctgcagtctagcggcctgtatagtctgagctccgtggtcaccgtgccttcttcctctcttggaacaaagacatacacctgcaacgtggaccacaagccctctaacaccaaggtggataagagagtggagtccaagtacggccccccttgccctccttgtcctgctccagagtttctgggtggaccttctgtgttcctgttccctcctaagcccaaggacaccctgatgatcagcagaacccctgaggtgacctgtgtggtggtcgacgtgtctcaagaggaccctgaagtgcagttcaactggtacgtggatggcgtggaagtgcacaacgccaagaccaagcctcgggaagagcagttcaactccacctacagagtggtctctgttctggctgtcctgcaccaggactggctgaacggcaaagagtacaagtgcaaggtgtccaacaaagggctcccatcttctatcgagaagaccatctccaaggccaagggccaacctagagagcctcaggtgtacaccctgcctccatctcaagaggaaatgaccaagaaccaggtgtctctgacctgtctcgtgaagggcttctaccccagcgatatcgccgtggcctgggagtccaacggccagcctgagaacaactataaaactacacctccagtgctggactccgacggctccttcttcctgtactccagactgaccgtggacaagtctagatggcaggaaggcaacgtgttcagctgttccgtgatgcacgaggccctgcacgcccactacacccagaaaagcctgagcctgtccttgggcaag

SEQ ID NO: 231 - DNA, 1785 bp, synthetic construct
  misc_feature 1..1785: note = Artificial
  source 1..1785: mol_type = other DNA
atgggttggagttgcatcatcctatttctagtggccaccgctaccggcgtgcactccgtgatccacgtgacaaaagaggttaaagaagtggctacactgtcttgcggccataatgtgtctgtggaagagttggctcagaccagaatctactggcagaaagagaagaagatggtgctgaccatgatgagtggcgacgccaatatctggcctgagtacaaaaaccggacgatcttcgacatcacgaacaacctgtctatcgtgtacctggaactgcggccttctgacgagggaacctacgagtgcctggtgctgaagtacgagaaggatgccttcaagagagagcacctggctgaggtgacactgtccgtgaaggccgacggcggcgggggttctggcggcggcggctctggcggaggaggatctggcggcggaggctccggcgaggtgcagctgctggaaagcggaggcggactggtccagcctggcggctccctgagactgagctgtgctgccagcgggttcacattttcctcctacgccatgtcctgggtccggcaggcccccggcaagggcctggaatgggtgtccggcatctccggctctggcggctttacctactacgccgattccgtgaagggcagattcaccatctcccgggacaactctaagaacaccctgtacctgcagatgaactctctgagagctgaggacaccgccgtgtactactgcgccaagccacctagaggctacaactatggccccttcgattactggggacagggcaccctcgtgaccgtgtcctctgcctctactaagggcccatctgtgttccctctggctccttgctccagatctacctccgagtctaccgctgccctgggctgcctggtgaaggactacttccccgagcctgtgaccgtctcttggaactccggcgccctgacctctggcgtgcacacctttcctgctgtgctccagtccagcggcctgtacagcctctcttctgtcgtgaccgtgccaagctcctcactcggcaccaagacctacacctgcaacgtggaccacaagccatccaatacaaaagtggacaagcgggtggaatccaagtacggccctccctgtcctccctgccctgctcctgagttcctgggcggaccttctgtgtttctgttccctcctaagcccaaggacaccctgatgatctcccggacacccgaagtgacatgcgtggtggtcgacgtgtctcaggaagatcctgaggtgcagttcaactggtacgtggacggcgtcgaggtgcacaacgccaagaccaagcctagagaagaacagttcaactccacctacagagtggtgtccgtgctggctgttctgcatcaggactggctaaacggcaaggaatacaagtgcaaggtgtccaacaagggcctgccttcttctatcgagaagaccatttccaaggctaagggccagcctcgcgaacctcaagtgtacaccctgcctccgtcccaagaggagatgaccaagaaccaggtgtccctgacctgtctggtgaaaggcttctacccttccgacatcgccgtggcctgggagtccaacggccagcctgagaacaattataaaaccacccctcccgtgctggactctgatggctccttcttcctgtatagccggctgaccgtggataagtccagatggcaagagggcaacgtcttcagctgtagcgtgatgcacgaggccctgcacgcccactacacccagaagtccctgtccctgtccctgggcaag

SEQ ID NO: 232 - DNA, 1785 bp, synthetic construct
  misc_feature 1..1785: note = Artificial
  source 1..1785: mol_type = other DNA
atgggttggagttgcatcatcctatttctagtggccaccgctacaggcgtccactccgtgatccacgtgaccaaagaagtgaaagaggtggccaccctgtcctgtggccataatgtgtccgtggaagagctcgctcagaccagaatctactggcagaaagagaagaagatggtgctgaccatgatgtccggcgacgccaacatctggcctgagtacaagaatcggaccattttcgacatcaccaacaacctgtcgatcgtgtggctggaactgagaccctctgacgagggcacctacgagtgcctggtgctgaagtacgaaaaggatgccttcaagcgcgagcacctggctgaggtgacactgtctgtgaaggccgacggcggtggcggatctggcggcggcggcagcggcggcggcggatctggcggcggaggctctggcgaggtgcagctgctggaatccggcgggggcctggtgcagcctggcggctccctgcggctgtcttgcgccgcctctggctttaccttcagctcttacgccatgtcttgggtgcggcaggccccaggaaagggcctggaatgggtctctggcatctccggctctggaggcttcacctattacgctgatagcgtgaagggcagattcaccatcagccgggacaacagcaagaacaccctgtacctgcagatgaacagcctgagagccgaggacaccgctgtgtactactgtgccaagccccctagaggctacaattacggacctttcgactactggggccagggcaccctggtcacagtttcctccgcttctaccaagggcccgtccgtgttccctctggctccttgctcccggagtacctccgagtccaccgccgctctgggctgcctggtgaaggactacttccccgaacctgtgaccgtgtcctggaacagcggcgctctgacctctggcgtgcatacttttcctgctgtgctgcagtcttctggcctgtattctctgtcttccgtcgtgacagtgcctagttcctctctgggaaccaagacctacacctgcaacgtggaccacaagccctccaacaccaaagtggataagagggtggagtctaagtacggccctccttgccctccatgtcctgcccctgagttcctgggcggcccttctgtgttcctgttccctcccaagcctaaggataccctgatgatctctcggacacccgaggtgacctgcgtggtggtggacgtgtcccaagaggatcctgaagtgcagttcaactggtacgtggacggagtggaagtgcacaacgccaaaaccaagcctcgggaggaacagttcaactccacctacagagtcgtttctgtcctggccgtgctgcaccaggactggctgaacggcaaggagtacaagtgcaaggtgtccaacaagggcctgccaagctcaatcgagaaaacaatctccaaggctaaaggccagcctagagagcctcaggtgtacaccttaccaccttctcaggaggagatgaccaagaaccaggtgtccctcacctgtctggtcaagggcttctacccttccgacatcgccgtggcttgggagtccaatggacaacctgagaacaactataagacaacccctcccgtgctggactcggatggttccttctttctgtactccagactgaccgtggacaagtctagatggcaagaaggcaacgtgttctcctgctctgtgatgcacgaggccctgcacgcccactacacccagaagtccctgtccctgtccctgggcaag

SEQ ID NO: 233 - DNA, 1785 bp, synthetic construct
  misc_feature 1..1785: note = Artificial
  source 1..1785: mol_type = other DNA
atgggttggagttgcatcatcctatttctagtggctacagccaccggcgtgcactccgtgatccacgtgaccaaagaagtgaaagaggttgctaccttgtcctgcggccacaacgtttccgtggaagagctggcccagaccagaatctactggcagaaagagaagaagatggtgctgaccatgatgtctggcgacgccaacatctggcctgaatacaagaaccggaccatcttcgacatcaccaacaacctgagtattgtgtacctggaactgagaccttctgacgagggcacgtacgagtgtgtggtcctgaagtacgagaaggatgccttcaagcgggagcacctggctgaggtgaccctgtctgtgaaggccgatggaggcggcggctccggcggcggcggctccggaggaggcggctctggcggaggcggctctggcgaggtgcagctgctggaatcaggtggaggcctggtgcagcccggcggctccctgagactgtcttgtgccgcctctggctttaccttctcttcctacgccatgtcctgggtgcggcaggcccctggcaagggcctggagtgggtcagcggcatctccggctccggcggttttacctactacgctgactccgtgaaaggcagattcaccatctcccgggacaacagcaagaataccctgtacctgcagatgaactccctgagagccgaggataccgccgtgtactactgcgctaagcctcctagaggctacaactacggccctttcgactactggggccagggcaccctggtgactgttagttctgcttctaccaaggggccttctgtctttcctctggctccatgctctcggtccacatccgagtccaccgctgctctgggctgcctcgtgaaggactacttccctgagcctgtgaccgtgtcttggaactctggcgccctgacctctggcgtgcatacatttcctgccgtgctgcagtcctctggcctgtactccctgtcctccgtggtgaccgtgccctccagctccctgggaaccaagacctatacatgcaacgtggaccacaagcctagcaacaccaaagtggacaagcgggtggaatccaagtacggccccccttgccccccttgtcctgctcctgagttcctgggcggcccttctgtgttcctgttccctcctaagcccaaggacaccctgatgatctctagaacccctgaagtcacctgtgtggtggtggacgtgtcccaagaggatcccgaggtccagttcaactggtacgtggatggtgtggaagtgcataacgccaagaccaagcccagagaagaacagttcaactcaacatacagagtggtgtccgtgctggctgtgctgcaccaggactggctgaacggcaaggagtataagtgcaaggtgtccaataagggcctgccttcctccatcgagaaaaccatcagcaaggccaagggccagccccgcgagccccaagtgtacaccctgcctccatctcaggaggaaatgaccaagaaccaggtgtcgctgacatgcctggtcaaaggattctaccctagcgacatcgccgtggcttgggagtctaatggccagcctgagaacaactataagaccacacctccagtgctggactccgacggctctttcttcctgtacagccggctgaccgtggataagagcagatggcaagaaggcaacgtgttctcctgctccgtaatgcacgaggccctgcacgcccactacacccagaagtctctcagcctgagcttaggcaag

SEQ ID NO: 234 - DNA, 1785 bp, synthetic construct
  misc_feature 1..1785: note = Artificial
  source 1..1785: mol_type = other DNA
atgggttggagttgcatcatcctatttctagtggctaccgccaccggcgtgcactccgtgatccacgtgacaaaagaagtcaaagaagtggctacactgtcttgcggccacaacgtgtccgtggaagagctggctcagaccagaatctactggcagaaagagaagaagatggtgctgaccatgatgtccggcgacgccaacatctggcctgaatataagaatcgcaccatcttcgatatcaccaacaatctgagcatcgtgtggctggaactgagaccttctgacgagggaacttatgagtgtgtggtgctgaagtacgagaaggatgccttcaagcgggagcacctggccgaggtcacactgagcgtgaaggccgacggcggcggcggatctggtggcggcggcagtggcggaggaggctccggtggcggcggcagcggcgaggtgcagctgctggaatccggcggcggcctcgtgcagcctggtggctctctgcggctgtcttgtgctgcctctggcttcaccttctcctcctacgccatgtcttgggttagacaggcccctggcaagggcctggagtgggtgtccggcatctccggctctggaggctttacctactacgctgactctgtgaaaggcaggttcaccatttcccgggacaactccaagaacaccctgtacctgcagatgaacagcctgagagccgaggacaccgctgtgtactactgcgccaagcctccccggggctacaactacggccccttcgactactggggccaaggcaccctggtgaccgtgtcgagcgcctccacaaaaggcccatccgtgttccctctggccccttgctcccggtctacctccgagtctacagctgctctgggctgcctggtgaaggactacttccccgaacctgtgaccgtgtcctggaactccggagctctgacctctggcgtgcacacctttcccgccgtgctgcagtcctccggtctgtactctctctcttctgtggtgacagtgccttccagttctctggggacaaaaacctatacatgcaacgtggaccacaagccctctaataccaaggtagataagagagtggaatccaagtacggccctccttgccccccttgtcctgctcctgagttcctgggcggcccctccgtctttctgttccctcctaagcccaaggacaccctgatgatctctcggacccctgaggtgacctgcgtggtcgtggacgtgtcccaagaagatcctgaggtccagttcaactggtacgtggacggcgtcgaagtgcataacgccaagaccaagccacgggaagagcagttcaactctacctacagagtggtgtctgtcctggccgtgctgcaccaggactggctgaacggcaaggaatacaagtgcaaggtgtccaacaagggcctgccttctagcatcgagaagaccatctccaaggccaaaggccagcctagagagcctcaggtgtacaccctgcctccatctcaggaggagatgaccaagaaccaggtttctctgacctgtctggtgaagggcttctaccctagcgacatcgccgtggcctgggagtccaacggccagcccgagaacaactacaagaccaccccacctgtgctggactccgatggctccttcttcctgtactccagactgaccgtggataagtccagatggcaagagggcaacgtgttctcctgctccgtgatgcacgaggccctgcatgctcactacacccagaagtctctgtccctgtccctgggaaag

SEQ ID NO: 235 - DNA, 1785 bp, synthetic construct
  misc_feature 1..1785: note = Artificial
  source 1..1785: mol_type = other DNA
atgggttggagttgcatcatcctatttctagtggctacagctaccggcgtgcactccgtgatccacgtgaccaaggaggtgaaagaggttgccactctctcctgcggccataacgtgtccgtggaggaactggcccagacccggatctattggcagaaagaaaagaagatggtgctcaccatgatgagcggcgacatgaacatctggcctgagtacaagaatcgcaccatcttcgacatcaccaacaacctgtctatcgtgtacctggagctgcggcctagcgacgagggaacctacgagtgcctggtcctgaagtacgagaaggacgccttcaagcgggagcacctggccgaggtgaccctgtctgtgaaggctgatggaggcggcggctccggcggcggcggctctggcggcggcggctccggaggcggtggcagtggcgaggtccagctgctggaatctggcggaggactggtgcagccaggcggatctctgagactgtcttgtgctgcttctgggttcaccttctcttcctacgctatgtcttgggttagacaggcccctggcaagggcctggaatgggtgtccggcatcagtggctctggcggcttcacctattacgccgacagcgtaaagggcagattcacaatctctcgggataactccaagaatacactgtacctgcagatgaactctctgagggctgaggacaccgctgtgtactactgcgccaagcctcctagaggctacaattacggccctttcgactactggggccagggcaccctggttaccgtgtccagcgcctctaccaagggaccatccgtgtttcctctggctccttgttctcggtccaccagcgagtctaccgccgccctgggctgcctggtgaaggattacttccccgagcccgtgaccgtgtcttggaactccggcgccctgacatccggcgtgcacacctttcctgccgtgctgcagtccagcggcctgtactccctgtccagcgtggtcacagtgccttcttccagcctgggcaccaagacctacacctgcaacgtggatcacaagccctccaacaccaaagtggacaagcgggtggaatccaagtacggccctccttgccctccttgtcctgctcctgaatttctggggggtccttctgtgttcctgtttcctcccaagcctaaggacaccctgatgatttccagaacccctgaagtgacctgcgtggtggttgacgtgtcccaagaggatcccgaagtgcagttcaattggtacgtggacggcgtggaagtccacaacgccaagaccaagcccagagaggaacagttcaactctacatacagagtggtctccgtgctggctgtgctgcaccaggactggctgaacggcaaagaatacaagtgcaaagtgtccaacaagggcctgccttccagcatcgagaaaaccatctccaaggccaaaggccagccaagagagcctcaggtgtataccctgcctccttctcaagaggagatgaccaagaaccaggtgtccctgacatgtctggtgaagggcttctacccctctgatatcgccgtggcctgggagtctaacggacagcccgagaacaactataagaccacacccccagtgctggactccgacggctccttcttcctgtactcccggctgactgtggacaagtctagatggcaagaaggcaacgtcttcagctgcagcgtgatgcacgaggccctgcatgcacactacacccagaagtccctgtctctgtccctgggcaag

SEQ ID NO: 236 - DNA, 1785 bp, synthetic construct
  misc_feature 1..1785: note = Artificial
  source 1..1785: mol_type = other DNA
atgggttggagttgcatcatcctatttctagtggccaccgctaccggcgtgcattccgtgatccacgtgaccaaggaagttaaagaagtggccaccctgtcttgcggccacaatgtgtccgtggaagagctggctcagaccagaatctactggcagaaagaaaagaagatggtgctgaccatgatgtcaggcgacatgaacatctggcctgaatacaagaatcggaccatcttcgacatcaccaacaacctctccatcgtgtggctggaattgcggcctagcgacgagggcacctacgagtgcctggtgctgaagtacgagaaggacgccttcaagagagagcacctggccgaggtcacactgtctgtgaaggctgatggaggcggcggctctggcggcggcggcagcggaggcggaggatcaggcggcggtggctccggcgaggtccagctgctggaatccggcggaggcctcgtgcagcccggcggctcactgagactgtcctgcgccgcttctggcttcaccttctcctcttacgccatgtcctgggtgcggcaggcccccggcaagggcctggagtgggtcagtggcatcagcggctccggtggctttacctactatgccgactctgtgaagggcagattcaccatttcccgggacaacagcaagaacacactgtacctgcagatgaactccctgagagccgaggacaccgccgtgtactactgcgctaagcctccaaggggctacaactacggacctttcgactactggggacagggcacactggtgaccgtgtcctccgcctccaccaaaggcccttctgtgttccctctggccccttgttccagatccacctccgagtctaccgctgctctgggatgtctggttaaagattacttccccgaacctgtcaccgtgtcttggaacagcggcgctctgacctctggggtgcacacctttcctgccgttctgcagtccagcggcctgtactccctgtccagcgtggttaccgtgccttcctcctctctgggcaccaagacctatacctgcaacgtggatcacaagccctccaacaccaaggtggacaagcgggtggagtccaagtacggcccaccttgccccccctgccctgctcctgagttcctgggcggcccttccgtgttcctgttcccacccaaacctaaggacacactgatgatctctcgcacacctgaggtgacctgtgtcgtggtggacgtgtctcaagaggatcctgaagtgcagttcaactggtacgtggacggcgtggaagtgcacaacgccaaaacaaagcctcgggaggaacaattcaactctacatacagagtggtgtctgtcctggctgtactgcaccaggactggctgaatggcaaagagtacaagtgcaaggtgtccaacaagggcctgccatcttccatcgagaagactatctccaaggccaagggccagcctagagagcctcaggtgtacaccctgcctccttcccaagaggagatgaccaagaaccaggtgtccctgacatgcctggtgaagggcttctacccctcggacatcgccgtggcctgggagtcgaacggccagcccgagaacaactacaagaccacccctcctgtgctggacagcgatgggtctttcttcctgtattccagactgaccgtggataagtctagatggcaggaaggcaacgtgttttcttgttctgtgatgcacgaggctctgcatgcccactacacccagaagtccttgtctctgagcctgggcaag

SEQ ID NO: 237 - DNA, 1785 bp, synthetic construct
  misc_feature 1..1785: note = Artificial
  source 1..1785: mol_type = other DNA
atgggttggagttgcatcatcctatttctagtggctaccgccaccggcgtgcattccgtgatccacgtgaccaaagaggtgaaagaggtagctacactgtcttgcggccacaatgtgtccgtggaagaactggcccagaccagaatctactggcagaaagaaaagaagatggtgctgaccatgatgtccggcgacatgaacatctggcctgagtacaagaaccggacaattttcgacatcaccaacaacctgtccatcgtgtacctggagctgcggccttccgacgagggtacctacgagtgcgtggtgctgaagtacgagaaggacgccttcaagagagagcacctggccgaggtgacactgtctgtcaaggctgacggcggcggcggcagtggcggaggcggctctggaggcgggggctctggaggaggcggctccggcgaggtgcagctgctggaatccggaggcggcctggtgcagcctggcggctccctgcggctgtcctgcgccgcctccggcttcaccttcagctcctacgccatgtcttgggtcagacaggcccctggcaaaggcctggaatgggtgtccggcatctccggcagtggcggatttacttactacgccgactctgtgaagggcagattcaccatctctcgggacaacagcaagaataccctgtacctgcagatgaactccctgagagccgaagataccgccgtgtactactgcgctaagccacctagaggctacaactacggccctttcgactactggggccagggcaccctggtcacggtctcctccgcttctaccaagggccccagcgtgtttcccctggctccttgctcccgcagcacctccgagtccaccgctgccctgggctgcctagtgaaggattacttccctgagcccgtgacagtgtcctggaactctggcgccctgacctctggcgtgcacacctttcccgctgtcctgcagtcctccggactgtactctctgagctctgttgtgaccgtgccttctagcagcctgggaactaagacctacacctgcaacgtggaccacaagccttccaacaccaaagtggataagcgggtggaatctaagtatggccctccttgtccaccttgtcctgcccctgagttcctgggtggcccatctgtctttctgttcccccctaagcctaaggacaccctgatgatcagccggacccctgaggtgacctgtgtggtggtggatgtgtctcaagaggaccctgaagtgcagttcaactggtacgtggacggagtggaagtgcacaacgccaagacaaagcccagagaagagcagttcaattccacctatagggtggtttcggtgctggctgtgttgcatcaggactggctgaacggcaaggaatacaagtgcaaggtgtctaacaagggcctgcctagctctatcgagaaaaccatctccaaggccaagggtcagcctcgggagcctcaagtctataccctgccaccatctcaggaagagatgacaaagaaccaggtgtccctgacctgcctggtgaagggcttctacccctctgatatcgccgtggcctgggagtccaacggccagcccgagaacaactacaaaaccaccccacctgtgctggactccgatggctccttcttcctgtactccagactcaccgtggacaagtccagatggcaagagggcaacgtgttctcctgttctgtcatgcacgaggctctgcacgcccactacacccagaagtctctcagtctttccctgggcaag

SEQ ID NO: 238 - DNA, 1785 bp, synthetic construct
  misc_feature 1..1785: note = Artificial
  source 1..1785: mol_type = other DNA
atgggttggagttgcatcatcctatttctagtggccacggctaccggcgtgcactccgtgatccacgtgaccaaggaagtgaaagaggtggctacactgtcctgcggccacaatgtgtccgtggaagaactggctcagaccagaatctactggcagaaagaaaagaagatggtgctgaccatgatgtccggcgacatgaacatctggcctgagtacaagaaccggaccatcttcgatatcaccaacaacctgtccatcgtgtggctggagctgagaccttctgacgagggcacctacgagtgcgtggtgctgaagtacgagaaggatgccttcaaacgggagcacctggccgaagtgacactgtctgtgaaggccgatggcggcggcggcagcggcggcggaggatctggcggcggaggctccggcggaggaggctctggcgaggtgcagctgctggaatctggcgggggcctggtgcagcccggcggctctctgcggctgtcctgtgccgcttctggcttcaccttctcctcctacgccatgtcctgggtgcggcaggcccctggcaagggcctggaatgggtctctggcatcagcggctccggcggctttacctactacgccgacagtgtgaagggcagattcaccatctctcgggacaactccaagaacaccctgtacctgcagatgaactccctcagagccgaggataccgccgtgtactactgcgccaagccccctagaggctacaactatggccctttcgactactggggccagggcacactggtcaccgtgtcctctgcctctacaaagggccccagcgtgttccctctggctccttgctctagatccacctccgagtctacagctgctctgggctgcctggtcaaggactacttccccgagcccgtgaccgtgtcttggaactctggcgctctgacctctggggtgcataccttcccagctgtgctgcagtccagcggactgtactccctgtccagcgtggtgaccgtgccctcctcttctctgggcactaaaacctatacctgcaacgtggaccacaagccttccaataccaaggtggacaagcgggtggaaagcaagtacggcccaccttgccctccttgtcctgctcccgagttcttgggcggtcctagcgtatttctgtttcctcctaaacctaaggacaccctgatgatcagcagaacccctgaggtcacctgtgtagtcgtggacgtgtctcaagaggaccctgaggtgcagttcaactggtacgtggacggcgtggaagtgcataacgccaagaccaagcctagagaagagcagttcaactccacctacagagtggtttccgtgctggctgtgctgcaccaggactggctgaacggcaaagagtacaaatgcaaggtttccaacaagggactgccctcatctatcgagaagaccatttcgaaggccaagggccagcctagggagcctcaggtgtacaccctgcctccaagccaagaagagatgaccaagaaccaggtgtccctgacctgtctggtgaagggattctacccttctgacatcgccgtggcctgggagtccaatggccagcctgagaacaactacaagaccacacctcctgtgctggactccgatggctccttcttcctgtattcgagactgacagtggataagtcccggtggcaagaaggcaacgtgttctcttgctccgtgatgcacgaggccctgcacgctcactacacccagaagagcctgtccctgtctctcggcaag

SEQ ID NO: 239 - DNA, 1785 bp, synthetic construct
  misc_feature 1..1785: note = Artificial
  source 1..1785: mol_type = other DNA
atgggttggagttgcatcatcctatttctagtagccaccgccaccggcgtgcactccgtcatccacgtgaccaaagaagtgaaagaggtggctacactgtcttgtggctggaatgtgtctgtggaagagctgatgcagacccggatctactggcagaaagagaagaagatggtgctgaccatgatgtccggagacatgaacatctggcctgagtataagaaccggaccattttcgacatcaccaacaacctctccatcgtgatcctggagctgcggccttctgacgagggcacctacgagtgcgtcgtgaacaagtacgagaaggacgccttcaagagggagcatctggccgaggtgaccctgtctgtgaaggctgatggcggcggaggctccggcggcggaggcagtggcggcggcggctccggagggggcggatctggcgaggtgcagctgctggaatccggcgggggcttggtgcagcccggcggctctctgagactgagctgcgctgcttctggcttcaccttttcttcctacgccatgtcttgggtgcggcaggcccctggcaagggcctggagtgggtctctggcatctctggcagcggcggatttacatattacgccgactctgtcaagggcagattcacaatctctcgggacaactccaagaacaccctgtacctgcagatgaattccctgagagctgaggataccgctgtgtactactgcgccaagcctcctagaggctacaactacggccctttcgattactggggacagggtaccctggtgacagtgtcctccgcctccaccaagggccccagcgtgtttcctctggctccatgctcccgctctacctccgagtccaccgccgccctgggctgcctggtgaaggactacttccccgaacctgttaccgtgtcctggaacagtggcgctctgacatctggcgtgcataccttcccagccgtgctgcagtcctctggactgtactccctgagctccgtggtgaccgtgccctccagcagcctgggcacaaagacctatacctgcaacgtggatcacaagccttctaataccaaagtggacaagcgggtggaatctaagtacggccctccttgtcctccttgccctgctccagagttcctcggcggcccctctgtgttcctgttccctcccaagcctaaggacaccctgatgatctccagaacccctgaagtgacctgcgtggtcgtggacgtgtcgcaagaggaccccgaagtgcagttcaactggtacgtggacggcgtcgaagtgcacaacgccaagaccaagcccagagaagagcagttcaactccacctacagagtggtgtccgtgctggccgtgctgcaccaggactggctgaacggcaaagagtacaagtgcaaggtgtccaacaagggcctgccatctagcatcgagaaaaccatctccaaggctaaaggccagcctagagagcctcaggtgtacaccctgcctccatctcaagaggagatgaccaagaaccaggtgtccctcacctgtctggtgaagggcttctacccttccgatatcgccgtggcctgggaaagcaatggtcagcctgagaacaactacaagaccacacctcctgtactggactccgacggctccttcttcctgtactctcggctgacagtcgataagtctagatggcaagaaggcaacgtgttctcgtgtagcgtgatgcacgaggctctgcacgcccactacacccagaagtccctgtccctgtccctgggcaag

SEQ ID NO: 240 - DNA, 1785 bp, synthetic construct
  misc_feature 1..1785: note = Artificial
  source 1..1785: mol_type = other DNA
atgggttggagttgcatcatcctatttctagttgctaccgctaccggtgtgcattctgtgatccatgtgacaaaagaagtgaaagaagtggccaccctgtcctgcggctggaatgtgtccgtggaagagctgatgcagactagaatctactggcagaaagaaaagaagatggtgctgaccatgatgtctggcgacatgaacatctggcctgagtacaagaaccggacaatcttcgacatcaccaacaacctgtccatcgtgattctggaactgagaccttctgacgagggcacatatgagtgcgtggtcgataagtacgagaaggacgccttcaagagagagcacctggccgaggtgacactgtctgtgaaagccgacggcggcggcggctctggaggaggcggctccggaggcgggggctcaggcggagggggctctggcgaggtgcagctgctggaatccggaggcggcctggtgcaacctggcggctcactgcggctgtcttgtgctgcttctggctttaccttcagctcctacgccatgtcctgggtgcggcaggcccccggcaagggcctggagtgggtctccggcatcagcggatctggaggcttcacctactacgccgatagcgttaaaggcagattcaccatctcccgggacaactccaagaataccctgtacctgcagatgaactccctgagagccgaggacaccgccgtgtactactgcgccaagccacctagaggctacaactacggccctttcgactactggggacagggcaccctggtcaccgtgtcctccgcctctaccaagggcccttccgtgtttccacttgccccttgctctcggtccacttccgagagcaccgctgctctgggctgcctggtgaaggactacttccccgaacccgtgaccgtgtcttggaatagcggcgctctgacatctggcgtgcacacctttcctgctgtcctccagagctctggcctgtactctctgtcctccgtggtgaccgtgccttcctcctctttaggcaccaagacctatacctgcaacgtggaccacaagccatccaacaccaaggtggacaagcgggtggaaagcaagtacggccccccatgtcctccttgccctgcccctgagttcctgggcggcccttcggtttttctcttccctcctaagcccaaggataccctgatgatctcaagaacccctgaagtgacctgtgtggtggtggacgtgtctcaggaggatcctgaagtgcagttcaactggtacgtggatggtgtggaagtgcacaacgccaagaccaaacctcgggaggagcagttcaactccacctatagagtggtctctgtgctggctgtgctgcaccaggactggctgaacggcaaagagtacaagtgcaaggtctccaacaagggactgccttcatccatcgagaagaccatctccaaggctaagggccagcctcgcgagcctcaggtgtacacattgccccccagccaagaagagatgaccaagaaccaggtgtccctgacctgtctggtgaagggcttctaccccagcgatatcgccgtagcttgggagtccaacggccaacctgagaacaactacaaaaccacacctcctgtgctggactccgacggctccttcttcctgtactccagactgaccgtcgacaagagcagatggcaggaaggcaacgtgttctcttgctccgtgatgcacgaggccctgcacgcccactacacccagaagtccctgtctctgtctctgggcaag

SEQ ID NO: 241 - DNA, 1785 bp, synthetic construct
  misc_feature 1..1785: note = Artificial
  source 1..1785: mol_type = other DNA
atgggttggagttgcatcatcctatttctagtcgctacagctaccggcgtccactccgtgatccacgtgaccaaggaagtgaaagaagtggccaccctctcctgcggctggaacgtgtctgtggaggaactgtgccagaccagaatctactggcagaaagaaaagaagatggtgctgaccatgatgtccggcgacatgaacatctggcctgaatacaagaatcggacaatcttcgacatcaccaacaacctctccatcgtgatcctggagctgagaccctccgacgagggcacctacgagtgcgtggtgaacaagtacgagaaggacgccttcaagcgcgagcatctggccgaggtgactctgtcggtgaaggccgacggcggaggaggaagcgggggcggcggctctggcggcggaggctccggcggcggcggctctggcgaggtgcagctcctggaatctggcggcggcctggtccagcctggcggctctctgaggctgtcctgtgctgcctctggctttaccttctcctcgtacgccatgtcttgggtgcggcaggctcctggaaagggcctggagtgggtctcaggcatctccggctctggcggcttcacctactacgccgactccgtgaagggcagattcaccatcagccgggacaactccaagaacacactgtacctgcagatgaacagcctgagagctgaggatacagctgtgtattactgcgccaagcctccaagaggctacaactatggcccattcgactactggggccagggcaccctggtgaccgtgtcctctgcttccaccaaaggaccttccgtgttccctctggccccttgctctcggtccacctctgagtctaccgctgctctgggctgcttggttaaagactacttccctgagcccgtgaccgtgtcctggaattccggcgctctgacctctggtgtccatacctttcctgccgtcctgcagagctctggtctgtactccctgtcctctgtggtgaccgtccctagctcatctctgggaacaaagacgtatacctgcaacgtggaccacaagccttccaacaccaaggtggacaagagagtggaatccaagtacggccctccttgtcctccttgtcccgccccagaattcctcggcggaccttctgtgtttctgttcccccccaagcctaaggacacactgatgatctccagaaccccagaagttacatgtgtggtcgtcgacgtgtctcaagaggaccccgaggtgcagttcaactggtacgtggatggcgtggaagtgcacaacgccaagaccaagcctagagaagagcagtttaactccacatacagagtggtgtccgtgctggctgtgctgcaccaggactggctgaacggcaaagagtacaagtgcaaggtgagcaacaagggcctgcccagctctatcgagaagaccattagcaaggccaaaggacagcctcgggagcctcaggtgtacaccctgcctccgtcccaagaggagatgaccaagaaccaggtgtctctgacctgcctggtgaaaggcttctacccttccgatatcgccgtggcctgggagtccaacggccagcccgagaacaactacaagaccacccctcctgtgctggattctgatggcagcttcttcctgtactcccggctgaccgtggataagtccagatggcaagaaggcaatgtgttctcctgctctgtgatgcacgaggccctgcacgcccactacacccagaagtccctgagtttgtctctggggaag

SEQ ID NO: 242 - DNA, 1785 bp, synthetic construct
  misc_feature 1..1785: note = Artificial
  source 1..1785: mol_type = other DNA
atgggttggagttgcatcatcctatttctagtggctaccgctacaggcgtgcattccgtgatccacgtgaccaaggaagtcaaggaagtggctacgctgtcctgcggctggaatgtgtctgtggaagagctgtgccagaccagaatctactggcagaaagagaagaagatggtgctgaccatgatgtccggcgacatgaacatctggcctgagtacaaaaaccggaccatcttcgacatcaccaacaacctgtctatcgtgatcctggaactgcggccttccgacgagggcacctatgagtgcgtggtggacaagtatgagaaggatgccttcaagcgggagcacctggctgaggtgacactgtctgtgaaagccgatggcggaggaggctccggcggaggcggatccgggggaggcggatctggcggcggcggatctggcgaggtgcagctgctggaaagcggaggcggcctggtgcagcctggcggcagtctgagactgtcttgtgccgcctccggctttaccttctcttcgtacgctatgtcttgggtgcggcaggcccctggcaagggcctggaatgggtctccggcatctccggctcaggcggcttcacctactacgccgactctgtgaaaggcagattcaccatttcccgggacaactccaagaacaccttgtacctgcagatgaacagcctgagagccgaggataccgccgtgtactactgcgccaagcctcccaggggctacaactacggccctttcgactactggggccagggcacactggtcacagtcagctccgcctctaccaagggccccagcgtgttccctctggctccttgttctagatccacctccgagtctaccgctgccctgggctgcctggtgaaggactacttccccgagcccgtgaccgtgtcctggaactctggcgccctgactagcggagtgcatacctttcctgctgtgctgcagtcgtccggcctgtactctctgagctccgtggtgaccgtgccttcttcttctctggggaccaaaacctacacctgcaacgtggaccacaagccttctaatactaaggtggataagagagtggaatccaagtatggccctccttgcccaccatgtcctgcccctgagttcctgggcggccctagcgtgtttctgtttccacccaagcctaaggacacactgatgatctccagaacccctgaagtgacctgcgtggtcgtggacgtgtctcaagaggaccctgaggttcagttcaactggtacgtggacggcgtggaggtgcacaacgccaagaccaagcctcgggaagaacagttcaacagtacctaccgcgtggtatccgtgctggctgtgctgcaccaggactggctgaacggcaaagagtacaagtgcaaggtctccaacaagggccttccctcctccatcgagaaaaccatctccaaggctaagggccagcctagagagcctcaggtgtacaccctgcctccttctcaagaggaaatgaccaagaaccaggttagcctgacatgtctggtgaagggcttctacccctctgatatcgccgtggcctgggagtctaatggccagcccgagaacaactacaagaccacaccacctgtgctggacagcgatggctccttcttcctgtactccagactgaccgtggacaagtctagatggcaagaaggcaacgtgttctcctgctccgtgatgcacgaggccctccacgctcactacacccagaagtccctgtccctgtccttgggcaag

SEQ ID NO: 243 - DNA, 1785 bp, synthetic construct
  misc_feature 1..1785: note = Artificial
  source 1..1785: mol_type = other DNA
atgggttggagttgcatcatcctatttctagtggctacagccaccggcgtgcactctgtgatccacgtgaccaaagaggtgaaagaggtggctaccctgtcctgcggccataatgtgtccgtggaagagctgatgcagacccggatctactggcagaaagaaaagaagatggtgctgaccatgatgtctggcgacatgaacatctggcctgagtacaagaaccgcacaatcttcgatatcaccaacaacctgtccatcgtgatcctggaactgcggccttctgacgagggcacctacgagtgcgtggtgaacaaatacgagaaggatgccttcaaacgggagcacctggctgaggtgaccctgtctgtgaaggccgacggtggcggaggctctggcggcggcggatccggcggcggcggatctggcggaggaggttctggcgaggtccagctgctggaatctggcggcggcctggtgcagcctggcggcagccttcggctgtcttgtgccgcttctggcttcaccttctcctcctacgccatgtcctgggtgcggcaggcccctggcaagggcctggagtgggtgtctggcatcagcggctccggcggctttacctactacgctgattccgtcaagggcagattcacaatttcccgggacaactccaagaacaccctgtacctgcagatgaattctctgagagccgaggataccgctgtctactactgcgccaagcctcctagaggctacaactacggccctttcgactactggggccagggcacactggtcaccgtgtcctccgcctctacaaaaggcccctctgtgttccctctggccccatgctccagatccaccagcgagtctaccgccgccctgggctgcctggtgaaggactactttcccgaacctgtgaccgtgtcttggaattctggggctctgacatccggagtgcacacctttcctgctgtgctgcagtcctctggactgtacagcctgagctctgtcgtgacagtcccttccagctccctgggcaccaagacctatacctgcaacgtggaccacaagcctagcaacactaaagtggacaagagagtggaatccaagtacggacccccttgtcctccttgccctgctcctgagttcctgggcggcccgtctgtgtttctgttcccacccaagcctaaggacaccctgatgatctccagaacacctgaagtgacctgtgtggtcgttgacgtgtcccaagaggaccctgaagtgcagttcaactggtacgtggatggcgtagaagtgcataacgccaagaccaagcccagagaagaacagttcaactccacctacagggtggtgtccgtgctggcagtgctgcaccaggactggctaaacggcaaggagtacaagtgcaaggtgtccaacaagggcctgccctcttccatcgagaagaccatctctaaggctaaggggcagcctagagagcctcaggtgtacaccctgcctccatcccaagaggagatgaccaagaaccaggtgagcctgacctgtctggtgaagggcttctatcctagcgatatcgccgtggcctgggagtccaatggccagcccgagaacaactataaaaccacccctccagtgctggactccgacggctccttcttcctgtactctaggctgaccgtggacaagtctagatggcaagaaggcaacgtgttctcttgctccgtgatgcacgaggccctgcacgcccactacacccagaagtccctcagcttgtccctgggaaag

SEQ ID NO: 244 - DNA, 1785 bp, synthetic construct
  misc_feature 1..1785: note = Artificial
  source 1..1785: mol_type = other DNA
atgggttggagttgcatcatcctatttctagtggctaccgccaccggcgtgcattccgtgatccacgtgaccaaagaggtgaaagaagtggccaccctgtcctgcggccacaatgtgtccgtggaagagctgatgcagaccagaatctactggcagaaggagaagaaaatggtgctgaccatgatgtctggcgacatgaacatctggcctgagtacaagaaccggaccatcttcgatatcaccaacaacctgtccatcgtgatcctggagctgagaccttctgacgagggcacctacgaatgcgtggtggataagtacgaaaaggacgccttcaagcgggagcacctggccgaggtgaccctgtctgtgaaggccgacggcggaggcggctctggaggtggtggcagcggcggcggaggctccggcggcggcggctctggcgaggtgcagctgctggaatctggcggcggactggtgcagcctggcggctccctcagactgtcttgtgctgcctcgggcttcacctttagctcctacgccatgtcctgggtgcggcaggccccaggcaagggactggagtgggtctccggcatctctggctccggcggatttacctactacgccgattctgtgaagggcagattcacaattagccgggacaactccaagaataccctgtacctccagatgaactctctgcgggctgaggacaccgccgtgtactactgcgccaagccccccagaggctacaactacggccctttcgactactggggccagggcacgctggtgaccgtgagctccgcctctaccaagggacctagcgtgtttcctctggctccctgctcccggtccacctccgagtctaccgctgctctgggctgcctggtgaaggactacttccccgaacctgtgaccgtgtcttggaactccggcgctttgacctctggcgtgcacaccttccctgctgtgctgcagtcctctggcctgtattctctgtcctctgtggtgaccgtgcctagcagctccctcggcaccaaaacctacacctgcaacgtggaccacaagccctctaacaccaaagtggacaagagagtggaaagcaagtacggcccaccttgccctccttgtcctgcccctgagttcctgggcggcccatctgtctttctgttcccacctaagcccaaggacacactgatgatctccagaacacctgaggtcacctgcgtcgtcgtggatgtgtctcaggaagatcctgaagttcagttcaactggtacgtggacggcgtcgaggtgcacaacgccaagacaaagcctagagaggaacagttcaatagcacctacagagtggtctccgtgctggccgtgctgcaccaggactggctgaacggaaaagagtataagtgcaaggtgtccaacaagggcctgccttcttctatcgagaagaccatctccaaggctaagggccagcctcgcgagcctcaagtgtacacactgcctccttcccaagaagagatgaccaagaaccaggtgtctctgacatgtctggttaagggcttctacccctcggacatcgccgtggcttgggagtccaacggccaacccgagaacaactacaagaccacccctcccgtgctggactccgatggctccttcttcctgtactctcggctgacagtggacaagtccagatggcaggaaggcaacgtgttctcctgtagcgtgatgcacgaggccctgcatgctcactacacacagaaaagcctgtccctatccctgggcaaa

SEQ ID NO: 245 - DNA, 1785 bp, synthetic construct
  misc_feature 1..1785: note = Artificial
  source 1..1785: mol_type = other DNA
atgggttggagttgcatcatcctatttctagtggccacagctaccggcgtgcactccgtgatccacgtgaccaaagaggtgaaggaggttgccaccctgtcttgtggccacaacgtgtccgtggaggaactgtgccagacacggatctactggcagaaagaaaagaagatggtgctgaccatgatgtccggcgacatgaacatctggcctgagtacaagaacagaaccatcttcgacatcaccaacaacctgtccatcgtgatcctggaacttagaccttccgacgagggaacctacgagtgcgtcgtggacaagtacgagaaggatgccttcaagagagagcacctggccgaggtgacgctatccgtcaaggccgatggcggcggcggctccggcggcggcggcagcggcggcggaggatccggcggcggcggttctggcgaggtgcagctgctggagtctggcggcggcctggttcagcctgggggcagcctgcggctgtcctgtgccgcttccggcttcaccttctcctcttacgccatgtcgtgggtgcggcaggcccctggcaaaggtctggaatgggtctccggcatctcgggctccggaggctttacctactatgccgactctgtgaagggcagattcaccatcagccgcgacaactccaaaaataccctgtacctgcagatgaactctctgagagctgaggacaccgccgtgtactactgcgccaagcctcctagaggttacaactacggacctttcgattattggggacagggcaccctggtgaccgtgtcctccgcctctaccaaaggccccagcgtgttcccactggctccctgctctcggtctacatccgagtccaccgctgccctgggctgcctggtgaaagactacttccccgagcctgtgaccgtgtcttggaacagcggcgctctgacctctggagtgcacacctttcctgccgtgctgcaaagcagtggcctgtactctctctctagcgttgtgacagtgccttcttcctccctgggcaccaagacctatacctgcaacgtggaccacaagccatccaacactaaggtggacaagagagtggagtccaagtacggccctccttgccctccttgtcctgctcctgagttcctgggcggcccttccgtgttcctgttccctcccaagcctaaggacaccctgatgatctcccggacccctgaagttacatgcgtggtcgtggatgtgtctcaggaggatcccgaagtgcagttcaactggtacgtggacggcgtggaagtgcataacgctaaaaccaaacccagagaggaacagtttaattctacctacagagtggtgtccgtgctggctgtgctccaccaggactggctgaacggcaaggaatacaagtgcaaggtgtccaacaagggcctgcccagctccatcgagaagaccatttctaaggccaagggccagcctcgggaaccgcaagtctacacactgcctccttcccaggaagagatgaccaagaaccaggtgtctctgacctgtctggtgaagggcttctacccttctgacatcgccgtggcctgggagagtaatggccagccagagaacaactataagaccacacccccagtgctggactctgacggatctttcttcctgtactccaggctgaccgtggataagtctagatggcaagagggcaacgtcttctcttgctccgtgatgcacgaggctctgcatgctcactacacccagaagtccctgtctctgagcctgggcaag

SEQ ID NO: 246 - DNA, 1785 bp, synthetic construct
  misc_feature 1..1785: note = Artificial
  source 1..1785: mol_type = other DNA
atgggttggagttgcatcatcctatttctagtggccaccgccaccggcgttcactctgtcatccacgtgaccaaagaggtgaaagaagtggctaccttgtcttgcggccataacgtcagcgtggaagagctgtgccagaccagaatctactggcagaaagagaagaagatggtgctgaccatgatgagcggggacatgaacatctggcccgagtacaagaaccggaccatcttcgacatcaccaacaacctgtccatcgtgatcctggaactgagaccttccgacgagggcacctacgagtgcgtggtgaacaagtacgagaaggatgccttcaagcgcgagcacctggccgaagtgaccctgtctgtgaaggccgacggcggcggtggcagcggaggaggcggctccggcggcggcggttctggcggcggcggatctggcgaggtgcagctgctggaatctggaggcggcctggtccagcctggaggctctctgcggctgtcctgtgccgcttccggcttcaccttctcctcctacgctatgtcttgggtgcggcaggcccctggcaagggcctggaatgggtctctggcatctccggcagcggcggctttacctactacgccgactccgtgaagggcagattcaccatctcccgggacaactccaagaacaccctgtacctgcagatgaactccctgagagccgaggacaccgctgtgtactactgcgccaagcctcctagaggctacaactatggcccattcgactactggggccaaggaactctggtgaccgtgagctccgcttctacaaaaggcccctccgtgttccctctggcaccttgctctcggagtacctccgagtccaccgccgccctgggctgcctggtcaaggactacttccctgaacccgttaccgtgtcctggaactctggcgctctgacctctggcgtgcacacctttcctgctgtgctgcagtcctctggcctgtactccttgtcttccgtggtgacagtgccttccagtagcctgggcaccaagacctacacctgcaatgtggaccacaaaccttccaatacaaaagtggacaagagagtggaaagcaagtacggccctccttgccctccttgtcctgctccagagttcctgggcggacctagcgtgtttctgttcccccccaagcctaaggacaccctgatgatctctagaacccctgaggtgacctgtgtggtcgtggacgtgagtcaagaggatcctgaggtgcagttcaactggtacgtggatggcgtggaagtgcacaacgccaagaccaagccccgggaagagcagtttaactctacctacagagtggtgtctgtgctggccgtgctgcaccaggattggctgaacggcaaggagtacaagtgcaaggtctccaacaagggcctcccatccagcatcgagaagacaatctccaaggctaaaggccagcctagagagcctcaggtgtatacactccctccctctcaagaggagatgaccaagaaccaggtctccctgacatgtctggtgaagggcttctacccttctgacattgccgtggcctgggagtctaatggccagcccgaaaacaactacaagacaaccccccctgtgctggactccgatggatccttcttcctgtactctagactgaccgtggataagtccaggtggcaggaaggcaacgtgttctcctgctccgtgatgcacgaggctctgcatgctcactacacccagaagtctctgagcctgtctctgggaaag

SEQ ID NO: 247 - DNA, 1785 bp, synthetic construct
  misc_feature 1..1785: note = Artificial
  source 1..1785: mol_type = other DNA
atgggttggagttgcatcatcctatttctagtcgctaccgctaccggcgtgcatagcgtgattcacgtgaccaaggaggtgaaagaggtggccacactgtcctgtggccataatgtgagcgtggaagaactggctcagacccggatctactggcagaaggaaaagaagatggtgctgaccatgatgtctggcgacatgaacatctggcctgagtacaagaacagaaccatcttcgacatcaccaacaacctgtccatcgtgctgctggagctgcggccttccgacgagggcacctacgagtgcctggtcctgaagtacgagaaggatgccttcaagcgggagcacctggctgaggtgactctgtctgtcaaagctgacggcggcggaggatccggcggcggcggctctggcggcggcggctctggcggcggcggctctggcgaggtgcagctgctggaatctgggggaggcctcgtgcagcctggcggatctctgagactgtcctgcgccgcctccggctttaccttctcctcctacgccatgtcctgggtgcggcaggcccccggcaagggactggagtgggtctcaggcatctccggcagcggaggcttcacctactacgccgactctgtgaaaggcagattcaccatctctcgggacaactccaagaacaccctgtacctgcagatgaacagcctgagagccgaggataccgcagtgtactactgcgctaagcctcctaggggctacaactacggccccttcgactattggggccagggcaccctagtgaccgtgtcctctgcctctaccaagggcccctctgtgtttcctctggccccttgtagccgcagtacctctgagtctaccgccgctctgggctgtctggtaaaggactacttcccagagcctgtgaccgtgtcttggaactccggcgctctgacctccggcgtgcacacctttcctgctgtgctgcagtccagcggtctgtacagcctcagttccgtcgtgacagtgccttcctcctccctgggaaccaagacctatacctgcaacgtggaccacaagcccagcaacaccaaagtggacaagagagtggaatccaagtacggccctccttgtccaccttgccccgctcctgagttcctcggcggcccctctgtgttcctgttcccccctaagcccaaggacaccctgatgatctccagaacacctgaagtgacctgcgtggtggtggatgtttctcaagaggacccagaggtgcagttcaactggtacgtggatggcgtcgaggtgcacaacgccaagaccaagcctagagaggaacaattcaattccacatacagagtggtctctgtgctggccgtgctgcaccaggactggctgaacggcaaagaatacaagtgcaaggtgtctaacaagggcctgccttcctctatcgagaagacaatctccaaggccaagggccagcctcgggaacctcaagtgtataccctgcctccatctcaggaagagatgacaaagaaccaggtgtcccttacatgcctggtgaagggattctacccttctgatatcgccgtggcctgggagtccaatggccagcccgagaacaactacaagaccacccctcctgtgctggactccgatggctccttcttcctgtactcccggctgaccgtggacaagtccagatggcaggaaggcaacgtgttcagctgctccgtgatgcacgaggccctgcacgcccactacacccagaaatctctgtccctgtcactgggcaag

SEQ ID NO: 248 - DNA, 1785 bp, synthetic construct
  misc_feature 1..1785: note = Artificial
  source 1..1785: mol_type = other DNA
atgggttggagttgcatcatcctatttctagtggccactgctaccggcgtgcactccgtgattcacgtgacaaaggaggtgaaagaagtggctacactgtcctgtggctggaacgtgtctgtggaagagctggtgcagaccagaatctactggcagaaaaataagaagatggtgctgaccatgatgtctggcgacatgaacatctggcctgaatacaagaaccggaccatctttgacatcaccaacaacctgtccatcgtgatcctggaactgcggcctagcgacgagggcacatatgagtgcgtggtgaataagtacgagaaggacgccttcaagcgggagcatctggccgaagtgaccctgtctgtcaaggccgacggcggcggcggctccggcggcggcggctctggaggaggcggcagcggcggcggaggatctggcgaggtccagctgctggaatccggcggcggcctcgtgcagcccggcggttctctgaggctgagctgcgctgcttctggcttcaccttctcctcctacgccatgtcctgggtgcggcaggcccctggcaaagggctggaatgggtctccggcatctccggctctggcggctttacctactacgccgattctgtgaagggcagattcacaatcagccgggacaactccaagaacaccctgtacctgcagatgaactctctgagagccgaggatactgccgtgtactattgcgccaagcctcctagaggctacaactacggccctttcgactactggggacagggcaccctggtgactgtttcttctgcctccaccaagggcccttccgtgttccctctggctccatgctctagaagcacctccgagtccaccgccgctctgggctgcctggtcaaagattacttccctgagcctgtgaccgtgtcttggaacagcggcgctctgacctctggcgtgcacacgtttcccgccgtgctgcagtcctcaggcctgtactccctcagctccgttgttacagtgccttcttcctccctcggcacaaagacctacacctgcaacgtggaccacaagcccagcaatacaaaagtggataagagagtggaatctaagtacggacctccttgccctccatgtcctgctcctgagttcctgggaggaccttctgtgtttctgttcccccccaaacctaaggacaccctgatgatctccagaacccccgaggtgacctgtgtggtcgtggacgtgtcccaggaggaccccgaggtccagttcaactggtacgtggatggcgtggaagtgcacaacgccaagaccaagcctagagaggaacagttcaattcaacctacagagtggtctccgtgcttgctgtgctgcaccaggactggctgaacggcaaagagtacaagtgcaaggtgtctaacaagggcctgccatccagcatcgagaagaccatcagcaaggctaagggccagccccgggaacctcaagtgtataccctgcctccttcccaagaggagatgaccaagaaccaggtgtctctgacctgtctggtgaagggcttctacccttctgatatcgccgtggcctgggagtccaacggccagcctgagaacaactacaagaccaccccccccgtgctggactccgacggctccttcttcctgtacagtcgcctgaccgtggacaagtctagatggcaagaaggcaacgtgttctcttgctccgtgatgcacgaggccctgcatgctcactacacccagaagtccctgtccctgtccctgggcaag

SEQ ID NO: 249 - DNA, 1785 bp, synthetic construct
  misc_feature 1..1785: note = Artificial
  source 1..1785: mol_type = other DNA
atgggttggagttgcatcatcctatttctagtggccaccgctaccggcgtgcactctgtgatccacgtgaccaaagaggtgaaagaagtggctaagctgtcttgtggccacaacgtcagcgtcgaggaactcgctcagacccggatctactggcagaaagaaaagaagatggtgctgacactgatgtccggcgaccacaacatctggcctgagtacaagaaccggacaatcttcgacatcaccaacaacctgtccatcgtgattctggaactgcggccatctgacgagggcacctacgagtgcgtggtcctgaagtacgagaaggacgccttcaagagagagcacctggccgaggtgaccctgtccgtgaaggccgacggcggaggaggctctggaggcggaggctctggcggaggaggctctggcggcggcggctccggcgaggtgcagctgctggagtccggtggcggcctggtgcagcccggcggaagcctgagactgtcctgtgctgcttctggcttcaccttctcttcctacgccatgtcttgggtccgccaggcgcctggcaagggcctggaatgggtgtctggcatcagcgggtccggcggctttacctactacgccgattctgtgaagggcagattcaccatctcccgggacaactccaagaataccctgtacctgcaaatgaacagcctcagagccgaggacaccgctgtgtactattgcgccaagccgccaagaggctacaactatggccctttcgattactggggccagggcaccctggttacagtgagctccgcctccaccaagggcccttccgtgtttcctctggctccttgctcccggtctacctctgagagcacagctgccctgggctgcctggtgaaggactacttccctgagcctgtgaccgtgtcctggaactccggcgctctgactagcggcgtgcacacctttcctgccgtgctgcagtcttctggcctgtactccctctcatccgtggtgaccgtgccttcatcttctctgggaacaaaaacctacacctgcaacgtggaccacaagccttctaacaccaaagtggataagcgcgtggaatctaagtacggccccccttgccctccttgtcctgctcctgagttccttggcggcccttccgtgttcctgttcccccccaagcctaaggataccctgatgatctccagaacacccgaggtcacatgtgtggttgtggacgtctcccaggaagatccagaggtgcagttcaactggtacgtggacggcgtggaagtgcataatgccaaaaccaagcccagagaggaacagtttaattccacctacagagtggtctcggttctggctgtgctccaccaggactggctgaacggaaaagagtacaagtgcaaggtgtccaacaagggactgcctagctccatcgagaagaccatctccaaggccaagggccagcccagggaacctcaggtttacaccctgcccccttcccaagaagagatgaccaagaaccaggtgtccctgacctgcctggtgaagggcttctacccttccgacatcgccgtggcctgggagagcaacggccaacctgagaacaactacaagaccacccctccagtgctggactccgatggctccttcttcctgtactctcggctgactgtggacaagtctagatggcaggaaggcaatgtgttctcttgctctgtgatgcatgaggccctgcacgcccactacacccagaagtccctgtctctgagcctgggcaaa

SEQ ID NO: 250 - DNA, 1785 bp, synthetic construct
  misc_feature 1..1785: note = Artificial
  source 1..1785: mol_type = other DNA
atgggttggagttgcatcatcctatttctagtggccaccgctaccggcgtgcatagcgtgatccacgtgaccaaggaagtgaaggaagtggctaagctgagttgcggccacaatgtgtccgtggaagaactggcccagaccagaatctactggcagaaagaaaagaagatggtgctgaccctgatgtctggcgaccagaacatctggcctgaatacaagaacagaactatctttgacatcaccaacaacctgtctatcgtgatcctggagctgcggccttcagatgaaggcacatacgagtgcgtggtgctgaagtacgagaaggacgcctttaagagagagcatctggctgaggtgacactcagcgtgaaggccgatggcggcggaggatctggcggcggcggcagcggcggaggcggctccggcggcggaggctccggcgaggtgcagctgctggaatctggcgggggactcgtgcagcctggcggctccctgagactgtcctgtgctgcctctggattcaccttctcttcctacgccatgtcctgggtcagacaggcccccggcaagggcctggaatgggtgtccggcatctccggatctggcggcttcacctactacgccgacagcgtcaagggcagattcaccatctctcgggacaactccaaaaacaccctgtacctgcagatgaactccctgagagccgaggataccgccgtgtactactgcgccaagccccctagaggctacaactacggccccttcgattactggggccaaggcaccctggtgaccgtgtcttccgcttctaccaagggcccttctgtgttccctctggctccttgctctcgctccacctccgagtccaccgccgctctgggctgcctggtgaaggactacttccccgagcctgtgacagtgtcttggaactccggcgctctgacctctggcgtgcacacctttcctgctgtgctgcagtccagcggcctgtattctctgagcagtgtggtcaccgtgcctagctctagcctgggcaccaaaacctacacctgcaacgtggaccacaagccttccaataccaaggtggataagcgggtggaatccaagtatggccccccttgtcctccttgccctgctcctgagttcctgggagggccttcggtgttcctgttccctcccaaacccaaggacaccctgatgatctcccggaccccagaagtgacctgtgtggtggtggacgtgtcccaagaggaccctgaggtgcagttcaactggtacgtggacggcgttgaagtgcacaacgccaaaacaaagcctcgggaagagcagttcaattctacatatcgggtcgtgtctgttctggccgtcctgcaccaggactggctgaacggcaaagagtacaagtgcaaggtctccaacaagggcctgccatcctccatcgagaagaccatttctaaggctaagggccagcctagagagcctcaggtgtacacactgcctccatcacaagaggagatgaccaagaaccaggtttctctgacctgtctggtgaaaggcttctacccctccgatatcgccgtggcctgggagtccaatggccagcccgagaacaactacaagaccacccctccagtactggactccgacggctccttcttcctgtactcccggctgacagtggacaagtctagatggcaggagggcaacgttttttcctgctccgtgatgcacgaggccctgcacgcccactacacccagaagtccctttctctgagcctgggcaaa

SEQ ID NO: 251 - DNA, 1785 bp, synthetic construct
  misc_feature 1..1785: note = Artificial
  source 1..1785: mol_type = other DNA
atgggttggagttgcatcatcctatttctagtggctaccgccaccggcgtgcattccgtgatccacgtgaccaaggaggtgaaagaggttgcaaagctgtcttgcggccataatgtgtccgtggaagaactggctcagaccagaatctactggcagaaggaaaaaaagatggtgctgaccctgatgtctggcgacatgaacatctggcctgagtacaagaaccggaccatctttgacatcaccaacaacctgtccatcgtgatcctggagctgcggcctagcgacgagggcacatacgagtgtgtggtgctgaagtacgagaaggatgccttcaagcgggaacacctggccgaagtgacgctgtccgtgaaggctgacggcggcggcggctctggcggcggaggctccggcggcggcggcagcggcggcggcggctctggcgaggtgcagctgctggaatccggtggcggcctggtgcagccaggaggatctctgagactgtcctgcgccgcttccggcttcaccttctcctcttacgccatgtcctgggtgcggcaggctcctggcaagggcctggaatgggtctccggcatctctggctctggcggctttacctactacgctgactccgtcaagggcagattcaccatctcccgggacaactctaagaacaccctctacctgcagatgaattccctgagagccgaggacacagccgtgtactactgcgctaaaccgcccagaggctacaactatggccctttcgactactggggacagggcaccctagtgacagtgtcttctgcctctacaaagggccccagcgtgttccctctggccccttgctccagatccacctctgagtctaccgctgctctgggctgtctggtgaaggactacttccccgagcctgtgaccgtgtcatggaactccggcgccctgacctccggcgtacacacctttcctgccgtgctgcagtcctccggactgtactccctgagctccgtcgtcaccgtgcctagttctagcctcggtacaaaaacctacacctgcaacgtggaccacaagccttctaacaccaaggtggacaagagagtggaatccaagtacggccctccatgtcctccttgtcctgctcccgagttcctgggaggacctagcgtgtttctgttcccaccaaagcccaaggacaccctgatgatctccagaacccctgaggtgacatgcgtggtggtcgacgtgtctcaggaggatcctgaagtgcagttcaactggtacgtggacggcgtggaagtgcacaacgccaagaccaagcctagagaggagcagttcaattccacctaccgggtggtgtccgtgctggctgttctgcaccaggattggctgaacggaaaagagtacaagtgcaaggtctccaacaagggcctgccctctagtatcgagaagaccattagcaaggccaaaggccagcccagggaaccacaagtgtatacactgcctcctagccaagaagagatgaccaagaaccaggtgtccctgacatgcctggtgaagggcttctacccctccgacatcgccgtggcctgggagtctaacggccagcctgagaacaactacaagaccacccctcctgtgctcgattccgatggatccttcttcctgtacagccggctgaccgtggataagtccagatggcaagagggcaacgtgttcagctgctctgtgatgcacgaggccctgcacgcccactacacccagaaatctctgagcctgtctctgggcaag

SEQ ID NO: 252 - DNA, 1785 bp, synthetic construct
  misc_feature 1..1785: note = Artificial
  source 1..1785: mol_type = other DNA
atgggttggagttgcatcatcctatttctagtggccaccgctaccggcgtgcattctgtgatccacgtgaccaaagaagtgaaggaggtggccaagctgagctgcggacataatgtgtccgtggaagagctggcccagaccagaatctactggcagaaagagaagaagatggtgctgaccacaatgtccggcgaccacaacatctggcctgagtacaagaaccggactatcttcgacatcaccaacaacctgtccatcgtgatcctggaactgcggccttccgacgagggaacatacgagtgcgtggtgctgaagtacgagaaagacgccttcaagagagagcacctggctgaagtgaccttatcagtgaaggctgacggcggaggcggctccggcggcggcggctctggcggaggtggctctggcggcggcggctccggcgaggtgcagctgctggaatccggcggcgggctggtgcagcctggaggatctttgagactgtcttgcgctgcttctggctttacattcagctcttacgccatgtcttgggtcaggcaggcccctggcaaaggcctggagtgggtgtctggcatctctggctccggcggctttacctactacgctgactccgtcaagggcagattcaccatctcccgggacaactccaaaaataccctgtacctgcagatgaactccctgagagccgaggacaccgccgtgtactactgcgccaagccccctagaggctacaactacggcccattcgactactggggccagggcaccctggtcaccgtgtcctccgcctctaccaagggcccttccgtgtttcctctggctccttgcagtcggtccacctccgagtctaccgccgctctgggctgcctggtgaaggattacttccccgagcccgtgaccgtgtcctggaacagcggcgctctgacaagtggagtgcacaccttccctgctgtgctgcagagctccggcctgtattccctgtcctctgtcgttaccgtgccctcctcctctctcggcaccaagacctatacctgcaacgtcgatcacaaaccttctaacaccaaagtggacaagcgggtggaatccaagtacggccctccttgtccaccttgtcctgctccagagttcctgggaggcccatctgtgtttctgttccctcctaagcctaaggacaccctgatgatcagccgcacacccgaagtgacatgtgtggtggtcgacgtgtctcaagaagatcctgaggtgcagttcaactggtatgtggatggcgtggaagtgcacaacgccaagacaaagcctcgggaagagcagttcaactctacatacagagtggttagcgtgctcgctgttctgcaccaggactggctgaacggcaaggagtacaagtgcaaggtgtccaacaagggcctgcccagctctatcgagaagaccatttccaaggccaagggacagcccagagagcctcaagtctacaccctgcctccatcccaggaagaaatgaccaagaaccaggtgtctctgacgtgtctggtgaagggcttctacccttctgatatcgccgtggcctgggagagcaatggccagcctgagaacaactacaagaccacccctcctgtgctagactctgatggatctttcttcctgtacagccggctgaccgtggacaagtccagatggcaagagggcaacgtgttctcctgctccgtgatgcacgaggccctgcacgcccactacacccagaagtctctgagcctctccctgggcaag

SEQ ID NO: 253 - DNA, 1785 bp, synthetic construct
  misc_feature 1..1785: note = Artificial
  source 1..1785: mol_type = other DNA
atgggttggagttgcatcatcctatttctagtggctaccgccaccggcgtgcactccgtgatccacgtgaccaaagaggtcaaggaggtggccaagctgtcctgcggccacaatgtgtctgtggaagagctggctcagaccagaatctactggcagaaagaaaaaaagatggtgctgacaaccatgtctggcgaccagaacatctggcctgagtacaagaacagaaccattttcgatatcaccaacaatctgtccatcgtgatcctggaactgcggccttctgacgagggcacatatgagtgcgtggtcctgaagtacgagaaggatgccttcaagagagaacacttggctgaggtgacactgtccgtcaaggccgacggcggcggaggcagcggtggcggcggctctggcggcggcggctctggaggaggcggatccggcgaagtgcagctgctagaatccggcggcggcctggtgcagcctggcggctctctgcggctgagctgcgccgcctctgggtttaccttctcctcctacgccatgtcctgggtgcggcaggcccctggcaaggggctggagtgggtctcaggcatcagcggaagcggcggcttcacctactacgctgattctgtgaaggggcggttcacaatctctcgcgacaactctaaaaacaccctgtacctgcagatgaactccctgcgggctgaggacaccgccgtgtactactgcgccaagcctcctagaggctacaactacggccctttcgattactggggccagggcacactggtcaccgtgagctctgcttccaccaagggcccatctgtgtttcctctggccccttgctccagatccacctccgaaagcaccgctgctctgggctgcctggtgaaggactacttccccgagccagtgaccgtgtcttggaactccggcgctctgacctctggagtgcacaccttccctgccgtgctgcagtccagcggactgtacagcctgtcatccgtggtcaccgtgccttcgtcctccctgggcacaaagacctacacctgcaacgtggatcacaagccctctaataccaaggtggacaagcgggtagaatccaaatacggccccccttgtcctccatgtcctgcacctgagtttctgggcggcccctctgtgtttctgttcccacctaagcccaaggacacactgatgatctctaggacacctgaagtgacctgtgtggtggtggacgtgtctcaagaagaccctgaggtgcagttcaactggtacgtggatggcgtggaagtgcataacgccaagaccaagcctagagaggagcagttcaattccacctatagagtggtgtctgttctcgctgtcctgcaccaggactggctgaacggaaaagagtataagtgcaaggtgtccaacaagggcctgccttccagcatcgagaaaaccatctcgaaggccaagggtcagcctagagagcctcaagtgtacaccctgcctccatctcaagaggagatgaccaagaaccaggtgtccttaacctgcctggtgaagggcttctacccctctgacatcgccgtggcctgggagtctaacggccagcccgagaacaactacaagaccacccctcccgtgctggactccgacggctccttcttcctgtactccagactcactgttgacaagtctagatggcaggaaggcaacgtgttcagttgttccgtgatgcacgaggccctgcatgctcactacacccagaagtccctgtccctgtccctcggcaag

SEQ ID NO: 254 - DNA, 1785 bp, synthetic construct
  misc_feature 1..1785: note = Artificial
  source 1..1785: mol_type = other DNA
atgggttggagttgcatcatcctatttctagtggctaccgccaccggcgtgcactccgtgatccacgtgaccaaagaagtgaaagaggtggccaagctgtcttgcggccataatgtgtctgttgaagagctggctcagactagaatctactggcagaaagagaagaagatggtcttgaccaccatgtctggcgacatgaacatctggcctgagtacaagaacagaaccatcttcgacatcaccaacaacctgtctatcgtgatcctggaactgagaccttctgacgagggaacatacgagtgtgtggtcctgaagtacgagaaagacgccttcaagcgggagcacctggctgaggtaaccctgagcgtgaaggctgatggcggcggcggcagcggcggcggtggctccggcggcggcggctccggcggaggcggctctggagaagtgcagctgctggaaagcggcggcggcctggtgcagcccggaggaagcttgcggctgtcctgtgctgcctctggcttcaccttctcttcctacgctatgtcttgggtgcggcaggcccctggcaagggactggaatgggtgtccggcatctctggatctggcggcttcacctactacgccgattccgtgaagggccggttcacaatctcccgggacaactctaagaatacactgtacctgcagatgaactccctcagagccgaggatacggctgtgtactattgcgccaagcctccaagaggctacaactacggccctttcgactactggggacagggcaccctggtcaccgtgtcctccgcctccaccaagggccccagcgtgtttcctctggccccctgctccagatctacctctgagtccacagctgctctgggctgcctggtgaaggattacttccccgaacccgtgaccgtgtcttggaactctggcgccctgacctccggcgtgcacacctttcccgccgtgctgcagtcctctggcctgtactctctgagctccgtggtcaccgtgcctagctcctctctgggcaccaaaacctacacctgcaacgtggaccacaagccatctaacaccaaggttgacaagagagtggaatccaagtatggacccccttgtcctccttgccctgctcctgagttcctggggggaccttccgtgttcctgttccctcctaagccgaaggacaccctgatgatttcccggacccctgaggtgacctgcgtggtcgtggacgtgtcccaggaggaccctgaagtgcagttcaactggtacgtggacggcgtggaagtgcataatgctaagacaaagcctagagaggaacagtttaactcgacctatcgcgtcgtgtctgtgctggcagtgctgcaccaggactggctgaacggcaaagagtacaagtgcaaggtgtccaacaagggcctgccctcctccatcgagaagaccatctccaaggccaaaggtcagcctagagagcctcaagtgtacacactgccacctagccaagaagagatgaccaagaaccaggtctctctgacctgtctggtgaagggcttctacccttccgatatcgccgtggcctgggagagcaacggccagccagagaacaactacaaaaccacccctcctgtgctggactccgacggctccttctttctgtacagcaggctgaccgtcgataagagcagatggcaggaaggcaacgtgttctcctgctccgtgatgcacgaggccctgcacgcccactacacccagaagtccctgtctctgtccctgggcaag

SEQ ID NO: 255 - DNA, 1785 bp, synthetic construct
  misc_feature 1..1785: note = Artificial
  source 1..1785: mol_type = other DNA
atgggttggagttgcatcatcctatttctagtggccaccgctacaggcgtgcatagcgtgatccacgtcacaaaagaagttaaagaggtggctaccctgtcctgcggccacaatgtgtcggtggaagagctggctcagacccggatctactggcagaaagagaagaagatggtgttgaccatgatgtctggcgaccataacatctggcctgagtacaagaacaggaccatcttcgacatcaccaacaacctgtccatcgtgtacctggaactgcggccttctgacgagggcacctatgagtgcctcgtgctgaagtacgagaaggatgccttcaagagagagcacctggccgaagtgacactgtctgtcaaggccgatggaggaggcggttccggcggcggcggctctggcgggggcggctctggcggcggcggctccggcgaggtgcagctgctggaatctggcggaggcctggtccagcctggcggatctctgagactgagctgtgctgcctctggcttcaccttctcctcttacgccatgtcctgggtgcggcaggcccctggcaaaggactggagtgggtctccggcatctccggcagcggcggctttacctattatgctgactccgtgaagggcagattcacaatctcccgcgacaatagcaagaacacactgtacctgcagatgaactccctgagagccgaggacacagccgtgtactactgcgccaagcctccaagaggctacaactacggcccctttgactactggggccagggcaccctcgtcaccgtgtcctctgcttctaccaagggcccttccgtgttccctctggctccttgctccagatccacctctgagtctaccgctgccctgggctgcctggtgaaggactacttccccgagcccgtgaccgtgtcttggaactctggcgctctgacctccggcgtgcacacctttccagctgtgctgcagtcctccggactgtactccctatcttctgtggttacagtgccttcctctagcctgggcaccaagacctacacctgcaacgtggatcacaagcccagcaataccaaagtggacaaacgggtggaatccaagtacggcccaccctgtcctccttgtcctgctcctgagttcctgggaggcccttccgtctttctgttcccccccaagcctaaggacaccctgatgatctctcgaacccctgaagtgacttgcgtggtcgtggacgtgtcccaagaggatcctgaagtgcagttcaactggtacgtggatggcgtggaggtacacaacgccaagacaaagcctagagaggaacagttcaacagcacctatagagtggtgtccgtgctggccgtactgcaccaggactggctgaacgggaaggagtacaagtgcaaggtgtccaacaagggcctgccttcgtccatcgagaagaccatttctaaggctaaaggacagcctcgggaacctcaagtgtacaccctgccaccttcccaagaagagatgaccaagaaccaggtgtccctgacttgtctggtgaaaggcttctacccctctgatatcgccgtggcctgggagtccaacggccagcccgagaacaactacaagaccacccctcctgtgctggactccgacggctctttcttcctgtacagccggctgaccgtggacaagtccagatggcaggaaggcaacgtgttctcctgctccgtgatgcacgaggccctgcacgcccactacacccagaagtctctgtccctcagcctgggaaag

SEQ ID NO: 256 - DNA, 1785 bp, synthetic construct
  misc_feature 1..1785: note = Artificial
  source 1..1785: mol_type = other DNA
atgggttggagttgcatcatcctatttctagtcgccacagctacaggcgtgcattccgtgatccacgtgaccaaagaggtgaaagaagtggctaccctgtcttgcggccacaatgtgtctgttgaggagctggctcagaccagaatctactggcagaaagaaaagaagatggtgctgaccatgatgtctggcgaccagaacatctggcctgagtataagaatcggaccatcttcgacatcaccaacaacctgtccattgtgtacctggaactcagaccttctgacgagggcacctatgagtgtcttgtgctgaagtacgagaaggacgccttcaagcgggagcacctggctgaggttaccctgtccgtgaaggccgatggcggcggaggctctggtggcgggggctctggcggcggaggctccggaggaggaggaagtggagaggtgcagctgctggaaagcggcggcggcctggtgcagcctggcggctccctgcggctgtcctgcgccgcttctggctttaccttttcctcctacgccatgtcctgggtgcggcaggcccctggcaagggcctggaatgggtctctggcatctccggcagcggcggcttcacctactacgccgacagcgtgaaaggcagattcaccatctctcgggacaattctaagaataccctgtacctgcagatgaactccctgagagccgaggacaccgctgtgtactactgcgctaagcctcctcggggctacaactacggacctttcgactactgggggcaggggacactcgtgaccgtgtcctctgcctccactaagggccctagcgtgtttcctctggctccttgttctcgctctacctccgagtctaccgccgccctgggctgcctggtgaaggactacttccccgagcctgtgaccgtgtcttggaacagcggcgctctgacatctggcgtgcacaccttccccgccgtcctgcagtcctccggcctgtattctctgagcagcgtggtgacggtgccatcctcttctctgggcaccaagacatacacctgcaacgtggatcacaagcccagcaacaccaaggtggacaagagagtggaatccaagtacggccctccttgtcctccttgcccagctcctgagttcctgggcggcccttccgtgtttctgttcccacccaagcctaaggatacactgatgatctcccggacacctgaagtgacctgcgtggtggtggatgtgtcccaagaggatccagaagtccagttcaactggtacgtggacggcgtggaagtgcacaacgccaagacaaaacctagggaggaacagttcaactccacctacagagtggtctctgtgctggctgtgctgcatcaggactggctgaacggcaaagagtacaagtgcaaggtgtccaacaagggcctgccttcctctatcgagaagaccatcagtaaggccaagggccagcccagagagcctcaggtgtacaccctgcccccctctcaagaagagatgaccaagaaccaggtttccctgacctgtctggtcaagggcttctacccttccgatatcgccgtggcctgggagtccaacggccagcctgagaacaactacaagaccacccctccagtgctggactccgacggcagcttcttcctgtacagcagactgaccgtggacaagtccagatggcaggaaggcaacgtgttctcctgctccgtgatgcacgaggccctgcacgcccactacacccaaaagagcttgtctctgtccctgggcaag

SEQ ID NO: 257 - DNA, 1785 bp, synthetic construct
  misc_feature 1..1785: note = Artificial
  source 1..1785: mol_type = other DNA
atgggttggagttgcatcatcctatttctagttgccaccgctaccggcgtccatagcgtgatccacgtgacaaaagaagtgaaagaagtggctacactgtcctgcggccacaatgtgagtgtcgaagagctggctcagaccagaatctactggcagaaagagaagaagatggtgctgaccatgatgtccggtgacaagaacatctggcctgaatacaagaacagaaccatcttcgatatcaccaacaacctgagcatcgtgtatctggaactgagaccttctgacgagggcacctacgagtgccttgtactgaagtatgaaaaggacgccttcaagcgcgaacatctggctgaggtgaccctcagcgtgaaggccgacggcggaggaggctccggcggaggcggatctggcggaggcggctccggcggaggcggctctggcgaggtgcagctgctggaatctggcggcggcctggtgcagcctggcggatctctgcggctgtcctgcgctgcctctggcttcaccttttcctcctacgccatgtcctgggtgcggcaggctccaggtaaagggctggagtgggtgtctggcatctctggctccggcggctttacctactacgccgattcagtcaagggcagattcaccatttcccgggacaactccaagaacaccctgtacctgcagatgaactcgctgcgggctgaggacacggccgtgtactactgtgctaagccccctagaggctacaactacggccctttcgactactggggccagggcaccctcgtgaccgtctcttccgccagcaccaagggcccctctgtgtttcctctggccccctgctcaagatccacctccgagtctaccgccgctctgggctgcctggtgaaggactacttccccgagcccgtaacagtgtcctggaactccggcgctctgacatccggcgtgcacaccttccccgctgtcctgcagtcttctggtctgtactctctgtcttccgtggtgaccgtgccttccagcagcctgggcacaaagacctatacctgcaacgtggaccacaagccttctaataccaaagtggacaagagagtggagtccaagtacggccctccttgtcctccttgccctgcccctgagttcctgggcggcccgtctgtgtttctgttcccacctaagcccaaggataccctgatgatcagccggacacctgaagtgacatgtgtggtggtggacgtgtcccaagaggatcctgaagtgcagttcaattggtacgtggacggcgtggaagtgcacaacgccaaaaccaagccccgggaggagcagttcaactctacttacagagtggtgtccgtgctggccgtgctgcaccaggactggctgaacggcaaggagtacaagtgcaaggtgtccaacaagggcctgccatcttctatcgagaagacaatctccaaagccaagggccaacctcgggagcctcaggtgtacaccctgcctccctcccaggaagagatgaccaagaatcaggtttctctgacctgtctggtcaagggcttctacccctccgacatcgccgtggcttgggagagcaacggacagcctgagaacaactacaagaccacccctcctgtgctggactccgatggctccttcttcctgtactccagactgaccgtggataagtccagatggcaagagggcaacgtgttctcctgcagcgtgatgcacgaggccctgcacgcccactacacccagaagtctctgtccctgtccctcggcaag

SEQ ID NO: 258 - DNA, 1785 bp, synthetic construct
  misc_feature 1..1785: note = Artificial
  source 1..1785: mol_type = other DNA
atgggttggagttgcatcatcctatttctagtggccacagctaccggcgtgcactctgtgatccacgtgaccaaagaagtgaaagaagtcgctacactttcctgcggccacaacgtgtccgtcgaggagctggcccagacccggatttactggcagaaagagaagaagatggtgctgaccatgatgtctggcgacatgaacatctggcctgaatacaagaacaggaccatcttcgacatcaccaacaacctgtctatcgtgatcctggccctgcggccttccgacgaaggcacctacgagtgcgtcgtgctcaagtacgagaaggacgccttcaagcgggagcacctggccgaggttacactgtccgtgaaggccgacggcggtggcggctctggtggcggcggctccggcggcggaggatctggcggaggaggcagtggcgaggtgcagctgctggaatctggcggcggcctggtgcaaccagggggatctctgagactgtcctgtgctgccagcggcttcaccttctcctcctacgccatgtcctgggtgcggcaggcccctggcaaggggctggaatgggtctccggcatctctggctccggcggctttacctactacgctgattctgtgaagggcagattcaccatcagccgcgacaactctaagaacaccctgtacctgcagatgaactctctgagagctgaggacaccgctgtgtactactgcgccaagccacctagaggctacaactacggaccttttgactactggggccagggcacactggtcaccgtgtcctctgcctctacgaaaggcccctccgtgtttcctctggctccctgttctagatccacatccgagtccaccgccgctctgggctgcctggtcaaggactacttccccgagcctgtgacagtgtcttggaactccggcgccctgacttccggcgtgcacacctttcccgccgtgctgcagtcctcaggcctgtactccttgtcctccgtggtgaccgtgcctagctcaagcctgggcaccaagacctatacctgcaatgtggaccacaagccaagcaataccaaagtggacaagagagtggaatccaagtacggccctccttgccctccttgtcccgctcctgagttcctcggcggaccttctgtgttcctgttcccccccaagcctaaggataccctgatgatctcccggacccctgaagtgacctgcgtggtcgtcgacgtgagccaagaggatcctgaggtgcagttcaactggtacgtggatggcgtggaagtgcataacgccaagaccaagccaagagaggaacagttcaactcaacctatagagtggtgtctgttctaacagtgctgcatcaggactggctgaacggcaaggagtacaagtgcaaggtgtccaacaagggcctgcccagctccatcgagaaaaccatctccaaggctaagggccagcctcgggaacctcaagtgtataccctgcctccttctcaggaagagatgaccaagaaccaggtgtcgctgacctgtctggtgaagggattctacccttctgatatcgccgtggagtgggagtccaatggccagcccgagaacaactacaaaaccacacctcctgtgctggattctgacggctccttcttcctgtactctcggttgaccgtggacaagtccagatggcaggagggcaacgtgttcagctgctcggtgatgcacgaggctctgcacaaccactacacccagaagtctctgtcactgtccctgggcaag

SEQ ID NO: 259 - DNA, 2031 bp, synthetic construct
  misc_feature 1..2031: note = Artificial
  source 1..2031: mol_type = other DNA
gtgatccatgtgactaaggaagtgaaggaagtggccacactgtcctgcggccataatgtgtccgtggaagagctggctcagaccagaatctactggcagaaaaacaagaagatggtgctgaccatgatgtctggcgacatgaacatctggcctgagtacaagaaccggaccatcttcgacatcaccaacaacctgtccatcgtgatcctggaactgagaccttccgacgagggaacctatgagtgtgtggtcctgaagtacgagaaggacgccttcaagcgggagcatctggccgaggtgaccctgtccgtgaaggccgatttccccaccccctccatctccgacttcgagatccctacctctaacatccggcggattatctgctcgaccagcggcggctttccagagcctcacctgagctggctggaaaacggcgaagaactgaacgccatcaacaccaccgtgtctcaggatcctgagaccgagctgtatgctgtgtcaagcaagctggatttcaacatgacaaccaaccactccttcatgtgcctgatcaagtacggccacctgagagtgaaccagaccttcaattggaataccaccaagcaggagcacttccccgacaacggcggcggaggctcaggcggagggggctccggcggcggcggtagcgggggcggcggctccggcgaggtgcagctgctggaatctggcggcggactggtccagcctggcggatccctccggctgtcttgtgccgcctctggattcaccttcagctcctacgccatgtcctgggtcagacaggcccctggcaagggcctggagtgggtgtccggcatctccggatctggcggctttacatactacgccgactctgtgaaaggcagattcaccatcagccgggacaacagcaaaaacacgctctacctgcagatgaactccttgcgggctgaggataccgccgtgtactactgcgccaagcccccaagaggctacaactacggccctttcgactactggggccagggcacactggtgaccgtctcttccgctagcaccaaaggaccttccgtgtttcctctggccccttgctctagatccacctccgaatccaccgctgctctgggctgtctcgtgaaggactacttccctgaacctgtgaccgtgtcttggaactctggcgctctgacctctggcgtgcacaccttcccagccgttttacagtccagcgggctgtactccctgtcttctgtggtgaccgtcccttcctcctccctgggcacaaagacctacacctgcaacgtggatcacaagccctctaacaccaaggtcgacaagagggtggagagtaaatacggcccgccttgtcctccttgccctgctcccgagttcctgggcggccctagtgtgtttctgttccccccaaagcctaaggataccctgatgatctccagaacccctgaagtgacatgcgtggtggtggacgtgagccaagaagaccctgaggtgcagtttaactggtacgtggacggcgtggaagtgcacaacgctaagaccaagcctagagaggagcagttcaactccacctaccgggtggttagcgtactcgccgtgctgcaccaggactggctgaatggcaaagaatacaagtgcaaggtgtccaacaagggcctgccttcctctatcgagaagaccatctctaaggccaaggggcagcctcgcgagcctcaggtgtacacactgccaccctcccaagaagagatgaccaagaatcaagtgtctctgacctgcctggtgaagggcttctacccttccgacatcgctgtggcttgggagtccaacggccagcccgagaacaactacaaaactacacctcctgtcctggactccgatggctctttcttcctgtattctagactgacagtggacaaatctagatggcaggaaggcaacgtgttctcctgctctgtgatgcacgaggccctgcacgcccactacacccagaagtccctgtctctgtctctgggaaag

SEQ ID NO: 260 - DNA, 2031 bp, synthetic construct
  misc_feature 1..2031: note = Artificial
  source 1..2031: mol_type = other DNA
gtgatccatgtgactaaggaagtgaaggaagtggccaccctgtcttgcggccacaacgtgtctgtggaggaactggcccagaccagaatctactggcagaaaaacaagaagatggtgctgaccatgatgtccggcgatatgaacatctggcctgagtacaagaaccggaccatcttcgacatcaccaacaacctgtccatcgtgatcctgaatctgcggcctagcgacgagggcacctacgagtgcgtggtgctgaagtacgagaaggatgccttcaagcgggaacacctggctgaggtcaccctaagtgtgaaggctgacttccctaccccttcgatctccgatttcgagatccccacctctaacatcagacggatcatctgctccacctccggtggctttcccgaacctcatctgagctggctcgaaaacggcgaggagctgaacgccatcaacaccaccgtgtctcaggaccctgaaaccgagctgtacgctgtgtcctctaagctggacttcaacatgaccaccaaccactcctttatgtgcctgatcaagtatggccatctgagagtgaaccagaccttcaattggaacaccaccaagcaggagcacttccctgacaacggaggcgggggctccggtggaggcggatctggaggaggcggcagcgggggcggcggatctggcgaagtgcagctgctggaatccggaggcggactggtgcagcctggcggctctctgcggctgtcctgtgccgcttccggcttcaccttctcttcctacgccatgtcttgggtcagacaggccccaggaaaaggcctggaatgggtgagcggcatctctggctctggcggcttcacctattacgccgactccgtcaaaggcagattcaccatttcccgggacaactccaagaatacactgtacctgcagatgaactccctgcgggcggaggacaccgctgtgtactactgcgccaagccacctcggggctacaactacggccctttcgactactggggccagggcaccctggtgaccgtgtcctccgcctctacaaaaggcccctccgtgtttcctctggccccttgctctcgcagcacctccgagtctacagccgctctgggctgcctggtgaaggactacttcccagagcccgtgacagtgtcctggaactctggcgctctgacctctggcgtgcacacctttcctgccgtgctgcagtcctccggcctgtattccctgtctagcgtggtgaccgtgccttcatctagcctcggcaccaaaacctacacctgcaacgtggaccacaagccttctaacaccaaggtggacaagagagtggaatctaagtacggccctccttgtcctccttgccctgctcccgagttcctgggcggcccttccgtgttcctgttcccccctaagcccaaggacacgctgatgatctccagaacccctgaggtcacatgcgtggtcgtggacgtgagccaagaggatcctgaggtgcagttcaactggtacgtggatggcgtggaagtgcacaatgctaagacaaaacctagggaagagcagttcaactctacttacagagtcgtgtccgtgctggctgtgctgcaccaggattggctgaacggcaaagagtacaagtgcaaggtttccaacaagggcctgcccagcagcatcgagaagaccatctccaaggccaagggccagcccagagagcctcaggtttacacactgcctccatctcaagaagagatgaccaagaaccaggtgtctctgacctgtctggtgaagggcttctacccttccgacatcgccgtggcttgggagtccaatggccagcctgagaacaactacaagaccactcctccagtgctggattccgacggcagcttctttctctactccagactgacagtggacaagtctagatggcaagaaggcaacgtgttctcctgttccgtgatgcacgaggccctgcacgcccactacacccagaagtccctttcgctgtccctgggcaaa

SEQ ID NO: 261 - DNA, 2031 bp, synthetic construct
  misc_feature 1..2031: note = Artificial
  source 1..2031: mol_type = other DNA
gtgatccatgtgactaaggaagtgaaggaagtggccaccctgagctgcggccacaacgtgtctgtggaagaactggctcagaccagaatctactggcagaagaacaagaagatggtgctaaccatgatgtctggcgacatgaatatctggcctgaatacaagaaccggaccatcttcgatatcaccaacaacctgtctatcgtgatcctgcagctgagaccttccgacgagggcacctacgagtgcgtggtcctgaagtacgagaaggacgccttcaagagagagcacctcgctgaggtgacactcagcgtgaaggctgatttccctaccccttccattagcgacttcgagatccccacctccaacatcagacggatcatctgctccacctctggaggctttccagaacctcacctgtcttggctggaaaacggcgaagaactgaacgccatcaacaccaccgtgagtcaagaccctgaaaccgagctgtacgctgtgtcctccaagctggactttaacatgaccaccaaccactccttcatgtgcctgatcaagtacggccatctgcgcgtgaaccagacattcaattggaacaccacaaaacaggagcacttccctgacaatggcggcggaggttctggcggaggcggctctggcggaggcggatctggcggcggcggatccggcgaggtgcagctgctggaatctggaggcggcctggtgcagcctggcggctctctgcggctgtcctgcgccgcctccggcttcaccttcagctcctacgccatgtcctgggtgcggcaggcccctggcaagggactggagtgggtctccggaatctcaggctctggcggcttcacctactacgctgacagcgtgaaaggcagattcactatctcccgggacaactccaagaacacactgtacctgcagatgaacagtctgagagccgaagacaccgctgtgtactactgcgctaaaccccccagaggctacaactacggacctttcgactactggggccagggcacactggtaaccgtttcttctgcctctaccaagggcccctccgtgttccctctggctccttgctctagatctacctccgagtccaccgccgctctgggctgcctggtgaaggattacttcccagaacccgtgaccgtgtcttggaacagtggcgctctgacatctggcgtgcacacctttcctgccgtgctgcagtcctctggcctgtacagcctgtccagcgttgtgaccgtgccttcctcctctctgggcaccaaaacctatacctgcaacgtggaccacaagccatctaacaccaaagtggacaagcgggtggagtccaagtacggtcctccttgtcctccttgccctgctcctgagttcctgggcggcccttccgtgtttctgttcccccccaagcctaaggacaccctcatgatcagccggacacctgaggtgacctgtgtggtggtggacgtgagccaagaggatcctgaggtgcagtttaactggtacgtggacggcgtggaagtgcataatgccaagacaaagcctagggaggagcagttcaactccacctacagagtcgtgtccgtgctggccgtgctgcatcaggactggctgaacgggaaagagtataagtgcaaggtgtccaacaagggcctgccctccagcatcgagaagaccatctctaaggccaagggccagcctcgggagcctcaggtctacaccctgcctccttcccaggaggagatgaccaagaatcaagtgtcgctgacctgtctggtcaagggcttctacccctccgacatcgccgtggcctgggagagcaacggccagcccgaaaacaactataagacaaccccacctgtgctggattccgatggctctttcttcctgtactccagactgaccgttgataagtccagatggcaagaaggcaacgtgttctcctgttccgtgatgcacgaggccctgcacgcccactacacccagaaatctctgagcctgagtctgggcaag

SEQ ID NO: 262 - DNA, 2031 bp, synthetic construct
  misc_feature 1..2031: note = Artificial
  source 1..2031: mol_type = other DNA
gtgatccatgtgactaaggaagtgaaggaagtggccaccttgtcctgcggacacaacgtgtccgtggaggagctggcccagaccagaatctactggcagaaaaacaagaagatggtgctgaccatgatgtccggcgacatgaacatctggcctgaatacaagaaccggaccatcttcgacatcaccaacaacctgtccatcgtgatcctgacactccggccttctgacgagggcacctacgagtgcgtggtgctgaagtacgagaaggacgccttcaagagagagcacctggccgaagtgactctgtccgtgaaggccgacttccctaccccttctatttccgactttgagatccctacctctaatatccggcggatcatctgctccacatctggtggcttccccgagcctcatctcagctggctggaaaatggcgaggaactgaacgccatcaacaccaccgtttctcaggaccccgagacagagctgtacgccgtgtcttccaagctggatttcaacatgaccaccaaccactccttcatgtgcctgatcaagtacggccaccttagagtgaaccagaccttcaactggaataccacaaagcaggaacacttccctgacaacggcggcggcggcagcggcggaggcggttccggcggcggcggaagcggcggcggcggcagtggagaagtgcagctgctggaatccggcggcggcctggtgcagcctggcggatctctgcggctgtcatgtgctgcttctggcttcaccttctcctcctacgccatgtcctgggtgcggcaggcccctggcaaaggcctggaatgggtgtccggcatctccggatctggcggctttacctactacgctgattctgtgaagggcagattcaccatctccagggataactccaagaacaccctgtacctgcagatgaactctctgagagccgaggacaccgccgtgtactactgtgccaagccgcctagaggctacaactacggtcctttcgactactggggccagggcaccctggtcaccgtgtcctccgcctctaccaagggaccatctgtttttcctctggctccatgctctcggtctacatccgagtcaacagctgctctgggctgcctggtgaaggactacttcccagaacctgtgacagtgtcttggaactccggagctctgacctccggcgtgcacacctttccagctgtgctgcagtccagcggcctgtactccctgtctagtgtggtgaccgtgccctcgtcttctctgggaacaaaaacctatacctgcaacgtggaccacaagcccagcaacaccaaagtggacaagcgggtcgagtctaaatacggccccccctgccctccttgtcctgctcctgagttcctgggcggccctagcgtgtttctgttccctcctaagcctaaggataccctgatgatcagcagaacccctgaggtgacctgtgtggtcgtggacgtgtcccaggaagaccctgaggtacagttcaactggtacgtggatggcgtggaagtgcataacgctaagaccaagcctagagaagaacagttcaattctacgtacagagtggtgtctgtgctggctgttctgcaccaggattggctgaacggcaaagagtataagtgcaaggtgtccaacaagggcctgccttcttctatcgagaagacaatctctaaggccaagggccaaccccgcgagccccaggtgtacaccctgccccctagccaagaggagatgaccaaaaatcaagtgtccctgacctgtctggtcaagggcttctacccttccgacatcgccgtggcttgggagtccaatggccagcctgagaacaactacaagaccaccccacccgtgctggactccgacggcagcttcttcctgtattctagactgaccgtggataagtccagatggcaggaagggaacgtgttctcttgcagcgtgatgcacgaggccctgcacgcccactacacccagaagagcctctccctgagcctgggcaag

SEQ ID NO: 263 - protein, 677 aa, synthetic construct
  REGION 1..677: note = Artificial
VIHVTKEVKEVATLSCGHNVSVEELAQTRIYWQKEKKMVLTMMSGDMNIWPEYKNRTIFDITNNLSIVILALRPSDEGTYECVVLKYEKDAFKREHLAEVTLSVKADFPTPSISDFEIPTSNIRRIICSTSGGFPEPHLSWLENGEELNAINTTVSQDPETELYAVSSKLDFNMTTNHSFMCLIKYGHLRVNQTFNWNTTKQEHFPDNGGGGSGGGGSGGGGSGGGGSGEVQLLESGGGLVQPGGSLRLSCAASGFTFSSYAMSWVRQAPGKGLEWVSGISGSGGFTYYADSVKGRFTISRDNSKNTLYLQMNSLRAEDTAVYYCAKPPRGYNYGPFDYWGQGTLVTVSSASTKGPSVFPLAPCSRSTSESTAALGCLVKDYFPEPVTVSWNSGALTSGVHTFPAVLQSSGLYSLSSVVTVPSSSLGTKTYTCNVDHKPSNTKVDKRVESKYGPPCPPCPAPEFLGGPSVFLFPPKPKDTLMISRTPEVTCVVVDVSQEDPEVQFNWYVDGVEVHNAKTKPREEQFNSTYRVVSVLAVLHQDWLNGKEYKCKVSNKGLPSSIEKTISKAKGQPREPQVYTLPPSQEEMTKNQVSLTCLVKGFYPSDIAVAWESNGQPENNYKTTPPVLDSDGSFFLYSRLTVDKSRWQEGNVFSCSVMHEALHAHYTQKSLSLSLGK

SEQ ID NO: 264 - DNA, 2088 bp, synthetic construct
  misc_feature 1..2088: note = Artificial
  source 1..2088: mol_type = other DNA
atgggctggtcctgcatcattctgttcctggtggccacagccaccggcgtccacagcgtgatccacgtgacaaaagaggtgaaagaggttgctacactgagctgcggccacaacgtgtctgtggaagagctcgcccagaccagaatctactggcagaaagaaaaaaagatggtgctgaccatgatgtctggagatatgaacatctggcctgaatacaagaacagaacaatcttcgacatcaccaacaacctgagcatcgtgatcctggctctgcggccttcagacgagggcacctacgagtgcgtggtgctgaagtatgagaaggacgccttcaagagagagcacctggcagaagtgacactgtccgtgaaggccgacttccctacacctagcatcagcgatttcgagatccctaccagcaatatccggagaatcatttgctccacatctggaggctttccggagccccacctgagctggctggaaaacggagaggaactgaacgccatcaacaccacagtgagccaggaccccgaaaccgagctgtacgccgtgtccagcaagctggactttaacatgacaacaaaccattcttttatgtgcctgatcaagtacgggcacctgagagtgaaccagacattcaactggaacactaccaagcaggagcatttcccagacaacggcggaggtggaagcggcggcggcggctctggcggcggaggctctggcggcggcggttccggcgaggtgcagctgctggaaagcggcggcggcctggtgcaaccaggcggaagcctgagactgagctgtgccgccagcggctttaccttttctagctacgccatgagctgggtgcggcaggcccctggaaaaggcctggaatgggtcagcggcattagcggcagcggcggcttcacgtactacgctgattctgtgaagggcagattcaccatctcacgcgacaactccaaaaacaccctgtacctgcaaatgaacagcctgagagcggaggataccgccgtgtactactgcgccaagccccctaggggctacaactacggcccattcgactactggggccaaggcaccctggtgacagtgagttccgccagcaccaagggcccatccgtgttccctctggctccttgtagccggagcaccagcgagagtacagccgctctgggctgcctggtgaaagactacttccccgagcctgtgaccgtgtcttggaacagcggcgccctgacaagcggagtgcacaccttccccgccgtgctgcagagcagcggcctgtacagcctgtctagcgtggtcaccgtgcctagcagctctctgggcaccaagacatatacatgcaacgtggaccacaaacccagcaacaccaaggtggacaagcgggtggaaagcaagtacggccccccatgccctccatgtcctgctcccgagttcctgggcggccctagcgtgttcctgtttccccccaagcctaaggataccctcatgatcagccggacccctgaagtgacatgtgtggtggtggacgtgtctcaggaagatcctgaggttcagttcaactggtacgtggatggagtggaagtccacaacgccaagaccaagccaagagaagagcagttcaacagcacatacagagtggtgtcagtgctgaccgtcctgcaccaggattggctgaatggcaaggagtataagtgcaaggtgagcaacaagggccttccttcttccatcgagaagaccatcagcaaggccaaaggccagcccagagagcctcaggtgtacaccctgcctcctagccaggaggaaatgaccaagaatcaggtgtctctcacctgcctggttaagggcttctacccctccgacatcgccgtggaatgggagtcaaatggacagcctgagaacaactacaagaccacccctcccgtgctggacagcgacggcagcttcttcctgtatagcagactgaccgttgacaagtccagatggcaggagggaaatgtgttcagctgttctgtcatgcacgaggccctgcacaatcactacacccagaagagcctgagcctcagcctgggaaag

SEQ ID NO: 265 - DNA, 1359 bp, synthetic construct
  misc_feature 1..1359: note = Artificial
  source 1..1359: mol_type = other DNA
atgggttggagttgcatcatcctatttctagtggctacagccaccggcgtgcacagcgtgatccacgtcaccaaagaagtgaaagaggtggccacactgagctgcggccataacgtgagcgtggaagagctggctcagaccagaatctactggcagaaaaacaagaagatggtcctgaccatgatgtccggcgatatgaacatctggcctgagtataagaacagaaccatcttcgacatcaccaacaacctgtctatcgtgatcctggaactgcggccttctgacgaaggcacctacgagtgcgtggtgctgaagtacgagaaggacgccttcaagcgggaacatctggccgaggtgaccctctccgtgaaggccgacttccctacaccttccatcagcgatttcgagatccctacgtccaacatcagacggatcatctgctctacctctggcggatttcctgaacctcacctgtcttggctggagaacggcgaggagctgaacgccatcaacacaaccgtgtctcaggatcctgagacagagctgtacgccgttagttctaagctggattttaacatgaccacaaaccactctttcatgtgcctgatcaagtacggccacctgagagtgaaccagaccttcaattggaacaccaccaagcaagagcacttccccgacaacgataagacccacacctgtcctccatgccctgctcccgagctgctgggcggcccttccgtgtttctgttcccacctaaacccaaggacaccctgatgatttctcggacccctgaagtgacctgtgttgtcgtggacgtgtctcacgaggaccccgaggtgaagttcaactggtacgtggatggcgtggaagtgcacaatgccaagaccaagcctagggaagagcagtacaactccacctacagagtggtgtccgtcctcacagtgctgcaccaggactggctgaatggcaaggagtataagtgcaaggtgagcaacaaggccctgcctgctcctatcgagaaaaccatctccaaggctaagggacagccaagagagcctcaggtgtacactctgcccccttcccgggacgaactgaccaagaaccaagtgtctctgacctgtctggtgaagggcttctacccttccgacatcgccgtggaatgggagtctaacggccagcccgaaaacaactacaagaccacccccccagtgctggactccgacggatccttcttcctgtactccaagctgaccgtcgacaagtccagatggcagcagggcaacgtgttctcctgctccgtgatgcacgaggctctgcataatcactacacccagaagtctctgtcactgtcccctggc

SEQ ID NO: 266 - DNA, 1359 bp, synthetic construct
  misc_feature 1..1359: note = Artificial
  source 1..1359: mol_type = other DNA
atgggttggagttgcatcatcctatttctagttgctacagctaccggcgtgcactctgtgatccacgtgaccaaggaggtgaaagaagtggccaccctatcttgcggccataatgtcagcgtggaagagctggctcagaccagaatctattggcagaaaaacaagaagatggtgctgaccatgatgtctggcgacatgaacatctggcctgagtataagaaccggaccatcttcgacatcaccaacaacctgtccatcgtgatcctgaacctgcggccttctgacgagggcacctacgagtgcgtggtgctgaagtacgagaaggatgccttcaagagagaacacctggccgaggtgaccctgtctgtgaaggccgactttccaacaccttctatctctgacttcgagatccctacctctaacatccggcggatcatctgctctacctccggcggctttcccgaacctcatctctcctggctggaaaacggcgaggaacttaacgccatcaacaccacagtgtctcaggatccagaaacagaactgtacgccgtctccagcaagctggattttaacatgaccaccaatcactccttcatgtgcctgatcaagtacggccatctgagagtgaaccagaccttcaattggaacacaaccaagcaagagcacttccccgacaacgacaagacccacacctgtcctccttgccctgcccctgagctgctgggaggaccttccgtgttcctgttccctcccaagcctaaggacaccctgatgatctcccgcactcccgaagtgacctgtgtggtcgtggacgtgtctcacgaggaccccgaggtcaagttcaactggtacgtggatggagtggaagtgcacaacgccaagacaaaacctcgggaagagcagtacaactccacctacagagtggtgtccgtactgaccgtgctgcaccaggactggctgaatggcaaggagtacaagtgcaaggtgtccaacaaagccctgcctgctcctatcgagaaaaccatttccaaggctaaaggccagcctagagagccccaagtgtacaccctgccgcctagcagagatgagctgaccaagaaccaggtgtccctgacctgtctggtgaagggcttctaccccagcgatatcgccgtggagtgggagtcgaacggccagcctgagaacaactacaagaccaccccacctgtgctcgactccgacggcagtttcttcctgtactccaagctgacagtggacaagtctagatggcagcagggcaacgtgttctcctgctccgtgatgcacgaggctctgcacaaccactacacccagaagtccctgagcctgtctcctggc

SEQ ID NO: 267 - DNA, 1359 bp, synthetic construct
  misc_feature 1..1359: note = Artificial
  source 1..1359: mol_type = other DNA
atgggttggagttgcatcatcctatttctagtggccaccgctaccggcgtgcactccgtgatccacgtgaccaaagaagtgaaagaggtggctaccctctcctgcggccataatgtgtccgtcgaggaactggcccagacaagaatctactggcagaaaaacaagaagatggtgctgaccatgatgtccggcgacatgaacatctggcctgaatacaagaaccggaccatcttcgacatcaccaacaacctgtccatcgtgatcctgcagctgcggccttctgacgagggaacctatgagtgcgtggttctgaagtacgagaaagacgccttcaagagagaacatctggccgaggtgactctgtctgtcaaggccgattttcctaccccttccatctccgacttcgagatccccacctccaacatcagacggatcatctgcagcacctctggcggatttcccgagcctcacctgtcttggctggaaaacggcgaggaactcaatgccatcaacaccaccgtgtctcaggatcctgaaaccgagctgtacgccgtctcttctaagctggatttcaacatgaccaccaaccattctttcatgtgcctgatcaagtacggccacctgagagtgaaccagaccttcaactggaacaccaccaagcaagagcacttccccgacaacgacaagacccacacctgtcctccctgcccagctcccgagctgctgggcggcccttctgtgtttctgttcccccctaagccaaaggacaccctgatgatctctagaacaccagaagtgacatgtgtggtggtggatgtgtctcacgaggacccagaagtgaagttcaattggtacgtggacggcgtggaagtgcacaacgctaaaaccaaacctcgggaagagcagtacaactccacctacagagtggtgtccgtcctgacagtgctgcaccaggactggctgaacggcaaggaatataagtgcaaggtgtccaacaaggctctgcctgcccctatcgagaagacaattagcaaggccaagggccagcctagagagcctcaagtgtacacactgcctccttcccgggatgagctgaccaaaaaccaggtctctctgacctgcctggtgaagggtttctacccctccgacatcgctgtggagtgggagtctaatggacagcctgagaacaactacaagaccacacctcctgttctggactccgatggctccttcttcctgtactccaagctgaccgtggacaagagccgctggcagcagggcaacgtgttcagctgttccgtgatgcacgaggccctgcacaaccactacacccagaagtccctgagcctgagccctggc

SEQ ID NO: 268 - DNA, 1359 bp, synthetic construct
  misc_feature 1..1359: note = Artificial
  source 1..1359: mol_type = other DNA
atgggttggagttgcatcatcctatttctagtggctaccgctaccggcgtgcactccgtgatccacgtgaccaaagaggtgaaagaagtggctacactgtcctgcggccacaacgtgtccgtcgaggaactggctcagaccagaatctactggcagaaaaacaagaagatggtgctgaccatgatgtccggcgacatgaacatctggcctgagtataagaaccggaccatcttcgacatcaccaataacctgtccatcgtgatcctgacactgagaccttctgacgagggcacctacgagtgcgtggtcctgaagtacgagaaggacgccttcaagcgggaacatctggccgaggtcaccctcagcgtgaaagccgactttcctaccccatctatctccgacttcgagatccccacatctaacatcagacggatcatctgctctacctctggcggattcccagagcctcacctgtcttggctggaaaacggcgaagagctgaacgccatcaacaccaccgtgtctcaggatcccgaaaccgagctgtacgccgtgagctccaagctggattttaacatgaccaccaaccattccttcatgtgtctgatcaagtacggccatctgcgcgtgaaccagaccttcaactggaacaccacaaagcaagagcacttccctgacaatgacaagacccacacctgtcctccttgcccagcccctgaactgctgggaggcccttctgtttttctgttcccccctaagcccaaggacaccctgatgatctctcggacccctgaggtgacatgtgtggttgtggatgtgtctcacgaggaccctgaagtgaagttcaattggtacgtcgacggcgtggaagtgcacaacgctaaaacgaagcctcgggaagagcagtacaactctacctacagagtggtgtccgtgctgaccgtgctgcaccaggactggctgaacggcaaggagtacaagtgcaaggtgtccaacaaggccctgcctgctcccatcgagaagaccattagcaaggccaagggccagcctagagagccccaagtgtacacactcccaccttccagagatgagctgaccaagaaccaggtgagtctgacctgcctggtgaagggcttctaccctagcgatatcgccgtggaatgggagtccaatggccagcccgagaacaactacaaaaccacacctcctgtgctggactccgacggatctttcttcctgtattccaagctgaccgtggacaagtctagatggcagcagggcaacgtgttctcctgctccgtgatgcacgaggctttgcacaaccactacacccagaagtccctgtccctgtctcctggc

SEQ ID NO: 269 - DNA, 1377 bp, synthetic construct
  misc_feature 1..1377: note = Artificial
  source 1..1377: mol_type = other DNA
atgggttggagttgcatcatcctatttctagtggccaccgccaccggcgtgcactccgtgatccacgtgaccaaggaagtgaaagaggtggctaccctatcttgcggccacaacgtgtctgtggaagagttggcccagaccagaatctactggcagaaagaaaagaagatggtgctgacaatgatgtccggcgacatgaacatctggcctgagtacaagaacagaaccatcttcgatatcaccaacaacctgtccatcgtgatcctggccctgcggccttctgatgagggcacctacgaatgcgtggtgctgaagtacgagaaggacgccttcaagcgggaacatctggctgaggttacactgtccgtgaaggctgactttcctacaccctctatctccgacttcgagatccctacatccaacatcagacggatcatctgctctacctctggaggctttccagagcctcatctgtcctggctggaaaacggcgaggaactgaacgccatcaacaccaccgtgtctcaggatcctgaaaccgagctgtacgccgtgtcctccaagctggacttcaacatgaccaccaatcactctttcatgtgcctgatcaagtacggccatctgagagtgaaccagaccttcaattggaacaccaccaagcaagagcacttccctgacaacgagccaaagtcctgcgacaagacccacacctgtcctccttgccctgcccctgaactgctgggcggccctagcgtgtttctgttcccccctaagcccaaggacaccctgatgatctccagaacccctgaagtgacctgtgtcgtggtggacgtgtctcacgaggaccctgaagtcaagttcaactggtacgtggatggcgtggaggtgcacaatgccaagacaaagcctcgggaggagcagtacaactccacctacagagtggtctctgtgctgaccgttctgcaccaggactggctgaatggtaaagagtataagtgcaaggtgtctaacaaggctctgcctgctcctatcgagaaaaccatttctaaagctaaaggacagccccgggagcctcaagtgtacaccctgccccccagccgcgacgaactgactaagaaccaggtcagcctgacctgcctggtgaagggcttctaccctagcgatatcgccgtagaatgggagtccaacggccagcccgagaacaactacaagaccacaccacctgtgctggactccgacggctccttcttcctgtactccaagctgaccgtggataagtctagatggcagcagggcaacgtgttctcctgtagcgtgatgcacgaggctctgcacaaccactatacacagaagtccctgagcctctctccaggcaag

SEQ ID NO: 270 - DNA, 1056 bp, synthetic construct
  misc_feature 1..1056: note = Artificial
  source 1..1056: mol_type = other DNA
atgggttggagttgcatcatcctatttctagtggctaccgctacaggcgtgcactccgtgatccacgtgaccaaagaagttaaagaggtggccaccctgtcttgtggccataatgtgagcgtggaagaactggctcagaccagaatctactggcagaaaaacaagaagatggtgctgaccatgatgtccggcgacatgaacatctggcctgagtacaagaatagaaccatcttcgacatcaccaacaacctgtccatcgtcatcctggaactgagaccttctgatgagggcacctatgagtgcgtggttctgaagtacgagaaagatgccttcaagcgggagcacctggccgaggtgacactctctgtgaaggctgacgacaagacccacacctgtcctccttgccctgcccctgagctgctgggaggccccagcgtgtttctgttcccccctaagcccaaggacaccctgatgatctcccggacccctgaagtcacctgcgtggtggtggacgtgtctcacgaggaccccgaagtgaagttcaactggtacgtggatggcgtcgaagtgcataacgccaaaaccaagcctcgggaagagcagtacaactccacctaccgggtggtctctgtgctgaccgtgctccaccaggactggctgaacggcaaggagtacaagtgcaaggtgtctaacaaggctctgcctgctcctatcgagaagaccatctctaaggccaagggccagcctagagagcctcaagtgtacaccctgccaccctctcgcgacgagctgacaaagaaccaggtgtctctgacttgcctggtgaaaggcttttaccctagcgatattgccgtggaatgggagtccaatggccaacccgagaacaactacaagaccacacctcctgtgctggattccgacggctctttcttcttgtactccaagctgacagtggacaagtccagatggcagcagggcaacgtgttctcctgctccgtgatgcacgaggccctgcacaaccactacacccagaagtccctgagcctgagcccagga

SEQ ID NO: 271 - DNA, 1056 bp, synthetic construct
  misc_feature 1..1056: note = Artificial
  source 1..1056: mol_type = other DNA
atgggttggagttgcatcatcctatttctagtggccaccgctaccggcgtgcactccgtgatccacgtgacaaaagaggtgaaagaagtggctacactgtcctgcggccataatgtgtctgtcgaggaactggctcagaccagaatctactggcagaaaaacaagaagatggtgctgaccatgatgtccggcgacatgaacatctggcctgagtacaagaaccggaccatcttcgacatcaccaacaatctgtccatcgtgatcctgaacctgagaccttccgatgaaggcacctacgagtgcgtggtgctgaagtacgagaaggacgccttcaagcgggaacacctggccgaggttaccctgtctgtgaaggccgacgacaagacccacacctgtcctccttgccctgctcctgagctgttgggcggacctagcgtgtttctgttcccccccaagcctaaggataccctcatgatttcccggacccctgaggtgacctgcgtggtcgtggacgtgtctcacgaggaccccgaagtcaagttcaactggtacgtggatggcgtggaagtgcacaacgccaagacaaagccccgcgaagagcagtacaactccacctacagagtggtgtccgtgctgaccgtcctgcaccaggactggctgaacggcaaggaatataaatgcaaggtgtccaacaaggctctgcctgcccctatcgagaaaacaatctctaaagctaagggccagcctagagagcctcaagtgtataccctgcccccatctcgggacgagctgaccaagaaccaagtgagcctcacctgtctggtgaagggcttctacccttctgatatcgccgtggaatgggagagcaatggacagccagagaacaactacaagaccacaccacctgtgctggactccgacggctctttcttcctgtactccaagctgaccgtggacaagtctagatggcagcagggcaacgtgttttcttgctccgtgatgcacgaggccctgcataaccactacacccagaagtccctgagcctgtctcctggc

SEQ ID NO: 272 - DNA, 1056 bp, synthetic construct
  misc_feature 1..1056: note = Artificial
  source 1..1056: mol_type = other DNA
atgggttggagttgcatcatcctatttctagtggctaccgctacaggagtgcactctgtgatccacgtgaccaaagaagtgaaggaagtggccacactgtcttgcggccacaatgtgtctgtcgaggaactggctcagaccagaatctactggcagaagaataagaagatggtgctgaccatgatgtccggtgacatgaacatctggcctgaatataagaacagaaccatcttcgacatcaccaacaacctgtccatcgtgatcctgcagctgcggcccagcgatgagggcacctacgagtgcgtggtgctgaagtacgaaaaggacgccttcaagcgggagcacctggccgaggtgacactcagcgtcaaagccgacgacaagacccacacctgccctccttgtcctgccccagagctgctgggcggcccttccgtgttcctgttccctcctaagcccaaggacaccctgatgatctcccggacccctgaggtgacctgtgtggtggtggacgtgtctcatgaggaccccgaggtcaagttcaactggtacgtggatggcgtggaagtgcacaacgccaaaaccaagcctagagaagagcagtacaactccacctacagagtggtttctgtgctgaccgtgctgcaccaggactggctgaacggcaaagagtacaagtgcaaggtgtccaacaaggccctgcctgctcctatcgagaagacaattagcaaggccaagggccagcctcgcgagcctcaagtgtacaccctgcccccatctcgggatgagctgaccaagaaccaggtctctctgacctgcctggtgaaaggcttctacccttctgacatcgccgtggaatgggagtccaacggacaacccgagaacaactacaagactacccctcccgtgctggattccgacggctccttctttctgtactccaagctgacagttgataagtccagatggcagcagggcaacgtgtttagctgctccgtgatgcacgaggctctgcataatcactacacccagaaatctctctccctgtctcctggc

SEQ ID NO: 273 - DNA, 1056 bp, synthetic construct
  misc_feature 1..1056: note = Artificial
  source 1..1056: mol_type = other DNA
atgggttggagttgcatcatcctatttctagtggctacagctaccggcgtgcactctgtgattcacgtcaccaaagaggtgaaagaggtggccacgctgtcctgcggccacaatgtgtctgtggaggaactggctcagaccagaatctactggcagaagaacaagaagatggtgctgactatgatgtccggtgacatgaacatctggcctgagtataagaatcggaccatcttcgatatcaccaacaacctgtccatcgtgatcctgaccctgagaccaagcgacgagggcacctacgagtgcgtggtgctgaagtacgagaaggacgccttcaagcgcgaacatctggccgaggtgacactctccgtgaaggccgacgataagacacacacctgccctccttgtcctgcccctgagctgctgggcggaccttctgtttttctgtttcctcccaagcctaaggacaccctgatgatctctagaacccctgaagtgacctgtgtggtggttgacgtgtctcacgaggaccccgaagtgaagttcaactggtacgtggacggcgtggaagtgcacaacgccaagaccaagccgcgggaagaacagtacaactccacctacagagtggtctctgtgctcacagtgctgcaccaggactggctgaatggcaaggaatataagtgcaaggtgtccaacaaggccctgcctgctcctatcgagaagaccatctccaaagctaagggacagcctagagagcctcaggtgtacaccctgcctcccagccgggatgagctgaccaagaaccaagtctccctgacctgcctggtgaagggcttctacccctctgatatcgccgtggaatgggagagcaacggccaaccagagaacaactacaaaaccaccccccctgtgctggactccgatggctccttcttcctgtactccaagctgacagtggacaagtctcggtggcagcagggcaacgtcttctcctgctccgtgatgcacgaggctctgcataaccactacacccagaaatctctgtctctgagccctggc

SEQ ID NO: 274 - DNA, 1056 bp, synthetic construct
  misc_feature 1..1056: note = Artificial
  source 1..1056: mol_type = other DNA
atgggttggagttgcatcatcctatttctagtggccaccgctaccggcgtgcactccgtgatccacgtgacaaaagaggttaaagaagtggctacactgagctgcggccacaatgtgtctgtggaagagctggcccagaccagaatctactggcaaaaagagaagaagatggtgctgaccatgatgtctggcgacatgaacatctggcctgagtataagaaccggaccatcttcgacatcaccaacaacctgtccatcgtgatcctggctttgagaccatccgatgagggcacctacgagtgcgtggtcctgaagtacgagaaggacgccttcaagagagagcacctggccgaggtgacactctctgtcaaggccgacgacaagacccacacctgtcctccttgccctgcccctgagctgctgggtggacctagcgtctttctgtttccccctaagcccaaggacaccctgatgatttctcggacaccagaggtgacctgtgtcgtcgtggacgtgtcccatgaggatcctgaagtgaagttcaactggtacgtggatggcgtggaagtgcacaacgctaagaccaagcctagagaagaacagtacaactccacctatagagtggtgtccgtgctgaccgtgctgcaccaggactggctgaacggcaaggaatacaagtgcaaggtgtccaacaaggctctgcctgctcctatcgagaaaaccatctccaaggccaagggccagcctcgggaacctcaggtgtacaccctgccccccagccgggacgagctgacaaaaaatcaagtgagcctcacctgcctggtgaagggcttctacccatctgatatcgccgtggaatgggagtccaacggccagcccgagaacaactacaagaccacccctcctgtgctggactccgatggctccttcttcctgtactctaagctgaccgtggacaagtctcgctggcagcagggcaacgtgttctcctgctccgtgatgcacgaggccctgcataatcactacacccagaagtccctgtctctgtctcctgga

SEQ ID NO: 275 - DNA, 723 bp, synthetic construct
  misc_feature 1..723: note = Artificial
  source 1..723: mol_type = other DNA
gctagcgccgccaccatgggttggagttgcatcatcctatttctagtcgccaccgctaccggcgtgcattccgagatcgtgctgacccagtctcccgctactctgagcctgtctccaggcgaacgcgctacactgtcctgcagagcttctcagtccatctccagctacctggcctggtatcagcagaagcctggacaggcccctcggctgctgatctacgacgcctccaatcgggctaccggaatccccgctagattttccggctctggctccggcaccgacttcaccctgaccatctcttctctggaacctgaggattttgccgtgtactactgccagcagagatccaactggcctctgaccttcggccaaggcatcaacctggaaatcaagcggaccgtggccgctcctagcgtgttcatcttccctccttccgacgagcagctgaagtctggcacagcctccgtggtgtgcctgctgaacaacttctaccctagagaggccaaagtgcagtggaaggtggacaacgccctgcagagcggcaactcccaagagtctgtcacagaacaggattctaaggactccacctactccctgtccagcaccctcaccctgtccaaagccgactacgagaagcacaaggtgtacgcctgcgaggtgacccaccagggcctgtcttctcccgtgaccaagtccttcaacagaggcgagtgttgactcgag

SEQ ID NO: 276 - DNA, 1782 bp, synthetic construct
  misc_feature 1..1782: note = Artificial
  source 1..1782: mol_type = other DNA
atgggttggagttgcatcatcctatttctagtggccaccgctaccggcgtgcactccgtgatccacgtgaccaaagaagtgaaagaggtggccaccctgtcctgcggccacaacgtttctgtggaagagctggcccagacgagaatctactggcagaaaaacaagaagatggtgctgaccatgatgtccggcgacatgaacatctggcctgagtacaagaacagaaccattttcgacatcaccaacaacctgtccatcgtgatcctgaacctgcggccttccgacgagggcacctatgagtgcgtggtgctgaagtacgagaaggatgctttcaagcgggaacacctggccgaggtgaccctgtccgtgaaggccgatggcggcggcggctctggcggaggaggcagtggtggtggaggaagtggcggaggcggcagcggccaggtgcagctgcagcagtggggcgctggcctgctgaagccctcggagacactgtccttgacctgtgccgtgtacggcggctccttttctgactactactggaactggatcagacagcctcctggcaaaggcctggaatggatcggcgagatcaaccaccggggatctaccaactccaacccttccctgaagtctagagtgacactgtctctggacaccagcaagaaccagttctccctgaagctgagatctgtcaccgccgccgacaccgccgtgtactactgcgccttcggctactccgattacgaatacaactggttcgacccttggggccagggcaccctggtgaccgtgtcctccgcctctacaaaagggcccagcgtgtttcctctggctccttgctctagatccacctccgagtccaccgctgctctgggctgcctggtcaaggactacttccccgagcctgtgaccgtgtcttggaacagcggcgccctgacctctggcgtccataccttccctgctgtgctgcagtcctctggcctgtactccctgtcttctgtcgtgacagtgccttcttcctccctgggcacaaaaacctacacctgcaacgtggaccacaagcctagcaacaccaaggtggataagagagtggaatctaagtacggccccccctgcccaccttgtcctgcccctgagttcctcggcggcccttctgtctttctgttccctcctaagcccaaggacaccctgatgatctcccggacccctgaggttacctgtgtggtcgtggatgtgtcgcaagaggaccccgaagtgcagtttaattggtatgtggacggcgtggaagtgcacaacgccaagacaaagcctcgggaagaacagttcaacagcacttaccgggtggtttcggtgctcaccgtgctgcaccaggactggctgaacggcaaagagtacaagtgcaaggtgtccaacaagggcctgccttcttccatcgagaagaccatctccaaggctaagggacagcctcgcgaacctcaggtgtatacactgccaccttcccaagaggagatgaccaagaatcaagtatctctgacctgtctggtgaagggcttctacccctccgacatcgccgtggagtgggagtctaacggccagcccgagaacaactacaagacaaccccaccagtgctggattccgacggctctttcttcctgtacagcagattgaccgtggacaagagtagatggcaggaaggcaacgtgttcagctgctccgtgatgcacgaggctctgcataatcactacacccagaagtccctgagcctgtctctgggcaag

SEQ ID NO: 277 - DNA, 1725 bp, synthetic construct
  misc_feature 1..1725: note = Artificial
  source 1..1725: mol_type = other DNA
gtgatccatgtgactaaggaagtgaaggaagtggccaccctgtcttgcggccacaacgtctctgtggaagagctggcccagaccagaatctactggcagaaaaataagaagatggtgctgaccatgatgtccggcgacatgaacatctggcctgaatacaagaacagaaccatcttcgacatcaccaacaacctgtccatcgtgatcctgaacctgcggccttctgacgagggcacctacgagtgcgtggtgctgaagtacgaaaaggacgcctttaagagagagcatctggccgaggtgacactgtccgtgaaggccgatggcggaggcggatctggcggcgggggctccggcggcggcggctctggtggcggcggctctggacaagtgcagctgcagcagtggggcgctggcctgctgaagccctccgagacactgagcctaacctgtgccgtgtatggcggttctttctccgactactactggaattggatccggcagcctcctggcaagggcctggaatggatcggcgagattaaccaccggggctctaccaactccaaccccagcctcaagtctagagtgacactttccctggatacttctaagaaccagttttctctgaagctgaggtccgtgaccgccgctgacaccgctgtgtactactgcgccttcggctactccgattacgagtacaactggttcgacccttggggacagggcacactggtcacagtgagctccgcctcgacaaaaggcccttccgtgtttcctctggctccttgctctcggtccacctctgagagcaccgctgccctgggctgcctggtcaaagactacttccccgagcctgtgaccgtgtcttggaatagcggcgctctgacctccggcgtgcacaccttcccagctgtgctgcagtccagtggcctgtactccttaagctctgtcgtgaccgtgcctagctcctcactgggcaccaagacctatacctgcaacgtggaccacaagccttccaacaccaaagtggacaagcgggtcgaatccaagtacggccccccctgccctccttgtcctgctcccgagttcctgggaggaccatcggtgtttctgttccctccaaagcctaaggataccctgatgatctccagaacacctgaagtgacctgtgtggttgtggacgtgtcccaagaggaccccgaggttcagttcaactggtacgtggatggcgtggaagtgcacaacgccaagaccaagcctagagaggaacagttcaactccacctacagagtggtcagcgtgctgaccgttctgcaccaggactggctgaacggcaaagagtacaagtgcaaggtgtctaacaagggactgccttcctctatcgagaagaccatcagcaaggctaagggccagccccgcgaacctcaggtgtacaccctgcctccttctcaggaagagatgaccaagaaccaggtgtccctgacctgtctggtgaaaggcttctacccctctgatatcgccgtggagtgggagtctaacggccagcctgagaacaactacaaaaccacccctccagtgctggactccgacggctccttcttcctgtactctcggctgaccgtggacaagtccagatggcaagaaggcaacgtgttcagctgctccgtgatgcacgaggccctgcataatcactacacccagaagtccctgtccctgtctctgggcaag

SEQ ID NO: 278 - DNA, 1725 bp, synthetic construct
  misc_feature 1..1725: note = Artificial
  source 1..1725: mol_type = other DNA
gtgatccatgtgactaaggaagtgaaggaagtcgctacattgagctgcggccataacgtctccgtggaagagctggcccagacccggatctactggcagaaaaacaagaagatggtgctaaccatgatgtccggcgacatgaacatctggcctgaatacaagaaccggaccatcttcgacatcaccaacaacctgtccatcgtgatcctgcagctgcggccttccgatgagggcacctacgagtgcgtggtgctgaagtacgaaaaggacgccttcaagcgggagcacctggctgaggtgaccctctctgtgaaggccgacggcggcggcggcagcggcggaggcggctctggaggagggggatctggcggcggcggttccggccaggttcagctgcagcagtggggagctggtctgctgaagccctctgagacactgagcctgacctgcgccgtgtatggcggctccttctccgactactactggaattggatcagacagccacccggcaagggcctggaatggatcggcgagatcaaccacagaggctctaccaactccaaccccagcctgaagtccagggtgaccctgagtctggacacctctaagaaccagttttctttgaagctgagatctgtgaccgccgctgataccgctgtgtactactgcgcttttggctactctgactacgagtacaactggttcgatccttggggccagggaaccctggtcactgtgtcctctgccagtacaaaaggccccagcgtgttccctctggctccttgctcccggtccacatccgagtctaccgccgcactgggctgtctggtgaaggactacttccccgagcccgtgaccgtgtcctggaattctggcgccctgacctctggcgtccacaccttccctgctgtgctgcaatctagtggcctgtactccctgtcctctgtcgtgacagtgcctagttccagcctgggcaccaaaacatacacctgcaacgtggaccacaagccttccaacacaaaggttgataagcgggtggaatccaagtacggccctccttgtcctccatgtcctgcccctgagttcctgggaggcccaagcgtgtttctgttccctcctaagcccaaagacaccctgatgatctcccgcacacctgaagtgacctgtgtggtagtcgacgtgagccaagaggatcccgaggtgcagttcaactggtacgtggacggcgtggaagtgcacaacgccaagaccaagcctagagaggaacagttcaactccacctacagagtggtgagcgtgctgaccgtgctgcaccaggactggctgaacggcaaggagtacaagtgcaaggtgtccaacaagggcctgccttcctctatcgagaagaccatttccaaagccaagggacagcctagagaacctcaggtctataccctgcctccatctcaagaagagatgaccaaaaaccaggtgtctctgacatgcctggtgaagggcttctatccttctgatatcgccgtggagtgggagtccaatggccagcctgagaacaactacaagaccacccctcctgtgctggactccgatggctccttcttcctgtactccagactgaccgtggacaagtctagatggcaggaaggcaacgtgttctcctgctctgtgatgcacgaggccctgcataatcactacacccagaagtccctgtccctgtctctcggcaaa

SEQ ID NO: 279 - DNA, 1725 bp, synthetic construct
  misc_feature 1..1725: note = Artificial
  source 1..1725: mol_type = other DNA
gtgatccatgtgactaaggaagtgaaggaagtggccaccctgtcttgcggccacaatgtgtctgtggaggaactggctcagacccggatctactggcagaagaacaagaagatggtcctgaccatgatgtccggcgacatgaacatctggcctgagtacaagaaccggacaatcttcgacatcaccaacaacctgtccatcgtgatcctgaccctgcggccttctgacgagggcacctatgagtgcgtggtgctgaagtacgagaaagacgcattcaagcgggagcatctggccgaggtgaccctgtccgtgaaggccgatggcggcgggggctccggcggcggcggcagtggaggaggaggctccggtggaggcggctccggacaggtgcagctccagcagtggggcgctggcctgctgaaaccatctgagacactgtccctgacatgcgccgtgtatggaggctccttctccgactactactggaactggatcagacagcctcccggcaagggcctggaatggatcggcgaaatcaaccacaggggctccaccaactccaaccctagcctgaagtctagagtgacactgagcctggatacctctaagaatcagttcagcctcaagctgagatctgtgaccgctgccgacaccgctgtgtactactgcgccttcggctactccgactacgagtacaactggttcgatccttggggccagggcacactcgtgaccgtgagctctgcttctaccaagggcccatccgtgtttcctctggccccttgttcgagatccacctccgagtccaccgccgctctgggctgtctggtgaaggactacttcccggaaccagttacagtgtcctggaactctggcgccctgaccagcggcgtccacaccttccctgccgtgctgcagtcctctggcctgtacagcctgtcttccgtcgtgaccgtgccctcttcctccctgggcaccaaaacctacacctgcaacgtggaccacaagccttccaacaccaaagtggataagagagtcgaatccaagtacggccctccctgccctccttgtcctgctccagagttcctgggcggccccagcgtgtttctgttcccccctaagcccaaagacaccctgatgatcagccggacccccgaggtgacctgtgtggtggttgacgtgtcccaggaggaccctgaagtgcagtttaattggtacgtggatggcgtcgaagtgcataatgccaagaccaagcctagagaggagcagttcaactccacctacagagtggtgtctgttctgaccgtgctgcaccaggactggctgaacggaaaagagtacaagtgcaaggtgagcaacaagggcctgccttcctctatcgagaagaccatctccaaggctaagggccaacctcgcgagcctcaggtgtatacacttcccccttctcaggaagaaatgaccaagaaccaagtgtctctgacctgcctggtgaaaggcttttaccctagtgatattgccgtggaatgggaatctaacggccagcctgagaacaactacaagaccacacctcctgtgctggactccgacgggtctttcttcctgtactctcggctgaccgtggacaagtccagatggcaagaaggcaacgtgttctcctgctccgtcatgcacgaggccctgcacaaccactacacccagaagtccttatctctgtccctgggcaag

SEQ ID NO: 280 - DNA, 1782 bp, synthetic construct
  misc_feature 1..1782: note = Artificial
  source 1..1782: mol_type = other DNA
atgggttggagttgcatcatcctatttctagtggccaccgctaccggcgtgcactcggtcatccacgtgaccaaagaagtgaaagaagtggctacactgtcatgcggccacaacgtgtctgtggaagagctcgcccagaccagaatctactggcagaaggaaaagaagatggtgctgaccatgatgtccggcgacatgaacatctggcctgagtacaagaaccggacaatcttcgacatcaccaacaatctgtctatcgtgatcctggctctgcggccatctgacgagggcacctacgagtgcgtggtgctgaagtacgaaaaggacgccttcaagcgggagcacctggccgaggtgaccctgtccgtgaaggccgacggcggcggaggcagcggcggcgggggcagtggtggcggcggctctggcggcggcggatctggccaggtgcagctgcagcagtggggagctggactgctgaagccttccgagacactcagcctgacttgtgccgtgtacggcggcagcttttctgactactactggaactggatcagacagccacctggcaagggcctggaatggatcggcgagatcaaccacagaggctccacgaattccaacccttccctgaagtctagagtgacactgtccctggacacctctaagaatcagttctctctgaagctgagatccgtgaccgccgccgataccgctgtgtactactgcgccttcggctactccgattacgagtacaactggttcgatccttggggccagggcaccctggtcaccgtgtcttctgcttctactaagggccccagcgtgtttcctctggccccttgcagccgctccacctccgaatccaccgctgctctgggctgcctggtgaaagactacttccccgagcctgtgacagtttcctggaactccggcgccctcacctctggcgtgcacaccttccctgccgtgctgcagtcctctggcctgtactccctgtccagcgtggtcaccgtgcccagctcctctctgggcaccaagacctacacctgcaacgtggaccacaagccctccaacaccaaggtggacaagagagtggagtccaagtacggacctccatgtccaccttgtcctgctcctgagttcctgggcggccctagcgtgttcctgtttcctcccaagcctaaggacaccctgatgatctctcggacccctgaagtgacctgcgtggtcgtggacgtttctcaggaggaccccgaagtgcagttcaattggtacgtggatggcgtggaggtgcataacgccaaaacaaagccccgggaagagcaattcaactccacctacagagtggtctctgtcctgaccgtgctgcaccaggactggctgaacggaaaagagtacaagtgcaaggtgtccaacaagggcctgcctagctccatcgagaaaaccatctccaaggccaagggacagcctagagaacctcaggtgtataccctgcctccatctcaagaggagatgaccaagaaccaggtctccctgacatgtctggtgaagggcttctacccttctgatattgccgttgagtgggagtctaacggccagcctgagaacaactacaagaccaccccccctgtgctggactccgacggctcttttttcctgtattcccggttgaccgtcgataagtccagatggcaagaaggcaacgtgttctcctgctccgtgatgcacgaggccctgcataaccactacacccagaaatctctgtctctgtccctgggaaag

SEQ ID NO: 281 - DNA, 702 bp, synthetic construct
  misc_feature 1..702: note = Artificial
  source 1..702: mol_type = other DNA
atgggttggagttgcatcatcctatttctagtcgccaccgccaccggagtgcactctcagaccgtggtgactcaagagcccagcctgacagtgtccccaggcggaaccgtcaccctcacctgtcggtcctctaccggcgccgtgaccacctccaactacgctaattgggtccagcagaagcctggtcaggctcctagaggcctgatcggcggcaccaacaagagagcccctggcacccctgccagattctccggctctctgctgggcggcaaggctgctctgacactgtctggcgtgcagcccgaagacgaggccgagtactactgcgccctgtggtattctaacctgtgggtgttcggcggaggcaccaagctgaccgtgctgggccagcctaaggccgctccatccgtgaccctgtttcctccttcttctgaggaactgcaggccaacaaagctaccctggtgtgcctgatctccgacttctaccccggcgctgtgacagtggcctggaaagccgatagcagccctgtgaaggctggcgtggaaacaaccacaccttccaagcagtccaacaacaagtacgccgcctcttcctacctgtccctgacccctgagcagtggaagtcccatcggtcttactcctgccaggtgacccacgagggctccaccgtggaaaagaccgtggctcccaccgagtgcagc

SEQ ID NO: 282 - DNA, 1806 bp, synthetic construct
  misc_feature 1..1806: note = Artificial
  source 1..1806: mol_type = other DNA
atgggttggagttgcatcatcctatttctagtggctaccgccaccggcgtgcactccgtgatccacgtgaccaaggaagtgaaagaggtggctaccctgtcttgtggccacaacgtgtctgtcgaggaactggcccagaccagaatctactggcagaagaacaagaagatggtgctgaccatgatgtccggcgacatgaacatctggcctgaatacaagaacagaaccatcttcgacatcaccaacaacctgtccatcgtgatcctgaatctgagaccttccgacgagggcacctatgagtgcgtggtcctgaagtacgagaaggacgccttcaagagagagcacctcgctgaggtgacactgtcggtgaaggccgacggcggcggaggcagcggtggaggcggcagcggcggagggggctctggcggcggcggctctggcgaggtgcagctggtggaatctggcggcggactggtgcagcctggcggctctctgcggctgtcttgcgccgcttctggctttaccttcaacacctacgccatgaattgggtgcggcaggcccctggaaagggcctggaatgggtggcccgcatccggtccaagtacaacaactacgccacctactacgctgcctccgtcaagggcagattcaccatctctagagatgattctaagaattctctgtacctccagatgaactccctgaaaaccgaggataccgctgtgtactactgcgctagacacggcaacttcggcaactcctacgtgtcctggttcgcctactggggccaaggcacactggtgacagtcagttccgcctctacaaagggcccttccgtgtttcctctggctccatcctctaagagcacatccgggggaaccgccgccctcggctgtctggtgaaggattacttccctgagcccgtcaccgtgtcttggaactccggcgctctgacatctggcgtgcacacctttcctgctgtgctgcagagctccggcctgtattccctgtccagcgtggtgaccgtaccttcttctagtctgggcacacagacctacatctgcaacgtgaaccacaagccctctaacaccaaggtggataagaaagtggaacccaagtcctgcgacaaaacccatacctgtcctccttgccctgcccccgaactgctgggcggaccttccgtgttcctgttccccccaaagcctaaggacaccctgatgatctcccggaccccagaggtaacctgcgttgtcgtggacgtgagccatgaggaccccgaggtgaagttcaactggtacgtggacggcgtggaagtgcataacgccaagaccaagcctagagaagagcagtacaactccacctacagagtggtctctgtgctgaccgtgctgcaccaggactggctgaacggcaaagagtacaagtgcaaggtgtccaacaaggccctgcccgctcctatcgagaagacaatctccaaggctaagggccagcctcgggaacctcaagtgtacaccctgcctccatctcgggacgagctgaccaaaaaccaggtgagcctgacctgcctggtcaagggcttctacccttctgacattgccgtggagtgggagagcaacggccagcccgagaacaactacaagaccacccctcctgtgctggactccgatggcagcttcttcctgtattccaagctgaccgtggacaagtccagatggcagcagggcaatgtgttcagctgttccgtgatgcacgaggctctgcacaatcactacacccagaaatccctgtccttgtctcctggcaaa

SEQ ID NO: 283 - DNA, 1749 bp, synthetic construct
  misc_feature 1..1749: note = Artificial
  source 1..1749: mol_type = other DNA
gtgatccatgtgactaaggaagtgaaggaagtggccaccctgtcttgcggccacaacgtgtccgtggaagaactggctcagaccagaatctactggcagaaaaacaagaagatggtgctgaccatgatgtccggcgacatgaacatctggcctgagtacaagaatagaaccatcttcgacatcacgaacaacctgtccatcgtgatcctgaacctgagacctagcgacgagggcacctacgagtgtgtggtgctgaagtacgagaaggacgccttcaagcgggagcacctggccgaggtgaccttgtccgtgaaggctgacggaggcggcggctccggcggcggcggctctggcggcggaggttccggaggcggtggatctggcgaggtgcagctggtcgagtccggcggcggcctggtgcagcccggcggctctctgcggctgagttgtgccgctagcggctttaccttcaacacctacgccatgaactgggtgcggcaggctcctggcaagggcctggaatgggtcgctcggatcagatctaagtacaacaattacgctacctactacgccgccagcgtgaagggcagattcaccatttctcgggacgactccaagaactccctgtacctgcagatgaacagcctgaagacagaagataccgccgtgtactactgcgccagacacggcaacttcggcaattcctatgtgtcttggttcgcctactggggccagggcacactagttacagtttcttctgcctctaccaaaggcccttccgtgttccctctggccccatcgagcaagagcaccagcgggggcaccgctgctctgggctgcctggtgaaggactacttccctgagcctgtgaccgtgtcctggaactctggcgctctaacatctggcgtgcacacatttccagctgtgctgcagtcctctggactgtactccctgagcagtgtcgtgacagtgccttcgtcctctctgggcacccagacctacatctgcaacgtgaaccacaagccctccaacaccaaggtggataagaaagtggaacctaaatcctgcgacaagacccacacctgccccccttgccctgcccctgagctgctgggaggaccttccgtatttctgttccctcccaaacctaaggacaccctgatgatctcccgcacaccggaagtgacctgtgtggtggtggatgtgtcccacgaggaccccgaagtgaagttcaattggtacgtggacggcgtggaagtgcataacgccaagaccaagcctagagaggaacagtacaactccacctacagagtggtctctgtgctgaccgtgctgcaccaggactggctgaacgggaaagagtacaagtgcaaggtgtccaacaaggccctgcctgctcctatcgagaaaaccatctccaaggctaagggacagcctcgggaaccccaggtgtacaccctgcctccctctagggatgagctgaccaagaaccaagtctccctcacatgtctggtgaagggcttctacccttctgatatcgccgtggagtgggagtctaatggccagcctgagaacaactataagaccacccctccagtgctggactctgatggctccttcttcctctattccaagctgaccgtggacaagtccagatggcagcagggcaacgtgttctcctgcagcgtgatgcacgaggccctgcataaccactacacccaaaagagcctgtctctgtctcctggcaag

SEQ ID NO: 284 - DNA, 1749 bp, synthetic construct
  misc_feature 1..1749: note = Artificial
  source 1..1749: mol_type = other DNA
gtgatccatgtgactaaggaagtgaaggaagtggccaccctgtcctgtggccacaacgtctctgtggaagaactggcccagaccagaatttactggcagaaaaacaagaagatggtgctgaccatgatgtccggcgacatgaacatctggcccgaatacaagaacagaacaatcttcgacatcaccaacaacctgtccatcgtgatcctgcagctgagaccttctgatgagggcacctacgagtgcgtggtgctgaagtacgaaaaggacgccttcaagcgggagcacctggccgaggtgacactgtctgtgaaggccgacggcggcggaggcagcggaggcggcggctctggcggaggcggatccggaggcggcggatctggcgaggtacagctggtggaatctggtggaggactggtgcagcctggcggcagcctgagactgagctgcgccgcttccggctttaccttcaacacctatgccatgaattgggtgcggcaggcccctggcaagggcctggaatgggtcgcccggatccggtccaagtacaacaactacgccacctactacgccgcctctgtgaagggcagattcaccatctcccgcgacgactctaaaaattctctgtacctgcagatgaactctctgaagacagaggacaccgctgtgtactactgcgctagacacggcaacttcggcaactcctatgtgtcctggttcgcctactggggccagggcaccttggtcaccgtgtcctctgcttctaccaagggcccttctgtgttccctctggctccttcctccaagtccacatctggcggcacagctgctctgggctgcctcgtgaaggactacttcccggagcccgtgaccgtgtcctggaactctggcgctctgacctccggcgtgcatacctttcctgctgtgctccagtccagcggcctgtattctctctcttctgtggtcaccgtgccatccagttccctgggcacacaaacctacatctgcaacgtgaaccacaagccttccaatactaaagtggataaaaaggtggaacccaagtcctgcgacaagacccacacctgccctccatgtcctgctcctgaacttctgggcggcccctcggtgtttctgttcccacctaagcccaaggataccctgatgatctcccggacccctgaggtgacctgtgtggttgtggacgtgtcccacgaggatcctgaggtcaagttcaactggtacgtggacggcgtagaagtgcataacgccaagaccaagcctcgagaagagcagtacaacagcacctacagagtggtgagcgtgctgacagtgctgcaccaggattggctgaacggcaaagagtacaagtgcaaggtgagcaacaaggccctgcccgcacctatcgagaagaccatcagcaaggctaagggccaacctagagagcctcaagtttacaccctgcctcctagccgggacgagctgaccaagaatcaggtgtctctgacctgtctggtgaagggcttctacccttccgacatcgccgtcgagtgggagtccaacggacagcccgagaacaactacaaaaccacccctcctgtgctggactccgatggctccttcttcctgtactccaagctgaccgtggacaaatctagatggcagcagggcaatgtgttctcctgctctgtgatgcacgaggccctgcacaaccactacacccagaagtccctgtctctgtctcctggcaag

SEQ ID NO: 285 - DNA, 1749 bp, synthetic construct
  misc_feature 1..1749: note = Artificial
  source 1..1749: mol_type = other DNA
gtgatccatgtgactaaggaagtgaaggaagtggctaccctgtcttgcggccataatgtgtctgtggaggaactggctcagaccagaatctactggcagaaaaacaagaagatggtgttgaccatgatgtccggcgacatgaacatctggcccgaatacaagaaccggaccatcttcgacatcaccaacaacctgtccatcgtgatcctgaccctgcggccttcggacgagggcacatacgagtgcgtggtgctgaagtatgaaaaggacgccttcaagagagagcacctcgccgaggtgacccttagcgtgaaggccgacggaggcggcggctccggaggcggcggatcaggaggcggcggatccggcggcggcgggtccggcgaggtccagctggtggaatctggaggcggcctggtgcagcctggtggctctctgagactgtcttgcgctgcttctggctttaccttcaacacctatgccatgaactgggtgcggcaggcccctggcaagggactggaatgggtggcccggatcagaagcaagtacaacaactacgccacctactacgccgcttccgtcaagggccggttcaccatcagccgggacgactccaaaaactccctgtacctgcagatgaactccctgaagaccgaggacaccgctgtgtactactgcgccagacacggcaacttcggcaactcctacgtttcctggttcgcctactggggccagggcaccctggtcacagtgtctagcgcctctaccaaaggccctagcgtgttccctctcgctccttcttccaagtccacctccggcggcaccgccgctctgggctgtctggtgaaggactacttccctgaacccgtgaccgtgtcttggaactctggcgccctgaccagcggagtgcacacctttcctgctgtgctgcagtccagcggcctgtattctctgtcctctgtggtgaccgtgccttcttccagcctgggaacccagacctacatttgcaacgtgaaccacaagccctctaatacaaaagtggacaagaaagttgaacctaagtcctgcgacaaaacacacacctgtccaccttgtcctgccccagagctgctgggcggcccctccgtgtttctgttccctcccaagcctaaggataccctgatgatctccagaacccctgaagtgacctgtgtggtcgtggatgtgtctcacgaggatcctgaggtgaagttcaattggtacgtggacggcgtggaagtgcacaacgccaagaccaagcctagagaagagcagtacaacagcacctacagagtggtatccgttctgactgtgctgcaccaggactggctgaacggaaaagagtacaagtgcaaggtctccaacaaggccctgcccgctcctatcgagaagacaatctccaaggccaagggccagcctcgcgagcctcaagtgtacaccctgcctccatctagggatgagctgaccaagaaccaggtgtctctgacctgcctggtgaagggcttctacccttccgatatcgccgtggagtgggagtccaacggccaacccgagaacaactacaagaccacacctcctgtgctggactctgatggctccttcttcctgtactccaaactgacagtcgacaagagcagatggcagcagggcaatgtgttctcctgctccgtgatgcacgaggctctgcataaccactacacacagaagtctctcagcctgtctcccggcaag

SEQ ID NO: 286 - DNA, 1806 bp, synthetic construct
  misc_feature 1..1806: note = Artificial
  source 1..1806: mol_type = other DNA
atgggttggagttgcatcatcctatttctagtggccaccgccaccggcgtgcactccgtgatccacgtgacaaaagaagtgaaagaggtggcaaccctgtcctgtggacataatgtctctgtggaggaactggctcagaccagaatctactggcagaaggaaaagaagatggtgctgactatgatgtccggcgacatgaatatctggcctgagtataagaaccgcaccatcttcgacatcaccaacaacctgtccatcgtgatcctggctctgagaccttccgacgagggcacatacgagtgcgtggtgctgaagtacgagaaggacgccttcaagcgggagcatctggccgaggtgaccctgtctgtgaaggctgatggcggtggcggctctggcggcggcggctctggcggcggcggatctggcggcggtggcagcggcgaggtgcagctggtggaatctggaggcggactcgtgcaacctggaggctccctgcggctgtcctgcgccgcttccggctttacctttaacacctacgccatgaattgggtgcggcaggcccctggcaagggcctggaatgggtcgcccggatcagatccaagtacaacaactacgccacctactacgctgcttccgtgaagggcagattcaccatctctcgggacgactctaagaactccctgtacctgcagatgaactctctgaagaccgaggacaccgctgtgtactactgcgctagacacggcaacttcggcaattcctacgtgtcctggttcgcctactggggccagggcacactggtgaccgtgtcttccgcctctactaaagggcctagcgtcttccctctggctccttcttccaagtccacctccggcggcacagctgccctgggctgcctggtcaaggactacttccccgagcctgtcaccgtgtcttggaacagcggcgctctgacctctggcgtgcataccttccctgccgtgctgcagtcctccggcctgtactccctgtcttccgtggtgacagtgcctagctcttctctcggaacacagacctacatctgcaacgtgaaccacaagccctccaacaccaaggtggataagaaagtggaaccaaagtcctgcgacaagacacacacctgtcctccttgccccgctcctgagctgctgggcggcccttctgtgtttctgttcccccctaagccaaaggataccctgatgatctccagaacccctgaagtgacatgtgttgtggtcgacgtgagccacgaggatcccgaggtgaagttcaactggtacgtggacggcgtggaagtgcacaacgccaagaccaagcctagggaggaacagtacaattctacctacagagtggtgtcggtgctgaccgtgctgcaccaggactggctgaacggcaaagagtacaagtgcaaggtgagcaacaaggctctgccagcccccattgagaagaccatcagtaaggccaaaggccaacctcgggaacctcaagtgtataccttgcctccatccagagatgaactgaccaagaaccaggtaagcctgacctgcttggtgaagggcttctacccctctgacatcgccgtcgagtgggagtccaacggccagcctgagaacaactacaaaaccacacctcctgtcctggactccgatggatccttcttcctgtattccaagctgaccgtggacaagtctagatggcagcagggcaacgtgttctcctgttccgtaatgcacgaggccctgcacaaccactacacccagaaatctctgagcctgtctcctggtaag

SEQ ID NO: 287 - protein, 448 aa, synthetic construct
  REGION 1..448: note = Artificial
EVQLLESGGGLVQPGGSLRLSCAASGFTFSSYAMSWVRQAPGKGLEWVSGISGSGGFTYYADSVKGRFTISRDNSKNTLYLQMNSLRAEDTAVYYCAKPPRGYNYGPFDYWGQGTLVTVSSASTKGPSVFPLAPCSRSTSESTAALGCLVKDYFPEPVTVSWNSGALTSGVHTFPAVLQSSGLYSLSSVVTVPSSSLGTKTYTCNVDHKPSNTKVDKRVESKYGPPCPPCPAPEFLGGPSVFLFPPKPKDTLMISRTPEVTCVVVDVSQEDPEVQFNWYVDGVEVHNAKTKPREEQFNSTYRVVSVLAVLHQDWLNGKEYKCKVSNKGLPSSIEKTISKAKGQPREPQVYTLPPSQEEMTKNQVSLTCLVKGFYPSDIAVAWESNGQPENNYKTTPPVLDSDGSFFLYSRLTVDKSRWQEGNVFSCSVMHEALHAHYTQKSLSLSLGK

SEQ ID NO: 288 - DNA, 1398 bp, synthetic construct
  misc_feature 1..1398: note = Artificial
  source 1..1398: mol_type = other DNA
atgcacagctcagcactgctctgttgcctggtcctcctgactggggtgagggccgaggtgcagctgctggagagcggggggggactggtgcagccaggaggaagcctgagactgagctgtgccgccagcgggtttacatttagcagctatgccatgagctgggtgagacaggcccctggcaaaggcctggagtgggtgagcggaatctccggcagcgggggatttacatactacgccgatagtgtgaagggcagatttacaatcagcagagacaacagcaagaacacactgtacctgcagatgaacagcctgagagccgaggacaccgccgtgtactattgcgccaagccccccagaggatataactacggacccttcgactactggggacagggcaccctggtgacagtgtccagcgctagcaccaagggcccatcggtcttccccctggcgccctgctccaggagcacctccgagagcacagccgccctgggctgcctggtcaaggactacttccccgaaccggtgacggtgtcgtggaactcaggcgccctgaccagcggcgtgcacaccttcccggctgtcctacagtcctcaggactctactccctcagcagcgtggtgaccgtgccctccagcagcttgggcacgaagacctacacctgcaacgtagatcacaagcccagcaacaccaaggtggacaagagagttgagtccaaatatggtcccccatgcccaccatgcccagcacctgagttcctggggggaccatcagtcttcctgttccccccaaaacccaaggacactctcatgatctcccggacccctgaggtcacgtgcgtggtggtggacgtgagccaggaagaccccgaggtccagttcaactggtacgtggatggcgtggaggtgcataatgccaagacaaagccgcgggaggagcagttcaacagcacgtaccgtgtggtcagcgtcctcaccgtcctgcaccaggactggctgaacggcaaggagtacaagtgcaaggtctccaacaaaggcctcccgtcctccatcgagaaaaccatctccaaagccaaagggcagccccgagagccacaggtgtacaccctgcccccatcccaggaggagatgaccaagaaccaggtcagcctgacctgcctggtcaaaggcttctaccccagcgacatcgccgtggagtgggagagcaatgggcagccggagaacaactacaagaccacgcctcccgtgctggactccgacggctccttcttcctctacagcaggctaaccgtggacaagagcaggtggcaggaggggaatgtcttctcatgctccgtgatgcatgaggctctgcacaaccactacacacagaagagcctctccctgtctctgggtaaa

SEQ ID NO: 289 - protein, 447 aa, synthetic construct
  REGION 1..447: note = Artificial
QVQLQQWGAGLLKPSETLSLTCAVYGGSFSDYYWNWIRQPPGKGLEWIGEINHRGSTNSNPSLKSRVTLSLDTSKNQFSLKLRSVTAADTAVYYCAFGYSDYEYNWFDPWGQGTLVTVSSASTKGPSVFPLAPCSRSTSESTAALGCLVKDYFPEPVTVSWNSGALTSGVHTFPAVLQSSGLYSLSSVVTVPSSSLGTKTYTCNVDHKPSNTKVDKRVESKYGPPCPPCPAPEFLGGPSVFLFPPKPKDTLMISRTPEVTCVVVDVSQEDPEVQFNWYVDGVEVHNAKTKPREEQFNSTYRVVSVLTVLHQDWLNGKEYKCKVSNKGLPSSIEKTISKAKGQPREPQVYTLPPSQEEMTKNQVSLTCLVKGFYPSDIAVEWESNGQPENNYKTTPPVLDSDGSFFLYSRLTVDKSRWQEGNVFSCSVMHEALHNHYTQKSLSLSLGK

SEQ ID NO: 290 - DNA, 1422 bp, synthetic construct
  misc_feature 1..1422: note = Artificial
  source 1..1422: mol_type = other DNA
gctagcgccgccaccatgggttggagttgcatcatcctatttctagtggctacagccaccggcgtccatagtcaagtgcagctgcagcaatggggcgctggcctgctgaagccttctgaaaccctgtccctgacctgtgccgtgtacggcggatctttctctgattactactggaattggatccggcagcctcctggcaagggactggaatggatcggcgagatcaaccacagaggcagcaccaactccaaccctagcctgaaatcccgggtgaccctcagcctggacacctctaaaaaccagttttccttgaagctgcggtccgttacagctgccgacaccgctgtgtactactgcgccttcggctactccgactacgagtacaactggttcgacccttggggacagggcaccctggtcaccgtgtcctctgcctctaccaagggcccctctgtgtttcctctggctccttgcagccgctccacctccgagtccaccgctgctctgggctgcctggtgaaggactacttccctgaacccgtgaccgtttcctggaactctggcgccctgacaagcggcgtgcacaccttccccgctgtcctgcagtcctccggcctgtacagcctgtcttccgtggtgaccgtgccttcttcttcactgggcacaaagacctatacctgcaatgtggaccacaagccttccaacaccaaagtggataagagagtggaatccaagtacggccctccatgtcctccttgtcctgcccctgagttcctcggcggcccatctgtgtttctgttcccacctaagcctaaggatacactgatgatctctcggaccccagaagtgacatgcgtggtcgtggacgtgtcccaggaggaccccgaggtgcagttcaactggtacgtggatggagtggaagtgcacaacgccaagacaaagcccagagaagagcagttcaactccacctacagagtggtgtccgtgctgaccgtgctgcaccaggactggctgaacggcaaagagtacaagtgcaaggtgtctaacaagggcctgccttcctcgatcgagaagaccatctccaaggccaaaggacagcctagagagcctcaggtgtacaccctgccccccagccaagaggagatgaccaagaaccaggtttctctaacctgcctggtgaagggcttctacccttctgacatcgccgtggagtgggagtctaatggccagcccgagaacaactataagaccaccccccctgtgctggactccgatggcagcttcttcctgtactctcggctgactgtggacaagagcagatggcaggaaggcaacgtcttctcctgctccgtgatgcacgaggccctgcataaccactacacccagaagtccctgtccctgtctctgggcaagtgactcgag

SEQ ID NO: 291 - protein, 455 aa, synthetic construct
  REGION 1..455: note = Artificial
EVQLVESGGGLVQPGGSLRLSCAASGFTFNTYAMNWVRQAPGKGLEWVARIRSKYNNYATYYAASVKGRFTISRDDSKNSLYLQMNSLKTEDTAVYYCARHGNFGNSYVSWFAYWGQGTLVTVSSASTKGPSVFPLAPSSKSTSGGTAALGCLVKDYFPEPVTVSWNSGALTSGVHTFPAVLQSSGLYSLSSVVTVPSSSLGTQTYICNVNHKPSNTKVDKKVEPKSCDKTHTCPPCPAPELLGGPSVFLFPPKPKDTLMISRTPEVTCVVVDVSHEDPEVKFNWYVDGVEVHNAKTKPREEQYNSTYRVVSVLTVLHQDWLNGKEYKCKVSNKALPAPIEKTISKAKGQPREPQVYTLPPSRDELTKNQVSLTCLVKGFYPSDIAVEWESNGQPENNYKTTPPVLDSDGSFFLYSKLTVDKSRWQQGNVFSCSVMHEALHNHYTQKSLSLSPGK

SEQ ID NO: 292 - DNA, 1422 bp, synthetic construct
  misc_feature 1..1422: note = Artificial
  source 1..1422: mol_type = other DNA
atgggttggagttgcatcatcctatttctagtggctaccgccaccggcgtgcactccgaggtgcagctggtcgaatccggcggaggtctcgtgcagcctggcggctctctgagactgtcttgtgctgcttctggcttcaccttcaacacctacgccatgaattgggtcagacaggcccccggcaagggcctggaatgggtggcccggatccggtccaagtacaacaactacgccacatactacgctgcctctgtcaaaggacggttcaccatctcaagagacgactccaagaactccctgtacctgcagatgaacagcctgaagaccgaggacaccgctgtgtattattgcgccagacacggcaacttcggcaactcctacgtgtcttggttcgcctactggggccagggcaccctggtgaccgtgtcctccgcctccaccaaaggcccctctgtgtttcctctggcccctagcagcaaatctacatcaggaggcaccgccgctctgggctgcctggtgaaggactacttccccgaacctgttacagtgtcctggaactctggcgctctgacctccggagtgcatacctttccagccgtgctgcaatcttctggcctgtactccctgagcagcgtggtgaccgtgccttcttccagcctgggaacacagacctacatctgcaacgtgaaccacaagccttccaacaccaaggtggacaagaaagtggaacccaagtcttgcgacaagacccacacctgtcctccttgccctgctcccgaactgctgggcggcccttccgtgtttctgttcccacctaagcccaaggatacactgatgatctcccggacacctgaggttacctgcgtggtcgtggacgtgtctcacgaggatcctgaggtgaagttcaactggtacgtggacggcgtggaagtgcacaatgccaagaccaagcctcgcgaggaacagtacaactctacctacagagtggtgtccgtgctgaccgtgctgcaccaggactggctgaacggcaaagagtacaagtgcaaggtgtctaacaaggccctgcccgctcctatcgagaagaccatctctaaggctaagggccagcctagagagcctcaagtgtacaccctgcctccatctcgggacgagctgacaaagaaccaggtgtccctcacctgtctggtcaagggcttctacccctccgacatcgccgtggagtgggagtccaatggccagcctgagaacaactacaaaaccacccctcctgtgctggactctgatggctccttcttcctgtattctaagctgaccgtagataagtccagatggcagcagggcaatgtgttctcctgctccgtgatgcacgaggccctgcataaccactacacccagaagtccctgagcctatctcctggcaag

SEQ ID NO: 293 - protein, 1025 aa, synthetic construct
  REGION 1..1025: note = Artificial
VIHVTKEVKEVATLSCGHNVSVEELAQTRIYWQKNKKMVLTMMSGDMNIWPEYKNRTIFDITNNLSIVILELRPSDEGTYECVVLKYEKDAFKREHLAEVTLSVKADGGGGSGGGGSGGGGSGGGGSGEVQLLESGGGLVQPGGSLRLSCAASGFTFSSYAMSWVRQAPGKGLEWVSGISGSGGFTYYADSVKGRFTISRDNSKNTLYLQMNSLRAEDTAVYYCAKPPRGYNYGPFDYWGQGTLVTVSSASTKGPSVFPLAPCSRSTSESTAALGCLVKDYFPEPVTVSWNSGALTSGVHTFPAVLQSSGLYSLSSVVTVPSSSLGTKTYTCNVDHKPSNTKVDKRVESKYGPPCPPCPAPEFLGGPSVFLFPPKPKDTLMISRTPEVTCVVVDVSQEDPEVQFNWYVDGVEVHNAKTKPREEQFNSTYRVVSVLAVLHQDWLNGKEYKCKVSNKGLPSSIEKTISKAKGQPREPQVYTLPPSQEEMTKNQVSLTCLVKGFYPSDIAVAWESNGQPENNYKTTPPVLDSDGSFFLYSRLTVDKSRWQEGNVFSCSVMHEALHAHYTQKSLSLSLGAGGGGSGGGGSGGGGSGGGGSGLQPGAEVPVVWAQEGAPAQLPCSPTIPLQDLSLLRRAGVTWQHQPDSGPPAAAPGHPLAPGPHPAAPSSWGPRPRRYTVLSVGPGGLRSGRLPLQPRVQLDERGRQRGDFSLWLRPARRADAGEYRAAVHLRDRALSCRLRLRLGQASMTASPPGSLRASDWVILNCSFSRPDRPASVHWFRNRGQGRVPVRESPHHHLAESFLFLPQVSPMDSGPWGCILTYRDGFNVSIMYNLTVLGLEPPTPLTVYAGAGSRVGLPCRLPAGVGTRSFLTAKWTPPGGGPDLLVTGDNGDFTLRLEDVSQAQAGTYTCHIHLQEQQLNATVTLAIITVTPKSFGSPGSLGKLLCEVTPVSGQERFVWSSLDTPSQRSFSGPWLEAQEAQLLSQPWQCQLYQGERLLGAAVYFTELSSPGAQRSGRAPGALPAGHL

SEQ ID NO: 294 - DNA, 3075 bp, synthetic construct
  misc_feature 1..3075: note = Artificial
  source 1..3075: mol_type = other DNA
gtgatccatgtgactaaggaagtgaaggaagtggctaccctgtcttgtggacacaacgtctcggtggaagagctggcccagaccagaatctactggcagaaaaacaagaagatggtgctgaccatgatgtctggcgatatgaacatctggcctgagtacaagaaccggaccatcttcgacatcaccaacaacctgagcatcgtgatcctggaactgagaccttccgatgaggggacgtatgagtgcgtggtgttaaagtacgagaaggacgccttcaagcgggagcacctggctgaggtcaccctgtctgtgaaggccgacggaggcggcggcagtggcggtggcggctccggcgggggaggctccggcggtggcggctctggcgaagtgcagctgctggaaagcggcggcggcctggtgcaacctggaggctctctgagactgtcttgtgctgcctctggcttcaccttctccagctacgccatgtcttgggtcagacaggccccaggcaagggcctcgaatgggtgtccggtatttctggctctggcggcttcacctactacgctgactccgtgaagggccggttcaccatctccagggataactccaagaataccctgtacctgcagatgaactctctgagagccgaggataccgcggtgtactactgcgcaaagcctccccggggctacaactacggccccttcgactactggggccagggcaccctggtgaccgtaagctccgctagtacaaaaggcccctcagtgttccctctggccccttgctccagatctacctccgagtccactgctgctctgggttgtctggtgaaggactacttccccgaacctgtaaccgtgagctggaactccggcgccctgacctctggcgtgcatacctttcccgccgtgctgcagtcctccggcctgtactcgctgtctagcgtggtgacagtgccttcctcatccctgggcaccaaaacctacacgtgcaacgtggaccacaagccttccaacaccaaggtcgacaagagagttgagtccaagtatggcccaccatgtcctccttgcccggctcctgagttcctgggcgggccttccgtgttcctgtttcctcccaaacctaaggacacactgatgatctccagaacccccgaagttacctgtgtggtcgtggatgtgtctcaggaggaccctgaagtgcagttcaactggtacgtggatggcgtggaagtgcataacgctaagaccaagcccagagaggaacagttcaactccacctaccgggtggtgagcgtgctggctgtgctgcaccaggattggctgaacggcaaagagtacaagtgcaaggtgtctaataagggactgcctagtagcatcgagaagaccatcagtaaggccaaaggccagcctagagaacctcaggtgtacacactgcctccctctcaagaagagatgaccaagaaccaggtttctctgacctgccttgtcaagggcttctacccttctgatatcgccgtggcctgggagtccaatggccaacctgagaacaactacaagaccactcctcccgtcctggactccgacggctctttcttcctgtactcccggctgaccgtggacaagtctagatggcaagaaggcaacgtgttttcctgctccgtgatgcacgaggccctgcacgcccactacacccagaagtccctgtccctgtctctcggcgccggcggcggcggatccggagggggcggatcgggaggaggtggctctggcggcggagggtctggcctgcagcctggcgccgaggtgccagtcgtgtgggcccaggagggcgctcctgctcagctgccctgcagtcctaccatccctctgcaggacctatccctgctgcggagagctggcgtaacctggcagcaccagcccgactctggcccacctgcggctgcccctggccatcctctggcccctggccctcaccctgccgctccttcttcatggggcccccggcctagaagatacacagtgctgtccgtgggccccgggggcctgcggtccggcagactgcctctgcaacctagagtgcagctcgacgagcggggcagacagagaggcgacttttccctgtggctgcgccccgccagaagagccgacgctggcgagtaccgggctgctgtgcacctgagagaccgggctctgtcctgccgactgagactgagactgggccaggcctccatgaccgcctccccccctggctctctcagagcctccgactgggtcatcctgaactgcagcttctcccggcctgacagaccagcttctgtgcactggttcagaaatcggggccagggccgtgtgccagtgcgagagagcccacaccatcacctggccgagagctttctgttcctgcctcaggtgtctcctatggactccggcccttggggctgcatcctgacatacagagacggcttcaatgtgtccatcatgtacaacctgaccgtgctgggcctggaaccccctacacctctgaccgtgtacgctggcgctggtagcagggtgggcctgccttgtagactgcctgccggagtgggaacccggtccttcctgaccgccaagtggacccctcctggcggcggtcctgatctgttggtgaccggcgacaacggcgattttaccctgagactggaggacgtgtcccaggctcaagccggcacatatacctgccacattcacctgcaagagcagcagctgaacgccacagtgacactggccatcatcaccgtcacccctaaatccttcggctctcctggatctctgggaaagctgctgtgcgaggtgacccctgtgtctggccaggaacggttcgtgtggtcttccctggacaccccttcccagcggtccttctccggcccttggctggaggcccaggaggcccagctgctgtcccagccctggcagtgccagctataccagggcgaacggctgctgggagctgccgtgtacttcaccgagctgtccagccccggcgctcagcggagcgggagagcccctggcgctttgccagccggccacctg

SEQ ID NO: 295 - protein, 1025 aa, synthetic construct
  REGION 1..1025: note = Artificial
VIHVTKEVKEVATLSCGHNVSVEELAQTRIYWQKNKKMVLTMMSGDMNIWPEYKNRTIFDITNNLSIVILNLRPSDEGTYECVVLKYEKDAFKREHLAEVTLSVKADGGGGSGGGGSGGGGSGGGGSGEVQLLESGGGLVQPGGSLRLSCAASGFTFSSYAMSWVRQAPGKGLEWVSGISGSGGFTYYADSVKGRFTISRDNSKNTLYLQMNSLRAEDTAVYYCAKPPRGYNYGPFDYWGQGTLVTVSSASTKGPSVFPLAPCSRSTSESTAALGCLVKDYFPEPVTVSWNSGALTSGVHTFPAVLQSSGLYSLSSVVTVPSSSLGTKTYTCNVDHKPSNTKVDKRVESKYGPPCPPCPAPEFLGGPSVFLFPPKPKDTLMISRTPEVTCVVVDVSQEDPEVQFNWYVDGVEVHNAKTKPREEQFNSTYRVVSVLAVLHQDWLNGKEYKCKVSNKGLPSSIEKTISKAKGQPREPQVYTLPPSQEEMTKNQVSLTCLVKGFYPSDIAVAWESNGQPENNYKTTPPVLDSDGSFFLYSRLTVDKSRWQEGNVFSCSVMHEALHAHYTQKSLSLSLGAGGGGSGGGGSGGGGSGGGGSGLQPGAEVPVVWAQEGAPAQLPCSPTIPLQDLSLLRRAGVTWQHQPDSGPPAAAPGHPLAPGPHPAAPSSWGPRPRRYTVLSVGPGGLRSGRLPLQPRVQLDERGRQRGDFSLWLRPARRADAGEYRAAVHLRDRALSCRLRLRLGQASMTASPPGSLRASDWVILNCSFSRPDRPASVHWFRNRGQGRVPVRESPHHHLAESFLFLPQVSPMDSGPWGCILTYRDGFNVSIMYNLTVLGLEPPTPLTVYAGAGSRVGLPCRLPAGVGTRSFLTAKWTPPGGGPDLLVTGDNGDFTLRLEDVSQAQAGTYTCHIHLQEQQLNATVTLAIITVTPKSFGSPGSLGKLLCEVTPVSGQERFVWSSLDTPSQRSFSGPWLEAQEAQLLSQPWQCQLYQGERLLGAAVYFTELSSPGAQRSGRAPGALPAGHL

SEQ ID NO: 296 - DNA, 3075 bp, synthetic construct
  misc_feature 1..3075: note = Artificial
  source 1..3075: mol_type = other DNA
gtgatccatgtgactaaggaagtgaaggaagtggccacactgtcctgcggccataacgtgtccgtggaagagctggcccagacccggatctactggcagaaaaacaagaagatggtgctgaccatgatgtccggggacatgaacatctggcctgagtacaagaaccgaaccatcttcgacatcaccaacaacctgtctatcgtgatcctgaatctgcggccctctgacgaaggcacctacgagtgcgtggtgctgaagtacgagaaagacgccttcaagcgggagcacctggccgaggtgaccctgtctgtgaaggccgacggcggaggcggctctggcggcggcggctctggcggtggcggatcgggcggcggcggctctggcgaggtgcaactgctggaatctggcggcggcctggtccagcctggcggctcattacggctgtcttgtgctgcttctggcttcaccttctcctcctacgccatgtcttgggtgcggcaggccccaggcaaaggcctcgagtgggtgagtggcatcagcggctctggcggcttcacatactacgccgactccgtcaaaggcagattcaccatttcccgggataattccaagaacaccctgtacctgcagatgaactccctgcgggccgaggataccgctgtgtactactgcgctaagcctcctagaggctataactatggccctttcgactactggggccaaggcaccctggtgaccgtctcctctgcctctaccaagggcccttccgtgttccctctggctccttgtagccggagcacctctgagagtaccgccgctctcggctgcctggtgaaggactactttcctgagcctgtgaccgtgtcttggaactctggtgccctgacctccggcgtgcacaccttccctgccgtgctgcagtcttctggcctgtacagcctgtcttccgtggtgaccgtgccttcctcctctctgggcaccaaaacctacacatgcaacgtggaccacaagccttccaacaccaaagtggacaagagagtggaatccaagtacggccccccttgccctccttgtcctgctcccgagttcctgggaggcccttccgtgtttctgttcccccccaagcctaaggacaccctgatgatctccagaacccctgaagtgacctgtgtggtcgtggatgtgtcccaggaggaccccgaggtacagttcaactggtacgtggacggcgtggaagtgcacaacgccaagaccaagcccagagaggaacagttcaactccacctacagagtggtctctgttcttgccgtgctgcaccaggactggctgaacggcaaagagtacaagtgcaaggtgagcaacaagggcctgccttcctccatcgagaagactatctccaaggccaagggccagccccgcgaacctcaggtgtacaccctgcccccgagccaagaagagatgacaaagaaccaggtgagtctgacctgcctggtgaagggcttctacccctccgatatcgccgttgcctgggagtctaatggccaaccggaaaacaactacaagaccacacctcctgtgctggattccgatggctcgttcttcctgtactccagactgaccgtggacaaatcccgttggcaagagggcaacgtgttctcttgctccgtgatgcacgaggctctccacgcccactacacccagaagtccctgtccctgtccctgggcgctggcgggggcggtagcggcgggggaggctccggcgggggcggctcaggcgggggcggctcaggcctgcagcccggagctgaagtgcctgtggtgtgggctcaggaaggcgcccctgctcaactgccttgctctcctaccatccctctgcaggacctctctctgctgcggcgggccggcgtgacatggcagcaccagcctgattccggcccccccgccgctgctcccggccaccccctggcccctggacctcaccctgctgccccctcctcttggggccctaggcctcggagatacaccgtgctgagcgtgggcccaggcggcctgcggtccggcagactgcctctgcagcccagagtccagctggacgagagaggcagacagagaggcgattttagcctgtggctgcgcccagccagaagagccgatgccggcgagtatagagccgccgtgcacctgagagaccgggccctgtcttgcagactacggcttcggctcggccaggcttccatgaccgcttcccctccaggctctctgagagcttccgattgggtcatcctgaactgctccttctctcggcctgacagacctgctagtgtgcactggttccggaacagaggacagggcagagttccagtgagagagtcccctcatcaccatctggctgagtctttcctcttcctgccccaggtgtctcccatggacagcggaccttggggatgcatcctgacctacagagacggatttaatgtgtccatcatgtacaacctgacagttctgggcctggaaccacctacacctctgaccgtgtacgctggagccggatctagagtgggcctgccttgtagactgcctgcgggcgtgggaacccggtctttcctgaccgccaagtggacccctcctgggggcggacctgacctgctggtgaccggcgacaacggggacttcaccctgcggctggaggacgtgtcccaggcccaggctggcacatacacctgtcacatccacctgcaagagcagcagctgaacgccaccgtgacactggccatcatcaccgtcacccctaagtcattcggctctcccggctctctgggcaagctgctgtgcgaggtgacacctgtaagcggtcaggagcggttcgtctggtcctccctggataccccttcccagagatctttttccggaccgtggctggaagctcaggaagctcagctcttgtcccagccttggcagtgccagctgtaccagggcgaacggctgctcggcgccgctgtgtacttcaccgagctgtccagccctggagcccagagatccggacgggcgccaggcgctctgcctgccggccatctg